European Patent Application EP 4 295 862 A2, published December 27, 2023. Title: CORONAVIRUS VACCINE. Applicant: BioNTech SE. Application EP. The sequence listing filed with the application follows.

SEQUENCE LISTING (177 sequences)

SEQ ID NO: 1 - protein, 1273 aa, synthetic construct
  REGION 1..1273: note = S protein
MFVFLVLLPLVSSQCVNLTTRTQLPPAYTNSFTRGVYYPDKVFRSSVLHSTQDLFLPFFSNVTWFHAIHVSGTNGTKRFDNPVLPFNDGVYFASTEKSNIIRGWIFGTTLDSKTQSLLIVNNATNVVIKVCEFQFCNDPFLGVYYHKNNKSWMESEFRVYSSANNCTFEYVSQPFLMDLEGKQGNFKNLREFVFKNIDGYFKIYSKHTPINLVRDLPQGFSALEPLVDLPIGINITRFQTLLALHRSYLTPGDSSSGWTAGAAAYYVGYLQPRTFLLKYNENGTITDAVDCALDPLSETKCTLKSFTVEKGIYQTSNFRVQPTESIVRFPNITNLCPFGEVFNATRFASVYAWNRKRISNCVADYSVLYNSASFSTFKCYGVSPTKLNDLCFTNVYADSFVIRGDEVRQIAPGQTGKIADYNYKLPDDFTGCVIAWNSNNLDSKVGGNYNYLYRLFRKSNLKPFERDISTEIYQAGSTPCNGVEGFNCYFPLQSYGFQPTNGVGYQPYRVVVLSFELLHAPATVCGPKKSTNLVKNKCVNFNFNGLTGTGVLTESNKKFLPFQQFGRDIADTTDAVRDPQTLEILDITPCSFGGVSVITPGTNTSNQVAVLYQDVNCTEVPVAIHADQLTPTWRVYSTGSNVFQTRAGCLIGAEHVNNSYECDIPIGAGICASYQTQTNSPRRARSVASQSIIAYTMSLGAENSVAYSNNSIAIPTNFTISVTTEILPVSMTKTSVDCTMYICGDSTECSNLLLQYGSFCTQLNRALTGIAVEQDKNTQEVFAQVKQIYKTPPIKDFGGFNFSQILPDPSKPSKRSFIEDLLFNKVTLADAGFIKQYGDCLGDIAARDLICAQKFNGLTVLPPLLTDEMIAQYTSALLAGTITSGWTFGAGAALQIPFAMQMAYRFNGIGVTQNVLYENQKLIANQFNSAIGKIQDSLSSTASALGKLQDVVNQNAQALNTLVKQLSSNFGAISSVLNDILSRLDKVEAEVQIDRLITGRLQSLQTYVTQQLIRAAEIRASANLAATKMSECVLGQSKRVDFCGKGYHLMSFPQSAPHGVVFLHVTYVPAQEKNFTTAPAICHDGKAHFPREGVFVSNGTHWFVTQRNFYEPQIITTDNTFVSGNCDVVIGIVNNTVYDPLQPELDSFKEELDKYFKNHTSPDVDLGDISGINASVVNIQKEIDRLNEVAKNLNESLIDLQELGKYEQYIKWPWYIWLGFIAGLIAIVMVTIMLCCMTSCCSCLKGCCSCGSCCKFDEDDSEPVLKGVKLHYT

SEQ ID NO: 2 - RNA, 3819 nt, synthetic construct
  misc_feature 1..3819: note = Coding Sequence
  source 1..3819: mol_type = other RNA
atgtttgtgtttcttgtgctgctgcctcttgtgtcttctcagtgtgtgaatttgacaacaagaacacagctgccaccagcttatacaaattcttttaccagaggagtgtattatcctgataaagtgtttagatcttctgtgctgcacagcacacaggacctgtttctgccattttttagcaatgtgacatggtttcatgcaattcatgtgtctggaacaaatggaacaaaaagatttgataatcctgtgctgccttttaatgatggagtgtattttgcttcaacagaaaagtcaaatattattagaggatggatttttggaacaacactggattctaaaacacagtctctgctgattgtgaataatgcaacaaatgtggtgattaaagtgtgtgaatttcagttttgtaatgatccttttctgggagtgtattatcacaaaaataataaatcttggatggaatctgaatttagagtgtattcctctgcaaataattgtacatttgaatatgtgtctcagccttttctgatggatctggaaggaaaacagggcaattttaaaaatctgagagaatttgtgtttaaaaatattgatggatattttaaaatttattctaaacacacaccaattaatttagtgagagatctgcctcagggattttctgctctggaacctctggtggatctgccaattggcattaatattacaagatttcagacactgctggctctgcacagatcttatctgacacctggagattcttcttctggatggacagccggagctgcagcttattatgtgggctatctgcagccaagaacatttctgctgaaatataatgaaaatggaacaattacagatgctgtggattgtgctctggatcctctgtctgaaacaaaatgtacattaaaatcttttacagtggaaaaaggcatttatcagacatctaattttagagtgcagccaacagaatctattgtgagatttccaaatattacaaatctgtgtccatttggagaagtgtttaatgcaacaagatttgcatctgtgtatgcatggaatagaaaaagaatttctaattgtgtggctgattattctgtgctgtataatagtgcttctttttccacatttaaatgttatggagtgtctccaacaaaattaaatgatttatgttttacaaatgtgtatgctgattcttttgtgatcagaggtgatgaagtgagacagattgcccccggacagacaggaaaaattgctgattacaattacaaactgcctgatgattttacaggatgtgtgattgcttggaattctaataatttagattctaaagtgggaggaaattacaattatctgtacagactgtttagaaaatcaaatctgaaaccttttgaaagagatatttcaacagaaatttatcaggctggatcaacaccttgtaatggagtggaaggatttaattgttattttccattacagagctatggatttcagccaaccaatggtgtgggatatcagccatatagagtggtggtgctgtcttttgaactgctgcatgcacctgcaacagtgtgtggacctaaaaaatctacaaatttagtgaaaaataaatgtgtgaattttaattttaatggattaacaggaacaggagtgctgacagaatctaataaaaaatttctgccttttcagcagtttggcagagatattgcagataccacagatgcagtgagagatcctcagacattagaaattctggatattacaccttgttcttttgggggtgtgtctgtgattacacctggaacaaatacatctaatcaggtggctgtgctgtatcaggatgtgaattgtacagaagtgccagtggcaattcatgcagatcagctgacaccaacatggagagtgtattctacaggatctaatgtgtttcagacaagagcaggatgtctgattggagcagaacatgtgaataattcttatgaatgtgatattccaattggagcaggcatttgtgcatcttatcagacacagacaaattccccaaggagagcaagatctgtggcatctcagtctattattgcatacaccatgtctctgggagcagaaaattctgtggcatattctaataattctattgctattccaacaaattttaccatttctgtgacaacagaaattttacctgtgtctatgacaaaaacatctgtggattgtaccatgtacatttgtggagattctacagaatgttctaatctgctgctgcagtatggatctttttgtacacagctgaatagagctttaacaggaattgctgtggaacaggataaaaatacacaggaagtgtttgctcaggtgaaacagatttacaaaacaccaccaattaaagattttggaggatttaattttagccagattctgcctgatccttctaaaccttctaaaagatcttttattgaagatctgctgtttaataaagtgacactggcagatgcaggatttattaaacagtatggagattgcctgggtgatattgctgcaagagatctgatttgtgctcagaaatttaatggactgacagtgctgcctcctctgctgacagatgaaatgattgctcagtacacatctgctttactggctggaacaattacaagcggatggacatttggagctggagctgctctgcagattccttttgcaatgcagatggcttacagatttaatggaattggagtgacacagaatgtgttatatgaaaatcagaaactgattgcaaatcagtttaattctgcaattggcaaaattcaggattctctgtcttctacagcttctgctctgggaaaactgcaggatgtggtgaatcagaatgcacaggcactgaatactctggtgaaacagctgtctagcaattttggggcaatttcttctgtgctgaatgatattctgtctagactggataaagtggaagctgaagtgcagattgatagactgatcacaggaagactgcagtctctgcagacttatgtgacacagcagctgattagagctgctgaaattagagcttctgctaatctggctgctacaaaaatgtctgaatgtgtgctgggacagtcaaaaagagtggatttttgtggaaaaggatatcatctgatgtcttttccacagtctgctccacatggagtggtgtttttacatgtgacatatgtgccagcacaggaaaagaattttaccacagcaccagcaatttgtcatgatggaaaagcacattttccaagagaaggagtgtttgtgtctaatggaacacattggtttgtgacacagagaaatttttatgaacctcagattattacaacagataatacatttgtgtcaggaaattgtgatgtggtgattggaattgtgaataatacagtgtatgatccactgcagccagaactggattcttttaaagaagaactggataaatattttaaaaatcacacatctcctgatgtggatttaggagatatttctggaatcaatgcatctgtggtgaatattcagaaagaaattgatagactgaatgaagtggccaaaaatctgaatgaatctctgattgatctgcaggaacttggaaaatatgaacagtacattaaatggccttggtacatttggcttggatttattgcaggattaattgcaattgtgatggtgacaattatgttatgttgtatgacatcatgttgttcttgtttaaaaggatgttgttcttgtggaagctgttgtaaatttgatgaagatgattctgaacctgtgttaaaaggagtgaaattgcattacaca

SEQ ID NO: 3 - protein, 218 aa, synthetic construct
  REGION 1..218: note = S Protein RBD Fusion
MFVFLVLLPLVSSQCVVRFPNITNLCPFGEVFNATRFASVYAWNRKRISNCVADYSVLYNSASFSTFKCYGVSPTKLNDLCFTNVYADSFVIRGDEVRQIAPGQTGKIADYNYKLPDDFTGCVIAWNSNNLDSKVGGNYNYLYRLFRKSNLKPFERDISTEIYQAGSTPCNGVEGFNCYFPLQSYGFQPTNGVGYQPYRVVVLSFELLHAPATVCGPK

SEQ ID NO: 4 - RNA, 654 nt, synthetic construct
  misc_feature 1..654: note = Coding Sequence
  source 1..654: mol_type = other RNA
atgtttgtgtttcttgtgctgctgcctcttgtgtcttctcagtgtgtggtgagatttccaaatattacaaatctgtgtccatttggagaagtgtttaatgcaacaagatttgcatctgtgtatgcatggaatagaaaaagaatttctaattgtgtggctgattattctgtgctgtataatagtgcttctttttccacatttaaatgttatggagtgtctccaacaaaattaaatgatttatgttttacaaatgtgtatgctgattcttttgtgatcagaggtgatgaagtgagacagattgcccccggacagacaggaaaaattgctgattacaattacaaactgcctgatgattttacaggatgtgtgattgcttggaattctaataatttagattctaaagtgggaggaaattacaattatctgtacagactgtttagaaaatcaaatctgaaaccttttgaaagagatatttcaacagaaatttatcaggctggatcaacaccttgtaatggagtggaaggatttaattgttattttccattacagagctatggatttcagccaaccaatggtgtgggatatcagccatatagagtggtggtgctgtcttttgaactgctgcatgcacctgcaacagtgtgtggacctaaa

SEQ ID NO: 5 - protein, 266 aa, synthetic construct
  REGION 1..266: note = S Protein RBD Fusion
MFVFLVLLPLVSSQCVVRFPNITNLCPFGEVFNATRFASVYAWNRKRISNCVADYSVLYNSASFSTFKCYGVSPTKLNDLCFTNVYADSFVIRGDEVRQIAPGQTGKIADYNYKLPDDFTGCVIAWNSNNLDSKVGGNYNYLYRLFRKSNLKPFERDISTEIYQAGSTPCNGVEGFNCYFPLQSYGFQPTNGVGYQPYRVVVLSFELLHAPATVCGPKGSPGSGSGSGYIPEAPRDGQAYVRKDGEWVLLSTFLGRSLEVLFQGPG

SEQ ID NO: 6 - RNA, 798 nt, synthetic construct
  misc_feature 1..798: note = Coding Sequence
  source 1..798: mol_type = other RNA
atgtttgtgtttcttgtgctgctgcctcttgtgtcttctcagtgtgtggtgagatttccaaatattacaaatctgtgtccatttggagaagtgtttaatgcaacaagatttgcatctgtgtatgcatggaatagaaaaagaatttctaattgtgtggctgattattctgtgctgtataatagtgcttctttttccacatttaaatgttatggagtgtctccaacaaaattaaatgatttatgttttacaaatgtgtatgctgattcttttgtgatcagaggtgatgaagtgagacagattgcccccggacagacaggaaaaattgctgattacaattacaaactgcctgatgattttacaggatgtgtgattgcttggaattctaataatttagattctaaagtgggaggaaattacaattatctgtacagactgtttagaaaatcaaatctgaaaccttttgaaagagatatttcaacagaaatttatcaggctggatcaacaccttgtaatggagtggaaggatttaattgttattttccattacagagctatggatttcagccaaccaatggtgtgggatatcagccatatagagtggtggtgctgtcttttgaactgctgcatgcacctgcaacagtgtgtggacctaaaggctcccccggctccggctccggatctggttatattcctgaagctccaagagatgggcaagcttacgttcgtaaagatggcgaatgggtattactttctacctttttaggccggtccctggaggtgctgttccagggccccggc

SEQ ID NO: 7 - protein, 1273 aa, synthetic construct
  REGION 1..1273: note = S Protein Variant
MFVFLVLLPLVSSQCVNLTTRTQLPPAYTNSFTRGVYYPDKVFRSSVLHSTQDLFLPFFSNVTWFHAIHVSGTNGTKRFDNPVLPFNDGVYFASTEKSNIIRGWIFGTTLDSKTQSLLIVNNATNVVIKVCEFQFCNDPFLGVYYHKNNKSWMESEFRVYSSANNCTFEYVSQPFLMDLEGKQGNFKNLREFVFKNIDGYFKIYSKHTPINLVRDLPQGFSALEPLVDLPIGINITRFQTLLALHRSYLTPGDSSSGWTAGAAAYYVGYLQPRTFLLKYNENGTITDAVDCALDPLSETKCTLKSFTVEKGIYQTSNFRVQPTESIVRFPNITNLCPFGEVFNATRFASVYAWNRKRISNCVADYSVLYNSASFSTFKCYGVSPTKLNDLCFTNVYADSFVIRGDEVRQIAPGQTGKIADYNYKLPDDFTGCVIAWNSNNLDSKVGGNYNYLYRLFRKSNLKPFERDISTEIYQAGSTPCNGVEGFNCYFPLQSYGFQPTNGVGYQPYRVVVLSFELLHAPATVCGPKKSTNLVKNKCVNFNFNGLTGTGVLTESNKKFLPFQQFGRDIADTTDAVRDPQTLEILDITPCSFGGVSVITPGTNTSNQVAVLYQDVNCTEVPVAIHADQLTPTWRVYSTGSNVFQTRAGCLIGAEHVNNSYECDIPIGAGICASYQTQTNSPRRARSVASQSIIAYTMSLGAENSVAYSNNSIAIPTNFTISVTTEILPVSMTKTSVDCTMYICGDSTECSNLLLQYGSFCTQLNRALTGIAVEQDKNTQEVFAQVKQIYKTPPIKDFGGFNFSQILPDPSKPSKRSFIEDLLFNKVTLADAGFIKQYGDCLGDIAARDLICAQKFNGLTVLPPLLTDEMIAQYTSALLAGTITSGWTFGAGAALQIPFAMQMAYRFNGIGVTQNVLYENQKLIANQFNSAIGKIQDSLSSTASALGKLQDVVNQNAQALNTLVKQLSSNFGAISSVLNDILSRLDPPEAEVQIDRLITGRLQSLQTYVTQQLIRAAEIRASANLAATKMSECVLGQSKRVDFCGKGYHLMSFPQSAPHGVVFLHVTYVPAQEKNFTTAPAICHDGKAHFPREGVFVSNGTHWFVTQRNFYEPQIITTDNTFVSGNCDVVIGIVNNTVYDPLQPELDSFKEELDKYFKNHTSPDVDLGDISGINASVVNIQKEIDRLNEVAKNLNESLIDLQELGKYEQYIKWPWYIWLGFIAGLIAIVMVTIMLCCMTSCCSCLKGCCSCGSCCKFDEDDSEPVLKGVKLHYT

SEQ ID NO: 8 - RNA, 3819 nt, synthetic construct
  misc_feature 1..3819: note = Coding Sequence
  source 1..3819: mol_type = other RNA
atgtttgtgtttcttgtgctgctgcctcttgtgtcttctcagtgtgtgaatttgacaacaagaacacagctgccaccagcttatacaaattcttttaccagaggagtgtattatcctgataaagtgtttagatcttctgtgctgcacagcacacaggacctgtttctgccattttttagcaatgtgacatggtttcatgcaattcatgtgtctggaacaaatggaacaaaaagatttgataatcctgtgctgccttttaatgatggagtgtattttgcttcaacagaaaagtcaaatattattagaggatggatttttggaacaacactggattctaaaacacagtctctgctgattgtgaataatgcaacaaatgtggtgattaaagtgtgtgaatttcagttttgtaatgatccttttctgggagtgtattatcacaaaaataataaatcttggatggaatctgaatttagagtgtattcctctgcaaataattgtacatttgaatatgtgtctcagccttttctgatggatctggaaggaaaacagggcaattttaaaaatctgagagaatttgtgtttaaaaatattgatggatattttaaaatttattctaaacacacaccaattaatttagtgagagatctgcctcagggattttctgctctggaacctctggtggatctgccaattggcattaatattacaagatttcagacactgctggctctgcacagatcttatctgacacctggagattcttcttctggatggacagccggagctgcagcttattatgtgggctatctgcagccaagaacatttctgctgaaatataatgaaaatggaacaattacagatgctgtggattgtgctctggatcctctgtctgaaacaaaatgtacattaaaatcttttacagtggaaaaaggcatttatcagacatctaattttagagtgcagccaacagaatctattgtgagatttccaaatattacaaatctgtgtccatttggagaagtgtttaatgcaacaagatttgcatctgtgtatgcatggaatagaaaaagaatttctaattgtgtggctgattattctgtgctgtataatagtgcttctttttccacatttaaatgttatggagtgtctccaacaaaattaaatgatttatgttttacaaatgtgtatgctgattcttttgtgatcagaggtgatgaagtgagacagattgcccccggacagacaggaaaaattgctgattacaattacaaactgcctgatgattttacaggatgtgtgattgcttggaattctaataatttagattctaaagtgggaggaaattacaattatctgtacagactgtttagaaaatcaaatctgaaaccttttgaaagagatatttcaacagaaatttatcaggctggatcaacaccttgtaatggagtggaaggatttaattgttattttccattacagagctatggatttcagccaaccaatggtgtgggatatcagccatatagagtggtggtgctgtcttttgaactgctgcatgcacctgcaacagtgtgtggacctaaaaaatctacaaatttagtgaaaaataaatgtgtgaattttaattttaatggattaacaggaacaggagtgctgacagaatctaataaaaaatttctgccttttcagcagtttggcagagatattgcagataccacagatgcagtgagagatcctcagacattagaaattctggatattacaccttgttcttttgggggtgtgtctgtgattacacctggaacaaatacatctaatcaggtggctgtgctgtatcaggatgtgaattgtacagaagtgccagtggcaattcatgcagatcagctgacaccaacatggagagtgtattctacaggatctaatgtgtttcagacaagagcaggatgtctgattggagcagaacatgtgaataattcttatgaatgtgatattccaattggagcaggcatttgtgcatcttatcagacacagacaaattccccaaggagagcaagatctgtggcatctcagtctattattgcatacaccatgtctctgggagcagaaaattctgtggcatattctaataattctattgctattccaacaaattttaccatttctgtgacaacagaaattttacctgtgtctatgacaaaaacatctgtggattgtaccatgtacatttgtggagattctacagaatgttctaatctgctgctgcagtatggatctttttgtacacagctgaatagagctttaacaggaattgctgtggaacaggataaaaatacacaggaagtgtttgctcaggtgaaacagatttacaaaacaccaccaattaaagattttggaggatttaattttagccagattctgcctgatccttctaaaccttctaaaagatcttttattgaagatctgctgtttaataaagtgacactggcagatgcaggatttattaaacagtatggagattgcctgggtgatattgctgcaagagatctgatttgtgctcagaaatttaatggactgacagtgctgcctcctctgctgacagatgaaatgattgctcagtacacatctgctttactggctggaacaattacaagcggatggacatttggagctggagctgctctgcagattccttttgcaatgcagatggcttacagatttaatggaattggagtgacacagaatgtgttatatgaaaatcagaaactgattgcaaatcagtttaattctgcaattggcaaaattcaggattctctgtcttctacagcttctgctctgggaaaactgcaggatgtggtgaatcagaatgcacaggcactgaatactctggtgaaacagctgtctagcaattttggggcaatttcttctgtgctgaatgatattctgtctagactggatcctcctgaagctgaagtgcagattgatagactgatcacaggaagactgcagtctctgcagacttatgtgacacagcagctgattagagctgctgaaattagagcttctgctaatctggctgctacaaaaatgtctgaatgtgtgctgggacagtcaaaaagagtggatttttgtggaaaaggatatcatctgatgtcttttccacagtctgctccacatggagtggtgtttttacatgtgacatatgtgccagcacaggaaaagaattttaccacagcaccagcaatttgtcatgatggaaaagcacattttccaagagaaggagtgtttgtgtctaatggaacacattggtttgtgacacagagaaatttttatgaacctcagattattacaacagataatacatttgtgtcaggaaattgtgatgtggtgattggaattgtgaataatacagtgtatgatccactgcagccagaactggattcttttaaagaagaactggataaatattttaaaaatcacacatctcctgatgtggatttaggagatatttctggaatcaatgcatctgtggtgaatattcagaaagaaattgatagactgaatgaagtggccaaaaatctgaatgaatctctgattgatctgcaggaacttggaaaatatgaacagtacattaaatggccttggtacatttggcttggatttattgcaggattaattgcaattgtgatggtgacaattatgttatgttgtatgacatcatgttgttcttgtttaaaaggatgttgttcttgtggaagctgttgtaaatttgatgaagatgattctgaacctgtgttaaaaggagtgaaattgcattacaca

SEQ ID NO: 9 - RNA, 3819 nt, synthetic construct
  misc_feature 1..3819: note = Coding Sequence
  source 1..3819: mol_type = other RNA
atgttcgtgttcctggtgctgctgcctctggtgtccagccagtgtgtgaacctgaccaccagaacacagctgcctccagcctacaccaacagctttaccagaggcgtgtactaccccgacaaggtgttcagatccagcgtgctgcactctacccaggacctgttcctgcctttcttcagcaacgtgacctggttccacgccatccacgtgtccggcaccaatggcaccaagagattcgacaaccccgtgctgcccttcaacgacggggtgtactttgccagcaccgagaagtccaacatcatcagaggctggatcttcggcaccacactggacagcaagacccagagcctgctgatcgtgaacaacgccaccaacgtggtcatcaaagtgtgcgagttccagttctgcaacgaccccttcctgggcgtctactaccacaagaacaacaagagctggatggaaagcgagttccgggtgtacagcagcgccaacaactgcaccttcgagtacgtgtcccagcctttcctgatggacctggaaggcaagcagggcaacttcaagaacctgcgcgagttcgtgtttaagaacatcgacggctacttcaagatctacagcaagcacacccctatcaacctcgtgcgggatctgcctcagggcttctctgctctggaacccctggtggatctgcccatcggcatcaacatcacccggtttcagacactgctggccctgcacagaagctacctgacacctggcgatagcagcagcggatggacagctggtgccgccgcttactatgtgggctacctgcagcctagaaccttcctgctgaagtacaacgagaacggcaccatcaccgacgccgtggattgtgctctggatcctctgagcgagacaaagtgcaccctgaagtccttcaccgtggaaaagggcatctaccagaccagcaacttccgggtgcagcccaccgaatccatcgtgcggttccccaatatcaccaatctgtgccccttcggcgaggtgttcaatgccaccagattcgcctctgtgtacgcctggaaccggaagcggatcagcaattgcgtggccgactactccgtgctgtacaactccgccagcttcagcaccttcaagtgctacggcgtgtcccctaccaagctgaacgacctgtgcttcacaaacgtgtacgccgacagcttcgtgatccggggagatgaagtgcggcagattgcccctggacagacaggcaagatcgccgactacaactacaagctgcccgacgacttcaccggctgtgtgattgcctggaacagcaacaacctggactccaaagtcggcggcaactacaattacctgtaccggctgttccggaagtccaatctgaagcccttcgagcgggacatctccaccgagatctatcaggccggcagcaccccttgtaacggcgtggaaggcttcaactgctacttcccactgcagtcctacggctttcagcccacaaatggcgtgggctatcagccctacagagtggtggtgctgagcttcgaactgctgcatgcccctgccacagtgtgcggccctaagaaaagcaccaatctcgtgaagaacaaatgcgtgaacttcaacttcaacggcctgaccggcaccggcgtgctgacagagagcaacaagaagttcctgccattccagcagtttggccgggatatcgccgataccacagacgccgttagagatccccagacactggaaatcctggacatcaccccttgcagcttcggcggagtgtctgtgatcacccctggcaccaacaccagcaatcaggtggcagtgctgtaccaggacgtgaactgtaccgaagtgcccgtggccattcacgccgatcagctgacacctacatggcgggtgtactccaccggcagcaatgtgtttcagaccagagccggctgtctgatcggagccgagcacgtgaacaatagctacgagtgcgacatccccatcggcgctggaatctgcgccagctaccagacacagacaaacagccctcggagagccagaagcgtggccagccagagcatcattgcctacacaatgtctctgggcgccgagaacagcgtggcctactccaacaactctatcgctatccccaccaacttcaccatcagcgtgaccacagagatcctgcctgtgtccatgaccaagaccagcgtggactgcaccatgtacatctgcggcgattccaccgagtgctccaacctgctgctgcagtacggcagcttctgcacccagctgaatagagccctgacagggatcgccgtggaacaggacaagaacacccaagaggtgttcgcccaagtgaagcagatctacaagacccctcctatcaaggacttcggcggcttcaatttcagccagattctgcccgatcctagcaagcccagcaagcggagcttcatcgaggacctgctgttcaacaaagtgacactggccgacgccggcttcatcaagcagtatggcgattgtctgggcgacattgccgccagggatctgatttgcgcccagaagtttaacggactgacagtgctgcctcctctgctgaccgatgagatgatcgcccagtacacatctgccctgctggccggcacaatcacaagcggctggacatttggagcaggcgccgctctgcagatcccctttgctatgcagatggcctaccggttcaacggcatcggagtgacccagaatgtgctgtacgagaaccagaagctgatcgccaaccagttcaacagcgccatcggcaagatccaggacagcctgagcagcacagcaagcgccctgggaaagctgcaggacgtggtcaaccagaatgcccaggcactgaacaccctggtcaagcagctgtcctccaacttcggcgccatcagctctgtgctgaacgatatcctgagcagactggaccctcctgaggccgaggtgcagatcgacagactgatcacaggcagactgcagagcctccagacatacgtgacccagcagctgatcagagccgccgagattagagcctctgccaatctggccgccaccaagatgtctgagtgtgtgctgggccagagcaagagagtggacttttgcggcaagggctaccacctgatgagcttccctcagtctgcccctcacggcgtggtgtttctgcacgtgacatatgtgcccgctcaagagaagaatttcaccaccgctccagccatctgccacgacggcaaagcccactttcctagagaaggcgtgttcgtgtccaacggcacccattggttcgtgacacagcggaacttctacgagccccagatcatcaccaccgacaacaccttcgtgtctggcaactgcgacgtcgtgatcggcattgtgaacaataccgtgtacgaccctctgcagcccgagctggacagcttcaaagaggaactggacaagtactttaagaaccacacaagccccgacgtggacctgggcgatatcagcggaatcaatgccagcgtcgtgaacatccagaaagagatcgaccggctgaacgaggtggccaagaatctgaacgagagcctgatcgacctgcaagaactggggaagtacgagcagtacatcaagtggccctggtacatctggctgggctttatcgccggactgattgccatcgtgatggtcacaatcatgctgtgttgcatgaccagctgctgtagctgcctgaagggctgttgtagctgtggcagctgctgcaagttcgacgaggacgattctgagcccgtgctgaagggcgtgaaactgcactacaca

SEQ ID NO: 10 - protein, 41 aa, synthetic construct
  REGION 1..41: note = Foldon Sequence
GSGYIPEAPRDGQAYVRKDGEWVLLSTFLGRSLEVLFQGPG

SEQ ID NO: 11 - RNA, 123 nt, synthetic construct
  misc_feature 1..123: note = Coding Sequence
  source 1..123: mol_type = other RNA
ggatctggttatattcctgaagctccaagagatgggcaagcttacgttcgtaaagatggcgaatgggtattactttctacctttttaggccggtccctggaggtgctgttccagggccccggc

SEQ ID NO: 12 - RNA, 47 nt, synthetic construct
  misc_feature 1..47: note = 5'-UTR
  source 1..47: mol_type = other RNA
aactagtattcttctggtccccacagactcagagagaacccgccacc

SEQ ID NO: 13 - RNA, 278 nt, synthetic construct
  misc_feature 1..278: note = 3'-UTR
  source 1..278: mol_type = other RNA
ctggtactgcatgcacgcaatgctagctgcccctttcccgtcctgggtaccccgagtctcccccgacctcgggtcccaggtatgctcccacctccacctgccccactcaccacctctgctagttccagacacctcccaagcacgcagcaatgcagctcaaaacgcttagcctagccacacccccacgggaaacagcagtgattaacctttagcaataaacgaaagtttaactaagctatactaaccccagggttggtcaatttcgtgccagccacacc

SEQ ID NO: 14 - RNA, 110 nt, synthetic construct
  misc_feature 1..110: note = A30L70
  source 1..110: mol_type = other RNA
aaaaaaaaaaaaaaaaaaaaaaaaaaaaaagcatatgactaaaaaaaaaaaaaaaaaaaaaaaaaaaaaaaaaaaaaaaaaaaaaaaaaaaaaaaaaaaaaaaaaaaaaa

SEQ ID NO: 15 - RNA, 4282 nt, synthetic construct
  misc_feature 1..4282: note = RBL063.1
  source 1..4282: mol_type = other RNA
gggcgaactagtattcttctggtccccacagactcagagagaacccgccaccatgtttgtgtttcttgtgctgctgcctcttgtgtcttctcagtgtgtgaatttgacaacaagaacacagctgccaccagcttatacaaattcttttaccagaggagtgtattatcctgataaagtgtttagatcttctgtgctgcacagcacacaggacctgtttctgccattttttagcaatgtgacatggtttcatgcaattcatgtgtctggaacaaatggaacaaaaagatttgataatcctgtgctgccttttaatgatggagtgtattttgcttcaacagaaaagtcaaatattattagaggatggatttttggaacaacactggattctaaaacacagtctctgctgattgtgaataatgcaacaaatgtggtgattaaagtgtgtgaatttcagttttgtaatgatccttttctgggagtgtattatcacaaaaataataaatcttggatggaatctgaatttagagtgtattcctctgcaaataattgtacatttgaatatgtgtctcagccttttctgatggatctggaaggaaaacagggcaattttaaaaatctgagagaatttgtgtttaaaaatattgatggatattttaaaatttattctaaacacacaccaattaatttagtgagagatctgcctcagggattttctgctctggaacctctggtggatctgccaattggcattaatattacaagatttcagacactgctggctctgcacagatcttatctgacacctggagattcttcttctggatggacagccggagctgcagcttattatgtgggctatctgcagccaagaacatttctgctgaaatataatgaaaatggaacaattacagatgctgtggattgtgctctggatcctctgtctgaaacaaaatgtacattaaaatcttttacagtggaaaaaggcatttatcagacatctaattttagagtgcagccaacagaatctattgtgagatttccaaatattacaaatctgtgtccatttggagaagtgtttaatgcaacaagatttgcatctgtgtatgcatggaatagaaaaagaatttctaattgtgtggctgattattctgtgctgtataatagtgcttctttttccacatttaaatgttatggagtgtctccaacaaaattaaatgatttatgttttacaaatgtgtatgctgattcttttgtgatcagaggtgatgaagtgagacagattgcccccggacagacaggaaaaattgctgattacaattacaaactgcctgatgattttacaggatgtgtgattgcttggaattctaataatttagattctaaagtgggaggaaattacaattatctgtacagactgtttagaaaatcaaatctgaaaccttttgaaagagatatttcaacagaaatttatcaggctggatcaacaccttgtaatggagtggaaggatttaattgttattttccattacagagctatggatttcagccaaccaatggtgtgggatatcagccatatagagtggtggtgctgtcttttgaactgctgcatgcacctgcaacagtgtgtggacctaaaaaatctacaaatttagtgaaaaataaatgtgtgaattttaattttaatggattaacaggaacaggagtgctgacagaatctaataaaaaatttctgccttttcagcagtttggcagagatattgcagataccacagatgcagtgagagatcctcagacattagaaattctggatattacaccttgttcttttgggggtgtgtctgtgattacacctggaacaaatacatctaatcaggtggctgtgctgtatcaggatgtgaattgtacagaagtgccagtggcaattcatgcagatcagctgacaccaacatggagagtgtattctacaggatctaatgtgtttcagacaagagcaggatgtctgattggagcagaacatgtgaataattcttatgaatgtgatattccaattggagcaggcatttgtgcatcttatcagacacagacaaattccccaaggagagcaagatctgtggcatctcagtctattattgcatacaccatgtctctgggagcagaaaattctgtggcatattctaataattctattgctattccaacaaattttaccatttctgtgacaacagaaattttacctgtgtctatgacaaaaacatctgtggattgtaccatgtacatttgtggagattctacagaatgttctaatctgctgctgcagtatggatctttttgtacacagctgaatagagctttaacaggaattgctgtggaacaggataaaaatacacaggaagtgtttgctcaggtgaaacagatttacaaaacaccaccaattaaagattttggaggatttaattttagccagattctgcctgatccttctaaaccttctaaaagatcttttattgaagatctgctgtttaataaagtgacactggcagatgcaggatttattaaacagtatggagattgcctgggtgatattgctgcaagagatctgatttgtgctcagaaatttaatggactgacagtgctgcctcctctgctgacagatgaaatgattgctcagtacacatctgctttactggctggaacaattacaagcggatggacatttggagctggagctgctctgcagattccttttgcaatgcagatggcttacagatttaatggaattggagtgacacagaatgtgttatatgaaaatcagaaactgattgcaaatcagtttaattctgcaattggcaaaattcaggattctctgtcttctacagcttctgctctgggaaaactgcaggatgtggtgaatcagaatgcacaggcactgaatactctggtgaaacagctgtctagcaattttggggcaatttcttctgtgctgaatgatattctgtctagactggatcctcctgaagctgaagtgcagattgatagactgatcacaggaagactgcagtctctgcagacttatgtgacacagcagctgattagagctgctgaaattagagcttctgctaatctggctgctacaaaaatgtctgaatgtgtgctgggacagtcaaaaagagtggatttttgtggaaaaggatatcatctgatgtcttttccacagtctgctccacatggagtggtgtttttacatgtgacatatgtgccagcacaggaaaagaattttaccacagcaccagcaatttgtcatgatggaaaagcacattttccaagagaaggagtgtttgtgtctaatggaacacattggtttgtgacacagagaaatttttatgaacctcagattattacaacagataatacatttgtgtcaggaaattgtgatgtggtgattggaattgtgaataatacagtgtatgatccactgcagccagaactggattcttttaaagaagaactggataaatattttaaaaatcacacatctcctgatgtggatttaggagatatttctggaatcaatgcatctgtggtgaatattcagaaagaaattgatagactgaatgaagtggccaaaaatctgaatgaatctctgattgatctgcaggaacttggaaaatatgaacagtacattaaatggccttggtacatttggcttggatttattgcaggattaattgcaattgtgatggtgacaattatgttatgttgtatgacatcatgttgttcttgtttaaaaggatgttgttcttgtggaagctgttgtaaatttgatgaagatgattctgaacctgtgttaaaaggagtgaaattgcattacacatgatgactcgagctggtactgcatgcacgcaatgctagctgcccctttcccgtcctgggtaccccgagtctcccccgacctcgggtcccaggtatgctcccacctccacctgccccactcaccacctctgctagttccagacacctcccaagcacgcagcaatgcagctcaaaacgcttagcctagccacacccccacgggaaacagcagtgattaacctttagcaataaacgaaagtttaactaagctatactaaccccagggttggtcaatttcgtgccagccacaccctggagctagcaaaaaaaaaaaaaaaaaaaaaaaaaaaaaagcatatgactaaaaaaaaaaaaaaaaaaaaaaaaaaaaaaaaaaaaaaaaaaaaaaaaaaaaaaaaaaaaaaaaaaaaaa

SEQ ID NO: 16 - RNA, 4282 nt, synthetic construct
  misc_feature 1..4282: note = RBL063.2
  source 1..4282: mol_type = other RNA
gggcgaactagtattcttctggtccccacagactcagagagaacccgccaccatgttcgtgttcctggtgctgctgcctctggtgtccagccagtgtgtgaacctgaccaccagaacacagctgcctccagcctacaccaacagctttaccagaggcgtgtactaccccgacaaggtgttcagatccagcgtgctgcactctacccaggacctgttcctgcctttcttcagcaacgtgacctggttccacgccatccacgtgtccggcaccaatggcaccaagagattcgacaaccccgtgctgcccttcaacgacggggtgtactttgccagcaccgagaagtccaacatcatcagaggctggatcttcggcaccacactggacagcaagacccagagcctgctgatcgtgaacaacgccaccaacgtggtcatcaaagtgtgcgagttccagttctgcaacgaccccttcctgggcgtctactaccacaagaacaacaagagctggatggaaagcgagttccgggtgtacagcagcgccaacaactgcaccttcgagtacgtgtcccagcctttcctgatggacctggaaggcaagcagggcaacttcaagaacctgcgcgagttcgtgtttaagaacatcgacggctacttcaagatctacagcaagcacacccctatcaacctcgtgcgggatctgcctcagggcttctctgctctggaacccctggtggatctgcccatcggcatcaacatcacccggtttcagacactgctggccctgcacagaagctacctgacacctggcgatagcagcagcggatggacagctggtgccgccgcttactatgtgggctacctgcagcctagaaccttcctgctgaagtacaacgagaacggcaccatcaccgacgccgtggattgtgctctggatcctctgagcgagacaaagtgcaccctgaagtccttcaccgtggaaaagggcatctaccagaccagcaacttccgggtgcagcccaccgaatccatcgtgcggttccccaatatcaccaatctgtgccccttcggcgaggtgttcaatgccaccagattcgcctctgtgtacgcctggaaccggaagcggatcagcaattgcgtggccgactactccgtgctgtacaactccgccagcttcagcaccttcaagtgctacggcgtgtcccctaccaagctgaacgacctgtgcttcacaaacgtgtacgccgacagcttcgtgatccggggagatgaagtgcggcagattgcccctggacagacaggcaagatcgccgactacaactacaagctgcccgacgacttcaccggctgtgtgattgcctggaacagcaacaacctggactccaaagtcggcggcaactacaattacctgtaccggctgttccggaagtccaatctgaagcccttcgagcgggacatctccaccgagatctatcaggccggcagcaccccttgtaacggcgtggaaggcttcaactgctacttcccactgcagtcctacggctttcagcccacaaatggcgtgggctatcagccctacagagtggtggtgctgagcttcgaactgctgcatgcccctgccacagtgtgcggccctaagaaaagcaccaatctcgtgaagaacaaatgcgtgaacttcaacttcaacggcctgaccggcaccggcgtgctgacagagagcaacaagaagttcctgccattccagcagtttggccgggatatcgccgataccacagacgccgttagagatccccagacactggaaatcctggacatcaccccttgcagcttcggcggagtgtctgtgatcacccctggcaccaacaccagcaatcaggtggcagtgctgtaccaggacgtgaactgtaccgaagtgcccgtggccattcacgccgatcagctgacacctacatggcgggtgtactccaccggcagcaatgtgtttcagaccagagccggctgtctgatcggagccgagcacgtgaacaatagctacgagtgcgacatccccatcggcgctggaatctgcgccagctaccagacacagacaaacagccctcggagagccagaagcgtggccagccagagcatcattgcctacacaatgtctctgggcgccgagaacagcgtggcctactccaacaactctatcgctatccccaccaacttcaccatcagcgtgaccacagagatcctgcctgtgtccatgaccaagaccagcgtggactgcaccatgtacatctgcggcgattccaccgagtgctccaacctgctgctgcagtacggcagcttctgcacccagctgaatagagccctgacagggatcgccgtggaacaggacaagaacacccaagaggtgttcgcccaagtgaagcagatctacaagacccctcctatcaaggacttcggcggcttcaatttcagccagattctgcccgatcctagcaagcccagcaagcggagcttcatcgaggacctgctgttcaacaaagtgacactggccgacgccggcttcatcaagcagtatggcgattgtctgggcgacattgccgccagggatctgatttgcgcccagaagtttaacggactgacagtgctgcctcctctgctgaccgatgagatgatcgcccagtacacatctgccctgctggccggcacaatcacaagcggctggacatttggagcaggcgccgctctgcagatcccctttgctatgcagatggcctaccggttcaacggcatcggagtgacccagaatgtgctgtacgagaaccagaagctgatcgccaaccagttcaacagcgccatcggcaagatccaggacagcctgagcagcacagcaagcgccctgggaaagctgcaggacgtggtcaaccagaatgcccaggcactgaacaccctggtcaagcagctgtcctccaacttcggcgccatcagctctgtgctgaacgatatcctgagcagactggaccctcctgaggccgaggtgcagatcgacagactgatcacaggcagactgcagagcctccagacatacgtgacccagcagctgatcagagccgccgagattagagcctctgccaatctggccgccaccaagatgtctgagtgtgtgctgggccagagcaagagagtggacttttgcggcaagggctaccacctgatgagcttccctcagtctgcccctcacggcgtggtgtttctgcacgtgacatatgtgcccgctcaagagaagaatttcaccaccgctccagccatctgccacgacggcaaagcccactttcctagagaaggcgtgttcgtgtccaacggcacccattggttcgtgacacagcggaacttctacgagccccagatcatcaccaccgacaacaccttcgtgtctggcaactgcgacgtcgtgatcggcattgtgaacaataccgtgtacgaccctctgcagcccgagctggacagcttcaaagaggaactggacaagtactttaagaaccacacaagccccgacgtggacctgggcgatatcagcggaatcaatgccagcgtcgtgaacatccagaaagagatcgaccggctgaacgaggtggccaagaatctgaacgagagcctgatcgacctgcaagaactggggaagtacgagcagtacatcaagtggccctggtacatctggctgggctttatcgccggactgattgccatcgtgatggtcacaatcatgctgtgttgcatgaccagctgctgtagctgcctgaagggctgttgtagctgtggcagctgctgcaagttcgacgaggacgattctgagcccgtgctgaagggcgtgaaactgcactacacatgatgactcgagctggtactgcatgcacgcaatgctagctgcccctttcccgtcctgggtaccccgagtctcccccgacctcgggtcccaggtatgctcccacctccacctgccccactcaccacctctgctagttccagacacctcccaagcacgcagcaatgcagctcaaaacgcttagcctagccacacccccacgggaaacagcagtgattaacctttagcaataaacgaaagtttaactaagctatactaaccccagggttggtcaatttcgtgccagccacaccctggagctagcaaaaaaaaaaaaaaaaaaaaaaaaaaaaaagcatatgactaaaaaaaaaaaaaaaaaaaaaaaaaaaaaaaaaaaaaaaaaaaaaaaaaaaaaaaaaaaaaaaaaaaaaa

SEQ ID NO: 17 - RNA, 1261 nt, synthetic construct
  misc_feature 1..1261: note = RBL063.3
  source 1..1261: mol_type = other RNA
gggcgaactagtattcttctggtccccacagactcagagagaacccgccaccatgtttgtgtttcttgtgctgctgcctcttgtgtcttctcagtgtgtggtgagatttccaaatattacaaatctgtgtccatttggagaagtgtttaatgcaacaagatttgcatctgtgtatgcatggaatagaaaaagaatttctaattgtgtggctgattattctgtgctgtataatagtgcttctttttccacatttaaatgttatggagtgtctccaacaaaattaaatgatttatgttttacaaatgtgtatgctgattcttttgtgatcagaggtgatgaagtgagacagattgcccccggacagacaggaaaaattgctgattacaattacaaactgcctgatgattttacaggatgtgtgattgcttggaattctaataatttagattctaaagtgggaggaaattacaattatctgtacagactgtttagaaaatcaaatctgaaaccttttgaaagagatatttcaacagaaatttatcaggctggatcaacaccttgtaatggagtggaaggatttaattgttattttccattacagagctatggatttcagccaaccaatggtgtgggatatcagccatatagagtggtggtgctgtcttttgaactgctgcatgcacctgcaacagtgtgtggacctaaaggctcccccggctccggctccggatctggttatattcctgaagctccaagagatgggcaagcttacgttcgtaaagatggcgaatgggtattactttctacctttttaggccggtccctggaggtgctgttccagggccccggctgatgactcgagctggtactgcatgcacgcaatgctagctgcccctttcccgtcctgggtaccccgagtctcccccgacctcgggtcccaggtatgctcccacctccacctgccccactcaccacctctgctagttccagacacctcccaagcacgcagcaatgcagctcaaaacgcttagcctagccacacccccacgggaaacagcagtgattaacctttagcaataaacgaaagtttaactaagctatactaaccccagggttggtcaatttcgtgccagccacaccctggagctagcaaaaaaaaaaaaaaaaaaaaaaaaaaaaaagcatatgactaaaaaaaaaaaaaaaaaaaaaaaaaaaaaaaaaaaaaaaaaaaaaaaaaaaaaaaaaaaaaaaaaaaaaa

SEQ ID NO: 18 - protein, 250 aa, synthetic construct
  REGION 1..250: note = S Protein RBD Fusion
VRFPNITNLCPFGEVFNATRFASVYAWNRKRISNCVADYSVLYNSASFSTFKCYGVSPTKLNDLCFTNVYADSFVIRGDEVRQIAPGQTGKIADYNYKLPDDFTGCVIAWNSNNLDSKVGGNYNYLYRLFRKSNLKPFERDISTEIYQAGSTPCNGVEGFNCYFPLQSYGFQPTNGVGYQPYRVVVLSFELLHAPATVCGPKGSPGSGSGSGYIPEAPRDGQAYVRKDGEWVLLSTFLGRSLEVLFQGPG

SEQ ID NO: 19 - RNA, 4283 nt, synthetic construct
  misc_feature 1..4283: note = RBP020.1
  source 1..4283: mol_type = other RNA
agaataaactagtattcttctggtccccacagactcagagagaacccgccaccatgtttgtgtttcttgtgctgctgcctcttgtgtcttctcagtgtgtgaatttgacaacaagaacacagctgccaccagcttatacaaattcttttaccagaggagtgtattatcctgataaagtgtttagatcttctgtgctgcacagcacacaggacctgtttctgccattttttagcaatgtgacatggtttcatgcaattcatgtgtctggaacaaatggaacaaaaagatttgataatcctgtgctgccttttaatgatggagtgtattttgcttcaacagaaaagtcaaatattattagaggatggatttttggaacaacactggattctaaaacacagtctctgctgattgtgaataatgcaacaaatgtggtgattaaagtgtgtgaatttcagttttgtaatgatccttttctgggagtgtattatcacaaaaataataaatcttggatggaatctgaatttagagtgtattcctctgcaaataattgtacatttgaatatgtgtctcagccttttctgatggatctggaaggaaaacagggcaattttaaaaatctgagagaatttgtgtttaaaaatattgatggatattttaaaatttattctaaacacacaccaattaatttagtgagagatctgcctcagggattttctgctctggaacctctggtggatctgccaattggcattaatattacaagatttcagacactgctggctctgcacagatcttatctgacacctggagattcttcttctggatggacagccggagctgcagcttattatgtgggctatctgcagccaagaacatttctgctgaaatataatgaaaatggaacaattacagatgctgtggattgtgctctggatcctctgtctgaaacaaaatgtacattaaaatcttttacagtggaaaaaggcatttatcagacatctaattttagagtgcagccaacagaatctattgtgagatttccaaatattacaaatctgtgtccatttggagaagtgtttaatgcaacaagatttgcatctgtgtatgcatggaatagaaaaagaatttctaattgtgtggctgattattctgtgctgtataatagtgcttctttttccacatttaaatgttatggagtgtctccaacaaaattaaatgatttatgttttacaaatgtgtatgctgattcttttgtgatcagaggtgatgaagtgagacagattgcccccggacagacaggaaaaattgctgattacaattacaaactgcctgatgattttacaggatgtgtgattgcttggaattctaataatttagattctaaagtgggaggaaattacaattatctgtacagactgtttagaaaatcaaatctgaaaccttttgaaagagatatttcaacagaaatttatcaggctggatcaacaccttgtaatggagtggaaggatttaattgttattttccattacagagctatggatttcagccaaccaatggtgtgggatatcagccatatagagtggtggtgctgtcttttgaactgctgcatgcacctgcaacagtgtgtggacctaaaaaatctacaaatttagtgaaaaataaatgtgtgaattttaattttaatggattaacaggaacaggagtgctgacagaatctaataaaaaatttctgccttttcagcagtttggcagagatattgcagataccacagatgcagtgagagatcctcagacattagaaattctggatattacaccttgttcttttgggggtgtgtctgtgattacacctggaacaaatacatctaatcaggtggctgtgctgtatcaggatgtgaattgtacagaagtgccagtggcaattcatgcagatcagctgacaccaacatggagagtgtattctacaggatctaatgtgtttcagacaagagcaggatgtctgattggagcagaacatgtgaataattcttatgaatgtgatattccaattggagcaggcatttgtgcatcttatcagacacagacaaattccccaaggagagcaagatctgtggcatctcagtctattattgcatacaccatgtctctgggagcagaaaattctgtggcatattctaataattctattgctattccaacaaattttaccatttctgtgacaacagaaattttacctgtgtctatgacaaaaacatctgtggattgtaccatgtacatttgtggagattctacagaatgttctaatctgctgctgcagtatggatctttttgtacacagctgaatagagctttaacaggaattgctgtggaacaggataaaaatacacaggaagtgtttgctcaggtgaaacagatttacaaaacaccaccaattaaagattttggaggatttaattttagccagattctgcctgatccttctaaaccttctaaaagatcttttattgaagatctgctgtttaataaagtgacactggcagatgcaggatttattaaacagtatggagattgcctgggtgatattgctgcaagagatctgatttgtgctcagaaatttaatggactgacagtgctgcctcctctgctgacagatgaaatgattgctcagtacacatctgctttactggctggaacaattacaagcggatggacatttggagctggagctgctctgcagattccttttgcaatgcagatggcttacagatttaatggaattggagtgacacagaatgtgttatatgaaaatcagaaactgattgcaaatcagtttaattctgcaattggcaaaattcaggattctctgtcttctacagcttctgctctgggaaaactgcaggatgtggtgaatcagaatgcacaggcactgaatactctggtgaaacagctgtctagcaattttggggcaatttcttctgtgctgaatgatattctgtctagactggatcctcctgaagctgaagtgcagattgatagactgatcacaggaagactgcagtctctgcagacttatgtgacacagcagctgattagagctgctgaaattagagcttctgctaatctggctgctacaaaaatgtctgaatgtgtgctgggacagtcaaaaagagtggatttttgtggaaaaggatatcatctgatgtcttttccacagtctgctccacatggagtggtgtttttacatgtgacatatgtgccagcacaggaaaagaattttaccacagcaccagcaatttgtcatgatggaaaagcacattttccaagagaaggagtgtttgtgtctaatggaacacattggtttgtgacacagagaaatttttatgaacctcagattattacaacagataatacatttgtgtcaggaaattgtgatgtggtgattggaattgtgaataatacagtgtatgatccactgcagccagaactggattcttttaaagaagaactggataaatattttaaaaatcacacatctcctgatgtggatttaggagatatttctggaatcaatgcatctgtggtgaatattcagaaagaaattgatagactgaatgaagtggccaaaaatctgaatgaatctctgattgatctgcaggaacttggaaaatatgaacagtacattaaatggccttggtacatttggcttggatttattgcaggattaattgcaattgtgatggtgacaattatgttatgttgtatgacatcatgttgttcttgtttaaaaggatgttgttcttgtggaagctgttgtaaatttgatgaagatgattctgaacctgtgttaaaaggagtgaaattgcattacacatgatgactcgagctggtactgcatgcacgcaatgctagctgcccctttcccgtcctgggtaccccgagtctcccccgacctcgggtcccaggtatgctcccacctccacctgccccactcaccacctctgctagttccagacacctcccaagcacgcagcaatgcagctcaaaacgcttagcctagccacacccccacgggaaacagcagtgattaacctttagcaataaacgaaagtttaactaagctatactaaccccagggttggtcaatttcgtgccagccacaccctggagctagcaaaaaaaaaaaaaaaaaaaaaaaaaaaaaagcatatgactaaaaaaaaaaaaaaaaaaaaaaaaaaaaaaaaaaaaaaaaaaaaaaaaaaaaaaaaaaaaaaaaaaaaaa

SEQ ID NO: 20 - RNA, 4283 nt, synthetic construct
  misc_feature 1..4283: note = RBP020.2
  source 1..4283: mol_type = other RNA
agaataaactagtattcttctggtccccacagactcagagagaacccgccaccatgttcgtgttcctggtgctgctgcctctggtgtccagccagtgtgtgaacctgaccaccagaacacagctgcctccagcctacaccaacagctttaccagaggcgtgtactaccccgacaaggtgttcagatccagcgtgctgcactctacccaggacctgttcctgcctttcttcagcaacgtgacctggttccacgccatccacgtgtccggcaccaatggcaccaagagattcgacaaccccgtgctgcccttcaacgacggggtgtactttgccagcaccgagaagtccaacatcatcagaggctggatcttcggcaccacactggacagcaagacccagagcctgctgatcgtgaacaacgccaccaacgtggtcatcaaagtgtgcgagttccagttctgcaacgaccccttcctgggcgtctactaccacaagaacaacaagagctggatggaaagcgagttccgggtgtacagcagcgccaacaactgcaccttcgagtacgtgtcccagcctttcctgatggacctggaaggcaagcagggcaacttcaagaacctgcgcgagttcgtgtttaagaacatcgacggctacttcaagatctacagcaagcacacccctatcaacctcgtgcgggatctgcctcagggcttctctgctctggaacccctggtggatctgcccatcggcatcaacatcacccggtttcagacactgctggccctgcacagaagctacctgacacctggcgatagcagcagcggatggacagctggtgccgccgcttactatgtgggctacctgcagcctagaaccttcctgctgaagtacaacgagaacggcaccatcaccgacgccgtggattgtgctctggatcctctgagcgagacaaagtgcaccctgaagtccttcaccgtggaaaagggcatctaccagaccagcaacttccgggtgcagcccaccgaatccatcgtgcggttccccaatatcaccaatctgtgccccttcggcgaggtgttcaatgccaccagattcgcctctgtgtacgcctggaaccggaagcggatcagcaattgcgtggccgactactccgtgctgtacaactccgccagcttcagcaccttcaagtgctacggcgtgtcccctaccaagctgaacgacctgtgcttcacaaacgtgtacgccgacagcttcgtgatccggggagatgaagtgcggcagattgcccctggacagacaggcaagatcgccgactacaactacaagctgcccgacgacttcaccggctgtgtgattgcctggaacagcaacaacctggactccaaagtcggcggcaactacaattacctgtaccggctgttccggaagtccaatctgaagcccttcgagcgggacatctccaccgagatctatcaggccggcagcaccccttgtaacggcgtggaaggcttcaactgctacttcccactgcagtcctacggctttcagcccacaaatggcgtgggctatcagccctacagagtggtggtgctgagcttcgaactgctgcatgcccctgccacagtgtgcggccctaagaaaagcaccaatctcgtgaagaacaaatgcgtgaacttcaacttcaacggcctgaccggcaccggcgtgctgacagagagcaacaagaagttcctgccattccagcagtttggccgggatatcgccgataccacagacgccgttagagatccccagacactggaaatcctggacatcaccccttgcagcttcggcggagtgtctgtgatcacccctggcaccaacaccagcaatcaggtggcagtgctgtaccaggacgtgaactgtaccgaagtgcccgtggccattcacgccgatcagctgacacctacatggcgggtgtactccaccggcagcaatgtgtttcagaccagagccggctgtctgatcggagccgagcacgtgaacaatagctacgagtgcgacatccccatcggcgctggaatctgcgccagctaccagacacagacaaacagccctcggagagccagaagcgtggccagccagagcatcattgcctacacaatgtctctgggcgccgagaacagcgtggcctactccaacaactctatcgctatccccaccaacttcaccatcagcgtgaccacagagatcctgcctgtgtccatgaccaagaccagcgtggactgcaccatgtacatctgcggcgattccaccgagtgctccaacctgctgctgcagtacggcagcttctgcacccagctgaatagagccctgacagggatcgccgtggaacaggacaagaacacccaagaggtgttcgcccaagtgaagcagatctacaagacccctcctatcaaggacttcggcggcttcaatttcagccagattctgcccgatcctagcaagcccagcaagcggagcttcatcgaggacctgctgttcaacaaagtgacactggccgacgccggcttcatcaagcagtatggcgattgtctgggcgacattgccgccagggatctgatttgcgcccagaagtttaacggactgacagtgctgcctcctctgctgaccgatgagatgatcgcccagtacacatctgccctgctggccggcacaatcacaagcggctggacatttggagcaggcgccgctctgcagatcccctttgctatgcagatggcctaccggttcaacggcatcggagtgacccagaatgtgctgtacgagaaccagaagctgatcgccaaccagttcaacagcgccatcggcaagatccaggacagcctgagcagcacagcaagcgccctgggaaagctgcaggacgtggtcaaccagaatgcccaggcactgaacaccctggtcaagcagctgtcctccaacttcggcgccatcagctctgtgctgaacgatatcctgagcagactggaccctcctgaggccgaggtgcagatcgacagactgatcacaggcagactgcagagcctccagacatacgtgacccagcagctgatcagagccgccgagattagagcctctgccaatctggccgccaccaagatgtctgagtgtgtgctgggccagagcaagagagtggacttttgcggcaagggctaccacctgatgagcttccctcagtctgcccctcacggcgtggtgtttctgcacgtgacatatgtgcccgctcaagagaagaatttcaccaccgctccagccatctgccacgacggcaaagcccactttcctagagaaggcgtgttcgtgtccaacggcacccattggttcgtgacacagcggaacttctacgagccccagatcatcaccaccgacaacaccttcgtgtctggcaactgcgacgtcgtgatcggcattgtgaacaataccgtgtacgaccctctgcagcccgagctggacagcttcaaagaggaactggacaagtactttaagaaccacacaagccccgacgtggacctgggcgatatcagcggaatcaatgccagcgtcgtgaacatccagaaagagatcgaccggctgaacgaggtggccaagaatctgaacgagagcctgatcgacctgcaagaactggggaagtacgagcagtacatcaagtggccctggtacatctggctgggctttatcgccggactgattgccatcgtgatggtcacaatcatgctgtgttgcatgaccagctgctgtagctgcctgaagggctgttgtagctgtggcagctgctgcaagttcgacgaggacgattctgagcccgtgctgaagggcgtgaaactgcactacacatgatgactcgagctggtactgcatgcacgcaatgctagctgcccctttcccgtcctgggtaccccgagtctcccccgacctcgggtcccaggtatgctcccacctccacctgccccactcaccacctctgctagttccagacacctcccaagcacgcagcaatgcagctcaaaacgcttagcctagccacacccccacgggaaacagcagtgattaacctttagcaataaacgaaagtttaactaagctatactaaccccagggttggtcaatttcgtgccagccacaccctggagctagcaaaaaaaaaaaaaaaaaaaaaaaaaaaaaagcatatgactaaaaaaaaaaaaaaaaaaaaaaaaaaaaaaaaaaaaaaaaaaaaaaaaaaaaaaaaaaaaaaaaaaaaaa

SEQ ID NO: 21 - RNA, 1262 nt, synthetic construct
  misc_feature 1..1262: note = RBP020.3
  source 1..1262: mol_type = other RNA
agaataaactagtattcttctggtccccacagactcagagagaacccgccaccatgtttgtgtttcttgtgctgctgcctcttgtgtcttctcagtgtgtggtgagatttccaaatattacaaatctgtgtccatttggagaagtgtttaatgcaacaagatttgcatctgtgtatgcatggaatagaaaaagaatttctaattgtgtggctgattattctgtgctgtataatagtgcttctttttccacatttaaatgttatggagtgtctccaacaaaattaaatgatttatgttttacaaatgtgtatgctgattcttttgtgatcagaggtgatgaagtgagacagattgcccccggacagacaggaaaaattgctgattacaattacaaactgcctgatgattttacaggatgtgtgattgcttggaattctaataatttagattctaaagtgggaggaaattacaattatctgtacagactgtttagaaaatcaaatctgaaaccttttgaaagagatatttcaacagaaatttatcaggctggatcaacaccttgtaatggagtggaaggatttaattgttattttccattacagagctatggatttcagccaaccaatggtgtgggatatcagccatatagagtggtggtgctgtcttttgaactgctgcatgcacctgcaacagtgtgtggacctaaaggctcccccggctccggctccggatctggttatattcctgaagctccaagagatgggcaagcttacgttcgtaaagatggcgaatgggtattactttctacctttttaggccggtccctggaggtgctgttccagggccccggctgatgactcgagctggtactgcatgcacgcaatgctagctgcccctttcccgtcctgggtaccccgagtctcccccgacctcgggtcccaggtatgctcccacctccacctgccccactcaccacctctgctagttccagacacctcccaagcacgcagcaatgcagctcaaaacgcttagcctagccacacccccacgggaaacagcagtgattaacctttagcaataaacgaaagtttaactaagctatactaaccccagggttggtcaatttcgtgccagccacaccctggagctagcaaaaaaaaaaaaaaaaaaaaaaaaaaaaaagcatatgactaaaaaaaaaaaaaaaaaaaaaaaaaaaaaaaaaaaaaaaaaaaaaaaaaaaaaaaaaaaaaaaaaaaaaa

SEQ ID NO: 22 - protein, 1879 aa, synthetic construct
  REGION 1..1879: note = Viral Protein
MEKVHVDIEEDSPFLRALQRSFPQFEVEAKQVTDNDHANARAFSHLASKLIETEVDPSDTILDIGSAPARRMYSKHKYHCICPMRCAEDPDRLYKYATKLKKNCKEITDKELDKKMKELAAVMSDPDLETETMCLHDDESCRYEGQVAVYQDVYAVDGPTSLYHQANKGVRVAYWIGFDTTPFMFKNLAGAYPSYSTNWADETVLTARNIGLCSSDVMERSRRGMSILRKKYLKPSNNVLFSVGSTIYHEKRDLLRSWHLPSVFHLRGKQNYTCRCETIVSCDGYVVKRIAISPGLYGKPSGYAATMHREGFLCCKVTDTLNGERVSFPVCTYVPATLCDQMTGILATDVSADDAQKLLVGLNQRIVVNGRTQRNTNTMKNYLLPVVAQAFARWAKEYKEDQEDERPLGLRDRQLVMGCCWAFRRHKITSIYKRPDTQTIIKVNSDFHSFVLPRIGSNTLEIGLRTRIRKMLEEHKEPSPLITAEDVQEAKCAADEAKEVREAEELRAALPPLAADVEEPTLEADVDLMLQEAGAGSVETPRGLIKVTSYAGEDKIGSYAVLSPQAVLKSEKLSCIHPLAEQVIVITHSGRKGRYAVEPYHGKVVVPEGHAIPVQDFQALSESATIVYNEREFVNRYLHHIATHGGALNTDEEYYKTVKPSEHDGEYLYDIDRKQCVKKELVTGLGLTGELVDPPFHEFAYESLRTRPAAPYQVPTIGVYGVPGSGKSGIIKSAVTKKDLVVSAKKENCAEIIRDVKKMKGLDVNARTVDSVLLNGCKHPVETLYIDEAFACHAGTLRALIAIIRPKKAVLCGDPKQCGFFNMMCLKVHFNHEICTQVFHKSISRRCTKSVTSVVSTLFYDKKMRTTNPKETKIVIDTTGSTKPKQDDLILTCFRGWVKQLQIDYKGNEIMTAAASQGLTRKGVYAVRYKVNENPLYAPTSEHVNVLLTRTEDRIVWKTLAGDPWIKTLTAKYPGNFTATIEEWQAEHDAIMRHILERPDPTDVFQNKANVCWAKALVPVLKTAGIDMTTEQWNTVDYFETDKAHSAEIVLNQLCVRFFGLDLDSGLFSAPTVPLSIRNNHWDNSPSPNMYGLNKEVVRQLSRRYPQLPRAVATGRVYDMNTGTLRNYDPRINLVPVNRRLPHALVLHHNEHPQSDFSSFVSKLKGRTVLVVGEKLSVPGKMVDWLSDRPEATFRARLDLGIPGDVPKYDIIFVNVRTPYKYHHYQQCEDHAIKLSMLTKKACLHLNPGGTCVSIGYGYADRASESIIGAIARQFKFSRVCKPKSSLEETEVLFVFIGYDRKARTHNPYKLSSTLTNIYTGSRLHEAGCAPSYHVVRGDIATATEGVIINAANSKGQPGGGVCGALYKKFPESFDLQPIEVGKARLVKGAAKHIIHAVGPNFNKVSEVEGDKQLAEAYESIAKIVNDNNYKSVAIPLLSTGIFSGNKDRLTQSLNHLLTALDTTDADVAIYCRDKKWEMTLKEAVARREAVEEICISDDSSVTEPDAELVRVHPKSSLAGRKGYSTSDGKTFSYLEGTKFHQAAKDIAEINAMWPVATEANEQVCMYILGESMSSIRSKCPVEESEASTPPSTLPCLCIHAMTPERVQRLKASRPEQITVCSSFPLPKYRITGVQKIQCSQPILFSPKVPAYIHPRKYLVETPPVDETPEPSAENQSTEGTPEQPPLITEDETRTRTPEPIIIEEEEEDSISLLSDGPTHQVLQVEADIHGPPSVSSSSWSIPHASDFDVDSLSILDTLEGASVTSGATSAETNSYFAKSMEFLARPVPAPRTVFRNPPHPAPRTRTPSLAPSRACSRTSLVSTPPGVNRVITREELEALTPSRTPSRSVSRTSLVSNPPGVNRVITREEFEAFVAQQQ

SEQ ID NO: 23 - protein, 613 aa, synthetic construct
  REGION 1..613: note = Viral Protein
RFDAGAYIFSSDTGQGHLQQKSVRQTVLSEVVLERTELEISYAPRLDQEKEELLRKKLQLNPTPANRSRYQSRKVENMKAITARRILQGLGHYLKAEGKVECYRTLHPVPLYSSSVNRAFSSPKVAVEACNAMLKENFPTVASYCIIPEYDAYLDMVDGASCCLDTASFCPAKLRSFPKKHSYLEPTIRSAVPSAIQNTLQNVLAAATKRNCNVTQMRELPVLDSAAFNVECFKKYACNNEYWETFKENPIRLTEENVVNYITKLKGPKAAALFAKTHNLNMLQDIPMDRFVMDLKRDVKVTPGTKHTEERPKVQVIQAADPLATAYLCGIHRELVRRLNAVLLPNIHTLFDMSAEDFDAIIAEHFQPGDCVLETDIASFDKSEDDAMALTALMILEDLGVDAELLTLIEAAFGEISSIHLPTKTKFKFGAMMKSGMFLTLFVNTVINIVIASRVLRERLTGSPCAAFIGDDNIVKGVKSDKLMADRCATWLNMEVKIIDAVVGEKAPYFCGGFILCDSVTGTACRVADPLKRLFKLGKPLAADDEHDDDRRRALHEESTRWNRVGILSELCKAVESRYETVGTSIIVMAMTTLASSVKSFSYLRGAPITLYG

SEQ ID NO: 24 - RNA, 11917 nt, synthetic construct
  misc_feature 1..11917: note = RBS004.1
  source 1..11917: mol_type = other RNA
gatgggcggcgcatgagagaagcccagaccaattacctacccaaaatggagaaagttcacgttgacatcgaggaagacagcccattcctcagagctttgcagcggagcttcccgcagtttgaggtagaagccaagcaggtcactgataatgaccatgctaatgccagagcgttttcgcatctggcttcaaaactgatcgaaacggaggtggacccatccgacacgatccttgacattggaagtgcgcccgcccgcagaatgtattctaagcacaagtatcattgtatctgtccgatgagatgtgcggaagatccggacagattgtataagtatgcaactaagctgaagaaaaactgtaaggaaataactgataaggaattggacaagaaaatgaaggagctcgccgccgtcatgagcgaccctgacctggaaactgagactatgtgcctccacgacgacgagtcgtgtcgctacgaagggcaagtcgctgtttaccaggatgtatacgcggttgacggaccgacaagtctctatcaccaagccaataagggagttagagtcgcctactggataggctttgacaccaccccttttatgtttaagaacttggctggagcatatccatcatactctaccaactgggccgacgaaaccgtgttaacggctcgtaacataggcctatgcagctctgacgttatggagcggtcacgtagagggatgtccattcttagaaagaagtatttgaaaccatccaacaatgttctattctctgttggctcgaccatctaccacgaaaagagggacttactgaggagctggcacctgccgtctgtatttcacttacgtggcaagcaaaattacacatgtcggtgtgagactatagttagttgcgacgggtacgtcgttaaaagaatagctatcagtccaggcctgtatgggaagccttcaggctatgctgctacgatgcaccgcgagggattcttgtgctgcaaagtgacagacacattgaacggggagagggtctcttttcccgtgtgcacgtatgtgccagctacattgtgtgaccaaatgactggcatactggcaacagatgtcagtgcggacgacgcgcaaaaactgctggttgggctcaaccagcgtatagtcgtcaacggtcgcacccagagaaacaccaataccatgaaaaattaccttttgcccgtagtggcccaggcatttgctaggtgggcaaaggaatataaggaagatcaagaagatgaaaggccactaggactacgagatagacagttagtcatggggtgttgttgggcttttagaaggcacaagataacatctatttataagcgcccggatacccaaaccatcatcaaagtgaacagcgatttccactcattcgtgctgcccaggataggcagtaacacattggagatcgggctgagaacaagaatcaggaaaatgttagaggagcacaaggagccgtcacctctcattaccgccgaggacgtacaagaagctaagtgcgcagccgatgaggctaaggaggtgcgtgaagccgaggagttgcgcgcagctctaccacctttggcagctgatgttgaggagcccactctggaagccgatgtcgacttgatgttacaagaggctggggccggctcagtggagacacctcgtggcttgataaaggttaccagctacgctggcgaggacaagatcggctcttacgctgtgctttctccgcaggctgtactcaagagtgaaaaattatcttgcatccaccctctcgctgaacaagtcatagtgataacacactctggccgaaaagggcgttatgccgtggaaccataccatggtaaagtagtggtgccagagggacatgcaatacccgtccaggactttcaagctctgagtgaaagtgccaccattgtgtacaacgaacgtgagttcgtaaacaggtacctgcaccatattgccacacatggaggagcgctgaacactgatgaagaatattacaaaactgtcaagcccagcgagcacgacggcgaatacctgtacgacatcgacaggaaacagtgcgtcaagaaagagctagtcactgggctagggctcacaggcgagctggtcgatcctcccttccatgaattcgcctacgagagtctgagaacacgaccagccgctccttaccaagtaccaaccataggggtgtatggcgtgccaggatcaggcaagtctggcatcattaaaagcgcagtcaccaaaaaagatctagtggtgagcgccaagaaagaaaactgtgcagaaattataagggacgtcaagaaaatgaaagggctggacgtcaatgccagaactgtggactcagtgctcttgaatggatgcaaacaccccgtagagaccctgtatattgacgaggcttttgcttgtcatgcaggtactctcagagcgctcatagccattataagacctaaaaaggcagtgctctgcggagatcccaaacagtgcggtttttttaacatgatgtgcctgaaagtgcattttaaccacgagatttgcacacaagtcttccacaaaagcatctctcgccgttgcactaaatctgtgacttcggtcgtctcaaccttgttttacgacaaaaaaatgagaacgacgaatccgaaagagactaagattgtgattgacactaccggcagtaccaaacctaagcaggacgatctcattctcacttgtttcagagggtgggtgaagcagttgcaaatagattacaaaggcaacgaaataatgacggcagctgcctctcaagggctgacccgtaaaggtgtgtatgccgttcggtacaaggtgaatgaaaatcctctgtacgcacccacctcagaacatgtgaacgtcctactgacccgcacggaggaccgcatcgtgtggaaaacactagccggcgacccatggataaaaacactgactgccaagtaccctgggaatttcactgccacgatagaggagtggcaagcagagcatgatgccatcatgaggcacatcttggagagaccggaccctaccgacgtcttccagaataaggcaaacgtgtgttgggccaaggctttagtgccggtgctgaagaccgctggcatagacatgaccactgaacaatggaacactgtggattattttgaaacggacaaagctcactcagcagagatagtattgaaccaactatgcgtgaggttctttggactcgatctggactccggtctattttctgcacccactgttccgttatccattaggaataatcactgggataactccccgtcgcctaacatgtacgggctgaataaagaagtggtccgtcagctctctcgcaggtacccacaactgcctcgggcagttgccactggtagagtctatgacatgaacactggtacactgcgcaattatgatccgcgcataaacctagtacctgtaaacagaagactgcctcatgctttagtcctccaccataatgaacacccacagagtgacttttcttcattcgtcagcaaattgaagggcagaactgtcctggtggtcggggaaaagttgtccgtcccaggcaaaatggttgactggttgtcagaccggcctgaggctaccttcagagctcggctggatttaggcatcccaggtgatgtgcccaaatatgacataatatttgttaatgtgaggaccccatataaataccatcactatcagcagtgtgaagaccatgccattaagctaagcatgttgaccaagaaagcatgtctgcatctgaatcccggcggaacctgtgtcagcataggttatggttacgctgacagggccagcgaaagcatcattggtgctatagcgcggcagttcaagttttcccgagtatgcaaaccgaaatcctcacttgaggagacggaagttctgtttgtattcattgggtacgatcgcaaggcccgtacgcacaatccttacaagctatcatcaaccttgaccaacatttatacaggttccagactccacgaagccggatgtgcaccctcatatcatgtggtgcgaggggatattgccacggccaccgaaggagtgattataaatgctgctaacagcaaaggacaacctggcggaggggtgtgcggagcgctgtataagaaattcccggaaagtttcgatttacagccgatcgaagtaggaaaagcgcgactggtcaaaggtgcagctaaacatatcattcatgccgtaggaccaaacttcaacaaagtttcggaggttgaaggtgacaaacagttggcagaggcttatgagtccatcgctaagattgtcaacgataacaattacaagtcagtagcgattccactgttgtccaccggcatcttttccgggaacaaagatcgactaacccaatcattgaaccatttgctgacagctttagacaccactgatgcagatgtagccatatactgcagggacaagaaatgggaaatgactctcaaggaagcagtggctaggagagaagcagtggaggagatatgcatatccgacgattcttcagtgacagaacctgatgcagagctggtgagggtgcatcccaagagttctttggctggaaggaagggctacagcacaagcgatggcaaaactttctcatatttggaagggaccaagtttcaccaggcggccaaggatatagcagaaattaatgccatgtggcccgttgcaacggaggccaatgagcaggtatgcatgtatatcctcggagaaagcatgagcagtattaggtcgaaatgccccgtcgaggagtcggaagcctccacaccacctagcacgctgccttgcttgtgcatccatgccatgactccagaaagagtacagcgcctaaaagcctcacgtccagaacaaattactgtgtgctcatcctttccattgccgaagtatagaatcactggtgtgcagaagatccaatgctcccagcctatattgttctcaccgaaagtgcctgcgtatattcatccaaggaagtatctcgtggaaacaccaccggtagacgagactccggagccatcggcagagaaccaatccacagaggggacacctgaacaaccaccacttataaccgaggatgagaccaggactagaacgcctgagccgatcatcatcgaagaagaagaagaagatagcataagtttgctgtcagatggcccgacccaccaggtgctgcaagtcgaggcagacattcacgggccgccctctgtatctagctcatcctggtccattcctcatgcatccgactttgatgtggacagtttatccatacttgacaccctggagggagctagcgtgaccagcggggcaacgtcagccgagactaactcttacttcgcaaagagtatggagtttctggcgcgaccggtgcctgcgcctcgaacagtattcaggaaccctccacatcccgctccgcgcacaagaacaccgtcacttgcacccagcagggcctgctccagaaccagcctagtttccaccccgccaggcgtgaatagggtgatcactagagaggagctcgaagcgcttaccccgtcacgcactcctagcaggtcggtctccagaaccagcctggtctccaacccgccaggcgtaaatagggtgattacaagagaggagtttgaggcgttcgtagcacaacaacaatgacggtttgatgcgggtgcatacatcttttcctccgacaccggtcaagggcatttacaacaaaaatcagtaaggcaaacggtgctatccgaagtggtgttggagaggaccgaattggagatttcgtatgccccgcgcctcgaccaagaaaaagaagaattactacgcaagaaattacagttaaatcccacacctgctaacagaagcagataccagtccaggaaggtggagaacatgaaagccataacagctagacgtattctgcaaggcctagggcattatttgaaggcagaaggaaaagtggagtgctaccgaaccctgcatcctgttcctttgtattcatctagtgtgaaccgtgccttttcaagccccaaggtcgcagtggaagcctgtaacgccatgttgaaagagaactttccgactgtggcttcttactgtattattccagagtacgatgcctatttggacatggttgacggagcttcatgctgcttagacactgccagtttttgccctgcaaagctgcgcagctttccaaagaaacactcctatttggaacccacaatacgatcggcagtgccttcagcgatccagaacacgctccagaacgtcctggcagctgccacaaaaagaaattgcaatgtcacgcaaatgagagaattgcccgtattggattcggcggcctttaatgtggaatgcttcaagaaatatgcgtgtaataatgaatattgggaaacgtttaaagaaaaccccatcaggcttactgaagaaaacgtggtaaattacattaccaaattaaaaggaccaaaagctgctgctctttttgcgaagacacataatttgaatatgttgcaggacataccaatggacaggtttgtaatggacttaaagagagacgtgaaagtgactccaggaacaaaacatactgaagaacggcccaaggtacaggtgatccaggctgccgatccgctagcaacagcgtatctgtgcggaatccaccgagagctggttaggagattaaatgcggtcctgcttccgaacattcatacactgtttgatatgtcggctgaagactttgacgctattatagccgagcacttccagcctggggattgtgttctggaaactgacatcgcgtcgtttgataaaagtgaggacgacgccatggctctgaccgcgttaatgattctggaagacttaggtgtggacgcagagctgttgacgctgattgaggcggctttcggcgaaatttcatcaatacatttgcccactaaaactaaatttaaattcggagccatgatgaaatctggaatgttcctcacactgtttgtgaacacagtcattaacattgtaatcgcaagcagagtgttgagagaacggctaaccggatcaccatgtgcagcattcattggagatgacaatatcgtgaaaggagtcaaatcggacaaattaatggcagacaggtgcgccacctggttgaatatggaagtcaagattatagatgctgtggtgggcgagaaagcgccttatttctgtggagggtttattttgtgtgactccgtgaccggcacagcgtgccgtgtggcagaccccctaaaaaggctgtttaagctaggcaaacctctggcagcagacgatgaacatgatgatgacaggagaagggcattgcatgaggagtcaacacgctggaaccgagtgggtattctttcagagctgtgcaaggcagtagaatcaaggtatgaaaccgtaggaacttccatcatagttatggccatgactactctagctagcagtgttaaatcattcagctacctgagaggggcccctataactctctacggctaacctgaatggactacgacatagtctagtccgccaagactagtatgtttgtgtttcttgtgctgctgcctcttgtgtcttctcagtgtgtgaatttgacaacaagaacacagctgccaccagcttatacaaattcttttaccagaggagtgtattatcctgataaagtgtttagatcttctgtgctgcacagcacacaggacctgtttctgccattttttagcaatgtgacatggtttcatgcaattcatgtgtctggaacaaatggaacaaaaagatttgataatcctgtgctgccttttaatgatggagtgtattttgcttcaacagaaaagtcaaatattattagaggatggatttttggaacaacactggattctaaaacacagtctctgctgattgtgaataatgcaacaaatgtggtgattaaagtgtgtgaatttcagttttgtaatgatccttttctgggagtgtattatcacaaaaataataaatcttggatggaatctgaatttagagtgtattcctctgcaaataattgtacatttgaatatgtgtctcagccttttctgatggatctggaaggaaaacagggcaattttaaaaatctgagagaatttgtgtttaaaaatattgatggatattttaaaatttattctaaacacacaccaattaatttagtgagagatctgcctcagggattttctgctctggaacctctggtggatctgccaattggcattaatattacaagatttcagacactgctggctctgcacagatcttatctgacacctggagattcttcttctggatggacagccggagctgcagcttattatgtgggctatctgcagccaagaacatttctgctgaaatataatgaaaatggaacaattacagatgctgtggattgtgctctggatcctctgtctgaaacaaaatgtacattaaaatcttttacagtggaaaaaggcatttatcagacatctaattttagagtgcagccaacagaatctattgtgagatttccaaatattacaaatctgtgtccatttggagaagtgtttaatgcaacaagatttgcatctgtgtatgcatggaatagaaaaagaatttctaattgtgtggctgattattctgtgctgtataatagtgcttctttttccacatttaaatgttatggagtgtctccaacaaaattaaatgatttatgttttacaaatgtgtatgctgattcttttgtgatcagaggtgatgaagtgagacagattgcccccggacagacaggaaaaattgctgattacaattacaaactgcctgatgattttacaggatgtgtgattgcttggaattctaataatttagattctaaagtgggaggaaattacaattatctgtacagactgtttagaaaatcaaatctgaaaccttttgaaagagatatttcaacagaaatttatcaggctggatcaacaccttgtaatggagtggaaggatttaattgttattttccattacagagctatggatttcagccaaccaatggtgtgggatatcagccatatagagtggtggtgctgtcttttgaactgctgcatgcacctgcaacagtgtgtggacctaaaaaatctacaaatttagtgaaaaataaatgtgtgaattttaattttaatggattaacaggaacaggagtgctgacagaatctaataaaaaatttctgccttttcagcagtttggcagagatattgcagataccacagatgcagtgagagatcctcagacattagaaattctggatattacaccttgttcttttgggggtgtgtctgtgattacacctggaacaaatacatctaatcaggtggctgtgctgtatcaggatgtgaattgtacagaagtgccagtggcaattcatgcagatcagctgacaccaacatggagagtgtattctacaggatctaatgtgtttcagacaagagcaggatgtctgattggagcagaacatgtgaataattcttatgaatgtgatattccaattggagcaggcatttgtgcatcttatcagacacagacaaattccccaaggagagcaagatctgtggcatctcagtctattattgcatacaccatgtctctgggagcagaaaattctgtggcatattctaataattctattgctattccaacaaattttaccatttctgtgacaacagaaattttacctgtgtctatgacaaaaacatctgtggattgtaccatgtacatttgtggagattctacagaatgttctaatctgctgctgcagtatggatctttttgtacacagctgaatagagctttaacaggaattgctgtggaacaggataaaaatacacaggaagtgtttgctcaggtgaaacagatttacaaaacaccaccaattaaagattttggaggatttaattttagccagattctgcctgatccttctaaaccttctaaaagatcttttattgaagatctgctgtttaataaagtgacactggcagatgcaggatttattaaacagtatggagattgcctgggtgatattgctgcaagagatctgatttgtgctcagaaatttaatggactgacagtgctgcctcctctgctgacagatgaaatgattgctcagtacacatctgctttactggctggaacaattacaagcggatggacatttggagctggagctgctctgcagattccttttgcaatgcagatggcttacagatttaatggaattggagtgacacagaatgtgttatatgaaaatcagaaactgattgcaaatcagtttaattctgcaattggcaaaattcaggattctctgtcttctacagcttctgctctgggaaaactgcaggatgtggtgaatcagaatgcacaggcactgaatactctggtgaaacagctgtctagcaattttggggcaatttcttctgtgctgaatgatattctgtctagactggatcctcctgaagctgaagtgcagattgatagactgatcacaggaagactgcagtctctgcagacttatgtgacacagcagctgattagagctgctgaaattagagcttctgctaatctggctgctacaaaaatgtctgaatgtgtgctgggacagtcaaaaagagtggatttttgtggaaaaggatatcatctgatgtcttttccacagtctgctccacatggagtggtgtttttacatgtgacatatgtgccagcacaggaaaagaattttaccacagcaccagcaatttgtcatgatggaaaagcacattttccaagagaaggagtgtttgtgtctaatggaacacattggtttgtgacacagagaaatttttatgaacctcagattattacaacagataatacatttgtgtcaggaaattgtgatgtggtgattggaattgtgaataatacagtgtatgatccactgcagccagaactggattcttttaaagaagaactggataaatattttaaaaatcacacatctcctgatgtggatttaggagatatttctggaatcaatgcatctgtggtgaatattcagaaagaaattgatagactgaatgaagtggccaaaaatctgaatgaatctctgattgatctgcaggaacttggaaaatatgaacagtacattaaatggccttggtacatttggcttggatttattgcaggattaattgcaattgtgatggtgacaattatgttatgttgtatgacatcatgttgttcttgtttaaaaggatgttgttcttgtggaagctgttgtaaatttgatgaagatgattctgaacctgtgttaaaaggagtgaaattgcattacacatgatgactcgagctggtactgcatgcacgcaatgctagctgcccctttcccgtcctgggtaccccgagtctcccccgacctcgggtcccaggtatgctcccacctccacctgccccactcaccacctctgctagttccagacacctcccaagcacgcagcaatgcagctcaaaacgcttagcctagccacacccccacgggaaacagcagtgattaacctttagcaataaacgaaagtttaactaagctatactaaccccagggttggtcaatttcgtgccagccacaccgcggccgcatgaatacagcagcaattggcaagctgcttacatagaactcgcggcgattggcatgccgccttaaaatttttattttattttttcttttcttttccgaatcggattttgtttttaatatttcaaaaaaaaaaaaaaaaaaaaaaaaaaaaaagcatatgactaaaaaaaaaaaaaaaaaaaaaaaaaaaaaaaaaaaaaaaaaaaaaaaaaaaaaaaaaaaaaaaaaaaaaa

SEQ ID NO: 25 - RNA, 11917 nt, synthetic construct
  misc_feature 1..11917: note = RBS004.2
  source 1..11917: mol_type = other RNA
gatgggcggcgcatgagagaagcccagaccaattacctacccaaaatggagaaagttcacgttgacatcgaggaagacagcccattcctcagagctttgcagcggagcttcccgcagtttgaggtagaagccaagcaggtcactgataatgaccatgctaatgccagagcgttttcgcatctggcttcaaaactgatcgaaacggaggtggacccatccgacacgatccttgacattggaagtgcgcccgcccgcagaatgtattctaagcacaagtatcattgtatctgtccgatgagatgtgcggaagatccggacagattgtataagtatgcaactaagctgaagaaaaactgtaaggaaataactgataaggaattggacaagaaaatgaaggagctcgccgccgtcatgagcgaccctgacctggaaactgagactatgtgcctccacgacgacgagtcgtgtcgctacgaagggcaagtcgctgtttaccaggatgtatacgcggttgacggaccgacaagtctctatcaccaagccaataagggagttagagtcgcctactggataggctttgacaccaccccttttatgtttaagaacttggctggagcatatccatcatactctaccaactgggccgacgaaaccgtgttaacggctcgtaacataggcctatgcagctctgacgttatggagcggtcacgtagagggatgtccattcttagaaagaagtatttgaaaccatccaacaatgttctattctctgttggctcgaccatctaccacgaaaagagggacttactgaggagctggcacctgccgtctgtatttcacttacgtggcaagcaaaattacacatgtcggtgtgagactatagttagttgcgacgggtacgtcgttaaaagaatagctatcagtccaggcctgtatgggaagccttcaggctatgctgctacgatgcaccgcgagggattcttgtgctgcaaagtgacagacacattgaacggggagagggtctcttttcccgtgtgcacgtatgtgccagctacattgtgtgaccaaatgactggcatactggcaacagatgtcagtgcggacgacgcgcaaaaactgctggttgggctcaaccagcgtatagtcgtcaacggtcgcacccagagaaacaccaataccatgaaaaattaccttttgcccgtagtggcccaggcatttgctaggtgggcaaaggaatataaggaagatcaagaagatgaaaggccactaggactacgagatagacagttagtcatggggtgttgttgggcttttagaaggcacaagataacatctatttataagcgcccggatacccaaaccatcatcaaagtgaacagcgatttccactcattcgtgctgcccaggataggcagtaacacattggagatcgggctgagaacaagaatcaggaaaatgttagaggagcacaaggagccgtcacctctcattaccgccgaggacgtacaagaagctaagtgcgcagccgatgaggctaaggaggtgcgtgaagccgaggagttgcgcgcagctctaccacctttggcagctgatgttgaggagcccactctggaagccgatgtcgacttgatgttacaagaggctggggccggctcagtggagacacctcgtggcttgataaaggttaccagctacgctggcgaggacaagatcggctcttacgctgtgctttctccgcaggctgtactcaagagtgaaaaattatcttgcatccaccctctcgctgaacaagtcatagtgataacacactctggccgaaaagggcgttatgccgtggaaccataccatggtaaagtagtggtgccagagggacatgcaatacccgtccaggactttcaagctctgagtgaaagtgccaccattgtgtacaacgaacgtgagttcgtaaacaggtacctgcaccatattgccacacatggaggagcgctgaacactgatgaagaatattacaaaactgtcaagcccagcgagcacgacggcgaatacctgtacgacatcgacaggaaacagtgcgtcaagaaagagctagtcactgggctagggctcacaggcgagctggtcgatcctcccttccatgaattcgcctacgagagtctgagaacacgaccagccgctccttaccaagtaccaaccataggggtgtatggcgtgccaggatcaggcaagtctggcatcattaaaagcgcagtcaccaaaaaagatctagtggtgagcgccaagaaagaaaactgtgcagaaattataagggacgtcaagaaaatgaaagggctggacgtcaatgccagaactgtggactcagtgctcttgaatggatgcaaacaccccgtagagaccctgtatattgacgaggcttttgcttgtcatgcaggtactctcagagcgctcatagccattataagacctaaaaaggcagtgctctgcggagatcccaaacagtgcggtttttttaacatgatgtgcctgaaagtgcattttaaccacgagatttgcacacaagtcttccacaaaagcatctctcgccgttgcactaaatctgtgacttcggtcgtctcaaccttgttttacgacaaaaaaatgagaacgacgaatccgaaagagactaagattgtgattgacactaccggcagtaccaaacctaagcaggacgatctcattctcacttgtttcagagggtgggtgaagcagttgcaaatagattacaaaggcaacgaaataatgacggcagctgcctctcaagggctgacccgtaaaggtgtgtatgccgttcggtacaaggtgaatgaaaatcctctgtacgcacccacctcagaacatgtgaacgtcctactgacccgcacggaggaccgcatcgtgtggaaaacactagccggcgacccatggataaaaacactgactgccaagtaccctgggaatttcactgccacgatagaggagtggcaagcagagcatgatgccatcatgaggcacatcttggagagaccggaccctaccgacgtcttccagaataaggcaaacgtgtgttgggccaaggctttagtgccggtgctgaagaccgctggcatagacatgaccactgaacaatggaacactgtggattattttgaaacggacaaagctcactcagcagagatagtattgaaccaactatgcgtgaggttctttggactcgatctggactccggtctattttctgcacccactgttccgttatccattaggaataatcactgggataactccccgtcgcctaacatgtacgggctgaataaagaagtggtccgtcagctctctcgcaggtacccacaactgcctcgggcagttgccactggtagagtctatgacatgaacactggtacactgcgcaattatgatccgcgcataaacctagtacctgtaaacagaagactgcctcatgctttagtcctccaccataatgaacacccacagagtgacttttcttcattcgtcagcaaattgaagggcagaactgtcctggtggtcggggaaaagttgtccgtcccaggcaaaatggttgactggttgtcagaccggcctgaggctaccttcagagctcggctggatttaggcatcccaggtgatgtgcccaaatatgacataatatttgttaatgtgaggaccccatataaataccatcactatcagcagtgtgaagaccatgccattaagctaagcatgttgaccaagaaagcatgtctgcatctgaatcccggcggaacctgtgtcagcataggttatggttacgctgacagggccagcgaaagcatcattggtgctatagcgcggcagttcaagttttcccgagtatgcaaaccgaaatcctcacttgaggagacggaagttctgtttgtattcattgggtacgatcgcaaggcccgtacgcacaatccttacaagctatcatcaaccttgaccaacatttatacaggttccagactccacgaagccggatgtgcaccctcatatcatgtggtgcgaggggatattgccacggccaccgaaggagtgattataaatgctgctaacagcaaaggacaacctggcggaggggtgtgcggagcgctgtataagaaattcccggaaagtttcgatttacagccgatcgaagtaggaaaagcgcgactggtcaaaggtgcagctaaacatatcattcatgccgtaggaccaaacttcaacaaagtttcggaggttgaaggtgacaaacagttggcagaggcttatgagtccatcgctaagattgtcaacgataacaattacaagtcagtagcgattccactgttgtccaccggcatcttttccgggaacaaagatcgactaacccaatcattgaaccatttgctgacagctttagacaccactgatgcagatgtagccatatactgcagggacaagaaatgggaaatgactctcaaggaagcagtggctaggagagaagcagtggaggagatatgcatatccgacgattcttcagtgacagaacctgatgcagagctggtgagggtgcatcccaagagttctttggctggaaggaagggctacagcacaagcgatggcaaaactttctcatatttggaagggaccaagtttcaccaggcggccaaggatatagcagaaattaatgccatgtggcccgttgcaacggaggccaatgagcaggtatgcatgtatatcctcggagaaagcatgagcagtattaggtcgaaatgccccgtcgaggagtcggaagcctccacaccacctagcacgctgccttgcttgtgcatccatgccatgactccagaaagagtacagcgcctaaaagcctcacgtccagaacaaattactgtgtgctcatcctttccattgccgaagtatagaatcactggtgtgcagaagatccaatgctcccagcctatattgttctcaccgaaagtgcctgcgtatattcatccaaggaagtatctcgtggaaacaccaccggtagacgagactccggagccatcggcagagaaccaatccacagaggggacacctgaacaaccaccacttataaccgaggatgagaccaggactagaacgcctgagccgatcatcatcgaagaagaagaagaagatagcataagtttgctgtcagatggcccgacccaccaggtgctgcaagtcgaggcagacattcacgggccgccctctgtatctagctcatcctggtccattcctcatgcatccgactttgatgtggacagtttatccatacttgacaccctggagggagctagcgtgaccagcggggcaacgtcagccgagactaactcttacttcgcaaagagtatggagtttctggcgcgaccggtgcctgcgcctcgaacagtattcaggaaccctccacatcccgctccgcgcacaagaacaccgtcacttgcacccagcagggcctgctccagaaccagcctagtttccaccccgccaggcgtgaatagggtgatcactagagaggagctcgaagcgcttaccccgtcacgcactcctagcaggtcggtctccagaaccagcctggtctccaacccgccaggcgtaaatagggtgattacaagagaggagtttgaggcgttcgtagcacaacaacaatgacggtttgatgcgggtgcatacatcttttcctccgacaccggtcaagggcatttacaacaaaaatcagtaaggcaaacggtgctatccgaagtggtgttggagaggaccgaattggagatttcgtatgccccgcgcctcgaccaagaaaaagaagaattactacgcaagaaattacagttaaatcccacacctgctaacagaagcagataccagtccaggaaggtggagaacatgaaagccataacagctagacgtattctgcaaggcctagggcattatttgaaggcagaaggaaaagtggagtgctaccgaaccctgcatcctgttcctttgtattcatctagtgtgaaccgtgccttttcaagccccaaggtcgcagtggaagcctgtaacgccatgttgaaagagaactttccgactgtggcttcttactgtattattccagagtacgatgcctatttggacatggttgacggagcttcatgctgcttagacactgccagtttttgccctgcaaagctgcgcagctttccaaagaaacactcctatttggaacccacaatacgatcggcagtgccttcagcgatccagaacacgctccagaacgtcctggcagctgccacaaaaagaaattgcaatgtcacgcaaatgagagaattgcccgtattggattcggcggcctttaatgtggaatgcttcaagaaatatgcgtgtaataatgaatattgggaaacgtttaaagaaaaccccatcaggcttactgaagaaaacgtggtaaattacattaccaaattaaaaggaccaaaagctgctgctctttttgcgaagacacataatttgaatatgttgcaggacataccaatggacaggtttgtaatggacttaaagagagacgtgaaagtgactccaggaacaaaacatactgaagaacggcccaaggtacaggtgatccaggctgccgatccgctagcaacagcgtatctgtgcggaatccaccgagagctggttaggagattaaatgcggtcctgcttccgaacattcatacactgtttgatatgtcggctgaagactttgacgctattatagccgagcacttccagcctggggattgtgttctggaaactgacatcgcgtcgtttgataaaagtgaggacgacgccatggctctgaccgcgttaatgattctggaagacttaggtgtggacgcagagctgttgacgctgattgaggcggctttcggcgaaatttcatcaatacatttgcccactaaaactaaatttaaattcggagccatgatgaaatctggaatgttcctcacactgtttgtgaacacagtcattaacattgtaatcgcaagcagagtgttgagagaacggctaaccggatcaccatgtgcagcattcattggagatgacaatatcgtgaaaggagtcaaatcggacaaattaatggcagacaggtgcgccacctggttgaatatggaagtcaagattatagatgctgtggtgggcgagaaagcgccttatttctgtggagggtttattttgtgtgactccgtgaccggcacagcgtgccgtgtggcagaccccctaaaaaggctgtttaagctaggcaaacctctggcagcagacgatgaacatgatgatgacaggagaagggcattgcatgaggagtcaacacgctggaaccgagtgggtattctttcagagctgtgcaaggcagtagaatcaaggtatgaaaccgtaggaacttccatcatagttatggccatgactactctagctagcagtgttaaatcattcagctacctgagaggggcccctataactctctacggctaacctgaatggactacgacatagtctagtccgccaagactagtatgttcgtgttcctggtgctgctgcctctggtgtccagccagtgtgtgaacctgaccaccagaacacagctgcctccagcctacaccaacagctttaccagaggcgtgtactaccccgacaaggtgttcagatccagcgtgctgcactctacccaggacctgttcctgcctttcttcagcaacgtgacctggttccacgccatccacgtgtccggcaccaatggcaccaagagattcgacaaccccgtgctgcccttcaacgacggggtgtactttgccagcaccgagaagtccaacatcatcagaggctggatcttcggcaccacactggacagcaagacccagagcctgctgatcgtgaacaacgccaccaacgtggtcatcaaagtgtgcgagttccagttctgcaacgaccccttcctgggcgtctactaccacaagaacaacaagagctggatggaaagcgagttccgggtgtacagcagcgccaacaactgcaccttcgagtacgtgtcccagcctttcctgatggacctggaaggcaagcagggcaacttcaagaacctgcgcgagttcgtgtttaagaacatcgacggctacttcaagatctacagcaagcacacccctatcaacctcgtgcgggatctgcctcagggcttctctgctctggaacccctggtggatctgcccatcggcatcaacatcacccggtttcagacactgctggccctgcacagaagctacctgacacctggcgatagcagcagcggatggacagctggtgccgccgcttactatgtgggctacctgcagcctagaaccttcctgctgaagtacaacgagaacggcaccatcaccgacgccgtggattgtgctctggatcctctgagcgagacaaagtgcaccctgaagtccttcaccgtggaaaagggcatctaccagaccagcaacttccgggtgcagcccaccgaatccatcgtgcggttccccaatatcaccaatctgtgccccttcggcgaggtgttcaatgccaccagattcgcctctgtgtacgcctggaaccggaagcggatcagcaattgcgtggccgactactccgtgctgtacaactccgccagcttcagcaccttcaagtgctacggcgtgtcccctaccaagctgaacgacctgtgcttcacaaacgtgtacgccgacagcttcgtgatccggggagatgaagtgcggcagattgcccctggacagacaggcaagatcgccgactacaactacaagctgcccgacgacttcaccggctgtgtgattgcctggaacagcaacaacctggactccaaagtcggcggcaactacaattacctgtaccggctgttccggaagtccaatctgaagcccttcgagcgggacatctccaccgagatctatcaggccggcagcaccccttgtaacggcgtggaaggcttcaactgctacttcccactgcagtcctacggctttcagcccacaaatggcgtgggctatcagccctacagagtggtggtgctgagcttcgaactgctgcatgcccctgccacagtgtgcggccctaagaaaagcaccaatctcgtgaagaacaaatgcgtgaacttcaacttcaacggcctgaccggcaccggcgtgctgacagagagcaacaagaagttcctgccattccagcagtttggccgggatatcgccgataccacagacgccgttagagatccccagacactggaaatcctggacatcaccccttgcagcttcggcggagtgtctgtgatcacccctggcaccaacaccagcaatcaggtggcagtgctgtaccaggacgtgaactgtaccgaagtgcccgtggccattcacgccgatcagctgacacctacatggcgggtgtactccaccggcagcaatgtgtttcagaccagagccggctgtctgatcggagccgagcacgtgaacaatagctacgagtgcgacatccccatcggcgctggaatctgcgccagctaccagacacagacaaacagccctcggagagccagaagcgtggccagccagagcatcattgcctacacaatgtctctgggcgccgagaacagcgtggcctactccaacaactctatcgctatccccaccaacttcaccatcagcgtgaccacagagatcctgcctgtgtccatgaccaagaccagcgtggactgcaccatgtacatctgcggcgattccaccgagtgctccaacctgctgctgcagtacggcagcttctgcacccagctgaatagagccctgacagggatcgccgtggaacaggacaagaacacccaagaggtgttcgcccaagtgaagcagatctacaagacccctcctatcaaggacttcggcggcttcaatttcagccagattctgcccgatcctagcaagcccagcaagcggagcttcatcgaggacctgctgttcaacaaagtgacactggccgacgccggcttcatcaagcagtatggcgattgtctgggcgacattgccgccagggatctgatttgcgcccagaagtttaacggactgacagtgctgcctcctctgctgaccgatgagatgatcgcccagtacacatctgccctgctggccggcacaatcacaagcggctggacatttggagcaggcgccgctctgcagatcccctttgctatgcagatggcctaccggttcaacggcatcggagtgacccagaatgtgctgtacgagaaccagaagctgatcgccaaccagttcaacagcgccatcggcaagatccaggacagcctgagcagcacagcaagcgccctgggaaagctgcaggacgtggtcaaccagaatgcccaggcactgaacaccctggtcaagcagctgtcctccaacttcggcgccatcagctctgtgctgaacgatatcctgagcagactggaccctcctgaggccgaggtgcagatcgacagactgatcacaggcagactgcagagcctccagacatacgtgacccagcagctgatcagagccgccgagattagagcctctgccaatctggccgccaccaagatgtctgagtgtgtgctgggccagagcaagagagtggacttttgcggcaagggctaccacctgatgagcttccctcagtctgcccctcacggcgtggtgtttctgcacgtgacatatgtgcccgctcaagagaagaatttcaccaccgctccagccatctgccacgacggcaaagcccactttcctagagaaggcgtgttcgtgtccaacggcacccattggttcgtgacacagcggaacttctacgagccccagatcatcaccaccgacaacaccttcgtgtctggcaactgcgacgtcgtgatcggcattgtgaacaataccgtgtacgaccctctgcagcccgagctggacagcttcaaagaggaactggacaagtactttaagaaccacacaagccccgacgtggacctgggcgatatcagcggaatcaatgccagcgtcgtgaacatccagaaagagatcgaccggctgaacgaggtggccaagaatctgaacgagagcctgatcgacctgcaagaactggggaagtacgagcagtacatcaagtggccctggtacatctggctgggctttatcgccggactgattgccatcgtgatggtcacaatcatgctgtgttgcatgaccagctgctgtagctgcctgaagggctgttgtagctgtggcagctgctgcaagttcgacgaggacgattctgagcccgtgctgaagggcgtgaaactgcactacacatgatgactcgagctggtactgcatgcacgcaatgctagctgcccctttcccgtcctgggtaccccgagtctcccccgacctcgggtcccaggtatgctcccacctccacctgccccactcaccacctctgctagttccagacacctcccaagcacgcagcaatgcagctcaaaacgcttagcctagccacacccccacgggaaacagcagtgattaacctttagcaataaacgaaagtttaactaagctatactaaccccagggttggtcaatttcgtgccagccacaccgcggccgcatgaatacagcagcaattggcaagctgcttacatagaactcgcggcgattggcatgccgccttaaaatttttattttattttttcttttcttttccgaatcggattttgtttttaatatttcaaaaaaaaaaaaaaaaaaaaaaaaaaaaaagcatatgactaaaaaaaaaaaaaaaaaaaaaaaaaaaaaaaaaaaaaaaaaaaaaaaaaaaaaaaaaaaaaaaaaaaaaa

SEQ ID NO: 26 - RNA, 8896 nt, synthetic construct
  misc_feature 1..8896: note = RBS004.3
  source 1..8896: mol_type = other RNA
gatgggcggcgcatgagagaagcccagaccaattacctacccaaaatggagaaagttcacgttgacatcgaggaagacagcccattcctcagagctttgcagcggagcttcccgcagtttgaggtagaagccaagcaggtcactgataatgaccatgctaatgccagagcgttttcgcatctggcttcaaaactgatcgaaacggaggtggacccatccgacacgatccttgacattggaagtgcgcccgcccgcagaatgtattctaagcacaagtatcattgtatctgtccgatgagatgtgcggaagatccggacagattgtataagtatgcaactaagctgaagaaaaactgtaaggaaataactgataaggaattggacaagaaaatgaaggagctcgccgccgtcatgagcgaccctgacctggaaactgagactatgtgcctccacgacgacgagtcgtgtcgctacgaagggcaagtcgctgtttaccaggatgtatacgcggttgacggaccgacaagtctctatcaccaagccaataagggagttagagtcgcctactggataggctttgacaccaccccttttatgtttaagaacttggctggagcatatccatcatactctaccaactgggccgacgaaaccgtgttaacggctcgtaacataggcctatgcagctctgacgttatggagcggtcacgtagagggatgtccattcttagaaagaagtatttgaaaccatccaacaatgttctattctctgttggctcgaccatctaccacgaaaagagggacttactgaggagctggcacctgccgtctgtatttcacttacgtggcaagcaaaattacacatgtcggtgtgagactatagttagttgcgacgggtacgtcgttaaaagaatagctatcagtccaggcctgtatgggaagccttcaggctatgctgctacgatgcaccgcgagggattcttgtgctgcaaagtgacagacacattgaacggggagagggtctcttttcccgtgtgcacgtatgtgccagctacattgtgtgaccaaatgactggcatactggcaacagatgtcagtgcggacgacgcgcaaaaactgctggttgggctcaaccagcgtatagtcgtcaacggtcgcacccagagaaacaccaataccatgaaaaattaccttttgcccgtagtggcccaggcatttgctaggtgggcaaaggaatataaggaagatcaagaagatgaaaggccactaggactacgagatagacagttagtcatggggtgttgttgggcttttagaaggcacaagataacatctatttataagcgcccggatacccaaaccatcatcaaagtgaacagcgatttccactcattcgtgctgcccaggataggcagtaacacattggagatcgggctgagaacaagaatcaggaaaatgttagaggagcacaaggagccgtcacctctcattaccgccgaggacgtacaagaagctaagtgcgcagccgatgaggctaaggaggtgcgtgaagccgaggagttgcgcgcagctctaccacctttggcagctgatgttgaggagcccactctggaagccgatgtcgacttgatgttacaagaggctggggccggctcagtggagacacctcgtggcttgataaaggttaccagctacgctggcgaggacaagatcggctcttacgctgtgctttctccgcaggctgtactcaagagtgaaaaattatcttgcatccaccctctcgctgaacaagtcatagtgataacacactctggccgaaaagggcgttatgccgtggaaccataccatggtaaagtagtggtgccagagggacatgcaatacccgtccaggactttcaagctctgagtgaaagtgccaccattgtgtacaacgaacgtgagttcgtaaacaggtacctgcaccatattgccacacatggaggagcgctgaacactgatgaagaatattacaaaactgtcaagcccagcgagcacgacggcgaatacctgtacgacatcgacaggaaacagtgcgtcaagaaagagctagtcactgggctagggctcacaggcgagctggtcgatcctcccttccatgaattcgcctacgagagtctgagaacacgaccagccgctccttaccaagtaccaaccataggggtgtatggcgtgccaggatcaggcaagtctggcatcattaaaagcgcagtcaccaaaaaagatctagtggtgagcgccaagaaagaaaactgtgcagaaattataagggacgtcaagaaaatgaaagggctggacgtcaatgccagaactgtggactcagtgctcttgaatggatgcaaacaccccgtagagaccctgtatattgacgaggcttttgcttgtcatgcaggtactctcagagcgctcatagccattataagacctaaaaaggcagtgctctgcggagatcccaaacagtgcggtttttttaacatgatgtgcctgaaagtgcattttaaccacgagatttgcacacaagtcttccacaaaagcatctctcgccgttgcactaaatctgtgacttcggtcgtctcaaccttgttttacgacaaaaaaatgagaacgacgaatccgaaagagactaagattgtgattgacactaccggcagtaccaaacctaagcaggacgatctcattctcacttgtttcagagggtgggtgaagcagttgcaaatagattacaaaggcaacgaaataatgacggcagctgcctctcaagggctgacccgtaaaggtgtgtatgccgttcggtacaaggtgaatgaaaatcctctgtacgcacccacctcagaacatgtgaacgtcctactgacccgcacggaggaccgcatcgtgtggaaaacactagccggcgacccatggataaaaacactgactgccaagtaccctgggaatttcactgccacgatagaggagtggcaagcagagcatgatgccatcatgaggcacatcttggagagaccggaccctaccgacgtcttccagaataaggcaaacgtgtgttgggccaaggctttagtgccggtgctgaagaccgctggcatagacatgaccactgaacaatggaacactgtggattattttgaaacggacaaagctcactcagcagagatagtattgaaccaactatgcgtgaggttctttggactcgatctggactccggtctattttctgcacccactgttccgttatccattaggaataatcactgggataactccccgtcgcctaacatgtacgggctgaataaagaagtggtccgtcagctctctcgcaggtacccacaactgcctcgggcagttgccactggtagagtctatgacatgaacactggtacactgcgcaattatgatccgcgcataaacctagtacctgtaaacagaagactgcctcatgctttagtcctccaccataatgaacacccacagagtgacttttcttcattcgtcagcaaattgaagggcagaactgtcctggtggtcggggaaaagttgtccgtcccaggcaaaatggttgactggttgtcagaccggcctgaggctaccttcagagctcggctggatttaggcatcccaggtgatgtgcccaaatatgacataatatttgttaatgtgaggaccccatataaataccatcactatcagcagtgtgaagaccatgccattaagctaagcatgttgaccaagaaagcatgtctgcatctgaatcccggcggaacctgtgtcagcataggttatggttacgctgacagggccagcgaaagcatcattggtgctatagcgcggcagttcaagttttcccgagtatgcaaaccgaaatcctcacttgaggagacggaagttctgtttgtattcattgggtacgatcgcaaggcccgtacgcacaatccttacaagctatcatcaaccttgaccaacatttatacaggttccagactccacgaagccggatgtgcaccctcatatcatgtggtgcgaggggatattgccacggccaccgaaggagtgattataaatgctgctaacagcaaaggacaacctggcggaggggtgtgcggagcgctgtataagaaattcccggaaagtttcgatttacagccgatcgaagtaggaaaagcgcgactggtcaaaggtgcagctaaacatatcattcatgccgtaggaccaaacttcaacaaagtttcggaggttgaaggtgacaaacagttggcagaggcttatgagtccatcgctaagattgtcaacgataacaattacaagtcagtagcgattccactgttgtccaccggcatcttttccgggaacaaagatcgactaacccaatcattgaaccatttgctgacagctttagacaccactgatgcagatgtagccatatactgcagggacaagaaatgggaaatgactctcaaggaagcagtggctaggagagaagcagtggaggagatatgcatatccgacgattcttcagtgacagaacctgatgcagagctggtgagggtgcatcccaagagttctttggctggaaggaagggctacagcacaagcgatggcaaaactttctcatatttggaagggaccaagtttcaccaggcggccaaggatatagcagaaattaatgccatgtggcccgttgcaacggaggccaatgagcaggtatgcatgtatatcctcggagaaagcatgagcagtattaggtcgaaatgccccgtcgaggagtcggaagcctccacaccacctagcacgctgccttgcttgtgcatccatgccatgactccagaaagagtacagcgcctaaaagcctcacgtccagaacaaattactgtgtgctcatcctttccattgccgaagtatagaatcactggtgtgcagaagatccaatgctcccagcctatattgttctcaccgaaagtgcctgcgtatattcatccaaggaagtatctcgtggaaacaccaccggtagacgagactccggagccatcggcagagaaccaatccacagaggggacacctgaacaaccaccacttataaccgaggatgagaccaggactagaacgcctgagccgatcatcatcgaagaagaagaagaagatagcataagtttgctgtcagatggcccgacccaccaggtgctgcaagtcgaggcagacattcacgggccgccctctgtatctagctcatcctggtccattcctcatgcatccgactttgatgtggacagtttatccatacttgacaccctggagggagctagcgtgaccagcggggcaacgtcagccgagactaactcttacttcgcaaagagtatggagtttctggcgcgaccggtgcctgcgcctcgaacagtattcaggaaccctccacatcccgctccgcgcacaagaacaccgtcacttgcacccagcagggcctgctccagaaccagcctagtttccaccccgccaggcgtgaatagggtgatcactagagaggagctcgaagcgcttaccccgtcacgcactcctagcaggtcggtctccagaaccagcctggtctccaacccgccaggcgtaaatagggtgattacaagagaggagtttgaggcgttcgtagcacaacaacaatgacggtttgatgcgggtgcatacatcttttcctccgacaccggtcaagggcatttacaacaaaaatcagtaaggcaaacggtgctatccgaagtggtgttggagaggaccgaattggagatttcgtatgccccgcgcctcgaccaagaaaaagaagaattactacgcaagaaattacagttaaatcccacacctgctaacagaagcagataccagtccaggaaggtggagaacatgaaagccataacagctagacgtattctgcaaggcctagggcattatttgaaggcagaaggaaaagtggagtgctaccgaaccctgcatcctgttcctttgtattcatctagtgtgaaccgtgccttttcaagccccaaggtcgcagtggaagcctgtaacgccatgttgaaagagaactttccgactgtggcttcttactgtattattccagagtacgatgcctatttggacatggttgacggagcttcatgctgcttagacactgccagtttttgccctgcaaagctgcgcagctttccaaagaaacactcctatttggaacccacaatacgatcggcagtgccttcagcgatccagaacacgctccagaacgtcctggcagctgccacaaaaagaaattgcaatgtcacgcaaatgagagaattgcccgtattggattcggcggcctttaatgtggaatgcttcaagaaatatgcgtgtaataatgaatattgggaaacgtttaaagaaaaccccatcaggcttactgaagaaaacgtggtaaattacattaccaaattaaaaggaccaaaagctgctgctctttttgcgaagacacataatttgaatatgttgcaggacataccaatggacaggtttgtaatggacttaaagagagacgtgaaagtgactccaggaacaaaacatactgaagaacggcccaaggtacaggtgatccaggctgccgatccgctagcaacagcgtatctgtgcggaatccaccgagagctggttaggagattaaatgcggtcctgcttccgaacattcatacactgtttgatatgtcggctgaagactttgacgctattatagccgagcacttccagcctggggattgtgttctggaaactgacatcgcgtcgtttgataaaagtgaggacgacgccatggctctgaccgcgttaatgattctggaagacttaggtgtggacgcagagctgttgacgctgattgaggcggctttcggcgaaatttcatcaatacatttgcccactaaaactaaatttaaattcggagccatgatgaaatctggaatgttcctcacactgtttgtgaacacagtcattaacattgtaatcgcaagcagagtgttgagagaacggctaaccggatcaccatgtgcagcattcattggagatgacaatatcgtgaaaggagtcaaatcggacaaattaatggcagacaggtgcgccacctggttgaatatggaagtcaagattatagatgctgtggtgggcgagaaagcgccttatttctgtggagggtttattttgtgtgactccgtgaccggcacagcgtgccgtgtggcagaccccctaaaaaggctgtttaagctaggcaaacctctggcagcagacgatgaacatgatgatgacaggagaagggcattgcatgaggagtcaacacgctggaaccgagtgggtattctttcagagctgtgcaaggcagtagaatcaaggtatgaaaccgtaggaacttccatcatagttatggccatgactactctagctagcagtgttaaatcattcagctacctgagaggggcccctataactctctacggctaacctgaatggactacgacatagtctagtccgccaagactagtatgtttgtgtttcttgtgctgctgcctcttgtgtcttctcagtgtgtggtgagatttccaaatattacaaatctgtgtccatttggagaagtgtttaatgcaacaagatttgcatctgtgtatgcatggaatagaaaaagaatttctaattgtgtggctgattattctgtgctgtataatagtgcttctttttccacatttaaatgttatggagtgtctccaacaaaattaaatgatttatgttttacaaatgtgtatgctgattcttttgtgatcagaggtgatgaagtgagacagattgcccccggacagacaggaaaaattgctgattacaattacaaactgcctgatgattttacaggatgtgtgattgcttggaattctaataatttagattctaaagtgggaggaaattacaattatctgtacagactgtttagaaaatcaaatctgaaaccttttgaaagagatatttcaacagaaatttatcaggctggatcaacaccttgtaatggagtggaaggatttaattgttattttccattacagagctatggatttcagccaaccaatggtgtgggatatcagccatatagagtggtggtgctgtcttttgaactgctgcatgcacctgcaacagtgtgtggacctaaaggctcccccggctccggctccggatctggttatattcctgaagctccaagagatgggcaagcttacgttcgtaaagatggcgaatgggtattactttctacctttttaggccggtccctggaggtgctgttccagggccccggctgatgactcgagctggtactgcatgcacgcaatgctagctgcccctttcccgtcctgggtaccccgagtctcccccgacctcgggtcccaggtatgctcccacctccacctgccccactcaccacctctgctagttccagacacctcccaagcacgcagcaatgcagctcaaaacgcttagcctagccacacccccacgggaaacagcagtgattaacctttagcaataaacgaaagtttaactaagctatactaaccccagggttggtcaatttcgtgccagccacaccgcggccgcatgaatacagcagcaattggcaagctgcttacatagaactcgcggcgattggcatgccgccttaaaatttttattttattttttcttttcttttccgaatcggattttgtttttaatatttcaaaaaaaaaaaaaaaaaaaaaaaaaaaaaagcatatgactaaaaaaaaaaaaaaaaaaaaaaaaaaaaaaaaaaaaaaaaaaaaaaaaaaaaaaaaaaaaaaaaaaaaaa

SEQ ID NO: 27 - RNA, 9079 nt, synthetic construct
  misc_feature 1..9079: note = RBS004.4
  source 1..9079: mol_type = other RNA
gatgggcggcgcatgagagaagcccagaccaattacctacccaaaatggagaaagttcacgttgacatcgaggaagacagcccattcctcagagctttgcagcggagcttcccgcagtttgaggtagaagccaagcaggtcactgataatgaccatgctaatgccagagcgttttcgcatctggcttcaaaactgatcgaaacggaggtggacccatccgacacgatccttgacattggaagtgcgcccgcccgcagaatgtattctaagcacaagtatcattgtatctgtccgatgagatgtgcggaagatccggacagattgtataagtatgcaactaagctgaagaaaaactgtaaggaaataactgataaggaattggacaagaaaatgaaggagctcgccgccgtcatgagcgaccctgacctggaaactgagactatgtgcctccacgacgacgagtcgtgtcgctacgaagggcaagtcgctgtttaccaggatgtatacgcggttgacggaccgacaagtctctatcaccaagccaataagggagttagagtcgcctactggataggctttgacaccaccccttttatgtttaagaacttggctggagcatatccatcatactctaccaactgggccgacgaaaccgtgttaacggctcgtaacataggcctatgcagctctgacgttatggagcggtcacgtagagggatgtccattcttagaaagaagtatttgaaaccatccaacaatgttctattctctgttggctcgaccatctaccacgaaaagagggacttactgaggagctggcacctgccgtctgtatttcacttacgtggcaagcaaaattacacatgtcggtgtgagactatagttagttgcgacgggtacgtcgttaaaagaatagctatcagtccaggcctgtatgggaagccttcaggctatgctgctacgatgcaccgcgagggattcttgtgctgcaaagtgacagacacattgaacggggagagggtctcttttcccgtgtgcacgtatgtgccagctacattgtgtgaccaaatgactggcatactggcaacagatgtcagtgcggacgacgcgcaaaaactgctggttgggctcaaccagcgtatagtcgtcaacggtcgcacccagagaaacaccaataccatgaaaaattaccttttgcccgtagtggcccaggcatttgctaggtgggcaaaggaatataaggaagatcaagaagatgaaaggccactaggactacgagatagacagttagtcatggggtgttgttgggcttttagaaggcacaagataacatctatttataagcgcccggatacccaaaccatcatcaaagtgaacagcgatttccactcattcgtgctgcccaggataggcagtaacacattggagatcgggctgagaacaagaatcaggaaaatgttagaggagcacaaggagccgtcacctctcattaccgccgaggacgtacaagaagctaagtgcgcagccgatgaggctaaggaggtgcgtgaagccgaggagttgcgcgcagctctaccacctttggcagctgatgttgaggagcccactctggaagccgatgtcgacttgatgttacaagaggctggggccggctcagtggagacacctcgtggcttgataaaggttaccagctacgctggcgaggacaagatcggctcttacgctgtgctttctccgcaggctgtactcaagagtgaaaaattatcttgcatccaccctctcgctgaacaagtcatagtgataacacactctggccgaaaagggcgttatgccgtggaaccataccatggtaaagtagtggtgccagagggacatgcaatacccgtccaggactttcaagctctgagtgaaagtgccaccattgtgtacaacgaacgtgagttcgtaaacaggtacctgcaccatattgccacacatggaggagcgctgaacactgatgaagaatattacaaaactgtcaagcccagcgagcacgacggcgaatacctgtacgacatcgacaggaaacagtgcgtcaagaaagagctagtcactgggctagggctcacaggcgagctggtcgatcctcccttccatgaattcgcctacgagagtctgagaacacgaccagccgctccttaccaagtaccaaccataggggtgtatggcgtgccaggatcaggcaagtctggcatcattaaaagcgcagtcaccaaaaaagatctagtggtgagcgccaagaaagaaaactgtgcagaaattataagggacgtcaagaaaatgaaagggctggacgtcaatgccagaactgtggactcagtgctcttgaatggatgcaaacaccccgtagagaccctgtatattgacgaggcttttgcttgtcatgcaggtactctcagagcgctcatagccattataagacctaaaaaggcagtgctctgcggagatcccaaacagtgcggtttttttaacatgatgtgcctgaaagtgcattttaaccacgagatttgcacacaagtcttccacaaaagcatctctcgccgttgcactaaatctgtgacttcggtcgtctcaaccttgttttacgacaaaaaaatgagaacgacgaatccgaaagagactaagattgtgattgacactaccggcagtaccaaacctaagcaggacgatctcattctcacttgtttcagagggtgggtgaagcagttgcaaatagattacaaaggcaacgaaataatgacggcagctgcctctcaagggctgacccgtaaaggtgtgtatgccgttcggtacaaggtgaatgaaaatcctctgtacgcacccacctcagaacatgtgaacgtcctactgacccgcacggaggaccgcatcgtgtggaaaacactagccggcgacccatggataaaaacactgactgccaagtaccctgggaatttcactgccacgatagaggagtggcaagcagagcatgatgccatcatgaggcacatcttggagagaccggaccctaccgacgtcttccagaataaggcaaacgtgtgttgggccaaggctttagtgccggtgctgaagaccgctggcatagacatgaccactgaacaatggaacactgtggattattttgaaacggacaaagctcactcagcagagatagtattgaaccaactatgcgtgaggttctttggactcgatctggactccggtctattttctgcacccactgttccgttatccattaggaataatcactgggataactccccgtcgcctaacatgtacgggctgaataaagaagtggtccgtcagctctctcgcaggtacccacaactgcctcgggcagttgccactggtagagtctatgacatgaacactggtacactgcgcaattatgatccgcgcataaacctagtacctgtaaacagaagactgcctcatgctttagtcctccaccataatgaacacccacagagtgacttttcttcattcgtcagcaaattgaagggcagaactgtcctggtggtcggggaaaagttgtccgtcccaggcaaaatggttgactggttgtcagaccggcctgaggctaccttcagagctcggctggatttaggcatcccaggtgatgtgcccaaatatgacataatatttgttaatgtgaggaccccatataaataccatcactatcagcagtgtgaagaccatgccattaagctaagcatgttgaccaagaaagcatgtctgcatctgaatcccggcggaacctgtgtcagcataggttatggttacgctgacagggccagcgaaagcatcattggtgctatagcgcggcagttcaagttttcccgagtatgcaaaccgaaatcctcacttgaggagacggaagttctgtttgtattcattgggtacgatcgcaaggcccgtacgcacaatccttacaagctatcatcaaccttgaccaacatttatacaggttccagactccacgaagccggatgtgcaccctcatatcatgtggtgcgaggggatattgccacggccaccgaaggagtgattataaatgctgctaacagcaaaggacaacctggcggaggggtgtgcggagcgctgtataagaaattcccggaaagtttcgatttacagccgatcgaagtaggaaaagcgcgactggtcaaaggtgcagctaaacatatcattcatgccgtaggaccaaacttcaacaaagtttcggaggttgaaggtgacaaacagttggcagaggcttatgagtccatcgctaagattgtcaacgataacaattacaagtcagtagcgattccactgttgtccaccggcatcttttccgggaacaaagatcgactaacccaatcattgaaccatttgctgacagctttagacaccactgatgcagatgtagccatatactgcagggacaagaaatgggaaatgactctcaaggaagcagtggctaggagagaagcagtggaggagatatgcatatccgacgattcttcagtgacagaacctgatgcagagctggtgagggtgcatcccaagagttctttggctggaaggaagggctacagcacaagcgatggcaaaactttctcatatttggaagggaccaagtttcaccaggcggccaaggatatagcagaaattaatgccatgtggcccgttgcaacggaggccaatgagcaggtatgcatgtatatcctcggagaaagcatgagcagtattaggtcgaaatgccccgtcgaggagtcggaagcctccacaccacctagcacgctgccttgcttgtgcatccatgccatgactccagaaagagtacagcgcctaaaagcctcacgtccagaacaaattactgtgtgctcatcctttccattgccgaagtatagaatcactggtgtgcagaagatccaatgctcccagcctatattgttctcaccgaaagtgcctgcgtatattcatccaaggaagtatctcgtggaaacaccaccggtagacgagactccggagccatcggcagagaaccaatccacagaggggacacctgaacaaccaccacttataaccgaggatgagaccaggactagaacgcctgagccgatcatcatcgaagaagaagaagaagatagcataagtttgctgtcagatggcccgacccaccaggtgctgcaagtcgaggcagacattcacgggccgccctctgtatctagctcatcctggtccattcctcatgcatccgactttgatgtggacagtttatccatacttgacaccctggagggagctagcgtgaccagcggggcaacgtcagccgagactaactcttacttcgcaaagagtatggagtttctggcgcgaccggtgcctgcgcctcgaacagtattcaggaaccctccacatcccgctccgcgcacaagaacaccgtcacttgcacccagcagggcctgctccagaaccagcctagtttccaccccgccaggcgtgaatagggtgatcactagagaggagctcgaagcgcttaccccgtcacgcactcctagcaggtcggtctccagaaccagcctggtctccaacccgccaggcgtaaatagggtgattacaagagaggagtttgaggcgttcgtagcacaacaacaatgacggtttgatgcgggtgcatacatcttttcctccgacaccggtcaagggcatttacaacaaaaatcagtaaggcaaacggtgctatccgaagtggtgttggagaggaccgaattggagatttcgtatgccccgcgcctcgaccaagaaaaagaagaattactacgcaagaaattacagttaaatcccacacctgctaacagaagcagataccagtccaggaaggtggagaacatgaaagccataacagctagacgtattctgcaaggcctagggcattatttgaaggcagaaggaaaagtggagtgctaccgaaccctgcatcctgttcctttgtattcatctagtgtgaaccgtgccttttcaagccccaaggtcgcagtggaagcctgtaacgccatgttgaaagagaactttccgactgtggcttcttactgtattattccagagtacgatgcctatttggacatggttgacggagcttcatgctgcttagacactgccagtttttgccctgcaaagctgcgcagctttccaaagaaacactcctatttggaacccacaatacgatcggcagtgccttcagcgatccagaacacgctccagaacgtcctggcagctgccacaaaaagaaattgcaatgtcacgcaaatgagagaattgcccgtattggattcggcggcctttaatgtggaatgcttcaagaaatatgcgtgtaataatgaatattgggaaacgtttaaagaaaaccccatcaggcttactgaagaaaacgtggtaaattacattaccaaattaaaaggaccaaaagctgctgctctttttgcgaagacacataatttgaatatgttgcaggacataccaatggacaggtttgtaatggacttaaagagagacgtgaaagtgactccaggaacaaaacatactgaagaacggcccaaggtacaggtgatccaggctgccgatccgctagcaacagcgtatctgtgcggaatccaccgagagctggttaggagattaaatgcggtcctgcttccgaacattcatacactgtttgatatgtcggctgaagactttgacgctattatagccgagcacttccagcctggggattgtgttctggaaactgacatcgcgtcgtttgataaaagtgaggacgacgccatggctctgaccgcgttaatgattctggaagacttaggtgtggacgcagagctgttgacgctgattgaggcggctttcggcgaaatttcatcaatacatttgcccactaaaactaaatttaaattcggagccatgatgaaatctggaatgttcctcacactgtttgtgaacacagtcattaacattgtaatcgcaagcagagtgttgagagaacggctaaccggatcaccatgtgcagcattcattggagatgacaatatcgtgaaaggagtcaaatcggacaaattaatggcagacaggtgcgccacctggttgaatatggaagtcaagattatagatgctgtggtgggcgagaaagcgccttatttctgtggagggtttattttgtgtgactccgtgaccggcacagcgtgccgtgtggcagaccccctaaaaaggctgtttaagctaggcaaacctctggcagcagacgatgaacatgatgatgacaggagaagggcattgcatgaggagtcaacacgctggaaccgagtgggtattctttcagagctgtgcaaggcagtagaatcaaggtatgaaaccgtaggaacttccatcatagttatggccatgactactctagctagcagtgttaaatcattcagctacctgagaggggcccctataactctctacggctaacctgaatggactacgacatagtctagtccgccaagactagtatgtttgtgtttcttgtgctgctgcctcttgtgtcttctcagtgtgtggtgagatttccaaatattacaaatctgtgtccatttggagaagtgtttaatgcaacaagatttgcatctgtgtatgcatggaatagaaaaagaatttctaattgtgtggctgattattctgtgctgtataatagtgcttctttttccacatttaaatgttatggagtgtctccaacaaaattaaatgatttatgttttacaaatgtgtatgctgattcttttgtgatcagaggtgatgaagtgagacagattgcccccggacagacaggaaaaattgctgattacaattacaaactgcctgatgattttacaggatgtgtgattgcttggaattctaataatttagattctaaagtgggaggaaattacaattatctgtacagactgtttagaaaatcaaatctgaaaccttttgaaagagatatttcaacagaaatttatcaggctggatcaacaccttgtaatggagtggaaggatttaattgttattttccattacagagctatggatttcagccaaccaatggtgtgggatatcagccatatagagtggtggtgctgtcttttgaactgctgcatgcacctgcaacagtgtgtggacctaaaggctcccccggctccggctccggatctggttatattcctgaagctccaagagatgggcaagcttacgttcgtaaagatggcgaatgggtattactttctacctttttaggaagcggcagcggatctgaacagtacattaaatggccttggtacatttggcttggatttattgcaggattaattgcaattgtgatggtgacaattatgttatgttgtatgacatcatgttgttcttgtttaaaaggatgttgttcttgtggaagctgttgtaaatttgatgaagatgattctgaacctgtgttaaaaggagtgaaattgcattacacatgatgactcgagctggtactgcatgcacgcaatgctagctgcccctttcccgtcctgggtaccccgagtctcccccgacctcgggtcccaggtatgctcccacctccacctgccccactcaccacctctgctagttccagacacctcccaagcacgcagcaatgcagctcaaaacgcttagcctagccacacccccacgggaaacagcagtgattaacctttagcaataaacgaaagtttaactaagctatactaaccccagggttggtcaatttcgtgccagccacaccgcggccgcatgaatacagcagcaattggcaagctgcttacatagaactcgcggcgattggcatgccgccttaaaatttttattttattttttcttttcttttccgaatcggattttgtttttaatatttcaaaaaaaaaaaaaaaaaaaaaaaaaaaaaagcatatgactaaaaaaaaaaaaaaaaaaaaaaaaaaaaaaaaaaaaaaaaaaaaaaaaaaaaaaaaaaaaaaaaaaaaaa

SEQ ID NO: 28 - protein, 327 aa, synthetic construct
  REGION 1..327: note = Vaccine Antigen
MFVFLVLLPLVSSQCVVRFPNITNLCPFGEVFNATRFASVYAWNRKRISNCVADYSVLYNSASFSTFKCYGVSPTKLNDLCFTNVYADSFVIRGDEVRQIAPGQTGKIADYNYKLPDDFTGCVIAWNSNNLDSKVGGNYNYLYRLFRKSNLKPFERDISTEIYQAGSTPCNGVEGFNCYFPLQSYGFQPTNGVGYQPYRVVVLSFELLHAPATVCGPKGSPGSGSGSGYIPEAPRDGQAYVRKDGEWVLLSTFLGSGSGSEQYIKWPWYIWLGFIAGLIAIVMVTIMLCCMTSCCSCLKGCCSCGSCCKFDEDDSEPVLKGVKLHYT

SEQ ID NO: 29 - protein, 311 aa, synthetic construct
  REGION 1..311: note = BNT162b3c
MFVFLVLLPLVSSQCVNLTVRFPNITNLCPFGEVFNATRFASVYAWNRKRISNCVADYSVLYNSASFSTFKCYGVSPTKLNDLCFTNVYADSFVIRGDEVRQIAPGQTGKIADYNYKLPDDFTGCVIAWNSNNLDSKVGGNYNYLYRLFRKSNLKPFERDISTEIYQAGSTPCNGVEGFNCYFPLQSYGFQPTNGVGYQPYRVVVLSFELLHAPATVCGPKGSPGSGSGSGYIPEAPRDGQAYVRKDGEWVLLSTFLGSGSGSEQYIKWPWYIWLGFIAGLIAIVMVTIMLCCMTSCCSCLKGCCSCGSCC

SEQ ID NO: 30 - RNA, 1397 nt, synthetic construct
  misc_feature 1..1397: note = BNT162b3c
  source 1..1397: mol_type = other RNA
agaataaactagtattcttctggtccccacagactcagagagaacccgccaccatgtttgtgtttcttgtgctgctgcctcttgtgtcttctcagtgtgtgaatttgacagtgagatttccaaatattacaaatctgtgtccatttggagaagtgtttaatgcaacaagatttgcatctgtgtatgcatggaatagaaaaagaatttctaattgtgtggctgattattctgtgctgtataatagtgcttctttttccacatttaaatgttatggagtgtctccaacaaaattaaatgatttatgttttacaaatgtgtatgctgattcttttgtgatcagaggtgatgaagtgagacagattgcccccggacagacaggaaaaattgctgattacaattacaaactgcctgatgattttacaggatgtgtgattgcttggaattctaataatttagattctaaagtgggaggaaattacaattatctgtacagactgtttagaaaatcaaatctgaaaccttttgaaagagatatttcaacagaaatttatcaggctggatcaacaccttgtaatggagtggaaggatttaattgttattttccattacagagctatggatttcagccaaccaatggtgtgggatatcagccatatagagtggtggtgctgtcttttgaactgctgcatgcacctgcaacagtgtgtggacctaaaggctcccccggctccggctccggatctggttatattcctgaagctccaagagatgggcaagcttacgttcgtaaagatggcgaatgggtattactttctacctttttaggaagcggcagcggatctgaacagtacattaaatggccttggtacatttggcttggatttattgcaggattaattgcaattgtgatggtgacaattatgttatgttgtatgacatcatgttgttcttgtttaaaaggatgttgttcttgtggaagctgttgttgatgactcgagctggtactgcatgcacgcaatgctagctgcccctttcccgtcctgggtaccccgagtctcccccgacctcgggtcccaggtatgctcccacctccacctgccccactcaccacctctgctagttccagacacctcccaagcacgcagcaatgcagctcaaaacgcttagcctagccacacccccacgggaaacagcagtgattaacctttagcaataaacgaaagtttaactaagctatactaaccccagggttggtcaatttcgtgccagccacaccctggagctagcaaaaaaaaaaaaaaaaaaaaaaaaaaaaaagcatatgactaaaaaaaaaaaaaaaaaaaaaaaaaaaaaaaaaaaaaaaaaaaaaaaaaaaaaaaaaaaaaaaaaaaaaa

SEQ ID NO: 31 - protein, 314 aa, synthetic construct
  REGION 1..314: note = BNT162b3d
MDWIWRILFLVGAATGAHSQMQVRFPNITNLCPFGEVFNATRFASVYAWNRKRISNCVADYSVLYNSASFSTFKCYGVSPTKLNDLCFTNVYADSFVIRGDEVRQIAPGQTGKIADYNYKLPDDFTGCVIAWNSNNLDSKVGGNYNYLYRLFRKSNLKPFERDISTEIYQAGSTPCNGVEGFNCYFPLQSYGFQPTNGVGYQPYRVVVLSFELLHAPATVCGPKGSPGSGSGSGYIPEAPRDGQAYVRKDGEWVLLSTFLGSGSGSEQYIKWPWYIWLGFIAGLIAIVMVTIMLCCMTSCCSCLKGCCSCGSCC

SEQ ID NO: 32 - RNA, 1406 nt, synthetic construct
  misc_feature 1..1406: note = BNT162b3d
  source 1..1406: mol_type = other RNA
agaataaactagtattcttctggtccccacagactcagagagaacccgccaccatggattggatttggagaatcctgttcctcgtgggagccgctacaggagcccactcccagatgcaggtgagatttccaaatattacaaatctgtgtccatttggagaagtgtttaatgcaacaagatttgcatctgtgtatgcatggaatagaaaaagaatttctaattgtgtggctgattattctgtgctgtataatagtgcttctttttccacatttaaatgttatggagtgtctccaacaaaattaaatgatttatgttttacaaatgtgtatgctgattcttttgtgatcagaggtgatgaagtgagacagattgcccccggacagacaggaaaaattgctgattacaattacaaactgcctgatgattttacaggatgtgtgattgcttggaattctaataatttagattctaaagtgggaggaaattacaattatctgtacagactgtttagaaaatcaaatctgaaaccttttgaaagagatatttcaacagaaatttatcaggctggatcaacaccttgtaatggagtggaaggatttaattgttattttccattacagagctatggatttcagccaaccaatggtgtgggatatcagccatatagagtggtggtgctgtcttttgaactgctgcatgcacctgcaacagtgtgtggacctaaaggctcccccggctccggctccggatctggttatattcctgaagctccaagagatgggcaagcttacgttcgtaaagatggcgaatgggtattactttctacctttttaggaagcggcagcggatctgaacagtacattaaatggccttggtacatttggcttggatttattgcaggattaattgcaattgtgatggtgacaattatgttatgttgtatgacatcatgttgttcttgtttaaaaggatgttgttcttgtggaagctgttgttgatgactcgagctggtactgcatgcacgcaatgctagctgcccctttcccgtcctgggtaccccgagtctcccccgacctcgggtcccaggtatgctcccacctccacctgccccactcaccacctctgctagttccagacacctcccaagcacgcagcaatgcagctcaaaacgcttagcctagccacacccccacgggaaacagcagtgattaacctttagcaataaacgaaagtttaactaagctatactaaccccagggttggtcaatttcgtgccagccacaccctggagctagcaaaaaaaaaaaaaaaaaaaaaaaaaaaaaagcatatgactaaaaaaaaaaaaaaaaaaaaaaaaaaaaaaaaaaaaaaaaaaaaaaaaaaaaaaaaaaaaaaaaaaaaaa

SEQ ID NO: 33 - protein, 9 aa, synthetic construct
  REGION 1..9: note = Linker
GSPGSGSGS

SEQ ID NO: 34 - protein, 6 aa, synthetic construct
  REGION 1..6: note = Linker
GSGSGS

SEQ ID NO: 35 - protein, 9 aa, synthetic construct
  REGION 1..9: note = Epitope
YLQPRTFLL

SEQ ID NO: 36 - protein, 9 aa, synthetic construct
  REGION 1..9: note = Epitope
RLQSLQTYV

SEQ ID NO: 37 - protein, 9 aa, synthetic construct
  REGION 1..9: note = Epitope
QYIKWPWYI

SEQ ID NO: 38 - protein, 9 aa, synthetic construct
  REGION 1..9: note = Epitope
NYNYLYRLF

SEQ ID NO: 39 - protein, 10 aa, synthetic construct
  REGION 1..10: note = Epitope
KWPWYIWLGF

SEQ ID NO: 40 - protein, 9 aa, synthetic construct
  REGION 1..9: note = Epitope
QPTESIVRF

SEQ ID NO: 41 - protein, 9 aa, synthetic construct
  REGION 1..9: note = Epitope
IPFAMQMAY

SEQ ID NO: 42 - protein, 9 aa, synthetic construct
  REGION 1..9: note = Epitope
LPFNDGVYF

SEQ ID NO: 43 - protein, 9 aa, synthetic construct
  REGION 1..9: note = Epitope
GVYFASTEK

SEQ ID NO: 44 - protein, 9 aa, synthetic construct
  REGION 1..9: note = Epitope
CVADYSVLY

SEQ ID NO: 45 - protein, 9 aa, synthetic construct
  REGION 1..9: note = Epitope
KCYGVSPTK

SEQ ID NO: 46 - protein, 9 aa, synthetic construct
  REGION 1..9: note = Epitope
FQPTNGVGY

SEQ ID NO: 47 - protein, 9 aa, synthetic construct
  REGION 1..9: note = Epitope
GTHWFVTQR

SEQ ID NO: 48 - protein, 9 aa, synthetic construct
  REGION 1..9: note = Epitope
VYDPLQPEL

SEQ ID NO: 49 - protein, 1270 aa, synthetic construct
  REGION 1..1270: note = Vaccine sequence
MFVFLVLLPLVSSQCVNLTTRTQLPPAYTNSFTRGVYYPDKVFRSSVLHSTQDLFLPFFSNVTWFHVISGTNGTKRFDNPVLPFNDGVYFASIEKSNIIRGWIFGTTLDSKTQSLLIVNNATNVVIKVCEFQFCNDPFLDHKNNKSWMESEFRVYSSANNCTFEYVSQPFLMDLEGKQGNFKNLREFVFKNIDGYFKIYSKHTPIIVREPEDLPQGFSALEPLVDLPIGINITRFQTLLALHRSYLTPGDSSSGWTAGAAAYYVGYLQPRTFLLKYNENGTITDAVDCALDPLSETKCTLKSFTVEKGIYQTSNFRVQPTESIVRFPNITNLCPFDEVFNATRFASVYAWNRKRISNCVADYSVLYNLAPFFTFKCYGVSPTKLNDLCFTNVYADSFVIRGDEVRQIAPGQTGNIADYNYKLPDDFTGCVIAWNSNKLDSKVSGNYNYLYRLFRKSNLKPFERDISTEIYQAGNKPCNGVAGFNCYFPLRSYSFRPTYGVGHQPYRVVVLSFELLHAPATVCGPKKSTNLVKNKCVNFNFNGLKGTGVLTESNKKFLPFQQFGRDIADTTDAVRDPQTLEILDITPCSFGGVSVITPGTNTSNQVAVLYQGVNCTEVPVAIHADQLTPTWRVYSTGSNVFQTRAGCLIGAEYVNNSYECDIPIGAGICASYQTQTKSHRRARSVASQSIIAYTMSLGAENSVAYSNNSIAIPTNFTISVTTEILPVSMTKTSVDCTMYICGDSTECSNLLLQYGSFCTQLKRALTGIAVEQDKNTQEVFAQVKQIYKTPPIKYFGGFNFSQILPDPSKPSKRSFIEDLLFNKVTLADAGFIKQYGDCLGDIAARDLICAQKFKGLTVLPPLLTDEMIAQYTSALLAGTITSGWTFGAGAALQIPFAMQMAYRFNGIGVTQNVLYENQKLIANQFNSAIGKIQDSLSSTASALGKLQDVVNHNAQALNTLVKQLSSKFGAISSVLNDIFSRLDPPEAEVQIDRLITGRLQSLQTYVTQQLIRAAEIRASANLAATKMSECVLGQSKRVDFCGKGYHLMSFPQSAPHGVVFLHVTYVPAQEKNFTTAPAICHDGKAHFPREGVFVSNGTHWFVTQRNFYEPQIITTDNTFVSGNCDVVIGIVNNTVYDPLQPELDSFKEELDKYFKNHTSPDVDLGDISGINASVVNIQKEIDRLNEVAKNLNESLIDLQELGKYEQYIKWPWYIWLGFIAGLIAIVMVTIMLCCMTSCCSCLKGCCSCGSCCKFDEDDSEPVLKGVKLHYT

SEQ ID NO: 50 - RNA, 3816 nt, synthetic construct
  misc_feature 1..3816: note = Coding sequence
  source 1..3816: mol_type = other RNA
atgttcgtgttcctggtgctgctgcctctggtgtccagccagtgtgtgaacctgaccaccagaacacagctgcctccagcctacaccaacagctttaccagaggcgtgtactaccccgacaaggtgttcagatccagcgtgctgcactctacccaggacctgttcctgcctttcttcagcaacgtgacctggttccacgtgatctccggcaccaatggcaccaagagattcgacaaccccgtgctgcccttcaacgacggggtgtactttgccagcatcgagaagtccaacatcatcagaggctggatcttcggcaccacactggacagcaagacccagagcctgctgatcgtgaacaacgccaccaacgtggtcatcaaagtgtgcgagttccagttctgcaacgaccccttcctggaccacaagaacaacaagagctggatggaaagcgagttccgggtgtacagcagcgccaacaactgcaccttcgagtacgtgtcccagcctttcctgatggacctggaaggcaagcagggcaacttcaagaacctgcgcgagttcgtgtttaagaacatcgacggctacttcaagatctacagcaagcacacccctatcatcgtgagagagcccgaggatctgcctcagggcttctctgctctggaacccctggtggatctgcccatcggcatcaacatcacccggtttcagacactgctggccctgcacagaagctacctgacacctggcgatagcagcagcggatggacagctggtgccgccgcttactatgtgggctacctgcagcctagaaccttcctgctgaagtacaacgagaacggcaccatcaccgacgccgtggattgtgctctggatcctctgagcgagacaaagtgcaccctgaagtccttcaccgtggaaaagggcatctaccagaccagcaacttccgggtgcagcccaccgaatccatcgtgcggttccccaatatcaccaatctgtgccccttcgacgaggtgttcaatgccaccagattcgcctctgtgtacgcctggaaccggaagcggatcagcaattgcgtggccgactactccgtgctgtacaacctggcccccttcttcaccttcaagtgctacggcgtgtcccctaccaagctgaacgacctgtgcttcacaaacgtgtacgccgacagcttcgtgatccggggagatgaagtgcggcagattgcccctggacagacaggcaacatcgccgactacaactacaagctgcccgacgacttcaccggctgtgtgattgcctggaacagcaacaagctggactccaaagtcagcggcaactacaattacctgtaccggctgttccggaagtccaatctgaagcccttcgagcgggacatctccaccgagatctatcaggccggcaacaagccttgtaacggcgtggccggcttcaactgctacttcccactgcggtcctacagctttaggcccacatacggcgtgggccaccagccctacagagtggtggtgctgagcttcgaactgctgcatgcccctgccacagtgtgcggccctaagaaaagcaccaatctcgtgaagaacaaatgcgtgaacttcaacttcaacggcctgaagggcaccggcgtgctgacagagagcaacaagaagttcctgccattccagcagtttggccgggatatcgccgataccacagacgccgttagagatccccagacactggaaatcctggacatcaccccttgcagcttcggcggagtgtctgtgatcacccctggcaccaacaccagcaatcaggtggcagtgctgtaccagggcgtgaactgtaccgaagtgcccgtggccattcacgccgatcagctgacacctacatggcgggtgtactccaccggcagcaatgtgtttcagaccagagccggctgtctgatcggagccgagtacgtgaacaatagctacgagtgcgacatccccatcggcgctggaatctgcgccagctaccagacacagacaaagagccaccggagagccagaagcgtggccagccagagcatcattgcctacacaatgtctctgggcgccgagaacagcgtggcctactccaacaactctatcgctatccccaccaacttcaccatcagcgtgaccacagagatcctgcctgtgtccatgaccaagaccagcgtggactgcaccatgtacatctgcggcgattccaccgagtgctccaacctgctgctgcagtacggcagcttctgcacccagctgaaaagagccctgacagggatcgccgtggaacaggacaagaacacccaagaggtgttcgcccaagtgaagcagatctacaagacccctcctatcaagtacttcggcggcttcaatttcagccagattctgcccgatcctagcaagcccagcaagcggagcttcatcgaggacctgctgttcaacaaagtgacactggccgacgccggcttcatcaagcagtatggcgattgtctgggcgacattgccgccagggatctgatttgcgcccagaagtttaagggactgacagtgctgcctcctctgctgaccgatgagatgatcgcccagtacacatctgccctgctggccggcacaatcacaagcggctggacatttggagcaggcgccgctctgcagatcccctttgctatgcagatggcctaccggttcaacggcatcggagtgacccagaatgtgctgtacgagaaccagaagctgatcgccaaccagttcaacagcgccatcggcaagatccaggacagcctgagcagcacagcaagcgccctgggaaagctgcaggacgtggtcaaccacaatgcccaggcactgaacaccctggtcaagcagctgtcctccaagttcggcgccatcagctctgtgctgaacgatatcttcagcagactggaccctcctgaggccgaggtgcagatcgacagactgatcacaggcagactgcagagcctccagacatacgtgacccagcagctgatcagagccgccgagattagagcctctgccaatctggccgccaccaagatgtctgagtgtgtgctgggccagagcaagagagtggacttttgcggcaagggctaccacctgatgagcttccctcagtctgcccctcacggcgtggtgtttctgcacgtgacatatgtgcccgctcaagagaagaatttcaccaccgctccagccatctgccacgacggcaaagcccactttcctagagaaggcgtgttcgtgtccaacggcacccattggttcgtgacacagcggaacttctacgagccccagatcatcaccaccgacaacaccttcgtgtctggcaactgcgacgtcgtgatcggcattgtgaacaataccgtgtacgaccctctgcagcccgagctggacagcttcaaagaggaactggacaagtactttaagaaccacacaagccccgacgtggacctgggcgatatcagcggaatcaatgccagcgtcgtgaacatccagaaagagatcgaccggctgaacgaggtggccaagaatctgaacgagagcctgatcgacctgcaagaactggggaagtacgagcagtacatcaagtggccctggtacatctggctgggctttatcgccggactgattgccatcgtgatggtcacaatcatgctgtgttgcatgaccagctgctgtagctgcctgaagggctgttgtagctgtggcagctgctgcaagttcgacgaggacgattctgagcccgtgctgaagggcgtgaaactgcactacacatgatga

SEQ ID NO: 51 - RNA, 4274 nt, synthetic construct
  misc_feature 1..4274: note = Vaccine RNA
  source 1..4274: mol_type = other RNA
agaataaactagtattcttctggtccccacagactcagagagaacccgccaccatgttcgtgttcctggtgctgctgcctctggtgtccagccagtgtgtgaacctgaccaccagaacacagctgcctccagcctacaccaacagctttaccagaggcgtgtactaccccgacaaggtgttcagatccagcgtgctgcactctacccaggacctgttcctgcctttcttcagcaacgtgacctggttccacgtgatctccggcaccaatggcaccaagagattcgacaaccccgtgctgcccttcaacgacggggtgtactttgccagcatcgagaagtccaacatcatcagaggctggatcttcggcaccacactggacagcaagacccagagcctgctgatcgtgaacaacgccaccaacgtggtcatcaaagtgtgcgagttccagttctgcaacgaccccttcctggaccacaagaacaacaagagctggatggaaagcgagttccgggtgtacagcagcgccaacaactgcaccttcgagtacgtgtcccagcctttcctgatggacctggaaggcaagcagggcaacttcaagaacctgcgcgagttcgtgtttaagaacatcgacggctacttcaagatctacagcaagcacacccctatcatcgtgagagagcccgaggatctgcctcagggcttctctgctctggaacccctggtggatctgcccatcggcatcaacatcacccggtttcagacactgctggccctgcacagaagctacctgacacctggcgatagcagcagcggatggacagctggtgccgccgcttactatgtgggctacctgcagcctagaaccttcctgctgaagtacaacgagaacggcaccatcaccgacgccgtggattgtgctctggatcctctgagcgagacaaagtgcaccctgaagtccttcaccgtggaaaagggcatctaccagaccagcaacttccgggtgcagcccaccgaatccatcgtgcggttccccaatatcaccaatctgtgccccttcgacgaggtgttcaatgccaccagattcgcctctgtgtacgcctggaaccggaagcggatcagcaattgcgtggccgactactccgtgctgtacaacctggcccccttcttcaccttcaagtgctacggcgtgtcccctaccaagctgaacgacctgtgcttcacaaacgtgtacgccgacagcttcgtgatccggggagatgaagtgcggcagattgcccctggacagacaggcaacatcgccgactacaactacaagctgcccgacgacttcaccggctgtgtgattgcctggaacagcaacaagctggactccaaagtcagcggcaactacaattacctgtaccggctgttccggaagtccaatctgaagcccttcgagcgggacatctccaccgagatctatcaggccggcaacaagccttgtaacggcgtggccggcttcaactgctacttcccactgcggtcctacagctttaggcccacatacggcgtgggccaccagccctacagagtggtggtgctgagcttcgaactgctgcatgcccctgccacagtgtgcggccctaagaaaagcaccaatctcgtgaagaacaaatgcgtgaacttcaacttcaacggcctgaagggcaccggcgtgctgacagagagcaacaagaagttcctgccattccagcagtttggccgggatatcgccgataccacagacgccgttagagatccccagacactggaaatcctggacatcaccccttgcagcttcggcggagtgtctgtgatcacccctggcaccaacaccagcaatcaggtggcagtgctgtaccagggcgtgaactgtaccgaagtgcccgtggccattcacgccgatcagctgacacctacatggcgggtgtactccaccggcagcaatgtgtttcagaccagagccggctgtctgatcggagccgagtacgtgaacaatagctacgagtgcgacatccccatcggcgctggaatctgcgccagctaccagacacagacaaagagccaccggagagccagaagcgtggccagccagagcatcattgcctacacaatgtctctgggcgccgagaacagcgtggcctactccaacaactctatcgctatccccaccaacttcaccatcagcgtgaccacagagatcctgcctgtgtccatgaccaagaccagcgtggactgcaccatgtacatctgcggcgattccaccgagtgctccaacctgctgctgcagtacggcagcttctgcacccagctgaaaagagccctgacagggatcgccgtggaacaggacaagaacacccaagaggtgttcgcccaagtgaagcagatctacaagacccctcctatcaagtacttcggcggcttcaatttcagccagattctgcccgatcctagcaagcccagcaagcggagcttcatcgaggacctgctgttcaacaaagtgacactggccgacgccggcttcatcaagcagtatggcgattgtctgggcgacattgccgccagggatctgatttgcgcccagaagtttaagggactgacagtgctgcctcctctgctgaccgatgagatgatcgcccagtacacatctgccctgctggccggcacaatcacaagcggctggacatttggagcaggcgccgctctgcagatcccctttgctatgcagatggcctaccggttcaacggcatcggagtgacccagaatgtgctgtacgagaaccagaagctgatcgccaaccagttcaacagcgccatcggcaagatccaggacagcctgagcagcacagcaagcgccctgggaaagctgcaggacgtggtcaaccacaatgcccaggcactgaacaccctggtcaagcagctgtcctccaagttcggcgccatcagctctgtgctgaacgatatcttcagcagactggaccctcctgaggccgaggtgcagatcgacagactgatcacaggcagactgcagagcctccagacatacgtgacccagcagctgatcagagccgccgagattagagcctctgccaatctggccgccaccaagatgtctgagtgtgtgctgggccagagcaagagagtggacttttgcggcaagggctaccacctgatgagcttccctcagtctgcccctcacggcgtggtgtttctgcacgtgacatatgtgcccgctcaagagaagaatttcaccaccgctccagccatctgccacgacggcaaagcccactttcctagagaaggcgtgttcgtgtccaacggcacccattggttcgtgacacagcggaacttctacgagccccagatcatcaccaccgacaacaccttcgtgtctggcaactgcgacgtcgtgatcggcattgtgaacaataccgtgtacgaccctctgcagcccgagctggacagcttcaaagaggaactggacaagtactttaagaaccacacaagccccgacgtggacctgggcgatatcagcggaatcaatgccagcgtcgtgaacatccagaaagagatcgaccggctgaacgaggtggccaagaatctgaacgagagcctgatcgacctgcaagaactggggaagtacgagcagtacatcaagtggccctggtacatctggctgggctttatcgccggactgattgccatcgtgatggtcacaatcatgctgtgttgcatgaccagctgctgtagctgcctgaagggctgttgtagctgtggcagctgctgcaagttcgacgaggacgattctgagcccgtgctgaagggcgtgaaactgcactacacatgatgactcgagctggtactgcatgcacgcaatgctagctgcccctttcccgtcctgggtaccccgagtctcccccgacctcgggtcccaggtatgctcccacctccacctgccccactcaccacctctgctagttccagacacctcccaagcacgcagcaatgcagctcaaaacgcttagcctagccacacccccacgggaaacagcagtgattaacctttagcaataaacgaaagtttaactaagctatactaaccccagggttggtcaatttcgtgccagccacaccctggagctagcaaaaaaaaaaaaaaaaaaaaaaaaaaaaaagcatatgactaaaaaaaaaaaaaaaaaaaaaaaaaaaaaaaaaaaaaaaaaaaaaaaaaaaaaaaaaaaaaaaaaaaaaa

SEQ ID NO: 52 - protein, 1270 aa, synthetic construct
  REGION 1..1270: note = Vaccine sequence
MFVFLVLLPLVSSQCVNLTTRTQLPPAYTNSFTRGVYYPDKVFRSSVLHSTQDLFLPFFSNVTWFHVISGTNGTKRFDNPVLPFNDGVYFASIEKSNIIRGWIFGTTLDSKTQSLLIVNNATNVVIKVCEFQFCNDPFLDHKNNKSWMESEFRVYSSANNCTFEYVSQPFLMDLEGKQGNFKNLREFVFKNIDGYFKIYSKHTPIIVREPEDLPQGFSALEPLVDLPIGINITRFQTLLALHRSYLTPGDSSSGWTAGAAAYYVGYLQPRTFLLKYNENGTITDAVDCALDPLSETKCTLKSFTVEKGIYQTSNFRVQPTESIVRFPNITNLCPFDEVFNATRFASVYAWNRKRISNCVADYSVLYNLAPFFTFKCYGVSPTKLNDLCFTNVYADSFVIRGDEVRQIAPGQTGKIADYNYKLPDDFTGCVIAWNSNNLDSKVGGNYNYLYRLFRKSNLKPFERDISTEIYQAGNKPCNGVAGFNCYFPLRSYSFRPTYGVGHQPYRVVVLSFELLHAPATVCGPKKSTNLVKNKCVNFNFNGLKGTGVLTESNKKFLPFQQFGRDIADTTDAVRDPQTLEILDITPCSFGGVSVITPGTNTSNQVAVLYQGVNCTEVPVAIHADQLTPTWRVYSTGSNVFQTRAGCLIGAEYVNNSYECDIPIGAGICASYQTQTKSHRRARSVASQSIIAYTMSLGAENSVAYSNNSIAIPTNFTISVTTEILPVSMTKTSVDCTMYICGDSTECSNLLLQYGSFCTQLKRALTGIAVEQDKNTQEVFAQVKQIYKTPPIKYFGGFNFSQILPDPSKPSKRSFIEDLLFNKVTLADAGFIKQYGDCLGDIAARDLICAQKFKGLTVLPPLLTDEMIAQYTSALLAGTITSGWTFGAGAALQIPFAMQMAYRFNGIGVTQNVLYENQKLIANQFNSAIGKIQDSLSSTASALGKLQDVVNHNAQALNTLVKQLSSKFGAISSVLNDIFSRLDPPEAEVQIDRLITGRLQSLQTYVTQQLIRAAEIRASANLAATKMSECVLGQSKRVDFCGKGYHLMSFPQSAPHGVVFLHVTYVPAQEKNFTTAPAICHDGKAHFPREGVFVSNGTHWFVTQRNFYEPQIITTDNTFVSGNCDVVIGIVNNTVYDPLQPELDSFKEELDKYFKNHTSPDVDLGDISGINASVVNIQKEIDRLNEVAKNLNESLIDLQELGKYEQYIKWPWYIWLGFIAGLIAIVMVTIMLCCMTSCCSCLKGCCSCGSCCKFDEDDSEPVLKGVKLHYT

SEQ ID NO: 53 - RNA, 3816 nt, synthetic construct
  misc_feature 1..3816: note = Coding sequence
  source 1..3816: mol_type = other RNA
atgttcgtgttcctggtgctgctgcctctggtgtccagccagtgtgtgaacctgaccaccagaacacagctgcctccagcctacaccaacagctttaccagaggcgtgtactaccccgacaaggtgttcagatccagcgtgctgcactctacccaggacctgttcctgcctttcttcagcaacgtgacctggttccacgtgatctccggcaccaatggcaccaagagattcgacaaccccgtgctgcccttcaacgacggggtgtactttgccagcatcgagaagtccaacatcatcagaggctggatcttcggcaccacactggacagcaagacccagagcctgctgatcgtgaacaacgccaccaacgtggtcatcaaagtgtgcgagttccagttctgcaacgaccccttcctggaccacaagaacaacaagagctggatggaaagcgagttccgggtgtacagcagcgccaacaactgcaccttcgagtacgtgtcccagcctttcctgatggacctggaaggcaagcagggcaacttcaagaacctgcgcgagttcgtgtttaagaacatcgacggctacttcaagatctacagcaagcacacccctatcatcgtgagagagcccgaggatctgcctcagggcttctctgctctggaacccctggtggatctgcccatcggcatcaacatcacccggtttcagacactgctggccctgcacagaagctacctgacacctggcgatagcagcagcggatggacagctggtgccgccgcttactatgtgggctacctgcagcctagaaccttcctgctgaagtacaacgagaacggcaccatcaccgacgccgtggattgtgctctggatcctctgagcgagacaaagtgcaccctgaagtccttcaccgtggaaaagggcatctaccagaccagcaacttccgggtgcagcccaccgaatccatcgtgcggttccccaatatcaccaatctgtgccccttcgacgaggtgttcaatgccaccagattcgcctctgtgtacgcctggaaccggaagcggatcagcaattgcgtggccgactactccgtgctgtacaacctggcccccttcttcaccttcaagtgctacggcgtgtcccctaccaagctgaacgacctgtgcttcacaaacgtgtacgccgacagcttcgtgatccggggagatgaagtgcggcagattgcccctggacagacaggcaagatcgccgactacaactacaagctgcccgacgacttcaccggctgtgtgattgcctggaacagcaacaacctggactccaaagtcggcggcaactacaattacctgtaccggctgttccggaagtccaatctgaagcccttcgagcgggacatctccaccgagatctatcaggccggcaacaagccttgtaacggcgtggccggcttcaactgctacttcccactgcggtcctacagctttaggcccacatacggcgtgggccaccagccctacagagtggtggtgctgagcttcgaactgctgcatgcccctgccacagtgtgcggccctaagaaaagcaccaatctcgtgaagaacaaatgcgtgaacttcaacttcaacggcctgaagggcaccggcgtgctgacagagagcaacaagaagttcctgccattccagcagtttggccgggatatcgccgataccacagacgccgttagagatccccagacactggaaatcctggacatcaccccttgcagcttcggcggagtgtctgtgatcacccctggcaccaacaccagcaatcaggtggcagtgctgtaccagggcgtgaactgtaccgaagtgcccgtggccattcacgccgatcagctgacacctacatggcgggtgtactccaccggcagcaatgtgtttcagaccagagccggctgtctgatcggagccgagtacgtgaacaatagctacgagtgcgacatccccatcggcgctggaatctgcgccagctaccagacacagacaaagagccaccggagagccagaagcgtggccagccagagcatcattgcctacacaatgtctctgggcgccgagaacagcgtggcctactccaacaactctatcgctatccccaccaacttcaccatcagcgtgaccacagagatcctgcctgtgtccatgaccaagaccagcgtggactgcaccatgtacatctgcggcgattccaccgagtgctccaacctgctgctgcagtacggcagcttctgcacccagctgaaaagagccctgacagggatcgccgtggaacaggacaagaacacccaagaggtgttcgcccaagtgaagcagatctacaagacccctcctatcaagtacttcggcggcttcaatttcagccagattctgcccgatcctagcaagcccagcaagcggagcttcatcgaggacctgctgttcaacaaagtgacactggccgacgccggcttcatcaagcagtatggcgattgtctgggcgacattgccgccagggatctgatttgcgcccagaagtttaagggactgacagtgctgcctcctctgctgaccgatgagatgatcgcccagtacacatctgccctgctggccggcacaatcacaagcggctggacatttggagcaggcgccgctctgcagatcccctttgctatgcagatggcctaccggttcaacggcatcggagtgacccagaatgtgctgtacgagaaccagaagctgatcgccaaccagttcaacagcgccatcggcaagatccaggacagcctgagcagcacagcaagcgccctgggaaagctgcaggacgtggtcaaccacaatgcccaggcactgaacaccctggtcaagcagctgtcctccaagttcggcgccatcagctctgtgctgaacgatatcttcagcagactggaccctcctgaggccgaggtgcagatcgacagactgatcacaggcagactgcagagcctccagacatacgtgacccagcagctgatcagagccgccgagattagagcctctgccaatctggccgccaccaagatgtctgagtgtgtgctgggccagagcaagagagtggacttttgcggcaagggctaccacctgatgagcttccctcagtctgcccctcacggcgtggtgtttctgcacgtgacatatgtgcccgctcaagagaagaatttcaccaccgctccagccatctgccacgacggcaaagcccactttcctagagaaggcgtgttcgtgtccaacggcacccattggttcgtgacacagcggaacttctacgagccccagatcatcaccaccgacaacaccttcgtgtctggcaactgcgacgtcgtgatcggcattgtgaacaataccgtgtacgaccctctgcagcccgagctggacagcttcaaagaggaactggacaagtactttaagaaccacacaagccccgacgtggacctgggcgatatcagcggaatcaatgccagcgtcgtgaacatccagaaagagatcgaccggctgaacgaggtggccaagaatctgaacgagagcctgatcgacctgcaagaactggggaagtacgagcagtacatcaagtggccctggtacatctggctgggctttatcgccggactgattgccatcgtgatggtcacaatcatgctgtgttgcatgaccagctgctgtagctgcctgaagggctgttgtagctgtggcagctgctgcaagttcgacgaggacgattctgagcccgtgctgaagggcgtgaaactgcactacacatgatga

SEQ ID NO: 54 - RNA, 4274 nt, synthetic construct
  misc_feature 1..4274: note = Vaccine RNA
  source 1..4274: mol_type = other RNA
agaataaactagtattcttctggtccccacagactcagagagaacccgccaccatgttcgtgttcctggtgctgctgcctctggtgtccagccagtgtgtgaacctgaccaccagaacacagctgcctccagcctacaccaacagctttaccagaggcgtgtactaccccgacaaggtgttcagatccagcgtgctgcactctacccaggacctgttcctgcctttcttcagcaacgtgacctggttccacgtgatctccggcaccaatggcaccaagagattcgacaaccccgtgctgcccttcaacgacggggtgtactttgccagcatcgagaagtccaacatcatcagaggctggatcttcggcaccacactggacagcaagacccagagcctgctgatcgtgaacaacgccaccaacgtggtcatcaaagtgtgcgagttccagttctgcaacgaccccttcctggaccacaagaacaacaagagctggatggaaagcgagttccgggtgtacagcagcgccaacaactgcaccttcgagtacgtgtcccagcctttcctgatggacctggaaggcaagcagggcaacttcaagaacctgcgcgagttcgtgtttaagaacatcgacggctacttcaagatctacagcaagcacacccctatcatcgtgagagagcccgaggatctgcctcagggcttctctgctctggaacccctggtggatctgcccatcggcatcaacatcacccggtttcagacactgctggccctgcacagaagctacctgacacctggcgatagcagcagcggatggacagctggtgccgccgcttactatgtgggctacctgcagcctagaaccttcctgctgaagtacaacgagaacggcaccatcaccgacgccgtggattgtgctctggatcctctgagcgagacaaagtgcaccctgaagtccttcaccgtggaaaagggcatctaccagaccagcaacttccgggtgcagcccaccgaatccatcgtgcggttccccaatatcaccaatctgtgccccttcgacgaggtgttcaatgccaccagattcgcctctgtgtacgcctggaaccggaagcggatcagcaattgcgtggccgactactccgtgctgtacaacctggcccccttcttcaccttcaagtgctacggcgtgtcccctaccaagctgaacgacctgtgcttcacaaacgtgtacgccgacagcttcgtgatccggggagatgaagtgcggcagattgcccctggacagacaggcaagatcgccgactacaactacaagctgcccgacgacttcaccggctgtgtgattgcctggaacagcaacaacctggactccaaagtcggcggcaactacaattacctgtaccggctgttccggaagtccaatctgaagcccttcgagcgggacatctccaccgagatctatcaggccggcaacaagccttgtaacggcgtggccggcttcaactgctacttcccactgcggtcctacagctttaggcccacatacggcgtgggccaccagccctacagagtggtggtgctgagcttcgaactgctgcatgcccctgccacagtgtgcggccctaagaaaagcaccaatctcgtgaagaacaaatgcgtgaacttcaacttcaacggcctgaagggcaccggcgtgctgacagagagcaacaagaagttcctgccattccagcagtttggccgggatatcgccgataccacagacgccgttagagatccccagacactggaaatcctggacatcaccccttgcagcttcggcggagtgtctgtgatcacccctggcaccaacaccagcaatcaggtggcagtgctgtaccagggcgtgaactgtaccgaagtgcccgtggccattcacgccgatcagctgacacctacatggcgggtgtactccaccggcagcaatgtgtttcagaccagagccggctgtctgatcggagccgagtacgtgaacaatagctacgagtgcgacatccccatcggcgctggaatctgcgccagctaccagacacagacaaagagccaccggagagccagaagcgtggccagccagagcatcattgcctacacaatgtctctgggcgccgagaacagcgtggcctactccaacaactctatcgctatccccaccaacttcaccatcagcgtgaccacagagatcctgcctgtgtccatgaccaagaccagcgtggactgcaccatgtacatctgcggcgattccaccgagtgctccaacctgctgctgcagtacggcagcttctgcacccagctgaaaagagccctgacagggatcgccgtggaacaggacaagaacacccaagaggtgttcgcccaagtgaagcagatctacaagacccctcctatcaagtacttcggcggcttcaatttcagccagattctgcccgatcctagcaagcccagcaagcggagcttcatcgaggacctgctgttcaacaaagtgacactggccgacgccggcttcatcaagcagtatggcgattgtctgggcgacattgccgccagggatctgatttgcgcccagaagtttaagggactgacagtgctgcctcctctgctgaccgatgagatgatcgcccagtacacatctgccctgctggccggcacaatcacaagcggctggacatttggagcaggcgccgctctgcagatcccctttgctatgcagatggcctaccggttcaacggcatcggagtgacccagaatgtgctgtacgagaaccagaagctgatcgccaaccagttcaacagcgccatcggcaagatccaggacagcctgagcagcacagcaagcgccctgggaaagctgcaggacgtggtcaaccacaatgcccaggcactgaacaccctggtcaagcagctgtcctccaagttcggcgccatcagctctgtgctgaacgatatcttcagcagactggaccctcctgaggccgaggtgcagatcgacagactgatcacaggcagactgcagagcctccagacatacgtgacccagcagctgatcagagccgccgagattagagcctctgccaatctggccgccaccaagatgtctgagtgtgtgctgggccagagcaagagagtggacttttgcggcaagggctaccacctgatgagcttccctcagtctgcccctcacggcgtggtgtttctgcacgtgacatatgtgcccgctcaagagaagaatttcaccaccgctccagccatctgccacgacggcaaagcccactttcctagagaaggcgtgttcgtgtccaacggcacccattggttcgtgacacagcggaacttctacgagccccagatcatcaccaccgacaacaccttcgtgtctggcaactgcgacgtcgtgatcggcattgtgaacaataccgtgtacgaccctctgcagcccgagctggacagcttcaaagaggaactggacaagtactttaagaaccacacaagccccgacgtggacctgggcgatatcagcggaatcaatgccagcgtcgtgaacatccagaaagagatcgaccggctgaacgaggtggccaagaatctgaacgagagcctgatcgacctgcaagaactggggaagtacgagcagtacatcaagtggccctggtacatctggctgggctttatcgccggactgattgccatcgtgatggtcacaatcatgctgtgttgcatgaccagctgctgtagctgcctgaagggctgttgtagctgtggcagctgctgcaagttcgacgaggacgattctgagcccgtgctgaagggcgtgaaactgcactacacatgatgactcgagctggtactgcatgcacgcaatgctagctgcccctttcccgtcctgggtaccccgagtctcccccgacctcgggtcccaggtatgctcccacctccacctgccccactcaccacctctgctagttccagacacctcccaagcacgcagcaatgcagctcaaaacgcttagcctagccacacccccacgggaaacagcagtgattaacctttagcaataaacgaaagtttaactaagctatactaaccccagggttggtcaatttcgtgccagccacaccctggagctagcaaaaaaaaaaaaaaaaaaaaaaaaaaaaaagcatatgactaaaaaaaaaaaaaaaaaaaaaaaaaaaaaaaaaaaaaaaaaaaaaaaaaaaaaaaaaaaaaaaaaaaaaa

SEQ ID NO: 55 - protein, 1270 aa, synthetic construct
MFVFLVLLPLVSSQCVNFTTRTQLPPAYTNSFTRGVYYPDKVFRSSVLHSTQDLFLPFFSNVTWFHAIHVSGTNGTKRFANPVLPFNDGVYFASTEKSNIIRGWIFGTTLDSKTQSLLIVNNATNVVIKVCEFQFCNDPFLGVYYHKNNKSWMESEFRVYSSANNCTFEYVSQPFLMDLEGKQGNFKNLREFVFKNIDGYFKIYSKHTPINLVRGLPQGFSALEPLVDLPIGINITRFQTLHISYLTPGDSSSGWTAGAAAYYVGYLQPRTFLLKYNENGTITDAVDCALDPLSETKCTLKSFTVEKGIYQTSNFRVQPTESIVRFPNITNLCPFGEVFNATRFASVYAWNRKRISNCVADYSVLYNSASFSTFKCYGVSPTKLNDLCFTNVYADSFVIRGDEVRQIAPGQTGNIADYNYKLPDDFTGCVIAWNSNNLDSKVGGNYNYLYRLFRKSNLKPFERDISTEIYQAGSTPCNGVKGFNCYFPLQSYGFQPTYGVGYQPYRVVVLSFELLHAPATVCGPKKSTNLVKNKCVNFNFNGLTGTGVLTESNKKFLPFQQFGRDIADTTDAVRDPQTLEILDITPCSFGGVSVITPGTNTSNQVAVLYQGVNCTEVPVAIHADQLTPTWRVYSTGSNVFQTRAGCLIGAEHVNNSYECDIPIGAGICASYQTQTNSPRRARSVASQSIIAYTMSLGVENSVAYSNNSIAIPTNFTISVTTEILPVSMTKTSVDCTMYICGDSTECSNLLLQYGSFCTQLNRALTGIAVEQDKNTQEVFAQVKQIYKTPPIKDFGGFNFSQILPDPSKPSKRSFIEDLLFNKVTLADAGFIKQYGDCLGDIAARDLICAQKFNGLTVLPPLLTDEMIAQYTSALLAGTITSGWTFGAGAALQIPFAMQMAYRFNGIGVTQNVLYENQKLIANQFNSAIGKIQDSLSSTASALGKLQDVVNQNAQALNTLVKQLSSNFGAISSVLNDILSRLDPPEAEVQIDRLITGRLQSLQTYVTQQLIRAAEIRASANLAATKMSECVLGQSKRVDFCGKGYHLMSFPQSAPHGVVFLHVTYVPAQEKNFTTAPAICHDGKAHFPREGVFVSNGTHWFVTQRNFYEPQIITTDNTFVSGNCDVVIGIVNNTVYDPLQPELDSFKEELDKYFKNHTSPDVDLGDISGINASVVNIQKEIDRLNEVAKNLNESLIDLQELGKYEQYIKWPWYIWLGFIAGLIAIVMVTIMLCCMTSCCSCLKGCCSCGSCCKFDEDDSEPVLKGVKLHYT

SEQ ID NO: 56 - RNA, 3817 nt, synthetic construct
  source 1..3817: mol_type = other RNA
atgttcgtgttcctggtgctgctgcctctggtgtccagccagtgtgtgaacttcaccaccagaacacagctgcctccagcctacaccaacagctttaccagaggcgtgtactaccccgacaaggtgttcagatccagcgtgctgcactctacccaggacctgttcctgcctttcttcagcaacgtgacctggttccacgccatccacgtgtccggcaccaatggcaccaagagattcgccaaccccgtgctgcccttcaacgacggggtgtactttgccagcaccgagaagtccaacatcatcagaggctggatcttcggcaccacactggacagcaagacccagagcctgctgatcgtgaacaacgccaccaacgtggtcatcaaagtgtgcgagttccagttctgcaacgaccccttcctgggcgtctactaccacaagaacaacaagagctggatggaaagcgagttccgggtgtacagcagcgccaacaactgcaccttcgagtacgtgtcccagcctttcctgatggacctggaaggcaagcagggcaacttcaagaacctgcgcgagttcgtgtttaagaacatcgacggctacttcaagatctacagcaagcacacccctatcaacctcgtgcggggcctgcctcagggcttctctgctctggaacccctggtggatctgcccatcggcatcaacatcacccggtttcagacactgcacatcagctacctgacacctggcgatagcagcagcggatggacagctggtgccgccgcttactatgtgggctacctgcagcctagaaccttcctgctgaagtacaacgagaacggcaccatcaccgacgccgtggattgtgctctggatcctctgagcgagacaaagtgcaccctgaagtccttcaccgtggaaaagggcatctaccagaccagcaacttccgggtgcagcccaccgaatccatcgtgcggttccccaatatcaccaatctgtgccccttcggcgaggtgttcaatgccaccagattcgcctctgtgtacgcctggaaccggaagcggatcagcaattgcgtggccgactactccgtgctgtacaactccgccagcttcagcaccttcaagtgctacggcgtgtcccctaccaagctgaacgacctgtgcttcacaaacgtgtacgccgacagcttcgtgatccggggagatgaagtgcggcagattgcccctggacagacaggcaacatcgccgactacaactacaagctgcccgacgacttcaccggctgtgtgattgcctggaacagcaacaacctggactccaaagtcggcggcaactacaattacctgtaccggctgttccggaagtccaatctgaagcccttcgagcgggacatctccaccgagatctatcaggccggcagcaccccttgtaacggcgtgaagggcttcaactgctacttcccactgcagtcctacggctttcagcccacatacggcgtgggctatcagccctacagagtggtggtgctgagcttcgaactgctgcatgcccctgccacagtgtgcggccctaagaaaagcaccaatctcgtgaagaacaaatgcgtgaacttcaacttcaacggcctgaccggcaccggcgtgctgacagagagcaacaagaagttcctgccattccagcagtttggccgggatatcgccgataccacagacgccgttagagatccccagacactggaaatcctggacatcaccccttgcagcttcggcggagtgtctgtgatcacccctggcaccaacaccagcaatcaggtggcagtgctgtaccagggcgtgaactgtaccgaagtgcccgtggccattcacgccgatcagctgacacctacatggcgggtgtactccaccggcagcaatgtgtttcagaccagagccggctgtctgatcggagccgagcacgtgaacaatagctacgagtgcgacatccccatcggcgctggaatctgcgccagctaccagacacagacaaacagccctcggagagccagaagcgtggccagccagagcatcattgcctacacaatgtctctgggcgtcgagaacagcgtggcctactccaacaactctatcgctatccccaccaacttcaccatcagcgtgaccacagagatcctgcctgtgtccatgaccaagaccagcgtggactgcaccatgtacatctgcggcgattccaccgagtgctccaacctgctgctgcagtacggcagcttctgcacccagctgaatagagccctgacagggatcgccgtggaacaggacaagaacacccaagaggtgttcgcccaagtgaagcagatctacaagacccctcctatcaaggacttcggcggcttcaatttcagccagattctgcccgatcctagcaagcccagcaagcggagcttcatcgaggacctgctgttcaacaaagtgacactggccgacgccggcttcatcaagcagtatggcgattgtctgggcgacattgccgccagggatctgatttgcgcccagaagtttaacggactgacagtgctgcctcctctgctgaccgatgagatgatcgcccagtacacatctgccctgctggccggcacaatcacaagcggctggacatttggagcaggcgccgctctgcagatcccctttgctatgcagatggcctaccggttcaacggcatcggagtgacccagaatgtgctgtacgagaaccagaagctgatcgccaaccagttcaacagcgccatcggcaagatccaggacagcctgagcagcacagcaagcgccctgggaaagctgcaggacgtggtcaaccagaatgcccaggcactgaacaccctggtcaagcagctgtcctccaacttcggcgccatcagctctgtgctgaacgatatcctgagcagactggaccctcctgaggccgaggtgcagatcgacagactgatcacaggcagactgcagagcctccagacatacgtgacccagcagctgatcagagccgccgagattagagcctctgccaatctggccgccaccaagatgtctgagtgtgtgctgggccagagcaagagagtggacttttgcggcaagggctaccacctgatgagcttccctcagtctgcccctcacggcgtggtgtttctgcacgtgacatatgtgcccgctcaagagaagaatttcaccaccgctccagccatctgccacgacggcaaagcccactttcctagagaaggcgtgttcgtgtccaacggcacccattggttcgtgacacagcggaacttctacgagccccagatcatcaccaccgacaacaccttcgtgtctggcaactgcgacgtcgtgatcggcattgtgaacaataccgtgtacgaccctctgcagcccgagctggacagcttcaaagaggaactggacaagtactttaagaaccacacaagccccgacgtggacctgggcgatatcagcggaatcaatgccagcgtcgtgaacatccagaaagagatcgaccggctgaacgaggtggccaagaatctgaacgagagcctgatcgacctgcaagaactggggaagtacgagcagtacatcaagtggccctggtacatctggctgggctttatcgccggactgattgccatcgtgatggtcacaatcatgctgtgttgcatgaccagctgctgtagctgcctgaagggctgttgtagctgtggcagctgctgcaagttcgacgaggacgattctgagcccgtgctgaagggcgtgaaactgcactacacatgatgac

SEQ ID NO: 57 - RNA, 4274 nt, synthetic construct
  source 1..4274: mol_type = other RNA
agaataaactagtattcttctggtccccacagactcagagagaacccgccaccatgttcgtgttcctggtgctgctgcctctggtgtccagccagtgtgtgaacttcaccaccagaacacagctgcctccagcctacaccaacagctttaccagaggcgtgtactaccccgacaaggtgttcagatccagcgtgctgcactctacccaggacctgttcctgcctttcttcagcaacgtgacctggttccacgccatccacgtgtccggcaccaatggcaccaagagattcgccaaccccgtgctgcccttcaacgacggggtgtactttgccagcaccgagaagtccaacatcatcagaggctggatcttcggcaccacactggacagcaagacccagagcctgctgatcgtgaacaacgccaccaacgtggtcatcaaagtgtgcgagttccagttctgcaacgaccccttcctgggcgtctactaccacaagaacaacaagagctggatggaaagcgagttccgggtgtacagcagcgccaacaactgcaccttcgagtacgtgtcccagcctttcctgatggacctggaaggcaagcagggcaacttcaagaacctgcgcgagttcgtgtttaagaacatcgacggctacttcaagatctacagcaagcacacccctatcaacctcgtgcggggcctgcctcagggcttctctgctctggaacccctggtggatctgcccatcggcatcaacatcacccggtttcagacactgcacatcagctacctgacacctggcgatagcagcagcggatggacagctggtgccgccgcttactatgtgggctacctgcagcctagaaccttcctgctgaagtacaacgagaacggcaccatcaccgacgccgtggattgtgctctggatcctctgagcgagacaaagtgcaccctgaagtccttcaccgtggaaaagggcatctaccagaccagcaacttccgggtgcagcccaccgaatccatcgtgcggttccccaatatcaccaatctgtgccccttcggcgaggtgttcaatgccaccagattcgcctctgtgtacgcctggaaccggaagcggatcagcaattgcgtggccgactactccgtgctgtacaactccgccagcttcagcaccttcaagtgctacggcgtgtcccctaccaagctgaacgacctgtgcttcacaaacgtgtacgccgacagcttcgtgatccggggagatgaagtgcggcagattgcccctggacagacaggcaacatcgccgactacaactacaagctgcccgacgacttcaccggctgtgtgattgcctggaacagcaacaacctggactccaaagtcggcggcaactacaattacctgtaccggctgttccggaagtccaatctgaagcccttcgagcgggacatctccaccgagatctatcaggccggcagcaccccttgtaacggcgtgaagggcttcaactgctacttcccactgcagtcctacggctttcagcccacatacggcgtgggctatcagccctacagagtggtggtgctgagcttcgaactgctgcatgcccctgccacagtgtgcggccctaagaaaagcaccaatctcgtgaagaacaaatgcgtgaacttcaacttcaacggcctgaccggcaccggcgtgctgacagagagcaacaagaagttcctgccattccagcagtttggccgggatatcgccgataccacagacgccgttagagatccccagacactggaaatcctggacatcaccccttgcagcttcggcggagtgtctgtgatcacccctggcaccaacaccagcaatcaggtggcagtgctgtaccagggcgtgaactgtaccgaagtgcccgtggccattcacgccgatcagctgacacctacatggcgggtgtactccaccggcagcaatgtgtttcagaccagagccggctgtctgatcggagccgagcacgtgaacaatagctacgagtgcgacatccccatcggcgctggaatctgcgccagctaccagacacagacaaacagccctcggagagccagaagcgtggccagccagagcatcattgcctacacaatgtctctgggcgtcgagaacagcgtggcctactccaacaactctatcgctatccccaccaacttcaccatcagcgtgaccacagagatcctgcctgtgtccatgaccaagaccagcgtggactgcaccatgtacatctgcggcgattccaccgagtgctccaacctgctgctgcagtacggcagcttctgcacccagctgaatagagccctgacagggatcgccgtggaacaggacaagaacacccaagaggtgttcgcccaagtgaagcagatctacaagacccctcctatcaaggacttcggcggcttcaatttcagccagattctgcccgatcctagcaagcccagcaagcggagcttcatcgaggacctgctgttcaacaaagtgacactggccgacgccggcttcatcaagcagtatggcgattgtctgggcgacattgccgccagggatctgatttgcgcccagaagtttaacggactgacagtgctgcctcctctgctgaccgatgagatgatcgcccagtacacatctgccctgctggccggcacaatcacaagcggctggacatttggagcaggcgccgctctgcagatcccctttgctatgcagatggcctaccggttcaacggcatcggagtgacccagaatgtgctgtacgagaaccagaagctgatcgccaaccagttcaacagcgccatcggcaagatccaggacagcctgagcagcacagcaagcgccctgggaaagctgcaggacgtggtcaaccagaatgcccaggcactgaacaccctggtcaagcagctgtcctccaacttcggcgccatcagctctgtgctgaacgatatcctgagcagactggaccctcctgaggccgaggtgcagatcgacagactgatcacaggcagactgcagagcctccagacatacgtgacccagcagctgatcagagccgccgagattagagcctctgccaatctggccgccaccaagatgtctgagtgtgtgctgggccagagcaagagagtggacttttgcggcaagggctaccacctgatgagcttccctcagtctgcccctcacggcgtggtgtttctgcacgtgacatatgtgcccgctcaagagaagaatttcaccaccgctccagccatctgccacgacggcaaagcccactttcctagagaaggcgtgttcgtgtccaacggcacccattggttcgtgacacagcggaacttctacgagccccagatcatcaccaccgacaacaccttcgtgtctggcaactgcgacgtcgtgatcggcattgtgaacaataccgtgtacgaccctctgcagcccgagctggacagcttcaaagaggaactggacaagtactttaagaaccacacaagccccgacgtggacctgggcgatatcagcggaatcaatgccagcgtcgtgaacatccagaaagagatcgaccggctgaacgaggtggccaagaatctgaacgagagcctgatcgacctgcaagaactggggaagtacgagcagtacatcaagtggccctggtacatctggctgggctttatcgccggactgattgccatcgtgatggtcacaatcatgctgtgttgcatgaccagctgctgtagctgcctgaagggctgttgtagctgtggcagctgctgcaagttcgacgaggacgattctgagcccgtgctgaagggcgtgaaactgcactacacatgatgactcgagctggtactgcatgcacgcaatgctagctgcccctttcccgtcctgggtaccccgagtctcccccgacctcgggtcccaggtatgctcccacctccacctgccccactcaccacctctgctagttccagacacctcccaagcacgcagcaatgcagctcaaaacgcttagcctagccacacccccacgggaaacagcagtgattaacctttagcaataaacgaaagtttaactaagctatactaaccccagggttggtcaatttcgtgccagccacaccctggagctagcaaaaaaaaaaaaaaaaaaaaaaaaaaaaaagcatatgactaaaaaaaaaaaaaaaaaaaaaaaaaaaaaaaaaaaaaaaaaaaaaaaaaaaaaaaaaaaaaaaaaaaaaa

SEQ ID NO: 58 - protein, 1270 aa, synthetic construct
MFVFLVLLPLVSSQCVNLTTRTQLPPAYTNSFTRGVYYPDKVFRSSVLHSTQDLFLPFFSNVTWFHAISGTNGTKRFDNPVLPFNDGVYFASTEKSNIIRGWIFGTTLDSKTQSLLIVNNATNVVIKVCEFQFCNDPFLGVYHKNNKSWMESEFRVYSSANNCTFEYVSQPFLMDLEGKQGNFKNLREFVFKNIDGYFKIYSKHTPINLVRDLPQGFSALEPLVDLPIGINITRFQTLLALHRSYLTPGDSSSGWTAGAAAYYVGYLQPRTFLLKYNENGTITDAVDCALDPLSETKCTLKSFTVEKGIYQTSNFRVQPTESIVRFPNITNLCPFGEVFNATRFASVYAWNRKRISNCVADYSVLYNSASFSTFKCYGVSPTKLNDLCFTNVYADSFVIRGDEVRQIAPGQTGKIADYNYKLPDDFTGCVIAWNSNNLDSKVGGNYNYLYRLFRKSNLKPFERDISTEIYQAGSTPCNGVEGFNCYFPLQSYGFQPTYGVGYQPYRVVVLSFELLHAPATVCGPKKSTNLVKNKCVNFNFNGLTGTGVLTESNKKFLPFQQFGRDIDDTTDAVRDPQTLEILDITPCSFGGVSVITPGTNTSNQVAVLYQGVNCTEVPVAIHADQLTPTWRVYSTGSNVFQTRAGCLIGAEHVNNSYECDIPIGAGICASYQTQTNSHRRARSVASQSIIAYTMSLGAENSVAYSNNSIAIPINFTISVTTEILPVSMTKTSVDCTMYICGDSTECSNLLLQYGSFCTQLNRALTGIAVEQDKNTQEVFAQVKQIYKTPPIKDFGGFNFSQILPDPSKPSKRSFIEDLLFNKVTLADAGFIKQYGDCLGDIAARDLICAQKFNGLTVLPPLLTDEMIAQYTSALLAGTITSGWTFGAGAALQIPFAMQMAYRFNGIGVTQNVLYENQKLIANQFNSAIGKIQDSLSSTASALGKLQDVVNQNAQALNTLVKQLSSNFGAISSVLNDILARLDPPEAEVQIDRLITGRLQSLQTYVTQQLIRAAEIRASANLAATKMSECVLGQSKRVDFCGKGYHLMSFPQSAPHGVVFLHVTYVPAQEKNFTTAPAICHDGKAHFPREGVFVSNGTHWFVTQRNFYEPQIITTHNTFVSGNCDVVIGIVNNTVYDPLQPELDSFKEELDKYFKNHTSPDVDLGDISGINASVVNIQKEIDRLNEVAKNLNESLIDLQELGKYEQYIKWPWYIWLGFIAGLIAIVMVTIMLCCMTSCCSCLKGCCSCGSCCKFDEDDSEPVLKGVKLHYT

SEQ ID NO: 59 - RNA, 3816 nt, synthetic construct
  source 1..3816: mol_type = other RNA
atgttcgtgttcctggtgctgctgcctctggtgtccagccagtgtgtgaacctgaccaccagaacacagctgcctccagcctacaccaacagctttaccagaggcgtgtactaccccgacaaggtgttcagatccagcgtgctgcactctacccaggacctgttcctgcctttcttcagcaacgtgacctggttccacgccatctccggcaccaatggcaccaagagattcgacaaccccgtgctgcccttcaacgacggggtgtactttgccagcaccgagaagtccaacatcatcagaggctggatcttcggcaccacactggacagcaagacccagagcctgctgatcgtgaacaacgccaccaacgtggtcatcaaagtgtgcgagttccagttctgcaacgaccccttcctgggcgtctaccacaagaacaacaagagctggatggaaagcgagttccgggtgtacagcagcgccaacaactgcaccttcgagtacgtgtcccagcctttcctgatggacctggaaggcaagcagggcaacttcaagaacctgcgcgagttcgtgtttaagaacatcgacggctacttcaagatctacagcaagcacacccctatcaacctcgtgcgggatctgcctcagggcttctctgctctggaacccctggtggatctgcccatcggcatcaacatcacccggtttcagacactgctggccctgcacagaagctacctgacacctggcgatagcagcagcggatggacagctggtgccgccgcttactatgtgggctacctgcagcctagaaccttcctgctgaagtacaacgagaacggcaccatcaccgacgccgtggattgtgctctggatcctctgagcgagacaaagtgcaccctgaagtccttcaccgtggaaaagggcatctaccagaccagcaacttccgggtgcagcccaccgaatccatcgtgcggttccccaatatcaccaatctgtgccccttcggcgaggtgttcaatgccaccagattcgcctctgtgtacgcctggaaccggaagcggatcagcaattgcgtggccgactactccgtgctgtacaactccgccagcttcagcaccttcaagtgctacggcgtgtcccctaccaagctgaacgacctgtgcttcacaaacgtgtacgccgacagcttcgtgatccggggagatgaagtgcggcagattgcccctggacagacaggcaagatcgccgactacaactacaagctgcccgacgacttcaccggctgtgtgattgcctggaacagcaacaacctggactccaaagtcggcggcaactacaattacctgtaccggctgttccggaagtccaatctgaagcccttcgagcgggacatctccaccgagatctatcaggccggcagcaccccttgtaacggcgtggaaggcttcaactgctacttcccactgcagtcctacggctttcagcccacatacggcgtgggctatcagccctacagagtggtggtgctgagcttcgaactgctgcatgcccctgccacagtgtgcggccctaagaaaagcaccaatctcgtgaagaacaaatgcgtgaacttcaacttcaacggcctgaccggcaccggcgtgctgacagagagcaacaagaagttcctgccattccagcagtttggccgggatatcgacgataccacagacgccgttagagatccccagacactggaaatcctggacatcaccccttgcagcttcggcggagtgtctgtgatcacccctggcaccaacaccagcaatcaggtggcagtgctgtaccagggcgtgaactgtaccgaagtgcccgtggccattcacgccgatcagctgacacctacatggcgggtgtactccaccggcagcaatgtgtttcagaccagagccggctgtctgatcggagccgagcacgtgaacaatagctacgagtgcgacatccccatcggcgctggaatctgcgccagctaccagacacagacaaacagccaccggagagccagaagcgtggccagccagagcatcattgcctacacaatgtctctgggcgccgagaacagcgtggcctactccaacaactctatcgctatccccatcaacttcaccatcagcgtgaccacagagatcctgcctgtgtccatgaccaagaccagcgtggactgcaccatgtacatctgcggcgattccaccgagtgctccaacctgctgctgcagtacggcagcttctgcacccagctgaatagagccctgacagggatcgccgtggaacaggacaagaacacccaagaggtgttcgcccaagtgaagcagatctacaagacccctcctatcaaggacttcggcggcttcaatttcagccagattctgcccgatcctagcaagcccagcaagcggagcttcatcgaggacctgctgttcaacaaagtgacactggccgacgccggcttcatcaagcagtatggcgattgtctgggcgacattgccgccagggatctgatttgcgcccagaagtttaacggactgacagtgctgcctcctctgctgaccgatgagatgatcgcccagtacacatctgccctgctggccggcacaatcacaagcggctggacatttggagcaggcgccgctctgcagatcccctttgctatgcagatggcctaccggttcaacggcatcggagtgacccagaatgtgctgtacgagaaccagaagctgatcgccaaccagttcaacagcgccatcggcaagatccaggacagcctgagcagcacagcaagcgccctgggaaagctgcaggacgtggtcaaccagaatgcccaggcactgaacaccctggtcaagcagctgtcctccaacttcggcgccatcagctctgtgctgaacgatatcctggccagactggaccctcctgaggccgaggtgcagatcgacagactgatcacaggcagactgcagagcctccagacatacgtgacccagcagctgatcagagccgccgagattagagcctctgccaatctggccgccaccaagatgtctgagtgtgtgctgggccagagcaagagagtggacttttgcggcaagggctaccacctgatgagcttccctcagtctgcccctcacggcgtggtgtttctgcacgtgacatatgtgcccgctcaagagaagaatttcaccaccgctccagccatctgccacgacggcaaagcccactttcctagagaaggcgtgttcgtgtccaacggcacccattggttcgtgacacagcggaacttctacgagccccagatcatcaccacccacaacaccttcgtgtctggcaactgcgacgtcgtgatcggcattgtgaacaataccgtgtacgaccctctgcagcccgagctggacagcttcaaagaggaactggacaagtactttaagaaccacacaagccccgacgtggacctgggcgatatcagcggaatcaatgccagcgtcgtgaacatccagaaagagatcgaccggctgaacgaggtggccaagaatctgaacgagagcctgatcgacctgcaagaactggggaagtacgagcagtacatcaagtggccctggtacatctggctgggctttatcgccggactgattgccatcgtgatggtcacaatcatgctgtgttgcatgaccagctgctgtagctgcctgaagggctgttgtagctgtggcagctgctgcaagttcgacgaggacgattctgagcccgtgctgaagggcgtgaaactgcactacacatgatga

SEQ ID NO: 60 - RNA, 4274 nt, synthetic construct
  source 1..4274: mol_type = other RNA
agaataaactagtattcttctggtccccacagactcagagagaacccgccaccatgttcgtgttcctggtgctgctgcctctggtgtccagccagtgtgtgaacctgaccaccagaacacagctgcctccagcctacaccaacagctttaccagaggcgtgtactaccccgacaaggtgttcagatccagcgtgctgcactctacccaggacctgttcctgcctttcttcagcaacgtgacctggttccacgccatctccggcaccaatggcaccaagagattcgacaaccccgtgctgcccttcaacgacggggtgtactttgccagcaccgagaagtccaacatcatcagaggctggatcttcggcaccacactggacagcaagacccagagcctgctgatcgtgaacaacgccaccaacgtggtcatcaaagtgtgcgagttccagttctgcaacgaccccttcctgggcgtctaccacaagaacaacaagagctggatggaaagcgagttccgggtgtacagcagcgccaacaactgcaccttcgagtacgtgtcccagcctttcctgatggacctggaaggcaagcagggcaacttcaagaacctgcgcgagttcgtgtttaagaacatcgacggctacttcaagatctacagcaagcacacccctatcaacctcgtgcgggatctgcctcagggcttctctgctctggaacccctggtggatctgcccatcggcatcaacatcacccggtttcagacactgctggccctgcacagaagctacctgacacctggcgatagcagcagcggatggacagctggtgccgccgcttactatgtgggctacctgcagcctagaaccttcctgctgaagtacaacgagaacggcaccatcaccgacgccgtggattgtgctctggatcctctgagcgagacaaagtgcaccctgaagtccttcaccgtggaaaagggcatctaccagaccagcaacttccgggtgcagcccaccgaatccatcgtgcggttccccaatatcaccaatctgtgccccttcggcgaggtgttcaatgccaccagattcgcctctgtgtacgcctggaaccggaagcggatcagcaattgcgtggccgactactccgtgctgtacaactccgccagcttcagcaccttcaagtgctacggcgtgtcccctaccaagctgaacgacctgtgcttcacaaacgtgtacgccgacagcttcgtgatccggggagatgaagtgcggcagattgcccctggacagacaggcaagatcgccgactacaactacaagctgcccgacgacttcaccggctgtgtgattgcctggaacagcaacaacctggactccaaagtcggcggcaactacaattacctgtaccggctgttccggaagtccaatctgaagcccttcgagcgggacatctccaccgagatctatcaggccggcagcaccccttgtaacggcgtggaaggcttcaactgctacttcccactgcagtcctacggctttcagcccacatacggcgtgggctatcagccctacagagtggtggtgctgagcttcgaactgctgcatgcccctgccacagtgtgcggccctaagaaaagcaccaatctcgtgaagaacaaatgcgtgaacttcaacttcaacggcctgaccggcaccggcgtgctgacagagagcaacaagaagttcctgccattccagcagtttggccgggatatcgacgataccacagacgccgttagagatccccagacactggaaatcctggacatcaccccttgcagcttcggcggagtgtctgtgatcacccctggcaccaacaccagcaatcaggtggcagtgctgtaccagggcgtgaactgtaccgaagtgcccgtggccattcacgccgatcagctgacacctacatggcgggtgtactccaccggcagcaatgtgtttcagaccagagccggctgtctgatcggagccgagcacgtgaacaatagctacgagtgcgacatccccatcggcgctggaatctgcgccagctaccagacacagacaaacagccaccggagagccagaagcgtggccagccagagcatcattgcctacacaatgtctctgggcgccgagaacagcgtggcctactccaacaactctatcgctatccccatcaacttcaccatcagcgtgaccacagagatcctgcctgtgtccatgaccaagaccagcgtggactgcaccatgtacatctgcggcgattccaccgagtgctccaacctgctgctgcagtacggcagcttctgcacccagctgaatagagccctgacagggatcgccgtggaacaggacaagaacacccaagaggtgttcgcccaagtgaagcagatctacaagacccctcctatcaaggacttcggcggcttcaatttcagccagattctgcccgatcctagcaagcccagcaagcggagcttcatcgaggacctgctgttcaacaaagtgacactggccgacgccggcttcatcaagcagtatggcgattgtctgggcgacattgccgccagggatctgatttgcgcccagaagtttaacggactgacagtgctgcctcctctgctgaccgatgagatgatcgcccagtacacatctgccctgctggccggcacaatcacaagcggctggacatttggagcaggcgccgctctgcagatcccctttgctatgcagatggcctaccggttcaacggcatcggagtgacccagaatgtgctgtacgagaaccagaagctgatcgccaaccagttcaacagcgccatcggcaagatccaggacagcctgagcagcacagcaagcgccctgggaaagctgcaggacgtggtcaaccagaatgcccaggcactgaacaccctggtcaagcagctgtcctccaacttcggcgccatcagctctgtgctgaacgatatcctggccagactggaccctcctgaggccgaggtgcagatcgacagactgatcacaggcagactgcagagcctccagacatacgtgacccagcagctgatcagagccgccgagattagagcctctgccaatctggccgccaccaagatgtctgagtgtgtgctgggccagagcaagagagtggacttttgcggcaagggctaccacctgatgagcttccctcagtctgcccctcacggcgtggtgtttctgcacgtgacatatgtgcccgctcaagagaagaatttcaccaccgctccagccatctgccacgacggcaaagcccactttcctagagaaggcgtgttcgtgtccaacggcacccattggttcgtgacacagcggaacttctacgagccccagatcatcaccacccacaacaccttcgtgtctggcaactgcgacgtcgtgatcggcattgtgaacaataccgtgtacgaccctctgcagcccgagctggacagcttcaaagaggaactggacaagtactttaagaaccacacaagccccgacgtggacctgggcgatatcagcggaatcaatgccagcgtcgtgaacatccagaaagagatcgaccggctgaacgaggtggccaagaatctgaacgagagcctgatcgacctgcaagaactggggaagtacgagcagtacatcaagtggccctggtacatctggctgggctttatcgccggactgattgccatcgtgatggtcacaatcatgctgtgttgcatgaccagctgctgtagctgcctgaagggctgttgtagctgtggcagctgctgcaagttcgacgaggacgattctgagcccgtgctgaagggcgtgaaactgcactacacatgatgagatctgctggtactgcatgcacgcaatgctagctgcccctttcccgtcctgggtaccccgagtctcccccgacctcgggtcccaggtatgctcccacctccacctgccccactcaccacctctgctagttccagacacctcccaagcacgcagcaatgcagctcaaaacgcttagcctagccacacccccacgggaaacagcagtgattaacctttagcaataaacgaaagtttaactaagctatactaaccccagggttggtcaatttcgtgccagccacaccctggagctagcaaaaaaaaaaaaaaaaaaaaaaaaaaaaaagcatatgactaaaaaaaaaaaaaaaaaaaaaaaaaaaaaaaaaaaaaaaaaaaaaaaaaaaaaaaaaaaaaaaaaaaaaa

SEQ ID NO: 61 - protein, 1271 aa, synthetic construct
MFVFLVLLPLVSSQCVNLRTRTQLPPAYTNSFTRGVYYPDKVFRSSVLHSTQDLFLPFFSNVTWFHAIHVSGTNGTKRFDNPVLPFNDGVYFASTEKSNIIRGWIFGTTLDSKTQSLLIVNNATNVVIKVCEFQFCNDPFLDVYYHKNNKSWMESGVYSSANNCTFEYVSQPFLMDLEGKQGNFKNLREFVFKNIDGYFKIYSKHTPINLVRDLPQGFSALEPLVDLPIGINITRFQTLLALHRSYLTPGDSSSGWTAGAAAYYVGYLQPRTFLLKYNENGTITDAVDCALDPLSETKCTLKSFTVEKGIYQTSNFRVQPTESIVRFPNITNLCPFGEVFNATRFASVYAWNRKRISNCVADYSVLYNSASFSTFKCYGVSPTKLNDLCFTNVYADSFVIRGDEVRQIAPGQTGKIADYNYKLPDDFTGCVIAWNSNNLDSKVGGNYNYRYRLFRKSNLKPFERDISTEIYQAGSKPCNGVEGFNCYFPLQSYGFQPTNGVGYQPYRVVVLSFELLHAPATVCGPKKSTNLVKNKCVNFNFNGLTGTGVLTESNKKFLPFQQFGRDIADTTDAVRDPQTLEILDITPCSFGGVSVITPGTNTSNQVAVLYQGVNCTEVPVAIHADQLTPTWRVYSTGSNVFQTRAGCLIGAEHVNNSYECDIPIGAGICASYQTQTNSRRRARSVASQSIIAYTMSLGAENSVAYSNNSIAIPTNFTISVTTEILPVSMTKTSVDCTMYICGDSTECSNLLLQYGSFCTQLNRALTGIAVEQDKNTQEVFAQVKQIYKTPPIKDFGGFNFSQILPDPSKPSKRSFIEDLLFNKVTLADAGFIKQYGDCLGDIAARDLICAQKFNGLTVLPPLLTDEMIAQYTSALLAGTITSGWTFGAGAALQIPFAMQMAYRFNGIGVTQNVLYENQKLIANQFNSAIGKIQDSLSSTASALGKLQNVVNQNAQALNTLVKQLSSNFGAISSVLNDILSRLDPPEAEVQIDRLITGRLQSLQTYVTQQLIRAAEIRASANLAATKMSECVLGQSKRVDFCGKGYHLMSFPQSAPHGVVFLHVTYVPAQEKNFTTAPAICHDGKAHFPREGVFVSNGTHWFVTQRNFYEPQIITTDNTFVSGNCDVVIGIVNNTVYDPLQPELDSFKEELDKYFKNHTSPDVDLGDISGINASVVNIQKEIDRLNEVAKNLNESLIDLQELGKYEQYIKWPWYIWLGFIAGLIAIVMVTIMLCCMTSCCSCLKGCCSCGSCCKFDEDDSEPVLKGVKLHYT

SEQ ID NO: 62 - DNA, 3819 bp, synthetic construct
  source 1..3819: mol_type = other DNA
atgttcgtgttcctggtgctgctgcctctggtgtccagccagtgtgtgaacctgagaaccagaacacagctgcctccagcctacaccaacagctttaccagaggcgtgtactaccccgacaaggtgttcagatccagcgtgctgcactctacccaggacctgttcctgcctttcttcagcaacgtgacctggttccacgccatccacgtgtccggcaccaatggcaccaagagattcgacaaccccgtgctgcccttcaacgacggggtgtactttgccagcaccgagaagtccaacatcatcagaggctggatcttcggcaccacactggacagcaagacccagagcctgctgatcgtgaacaacgccaccaacgtggtcatcaaagtgtgcgagttccagttctgcaacgaccccttcctggacgtctactaccacaagaacaacaagagctggatggaaagcggcgtgtacagcagcgccaacaactgcaccttcgagtacgtgtcccagcctttcctgatggacctggaaggcaagcagggcaacttcaagaacctgcgcgagttcgtgtttaagaacatcgacggctacttcaagatctacagcaagcacacccctatcaacctcgtgcgggatctgcctcagggcttctctgctctggaacccctggtggatctgcccatcggcatcaacatcacccggtttcagacactgctggccctgcacagaagctacctgacacctggcgatagcagcagcggatggacagctggtgccgccgcttactatgtgggctacctgcagcctagaaccttcctgctgaagtacaacgagaacggcaccatcaccgacgccgtggattgtgctctggatcctctgagcgagacaaagtgcaccctgaagtccttcaccgtggaaaagggcatctaccagaccagcaacttccgggtgcagcccaccgaatccatcgtgcggttccccaatatcaccaatctgtgccccttcggcgaggtgttcaatgccaccagattcgcctctgtgtacgcctggaaccggaagcggatcagcaattgcgtggccgactactccgtgctgtacaactccgccagcttcagcaccttcaagtgctacggcgtgtcccctaccaagctgaacgacctgtgcttcacaaacgtgtacgccgacagcttcgtgatccggggagatgaagtgcggcagattgcccctggacagacaggcaagatcgccgactacaactacaagctgcccgacgacttcaccggctgtgtgattgcctggaacagcaacaacctggactccaaagtcggcggcaactacaattacaggtaccggctgttccggaagtccaatctgaagcccttcgagcgggacatctccaccgagatctatcaggccggcagcaagccttgtaacggcgtggaaggcttcaactgctacttcccactgcagtcctacggctttcagcccacaaatggcgtgggctatcagccctacagagtggtggtgctgagcttcgaactgctgcatgcccctgccacagtgtgcggccctaagaaaagcaccaatctcgtgaagaacaaatgcgtgaacttcaacttcaacggcctgaccggcaccggcgtgctgacagagagcaacaagaagttcctgccattccagcagtttggccgggatatcgccgataccacagacgccgttagagatccccagacactggaaatcctggacatcaccccttgcagcttcggcggagtgtctgtgatcacccctggcaccaacaccagcaatcaggtggcagtgctgtaccagggcgtgaactgtaccgaagtgcccgtggccattcacgccgatcagctgacacctacatggcgggtgtactccaccggcagcaatgtgtttcagaccagagccggctgtctgatcggagccgagcacgtgaacaatagctacgagtgcgacatccccatcggcgctggaatctgcgccagctaccagacacagacaaacagcaggcggagagccagaagcgtggccagccagagcatcattgcctacacaatgtctctgggcgccgagaacagcgtggcctactccaacaactctatcgctatccccaccaacttcaccatcagcgtgaccacagagatcctgcctgtgtccatgaccaagaccagcgtggactgcaccatgtacatctgcggcgattccaccgagtgctccaacctgctgctgcagtacggcagcttctgcacccagctgaatagagccctgacagggatcgccgtggaacaggacaagaacacccaagaggtgttcgcccaagtgaagcagatctacaagacccctcctatcaaggacttcggcggcttcaatttcagccagattctgcccgatcctagcaagcccagcaagcggagcttcatcgaggacctgctgttcaacaaagtgacactggccgacgccggcttcatcaagcagtatggcgattgtctgggcgacattgccgccagggatctgatttgcgcccagaagtttaacggactgacagtgctgcctcctctgctgaccgatgagatgatcgcccagtacacatctgccctgctggccggcacaatcacaagcggctggacatttggagcaggcgccgctctgcagatcccctttgctatgcagatggcctaccggttcaacggcatcggagtgacccagaatgtgctgtacgagaaccagaagctgatcgccaaccagttcaacagcgccatcggcaagatccaggacagcctgagcagcacagcaagcgccctgggaaagctgcagaacgtggtcaaccagaatgcccaggcactgaacaccctggtcaagcagctgtcctccaacttcggcgccatcagctctgtgctgaacgatatcctgagcagactggaccctcctgaggccgaggtgcagatcgacagactgatcacaggcagactgcagagcctccagacatacgtgacccagcagctgatcagagccgccgagattagagcctctgccaatctggccgccaccaagatgtctgagtgtgtgctgggccagagcaagagagtggacttttgcggcaagggctaccacctgatgagcttccctcagtctgcccctcacggcgtggtgtttctgcacgtgacatatgtgcccgctcaagagaagaatttcaccaccgctccagccatctgccacgacggcaaagcccactttcctagagaaggcgtgttcgtgtccaacggcacccattggttcgtgacacagcggaacttctacgagccccagatcatcaccaccgacaacaccttcgtgtctggcaactgcgacgtcgtgatcggcattgtgaacaataccgtgtacgaccctctgcagcccgagctggacagcttcaaagaggaactggacaagtactttaagaaccacacaagccccgacgtggacctgggcgatatcagcggaatcaatgccagcgtcgtgaacatccagaaagagatcgaccggctgaacgaggtggccaagaatctgaacgagagcctgatcgacctgcaagaactggggaagtacgagcagtacatcaagtggccctggtacatctggctgggctttatcgccggactgattgccatcgtgatggtcacaatcatgctgtgttgcatgaccagctgctgtagctgcctgaagggctgttgtagctgtggcagctgctgcaagttcgacgaggacgattctgagcccgtgctgaagggcgtgaaactgcactacacatgatga

SEQ ID NO: 63 - DNA, 4277 bp, synthetic construct
  source 1..4277: mol_type = other DNA
agaataaactagtattcttctggtccccacagactcagagagaacccgccaccatgttcgtgttcctggtgctgctgcctctggtgtccagccagtgtgtgaacctgagaaccagaacacagctgcctccagcctacaccaacagctttaccagaggcgtgtactaccccgacaaggtgttcagatccagcgtgctgcactctacccaggacctgttcctgcctttcttcagcaacgtgacctggttccacgccatccacgtgtccggcaccaatggcaccaagagattcgacaaccccgtgctgcccttcaacgacggggtgtactttgccagcaccgagaagtccaacatcatcagaggctggatcttcggcaccacactggacagcaagacccagagcctgctgatcgtgaacaacgccaccaacgtggtcatcaaagtgtgcgagttccagttctgcaacgaccccttcctggacgtctactaccacaagaacaacaagagctggatggaaagcggcgtgtacagcagcgccaacaactgcaccttcgagtacgtgtcccagcctttcctgatggacctggaaggcaagcagggcaacttcaagaacctgcgcgagttcgtgtttaagaacatcgacggctacttcaagatctacagcaagcacacccctatcaacctcgtgcgggatctgcctcagggcttctctgctctggaacccctggtggatctgcccatcggcatcaacatcacccggtttcagacactgctggccctgcacagaagctacctgacacctggcgatagcagcagcggatggacagctggtgccgccgcttactatgtgggctacctgcagcctagaaccttcctgctgaagtacaacgagaacggcaccatcaccgacgccgtggattgtgctctggatcctctgagcgagacaaagtgcaccctgaagtccttcaccgtggaaaagggcatctaccagaccagcaacttccgggtgcagcccaccgaatccatcgtgcggttccccaatatcaccaatctgtgccccttcggcgaggtgttcaatgccaccagattcgcctctgtgtacgcctggaaccggaagcggatcagcaattgcgtggccgactactccgtgctgtacaactccgccagcttcagcaccttcaagtgctacggcgtgtcccctaccaagctgaacgacctgtgcttcacaaacgtgtacgccgacagcttcgtgatccggggagatgaagtgcggcagattgcccctggacagacaggcaagatcgccgactacaactacaagctgcccgacgacttcaccggctgtgtgattgcctggaacagcaacaacctggactccaaagtcggcggcaactacaattacaggtaccggctgttccggaagtccaatctgaagcccttcgagcgggacatctccaccgagatctatcaggccggcagcaagccttgtaacggcgtggaaggcttcaactgctacttcccactgcagtcctacggctttcagcccacaaatggcgtgggctatcagccctacagagtggtggtgctgagcttcgaactgctgcatgcccctgccacagtgtgcggccctaagaaaagcaccaatctcgtgaagaacaaatgcgtgaacttcaacttcaacggcctgaccggcaccggcgtgctgacagagagcaacaagaagttcctgccattccagcagtttggccgggatatcgccgataccacagacgccgttagagatccccagacactggaaatcctggacatcaccccttgcagcttcggcggagtgtctgtgatcacccctggcaccaacaccagcaatcaggtggcagtgctgtaccagggcgtgaactgtaccgaagtgcccgtggccattcacgccgatcagctgacacctacatggcgggtgtactccaccggcagcaatgtgtttcagaccagagccggctgtctgatcggagccgagcacgtgaacaatagctacgagtgcgacatccccatcggcgctggaatctgcgccagctaccagacacagacaaacagcaggcggagagccagaagcgtggccagccagagcatcattgcctacacaatgtctctgggcgccgagaacagcgtggcctactccaacaactctatcgctatccccaccaacttcaccatcagcgtgaccacagagatcctgcctgtgtccatgaccaagaccagcgtggactgcaccatgtacatctgcggcgattccaccgagtgctccaacctgctgctgcagtacggcagcttctgcacccagctgaatagagccctgacagggatcgccgtggaacaggacaagaacacccaagaggtgttcgcccaagtgaagcagatctacaagacccctcctatcaaggacttcggcggcttcaatttcagccagattctgcccgatcctagcaagcccagcaagcggagcttcatcgaggacctgctgttcaacaaagtgacactggccgacgccggcttcatcaagcagtatggcgattgtctgggcgacattgccgccagggatctgatttgcgcccagaagtttaacggactgacagtgctgcctcctctgctgaccgatgagatgatcgcccagtacacatctgccctgctggccggcacaatcacaagcggctggacatttggagcaggcgccgctctgcagatcccctttgctatgcagatggcctaccggttcaacggcatcggagtgacccagaatgtgctgtacgagaaccagaagctgatcgccaaccagttcaacagcgccatcggcaagatccaggacagcctgagcagcacagcaagcgccctgggaaagctgcagaacgtggtcaaccagaatgcccaggcactgaacaccctggtcaagcagctgtcctccaacttcggcgccatcagctctgtgctgaacgatatcctgagcagactggaccctcctgaggccgaggtgcagatcgacagactgatcacaggcagactgcagagcctccagacatacgtgacccagcagctgatcagagccgccgagattagagcctctgccaatctggccgccaccaagatgtctgagtgtgtgctgggccagagcaagagagtggacttttgcggcaagggctaccacctgatgagcttccctcagtctgcccctcacggcgtggtgtttctgcacgtgacatatgtgcccgctcaagagaagaatttcaccaccgctccagccatctgccacgacggcaaagcccactttcctagagaaggcgtgttcgtgtccaacggcacccattggttcgtgacacagcggaacttctacgagccccagatcatcaccaccgacaacaccttcgtgtctggcaactgcgacgtcgtgatcggcattgtgaacaataccgtgtacgaccctctgcagcccgagctggacagcttcaaagaggaactggacaagtactttaagaaccacacaagccccgacgtggacctgggcgatatcagcggaatcaatgccagcgtcgtgaacatccagaaagagatcgaccggctgaacgaggtggccaagaatctgaacgagagcctgatcgacctgcaagaactggggaagtacgagcagtacatcaagtggccctggtacatctggctgggctttatcgccggactgattgccatcgtgatggtcacaatcatgctgtgttgcatgaccagctgctgtagctgcctgaagggctgttgtagctgtggcagctgctgcaagttcgacgaggacgattctgagcccgtgctgaagggcgtgaaactgcactacacatgatgatttcacctggtactgcatgcacgcaatgctagctgcccctttcccgtcctgggtaccccgagtctcccccgacctcgggtcccaggtatgctcccacctccacctgccccactcaccacctctgctagttccagacacctcccaagcacgcagcaatgcagctcaaaacgcttagcctagccacacccccacgggaaacagcagtgattaacctttagcaataaacgaaagtttaactaagctatactaaccccagggttggtcaatttcgtgccagccacaccctggagctagcaaaaaaaaaaaaaaaaaaaaaaaaaaaaaagcatatgactaaaaaaaaaaaaaaaaaaaaaaaaaaaaaaaaaaaaaaaaaaaaaaaaaaaaaaaaaaaaaaaaaaaaaa

SEQ ID NO: 64 - protein, 1270 aa, synthetic construct
MFVFLVLLPLVSSQCVNLITRTQSYTNSFTRGVYYPDKVFRSSVLHSTQDLFLPFFSNVTWFHAIHVSGTNGTKRFDNPVLPFNDGVYFASTEKSNIIRGWIFGTTLDSKTQSLLIVNNATNVVIKVCEFQFCNDPFLDVYYHKNNKSWMESEFRVYSSANNCTFEYVSQPFLMDLEGKQGNFKNLREFVFKNIDGYFKIYSKHTPINLGRDLPQGFSALEPLVDLPIGINITRFQTLLALHRSYLTPGDSSSGWTAGAAAYYVGYLQPRTFLLKYNENGTITDAVDCALDPLSETKCTLKSFTVEKGIYQTSNFRVQPTESIVRFPNITNLCPFDEVFNATRFASVYAWNRKRISNCVADYSVLYNFAPFFAFKCYGVSPTKLNDLCFTNVYADSFVIRGNEVSQIAPGQTGNIADYNYKLPDDFTGCVIAWNSNKLDSKVGGNYNYLYRLFRKSNLKPFERDISTEIYQAGNKPCNGVAGFNCYFPLRSYGFRPTYGVGHQPYRVVVLSFELLHAPATVCGPKKSTNLVKNKCVNFNFNGLTGTGVLTESNKKFLPFQQFGRDIADTTDAVRDPQTLEILDITPCSFGGVSVITPGTNTSNQVAVLYQGVNCTEVPVAIHADQLTPTWRVYSTGSNVFQTRAGCLIGAEYVNNSYECDIPIGAGICASYQTQTKSHRRARSVASQSIIAYTMSLGAENSVAYSNNSIAIPTNFTISVTTEILPVSMTKTSVDCTMYICGDSTECSNLLLQYGSFCTQLKRALTGIAVEQDKNTQEVFAQVKQIYKTPPIKYFGGFNFSQILPDPSKPSKRSFIEDLLFNKVTLADAGFIKQYGDCLGDIAARDLICAQKFNGLTVLPPLLTDEMIAQYTSALLAGTITSGWTFGAGAALQIPFAMQMAYRFNGIGVTQNVLYENQKLIANQFNSAIGKIQDSLSSTASALGKLQDVVNHNAQALNTLVKQLSSKFGAISSVLNDILSRLDPPEAEVQIDRLITGRLQSLQTYVTQQLIRAAEIRASANLAATKMSECVLGQSKRVDFCGKGYHLMSFPQSAPHGVVFLHVTYVPAQEKNFTTAPAICHDGKAHFPREGVFVSNGTHWFVTQRNFYEPQIITTDNTFVSGNCDVVIGIVNNTVYDPLQPELDSFKEELDKYFKNHTSPDVDLGDISGINASVVNIQKEIDRLNEVAKNLNESLIDLQELGKYEQYIKWPWYIWLGFIAGLIAIVMVTIMLCCMTSCCSCLKGCCSCGSCCKFDEDDSEPVLKGVKLHYT

SEQ ID NO: 65 - RNA, 3816 nt, synthetic construct
  source 1..3816: mol_type = other RNA
atgttcgtgttcctggtgctgctgcctctggtgtccagccagtgtgtgaacctgatcaccagaacacagtcatacaccaacagctttaccagaggcgtgtactaccccgacaaggtgttcagatccagcgtgctgcactctacccaggacctgttcctgcctttcttcagcaacgtgacctggttccacgccatccacgtgtccggcaccaatggcaccaagagattcgacaaccccgtgctgcccttcaacgacggggtgtactttgccagcaccgagaagtccaacatcatcagaggctggatcttcggcaccacactggacagcaagacccagagcctgctgatcgtgaacaacgccaccaacgtggtcatcaaagtgtgcgagttccagttctgcaacgaccccttcctggacgtctactaccacaagaacaacaagagctggatggaaagcgagttccgggtgtacagcagcgccaacaactgcaccttcgagtacgtgtcccagcctttcctgatggacctggaaggcaagcagggcaacttcaagaacctgcgcgagttcgtgtttaagaacatcgacggctacttcaagatctacagcaagcacacccctatcaacctcggccgggatctgcctcagggcttctctgctctggaacccctggtggatctgcccatcggcatcaacatcacccggtttcagacactgctggccctgcacagaagctacctgacacctggcgatagcagcagcggatggacagctggtgccgccgcttactatgtgggctacctgcagcctagaaccttcctgctgaagtacaacgagaacggcaccatcaccgacgccgtggattgtgctctggatcctctgagcgagacaaagtgcaccctgaagtccttcaccgtggaaaagggcatctaccagaccagcaacttccgggtgcagcccaccgaatccatcgtgcggttccccaatatcaccaatctgtgccccttcgacgaggtgttcaatgccaccagattcgcctctgtgtacgcctggaaccggaagcggatcagcaattgcgtggccgactactccgtgctgtacaacttcgcccccttcttcgcattcaagtgctacggcgtgtcccctaccaagctgaacgacctgtgcttcacaaacgtgtacgccgacagcttcgtgatccggggaaacgaagtgtcacagattgcccctggacagacaggcaacatcgccgactacaactacaagctgcccgacgacttcaccggctgtgtgattgcctggaacagcaacaagctggactccaaagtcggcggcaactacaattacctgtaccggctgttccggaagtccaatctgaagcccttcgagcgggacatctccaccgagatctatcaggccggcaacaagccttgtaacggcgtggcaggcttcaactgctacttcccactgaggtcctacggctttaggcccacatacggcgtgggccaccagccctacagagtggtggtgctgagcttcgaactgctgcatgcccctgccacagtgtgcggccctaagaaaagcaccaatctcgtgaagaacaaatgcgtgaacttcaacttcaacggcctgaccggcaccggcgtgctgacagagagcaacaagaagttcctgccattccagcagtttggccgggatatcgccgataccacagacgccgttagagatccccagacactggaaatcctggacatcaccccttgcagcttcggcggagtgtctgtgatcacccctggcaccaacaccagcaatcaggtggcagtgctgtaccagggcgtgaactgtaccgaagtgcccgtggccattcacgccgatcagctgacacctacatggcgggtgtactccaccggcagcaatgtgtttcagaccagagccggctgtctgatcggagccgagtacgtgaacaatagctacgagtgcgacatccccatcggcgctggaatctgcgccagctaccagacacagacaaagagccaccggagagccagaagcgtggccagccagagcatcattgcctacacaatgtctctgggcgccgagaacagcgtggcctactccaacaactctatcgctatccccaccaacttcaccatcagcgtgaccacagagatcctgcctgtgtccatgaccaagaccagcgtggactgcaccatgtacatctgcggcgattccaccgagtgctccaacctgctgctgcagtacggcagcttctgcacccagctgaaaagagccctgacagggatcgccgtggaacaggacaagaacacccaagaggtgttcgcccaagtgaagcagatctacaagacccctcctatcaagtacttcggcggcttcaatttcagccagattctgcccgatcctagcaagcccagcaagcggagcttcatcgaggacctgctgttcaacaaagtgacactggccgacgccggcttcatcaagcagtatggcgattgtctgggcgacattgccgccagggatctgatttgcgcccagaagtttaacggactgacagtgctgcctcctctgctgaccgatgagatgatcgcccagtacacatctgccctgctggccggcacaatcacaagcggctggacatttggagcaggcgccgctctgcagatcccctttgctatgcagatggcctaccggttcaacggcatcggagtgacccagaatgtgctgtacgagaaccagaagctgatcgccaaccagttcaacagcgccatcggcaagatccaggacagcctgagcagcacagcaagcgccctgggaaagctgcaggacgtggtcaaccacaatgcccaggcactgaacaccctggtcaagcagctgtcctccaagttcggcgccatcagctctgtgctgaacgatatcctgagcagactggaccctcctgaggccgaggtgcagatcgacagactgatcacaggcagactgcagagcctccagacatacgtgacccagcagctgatcagagccgccgagattagagcctctgccaatctggccgccaccaagatgtctgagtgtgtgctgggccagagcaagagagtggacttttgcggcaagggctaccacctgatgagcttccctcagtctgcccctcacggcgtggtgtttctgcacgtgacatatgtgcccgctcaagagaagaatttcaccaccgctccagccatctgccacgacggcaaagcccactttcctagagaaggcgtgttcgtgtccaacggcacccattggttcgtgacacagcggaacttctacgagccccagatcatcaccaccgacaacaccttcgtgtctggcaactgcgacgtcgtgatcggcattgtgaacaataccgtgtacgaccctctgcagcccgagctggacagcttcaaagaggaactggacaagtactttaagaaccacacaagccccgacgtggacctgggcgatatcagcggaatcaatgccagcgtcgtgaacatccagaaagagatcgaccggctgaacgaggtggccaagaatctgaacgagagcctgatcgacctgcaagaactggggaagtacgagcagtacatcaagtggccctggtacatctggctgggctttatcgccggactgattgccatcgtgatggtcacaatcatgctgtgttgcatgaccagctgctgtagctgcctgaagggctgttgtagctgtggcagctgctgcaagttcgacgaggacgattctgagcccgtgctgaagggcgtgaaactgcactacacatgatga

SEQ ID NO: 66 - DNA, 3816 bp, synthetic construct
  source 1..3816: mol_type = other DNA
atgttcgtgttcctggtgctgctgcctctggtgtccagccagtgtgtgaacctgatcaccagaacacagtcatacaccaacagctttaccagaggcgtgtactaccccgacaaggtgttcagatccagcgtgctgcactctacccaggacctgttcctgcctttcttcagcaacgtgacctggttccacgccatccacgtgtccggcaccaatggcaccaagagattcgacaaccccgtgctgcccttcaacgacggggtgtactttgccagcaccgagaagtccaacatcatcagaggctggatcttcggcaccacactggacagcaagacccagagcctgctgatcgtgaacaacgccaccaacgtggtcatcaaagtgtgcgagttccagttctgcaacgaccccttcctggacgtctactaccacaagaacaacaagagctggatggaaagcgagttccgggtgtacagcagcgccaacaactgcaccttcgagtacgtgtcccagcctttcctgatggacctggaaggcaagcagggcaacttcaagaacctgcgcgagttcgtgtttaagaacatcgacggctacttcaagatctacagcaagcacacccctatcaacctcggccgggatctgcctcagggcttctctgctctggaacccctggtggatctgcccatcggcatcaacatcacccggtttcagacactgctggccctgcacagaagctacctgacacctggcgatagcagcagcggatggacagctggtgccgccgcttactatgtgggctacctgcagcctagaaccttcctgctgaagtacaacgagaacggcaccatcaccgacgccgtggattgtgctctggatcctctgagcgagacaaagtgcaccctgaagtccttcaccgtggaaaagggcatctaccagaccagcaacttccgggtgcagcccaccgaatccatcgtgcggttccccaatatcaccaatctgtgccccttcgacgaggtgttcaatgccaccagattcgcctctgtgtacgcctggaaccggaagcggatcagcaattgcgtggccgactactccgtgctgtacaacttcgcccccttcttcgcattcaagtgctacggcgtgtcccctaccaagctgaacgacctgtgcttcacaaacgtgtacgccgacagcttcgtgatccggggaaacgaagtgtcacagattgcccctggacagacaggcaacatcgccgactacaactacaagctgcccgacgacttcaccggctgtgtgattgcctggaacagcaacaagctggactccaaagtcggcggcaactacaattacctgtaccggctgttccggaagtccaatctgaagcccttcgagcgggacatctccaccgagatctatcaggccggcaacaagccttgtaacggcgtggcaggcttcaactgctacttcccactgaggtcctacggctttaggcccacatacggcgtgggccaccagccctacagagtggtggtgctgagcttcgaactgctgcatgcccctgccacagtgtgcggccctaagaaaagcaccaatctcgtgaagaacaaatgcgtgaacttcaacttcaacggcctgaccggcaccggcgtgctgacagagagcaacaagaagttcctgccattccagcagtttggccgggatatcgccgataccacagacgccgttagagatccccagacactggaaatcctggacatcaccccttgcagcttcggcggagtgtctgtgatcacccctggcaccaacaccagcaatcaggtggcagtgctgtaccagggcgtgaactgtaccgaagtgcccgtggccattcacgccgatcagctgacacctacatggcgggtgtactccaccggcagcaatgtgtttcagaccagagccggctgtctgatcggagccgagtacgtgaacaatagctacgagtgcgacatccccatcggcgctggaatctgcgccagctaccagacacagacaaagagccaccggagagccagaagcgtggccagccagagcatcattgcctacacaatgtctctgggcgccgagaacagcgtggcctactccaacaactctatcgctatccccaccaacttcaccatcagcgtgaccacagagatcctgcctgtgtccatgaccaagaccagcgtggactgcaccatgtacatctgcggcgattccaccgagtgctccaacctgctgctgcagtacggcagcttctgcacccagctgaaaagagccctgacagggatcgccgtggaacaggacaagaacacccaagaggtgttcgcccaagtgaagcagatctacaagacccctcctatcaagtacttcggcggcttcaatttcagccagattctgcccgatcctagcaagcccagcaagcggagcttcatcgaggacctgctgttcaacaaagtgacactggccgacgccggcttcatcaagcagtatggcgattgtctgggcgacattgccgccagggatctgatttgcgcccagaagtttaacggactgacagtgctgcctcctctgctgaccgatgagatgatcgcccagtacacatctgccctgctggccggcacaatcacaagcggctggacatttggagcaggcgccgctctgcagatcccctttgctatgcagatggcctaccggttcaacggcatcggagtgacccagaatgtgctgtacgagaaccagaagctgatcgccaaccagttcaacagcgccatcggcaagatccaggacagcctgagcagcacagcaagcgccctgggaaagctgcaggacgtggtcaaccacaatgcccaggcactgaacaccctggtcaagcagctgtcctccaagttcggcgccatcagctctgtgctgaacgatatcctgagcagactggaccctcctgaggccgaggtgcagatcgacagactgatcacaggcagactgcagagcctccagacatacgtgacccagcagctgatcagagccgccgagattagagcctctgccaatctggccgccaccaagatgtctgagtgtgtgctgggccagagcaagagagtggacttttgcggcaagggctaccacctgatgagcttccctcagtctgcccctcacggcgtggtgtttctgcacgtgacatatgtgcccgctcaagagaagaatttcaccaccgctccagccatctgccacgacggcaaagcccactttcctagagaaggcgtgttcgtgtccaacggcacccattggttcgtgacacagcggaacttctacgagccccagatcatcaccaccgacaacaccttcgtgtctggcaactgcgacgtcgtgatcggcattgtgaacaataccgtgtacgaccctctgcagcccgagctggacagcttcaaagaggaactggacaagtactttaagaaccacacaagccccgacgtggacctgggcgatatcagcggaatcaatgccagcgtcgtgaacatccagaaagagatcgaccggctgaacgaggtggccaagaatctgaacgagagcctgatcgacctgcaagaactggggaagtacgagcagtacatcaagtggccctggtacatctggctgggctttatcgccggactgattgccatcgtgatggtcacaatcatgctgtgttgcatgaccagctgctgtagctgcctgaagggctgttgtagctgtggcagctgctgcaagttcgacgaggacgattctgagcccgtgctgaagggcgtgaaactgcactacacatgatga

SEQ ID NO: 67 - RNA, 4274 nt, synthetic construct
  source 1..4274: mol_type = other RNA
agaataaactagtattcttctggtccccacagactcagagagaacccgccaccatgttcgtgttcctggtgctgctgcctctggtgtccagccagtgtgtgaacctgatcaccagaacacagtcatacaccaacagctttaccagaggcgtgtactaccccgacaaggtgttcagatccagcgtgctgcactctacccaggacctgttcctgcctttcttcagcaacgtgacctggttccacgccatccacgtgtccggcaccaatggcaccaagagattcgacaaccccgtgctgcccttcaacgacggggtgtactttgccagcaccgagaagtccaacatcatcagaggctggatcttcggcaccacactggacagcaagacccagagcctgctgatcgtgaacaacgccaccaacgtggtcatcaaagtgtgcgagttccagttctgcaacgaccccttcctggacgtctactaccacaagaacaacaagagctggatggaaagcgagttccgggtgtacagcagcgccaacaactgcaccttcgagtacgtgtcccagcctttcctgatggacctggaaggcaagcagggcaacttcaagaacctgcgcgagttcgtgtttaagaacatcgacggctacttcaagatctacagcaagcacacccctatcaacctcggccgggatctgcctcagggcttctctgctctggaacccctggtggatctgcccatcggcatcaacatcacccggtttcagacactgctggccctgcacagaagctacctgacacctggcgatagcagcagcggatggacagctggtgccgccgcttactatgtgggctacctgcagcctagaaccttcctgctgaagtacaacgagaacggcaccatcaccgacgccgtggattgtgctctggatcctctgagcgagacaaagtgcaccctgaagtccttcaccgtggaaaagggcatctaccagaccagcaacttccgggtgcagcccaccgaatccatcgtgcggttccccaatatcaccaatctgtgccccttcgacgaggtgttcaatgccaccagattcgcctctgtgtacgcctggaaccggaagcggatcagcaattgcgtggccgactactccgtgctgtacaacttcgcccccttcttcgcattcaagtgctacggcgtgtcccctaccaagctgaacgacctgtgcttcacaaacgtgtacgccgacagcttcgtgatccggggaaacgaagtgtcacagattgcccctggacagacaggcaacatcgccgactacaactacaagctgcccgacgacttcaccggctgtgtgattgcctggaacagcaacaagctggactccaaagtcggcggcaactacaattacctgtaccggctgttccggaagtccaatctgaagcccttcgagcgggacatctccaccgagatctatcaggccggcaacaagccttgtaacggcgtggcaggcttcaactgctacttcccactgaggtcctacggctttaggcccacatacggcgtgggccaccagccctacagagtggtggtgctgagcttcgaactgctgcatgcccctgccacagtgtgcggccctaagaaaagcaccaatctcgtgaagaacaaatgcgtgaacttcaacttcaacggcctgaccggcaccggcgtgctgacagagagcaacaagaagttcctgccattccagcagtttggccgggatatcgccgataccacagacgccgttagagatccccagacactggaaatcctggacatcaccccttgcagcttcggcggagtgtctgtgatcacccctggcaccaacaccagcaatcaggtggcagtgctgtaccagggcgtgaactgtaccgaagtgcccgtggccattcacgccgatcagctgacacctacatggcgggtgtactccaccggcagcaatgtgtttcagaccagagccggctgtctgatcggagccgagtacgtgaacaatagctacgagtgcgacatccccatcggcgctggaatctgcgccagctaccagacacagacaaagagccaccggagagccagaagcgtggccagccagagcatcattgcctacacaatgtctctgggcgccgagaacagcgtggcctactccaacaactctatcgctatccccaccaacttcaccatcagcgtgaccacagagatcctgcctgtgtccatgaccaagaccagcgtggactgcaccatgtacatctgcggcgattccaccgagtgctccaacctgctgctgcagtacggcagcttctgcacccagctgaaaagagccctgacagggatcgccgtggaacaggacaagaacacccaagaggtgttcgcccaagtgaagcagatctacaagacccctcctatcaagtacttcggcggcttcaatttcagccagattctgcccgatcctagcaagcccagcaagcggagcttcatcgaggacctgctgttcaacaaagtgacactggccgacgccggcttcatcaagcagtatggcgattgtctgggcgacattgccgccagggatctgatttgcgcccagaagtttaacggactgacagtgctgcctcctctgctgaccgatgagatgatcgcccagtacacatctgccctgctggccggcacaatcacaagcggctggacatttggagcaggcgccgctctgcagatcccctttgctatgcagatggcctaccggttcaacggcatcggagtgacccagaatgtgctgtacgagaaccagaagctgatcgccaaccagttcaacagcgccatcggcaagatccaggacagcctgagcagcacagcaagcgccctgggaaagctgcaggacgtggtcaaccacaatgcccaggcactgaacaccctggtcaagcagctgtcctccaagttcggcgccatcagctctgtgctgaacgatatcctgagcagactggaccctcctgaggccgaggtgcagatcgacagactgatcacaggcagactgcagagcctccagacatacgtgacccagcagctgatcagagccgccgagattagagcctctgccaatctggccgccaccaagatgtctgagtgtgtgctgggccagagcaagagagtggacttttgcggcaagggctaccacctgatgagcttccctcagtctgcccctcacggcgtggtgtttctgcacgtgacatatgtgcccgctcaagagaagaatttcaccaccgctccagccatctgccacgacggcaaagcccactttcctagagaaggcgtgttcgtgtccaacggcacccattggttcgtgacacagcggaacttctacgagccccagatcatcaccaccgacaacaccttcgtgtctggcaactgcgacgtcgtgatcggcattgtgaacaataccgtgtacgaccctctgcagcccgagctggacagcttcaaagaggaactggacaagtactttaagaaccacacaagccccgacgtggacctgggcgatatcagcggaatcaatgccagcgtcgtgaacatccagaaagagatcgaccggctgaacgaggtggccaagaatctgaacgagagcctgatcgacctgcaagaactggggaagtacgagcagtacatcaagtggccctggtacatctggctgggctttatcgccggactgattgccatcgtgatggtcacaatcatgctgtgttgcatgaccagctgctgtagctgcctgaagggctgttgtagctgtggcagctgctgcaagttcgacgaggacgattctgagcccgtgctgaagggcgtgaaactgcactacacatgatgactcgagctggtactgcatgcacgcaatgctagctgcccctttcccgtcctgggtaccccgagtctcccccgacctcgggtcccaggtatgctcccacctccacctgccccactcaccacctctgctagttccagacacctcccaagcacgcagcaatgcagctcaaaacgcttagcctagccacacccccacgggaaacagcagtgattaacctttagcaataaacgaaagtttaactaagctatactaaccccagggttggtcaatttcgtgccagccacaccctggagctagcaaaaaaaaaaaaaaaaaaaaaaaaaaaaaagcatatgactaaaaaaaaaaaaaaaaaaaaaaaaaaaaaaaaaaaaaaaaaaaaaaaaaaaaaaaaaaaaaaaaaaaaaa

SEQ ID NO: 68 - DNA, 4274 bp, synthetic construct
  source 1..4274: mol_type = other DNA
agaataaactagtattcttctggtccccacagactcagagagaacccgccaccatgttcgtgttcctggtgctgctgcctctggtgtccagccagtgtgtgaacctgatcaccagaacacagtcatacaccaacagctttaccagaggcgtgtactaccccgacaaggtgttcagatccagcgtgctgcactctacccaggacctgttcctgcctttcttcagcaacgtgacctggttccacgccatccacgtgtccggcaccaatggcaccaagagattcgacaaccccgtgctgcccttcaacgacggggtgtactttgccagcaccgagaagtccaacatcatcagaggctggatcttcggcaccacactggacagcaagacccagagcctgctgatcgtgaacaacgccaccaacgtggtcatcaaagtgtgcgagttccagttctgcaacgaccccttcctggacgtctactaccacaagaacaacaagagctggatggaaagcgagttccgggtgtacagcagcgccaacaactgcaccttcgagtacgtgtcccagcctttcctgatggacctggaaggcaagcagggcaacttcaagaacctgcgcgagttcgtgtttaagaacatcgacggctacttcaagatctacagcaagcacacccctatcaacctcggccgggatctgcctcagggcttctctgctctggaacccctggtggatctgcccatcggcatcaacatcacccggtttcagacactgctggccctgcacagaagctacctgacacctggcgatagcagcagcggatggacagctggtgccgccgcttactatgtgggctacctgcagcctagaaccttcctgctgaagtacaacgagaacggcaccatcaccgacgccgtggattgtgctctggatcctctgagcgagacaaagtgcaccctgaagtccttcaccgtggaaaagggcatctaccagaccagcaacttccgggtgcagcccaccgaatccatcgtgcggttccccaatatcaccaatctgtgccccttcgacgaggtgttcaatgccaccagattcgcctctgtgtacgcctggaaccggaagcggatcagcaattgcgtggccgactactccgtgctgtacaacttcgcccccttcttcgcattcaagtgctacggcgtgtcccctaccaagctgaacgacctgtgcttcacaaacgtgtacgccgacagcttcgtgatccggggaaacgaagtgtcacagattgcccctggacagacaggcaacatcgccgactacaactacaagctgcccgacgacttcaccggctgtgtgattgcctggaacagcaacaagctggactccaaagtcggcggcaactacaattacctgtaccggctgttccggaagtccaatctgaagcccttcgagcgggacatctccaccgagatctatcaggccggcaacaagccttgtaacggcgtggcaggcttcaactgctacttcccactgaggtcctacggctttaggcccacatacggcgtgggccaccagccctacagagtggtggtgctgagcttcgaactgctgcatgcccctgccacagtgtgcggccctaagaaaagcaccaatctcgtgaagaacaaatgcgtgaacttcaacttcaacggcctgaccggcaccggcgtgctgacagagagcaacaagaagttcctgccattccagcagtttggccgggatatcgccgataccacagacgccgttagagatccccagacactggaaatcctggacatcaccccttgcagcttcggcggagtgtctgtgatcacccctggcaccaacaccagcaatcaggtggcagtgctgtaccagggcgtgaactgtaccgaagtgcccgtggccattcacgccgatcagctgacacctacatggcgggtgtactccaccggcagcaatgtgtttcagaccagagccggctgtctgatcggagccgagtacgtgaacaatagctacgagtgcgacatccccatcggcgctggaatctgcgccagctaccagacacagacaaagagccaccggagagccagaagcgtggccagccagagcatcattgcctacacaatgtctctgggcgccgagaacagcgtggcctactccaacaactctatcgctatccccaccaacttcaccatcagcgtgaccacagagatcctgcctgtgtccatgaccaagaccagcgtggactgcaccatgtacatctgcggcgattccaccgagtgctccaacctgctgctgcagtacggcagcttctgcacccagctgaaaagagccctgacagggatcgccgtggaacaggacaagaacacccaagaggtgttcgcccaagtgaagcagatctacaagacccctcctatcaagtacttcggcggcttcaatttcagccagattctgcccgatcctagcaagcccagcaagcggagcttcatcgaggacctgctgttcaacaaagtgacactggccgacgccggcttcatcaagcagtatggcgattgtctgggcgacattgccgccagggatctgatttgcgcccagaagtttaacggactgacagtgctgcctcctctgctgaccgatgagatgatcgcccagtacacatctgccctgctggccggcacaatcacaagcggctggacatttggagcaggcgccgctctgcagatcccctttgctatgcagatggcctaccggttcaacggcatcggagtgacccagaatgtgctgtacgagaaccagaagctgatcgccaaccagttcaacagcgccatcggcaagatccaggacagcctgagcagcacagcaagcgccctgggaaagctgcaggacgtggtcaaccacaatgcccaggcactgaacaccctggtcaagcagctgtcctccaagttcggcgccatcagctctgtgctgaacgatatcctgagcagactggaccctcctgaggccgaggtgcagatcgacagactgatcacaggcagactgcagagcctccagacatacgtgacccagcagctgatcagagccgccgagattagagcctctgccaatctggccgccaccaagatgtctgagtgtgtgctgggccagagcaagagagtggacttttgcggcaagggctaccacctgatgagcttccctcagtctgcccctcacggcgtggtgtttctgcacgtgacatatgtgcccgctcaagagaagaatttcaccaccgctccagccatctgccacgacggcaaagcccactttcctagagaaggcgtgttcgtgtccaacggcacccattggttcgtgacacagcggaacttctacgagccccagatcatcaccaccgacaacaccttcgtgtctggcaactgcgacgtcgtgatcggcattgtgaacaataccgtgtacgaccctctgcagcccgagctggacagcttcaaagaggaactggacaagtactttaagaaccacacaagccccgacgtggacctgggcgatatcagcggaatcaatgccagcgtcgtgaacatccagaaagagatcgaccggctgaacgaggtggccaagaatctgaacgagagcctgatcgacctgcaagaactggggaagtacgagcagtacatcaagtggccctggtacatctggctgggctttatcgccggactgattgccatcgtgatggtcacaatcatgctgtgttgcatgaccagctgctgtagctgcctgaagggctgttgtagctgtggcagctgctgcaagttcgacgaggacgattctgagcccgtgctgaagggcgtgaaactgcactacacatgatgactcgagctggtactgcatgcacgcaatgctagctgcccctttcccgtcctgggtaccccgagtctcccccgacctcgggtcccaggtatgctcccacctccacctgccccactcaccacctctgctagttccagacacctcccaagcacgcagcaatgcagctcaaaacgcttagcctagccacacccccacgggaaacagcagtgattaacctttagcaataaacgaaagtttaactaagctatactaaccccagggttggtcaatttcgtgccagccacaccctggagctagcaaaaaaaaaaaaaaaaaaaaaaaaaaaaaagcatatgactaaaaaaaaaaaaaaaaaaaaaaaaaaaaaaaaaaaaaaaaaaaaaaaaaaaaaaaaaaaaaaaaaaaaaa

SEQ ID NO: 69 - protein, 1268 aa, synthetic construct
MFVFLVLLPLVSSQCVNLITRTQSYTNSFTRGVYYPDKVFRSSVLHSTQDLFLPFFSNVTWFHAISGTNGTKRFDNPVLPFNDGVYFASTEKSNIIRGWIFGTTLDSKTQSLLIVNNATNVVIKVCEFQFCNDPFLDVYYHKNNKSWMESEFRVYSSANNCTFEYVSQPFLMDLEGKQGNFKNLREFVFKNIDGYFKIYSKHTPINLGRDLPQGFSALEPLVDLPIGINITRFQTLLALHRSYLTPGDSSSGWTAGAAAYYVGYLQPRTFLLKYNENGTITDAVDCALDPLSETKCTLKSFTVEKGIYQTSNFRVQPTESIVRFPNITNLCPFDEVFNATRFASVYAWNRKRISNCVADYSVLYNFAPFFAFKCYGVSPTKLNDLCFTNVYADSFVIRGNEVRQIAPGQTGNIADYNYKLPDDFTGCVIAWNSNKLDSKVGGNYNYRYRLFRKSNLKPFERDISTEIYQAGNKPCNGVAGVNCYFPLQSYGFRPTYGVGHQPYRVVVLSFELLHAPATVCGPKKSTNLVKNKCVNFNFNGLTGTGVLTESNKKFLPFQQFGRDIADTTDAVRDPQTLEILDITPCSFGGVSVITPGTNTSNQVAVLYQGVNCTEVPVAIHADQLTPTWRVYSTGSNVFQTRAGCLIGAEYVNNSYECDIPIGAGICASYQTQTKSHRRARSVASQSIIAYTMSLGAENSVAYSNNSIAIPTNFTISVTTEILPVSMTKTSVDCTMYICGDSTECSNLLLQYGSFCTQLKRALTGIAVEQDKNTQEVFAQVKQIYKTPPIKYFGGFNFSQILPDPSKPSKRSFIEDLLFNKVTLADAGFIKQYGDCLGDIAARDLICAQKFNGLTVLPPLLTDEMIAQYTSALLAGTITSGWTFGAGAALQIPFAMQMAYRFNGIGVTQNVLYENQKLIANQFNSAIGKIQDSLSSTASALGKLQDVVNHNAQALNTLVKQLSSKFGAISSVLNDILSRLDPPEAEVQIDRLITGRLQSLQTYVTQQLIRAAEIRASANLAATKMSECVLGQSKRVDFCGKGYHLMSFPQSAPHGVVFLHVTYVPAQEKNFTTAPAICHDGKAHFPREGVFVSNGTHWFVTQRNFYEPQIITTDNTFVSGNCDVVIGIVNNTVYDPLQPELDSFKEELDKYFKNHTSPDVDLGDISGINASVVNIQKEIDRLNEVAKNLNESLIDLQELGKYEQYIKWPWYIWLGFIAGLIAIVMVTIMLCCMTSCCSCLKGCCSCGSCCKFDEDDSEPVLKGVKLHYT

SEQ ID NO: 70 - RNA, 3810 nt, synthetic construct
  source 1..3810: mol_type = other RNA
atgttcgtgttcctggtgctgctgcctctggtgtccagccagtgtgtgaacctgatcaccagaacacagtcatacaccaacagctttaccagaggcgtgtactaccccgacaaggtgttcagatccagcgtgctgcactctacccaggacctgttcctgcctttcttcagcaacgtgacctggttccacgccatctccggcaccaatggcaccaagagattcgacaaccccgtgctgcccttcaacgacggggtgtactttgccagcaccgagaagtccaacatcatcagaggctggatcttcggcaccacactggacagcaagacccagagcctgctgatcgtgaacaacgccaccaacgtggtcatcaaagtgtgcgagttccagttctgcaacgaccccttcctggacgtctactaccacaagaacaacaagagctggatggaaagcgagttccgggtgtacagcagcgccaacaactgcaccttcgagtacgtgtcccagcctttcctgatggacctggaaggcaagcagggcaacttcaagaacctgcgcgagttcgtgtttaagaacatcgacggctacttcaagatctacagcaagcacacccctatcaacctcggccgggatctgcctcagggcttctctgctctggaacccctggtggatctgcccatcggcatcaacatcacccggtttcagacactgctggccctgcacagaagctacctgacacctggcgatagcagcagcggatggacagctggtgccgccgcttactatgtgggctacctgcagcctagaaccttcctgctgaagtacaacgagaacggcaccatcaccgacgccgtggattgtgctctggatcctctgagcgagacaaagtgcaccctgaagtccttcaccgtggaaaagggcatctaccagaccagcaacttccgggtgcagcccaccgaatccatcgtgcggttccccaatatcaccaatctgtgccccttcgacgaggtgttcaatgccaccagattcgcctctgtgtacgcctggaaccggaagcggatcagcaattgcgtggccgactactccgtgctgtacaacttcgcccccttcttcgcattcaagtgctacggcgtgtcccctaccaagctgaacgacctgtgcttcacaaacgtgtacgccgacagcttcgtgatccggggaaacgaagtgcggcagattgcccctggacagacaggcaacatcgccgactacaactacaagctgcccgacgacttcaccggctgtgtgattgcctggaacagcaacaagctggactccaaagtcggcggcaactacaattacaggtaccggctgttccggaagtccaatctgaagcccttcgagcgggacatctccaccgagatctatcaggccggcaacaagccttgtaacggcgtggcaggcgtgaactgctacttcccactgcagtcctacggctttaggcccacatacggcgtgggccaccagccctacagagtggtggtgctgagcttcgaactgctgcatgcccctgccacagtgtgcggccctaagaaaagcaccaatctcgtgaagaacaaatgcgtgaacttcaacttcaacggcctgaccggcaccggcgtgctgacagagagcaacaagaagttcctgccattccagcagtttggccgggatatcgccgataccacagacgccgttagagatccccagacactggaaatcctggacatcaccccttgcagcttcggcggagtgtctgtgatcacccctggcaccaacaccagcaatcaggtggcagtgctgtaccagggcgtgaactgtaccgaagtgcccgtggccattcacgccgatcagctgacacctacatggcgggtgtactccaccggcagcaatgtgtttcagaccagagccggctgtctgatcggagccgagtacgtgaacaatagctacgagtgcgacatccccatcggcgctggaatctgcgccagctaccagacacagacaaagagccaccggagagccagaagcgtggccagccagagcatcattgcctacacaatgtctctgggcgccgagaacagcgtggcctactccaacaactctatcgctatccccaccaacttcaccatcagcgtgaccacagagatcctgcctgtgtccatgaccaagaccagcgtggactgcaccatgtacatctgcggcgattccaccgagtgctccaacctgctgctgcagtacggcagcttctgcacccagctgaaaagagccctgacagggatcgccgtggaacaggacaagaacacccaagaggtgttcgcccaagtgaagcagatctacaagacccctcctatcaagtacttcggcggcttcaatttcagccagattctgcccgatcctagcaagcccagcaagcggagcttcatcgaggacctgctgttcaacaaagtgacactggccgacgccggcttcatcaagcagtatggcgattgtctgggcgacattgccgccagggatctgatttgcgcccagaagtttaacggactgacagtgctgcctcctctgctgaccgatgagatgatcgcccagtacacatctgccctgctggccggcacaatcacaagcggctggacatttggagcaggcgccgctctgcagatcccctttgctatgcagatggcctaccggttcaacggcatcggagtgacccagaatgtgctgtacgagaaccagaagctgatcgccaaccagttcaacagcgccatcggcaagatccaggacagcctgagcagcacagcaagcgccctgggaaagctgcaggacgtggtcaaccacaatgcccaggcactgaacaccctggtcaagcagctgtcctccaagttcggcgccatcagctctgtgctgaacgatatcctgagcagactggaccctcctgaggccgaggtgcagatcgacagactgatcacaggcagactgcagagcctccagacatacgtgacccagcagctgatcagagccgccgagattagagcctctgccaatctggccgccaccaagatgtctgagtgtgtgctgggccagagcaagagagtggacttttgcggcaagggctaccacctgatgagcttccctcagtctgcccctcacggcgtggtgtttctgcacgtgacatatgtgcccgctcaagagaagaatttcaccaccgctccagccatctgccacgacggcaaagcccactttcctagagaaggcgtgttcgtgtccaacggcacccattggttcgtgacacagcggaacttctacgagccccagatcatcaccaccgacaacaccttcgtgtctggcaactgcgacgtcgtgatcggcattgtgaacaataccgtgtacgaccctctgcagcccgagctggacagcttcaaagaggaactggacaagtactttaagaaccacacaagccccgacgtggacctgggcgatatcagcggaatcaatgccagcgtcgtgaacatccagaaagagatcgaccggctgaacgaggtggccaagaatctgaacgagagcctgatcgacctgcaagaactggggaagtacgagcagtacatcaagtggccctggtacatctggctgggctttatcgccggactgattgccatcgtgatggtcacaatcatgctgtgttgcatgaccagctgctgtagctgcctgaagggctgttgtagctgtggcagctgctgcaagttcgacgaggacgattctgagcccgtgctgaagggcgtgaaactgcactacacatgatga

SEQ ID NO: 71 - DNA, 3810 bp, synthetic construct
  source 1..3810: mol_type = other DNA
atgttcgtgttcctggtgctgctgcctctggtgtccagccagtgtgtgaacctgatcaccagaacacagtcatacaccaacagctttaccagaggcgtgtactaccccgacaaggtgttcagatccagcgtgctgcactctacccaggacctgttcctgcctttcttcagcaacgtgacctggttccacgccatctccggcaccaatggcaccaagagattcgacaaccccgtgctgcccttcaacgacggggtgtactttgccagcaccgagaagtccaacatcatcagaggctggatcttcggcaccacactggacagcaagacccagagcctgctgatcgtgaacaacgccaccaacgtggtcatcaaagtgtgcgagttccagttctgcaacgaccccttcctggacgtctactaccacaagaacaacaagagctggatggaaagcgagttccgggtgtacagcagcgccaacaactgcaccttcgagtacgtgtcccagcctttcctgatggacctggaaggcaagcagggcaacttcaagaacctgcgcgagttcgtgtttaagaacatcgacggctacttcaagatctacagcaagcacacccctatcaacctcggccgggatctgcctcagggcttctctgctctggaacccctggtggatctgcccatcggcatcaacatcacccggtttcagacactgctggccctgcacagaagctacctgacacctggcgatagcagcagcggatggacagctggtgccgccgcttactatgtgggctacctgcagcctagaaccttcctgctgaagtacaacgagaacggcaccatcaccgacgccgtggattgtgctctggatcctctgagcgagacaaagtgcaccctgaagtccttcaccgtggaaaagggcatctaccagaccagcaacttccgggtgcagcccaccgaatccatcgtgcggttccccaatatcaccaatctgtgccccttcgacgaggtgttcaatgccaccagattcgcctctgtgtacgcctggaaccggaagcggatcagcaattgcgtggccgactactccgtgctgtacaacttcgcccccttcttcgcattcaagtgctacggcgtgtcccctaccaagctgaacgacctgtgcttcacaaacgtgtacgccgacagcttcgtgatccggggaaacgaagtgcggcagattgcccctggacagacaggcaacatcgccgactacaactacaagctgcccgacgacttcaccggctgtgtgattgcctggaacagcaacaagctggactccaaagtcggcggcaactacaattacaggtaccggctgttccggaagtccaatctgaagcccttcgagcgggacatctccaccgagatctatcaggccggcaacaagccttgtaacggcgtggcaggcgtgaactgctacttcccactgcagtcctacggctttaggcccacatacggcgtgggccaccagccctacagagtggtggtgctgagcttcgaactgctgcatgcccctgccacagtgtgcggccctaagaaaagcaccaatctcgtgaagaacaaatgcgtgaacttcaacttcaacggcctgaccggcaccggcgtgctgacagagagcaacaagaagttcctgccattccagcagtttggccgggatatcgccgataccacagacgccgttagagatccccagacactggaaatcctggacatcaccccttgcagcttcggcggagtgtctgtgatcacccctggcaccaacaccagcaatcaggtggcagtgctgtaccagggcgtgaactgtaccgaagtgcccgtggccattcacgccgatcagctgacacctacatggcgggtgtactccaccggcagcaatgtgtttcagaccagagccggctgtctgatcggagccgagtacgtgaacaatagctacgagtgcgacatccccatcggcgctggaatctgcgccagctaccagacacagacaaagagccaccggagagccagaagcgtggccagccagagcatcattgcctacacaatgtctctgggcgccgagaacagcgtggcctactccaacaactctatcgctatccccaccaacttcaccatcagcgtgaccacagagatcctgcctgtgtccatgaccaagaccagcgtggactgcaccatgtacatctgcggcgattccaccgagtgctccaacctgctgctgcagtacggcagcttctgcacccagctgaaaagagccctgacagggatcgccgtggaacaggacaagaacacccaagaggtgttcgcccaagtgaagcagatctacaagacccctcctatcaagtacttcggcggcttcaatttcagccagattctgcccgatcctagcaagcccagcaagcggagcttcatcgaggacctgctgttcaacaaagtgacactggccgacgccggcttcatcaagcagtatggcgattgtctgggcgacattgccgccagggatctgatttgcgcccagaagtttaacggactgacagtgctgcctcctctgctgaccgatgagatgatcgcccagtacacatctgccctgctggccggcacaatcacaagcggctggacatttggagcaggcgccgctctgcagatcccctttgctatgcagatggcctaccggttcaacggcatcggagtgacccagaatgtgctgtacgagaaccagaagctgatcgccaaccagttcaacagcgccatcggcaagatccaggacagcctgagcagcacagcaagcgccctgggaaagctgcaggacgtggtcaaccacaatgcccaggcactgaacaccctggtcaagcagctgtcctccaagttcggcgccatcagctctgtgctgaacgatatcctgagcagactggaccctcctgaggccgaggtgcagatcgacagactgatcacaggcagactgcagagcctccagacatacgtgacccagcagctgatcagagccgccgagattagagcctctgccaatctggccgccaccaagatgtctgagtgtgtgctgggccagagcaagagagtggacttttgcggcaagggctaccacctgatgagcttccctcagtctgcccctcacggcgtggtgtttctgcacgtgacatatgtgcccgctcaagagaagaatttcaccaccgctccagccatctgccacgacggcaaagcccactttcctagagaaggcgtgttcgtgtccaacggcacccattggttcgtgacacagcggaacttctacgagccccagatcatcaccaccgacaacaccttcgtgtctggcaactgcgacgtcgtgatcggcattgtgaacaataccgtgtacgaccctctgcagcccgagctggacagcttcaaagaggaactggacaagtactttaagaaccacacaagccccgacgtggacctgggcgatatcagcggaatcaatgccagcgtcgtgaacatccagaaagagatcgaccggctgaacgaggtggccaagaatctgaacgagagcctgatcgacctgcaagaactggggaagtacgagcagtacatcaagtggccctggtacatctggctgggctttatcgccggactgattgccatcgtgatggtcacaatcatgctgtgttgcatgaccagctgctgtagctgcctgaagggctgttgtagctgtggcagctgctgcaagttcgacgaggacgattctgagcccgtgctgaagggcgtgaaactgcactacacatgatga

SEQ ID NO: 72 - RNA, 4268 nt, synthetic construct
  source 1..4268: mol_type = other RNA
agaataaactagtattcttctggtccccacagactcagagagaacccgccaccatgttcgtgttcctggtgctgctgcctctggtgtccagccagtgtgtgaacctgatcaccagaacacagtcatacaccaacagctttaccagaggcgtgtactaccccgacaaggtgttcagatccagcgtgctgcactctacccaggacctgttcctgcctttcttcagcaacgtgacctggttccacgccatctccggcaccaatggcaccaagagattcgacaaccccgtgctgcccttcaacgacggggtgtactttgccagcaccgagaagtccaacatcatcagaggctggatcttcggcaccacactggacagcaagacccagagcctgctgatcgtgaacaacgccaccaacgtggtcatcaaagtgtgcgagttccagttctgcaacgaccccttcctggacgtctactaccacaagaacaacaagagctggatggaaagcgagttccgggtgtacagcagcgccaacaactgcaccttcgagtacgtgtcccagcctttcctgatggacctggaaggcaagcagggcaacttcaagaacctgcgcgagttcgtgtttaagaacatcgacggctacttcaagatctacagcaagcacacccctatcaacctcggccgggatctgcctcagggcttctctgctctggaacccctggtggatctgcccatcggcatcaacatcacccggtttcagacactgctggccctgcacagaagctacctgacacctggcgatagcagcagcggatggacagctggtgccgccgcttactatgtgggctacctgcagcctagaaccttcctgctgaagtacaacgagaacggcaccatcaccgacgccgtggattgtgctctggatcctctgagcgagacaaagtgcaccctgaagtccttcaccgtggaaaagggcatctaccagaccagcaacttccgggtgcagcccaccgaatccatcgtgcggttccccaatatcaccaatctgtgccccttcgacgaggtgttcaatgccaccagattcgcctctgtgtacgcctggaaccggaagcggatcagcaattgcgtggccgactactccgtgctgtacaacttcgcccccttcttcgcattcaagtgctacggcgtgtcccctaccaagctgaacgacctgtgcttcacaaacgtgtacgccgacagcttcgtgatccggggaaacgaagtgcggcagattgcccctggacagacaggcaacatcgccgactacaactacaagctgcccgacgacttcaccggctgtgtgattgcctggaacagcaacaagctggactccaaagtcggcggcaactacaattacaggtaccggctgttccggaagtccaatctgaagcccttcgagcgggacatctccaccgagatctatcaggccggcaacaagccttgtaacggcgtggcaggcgtgaactgctacttcccactgcagtcctacggctttaggcccacatacggcgtgggccaccagccctacagagtggtggtgctgagcttcgaactgctgcatgcccctgccacagtgtgcggccctaagaaaagcaccaatctcgtgaagaacaaatgcgtgaacttcaacttcaacggcctgaccggcaccggcgtgctgacagagagcaacaagaagttcctgccattccagcagtttggccgggatatcgccgataccacagacgccgttagagatccccagacactggaaatcctggacatcaccccttgcagcttcggcggagtgtctgtgatcacccctggcaccaacaccagcaatcaggtggcagtgctgtaccagggcgtgaactgtaccgaagtgcccgtggccattcacgccgatcagctgacacctacatggcgggtgtactccaccggcagcaatgtgtttcagaccagagccggctgtctgatcggagccgagtacgtgaacaatagctacgagtgcgacatccccatcggcgctggaatctgcgccagctaccagacacagacaaagagccaccggagagccagaagcgtggccagccagagcatcattgcctacacaatgtctctgggcgccgagaacagcgtggcctactccaacaactctatcgctatccccaccaacttcaccatcagcgtgaccacagagatcctgcctgtgtccatgaccaagaccagcgtggactgcaccatgtacatctgcggcgattccaccgagtgctccaacctgctgctgcagtacggcagcttctgcacccagctgaaaagagccctgacagggatcgccgtggaacaggacaagaacacccaagaggtgttcgcccaagtgaagcagatctacaagacccctcctatcaagtacttcggcggcttcaatttcagccagattctgcccgatcctagcaagcccagcaagcggagcttcatcgaggacctgctgttcaacaaagtgacactggccgacgccggcttcatcaagcagtatggcgattgtctgggcgacattgccgccagggatctgatttgcgcccagaagtttaacggactgacagtgctgcctcctctgctgaccgatgagatgatcgcccagtacacatctgccctgctggccggcacaatcacaagcggctggacatttggagcaggcgccgctctgcagatcccctttgctatgcagatggcctaccggttcaacggcatcggagtgacccagaatgtgctgtacgagaaccagaagctgatcgccaaccagttcaacagcgccatcggcaagatccaggacagcctgagcagcacagcaagcgccctgggaaagctgcaggacgtggtcaaccacaatgcccaggcactgaacaccctggtcaagcagctgtcctccaagttcggcgccatcagctctgtgctgaacgatatcctgagcagactggaccctcctgaggccgaggtgcagatcgacagactgatcacaggcagactgcagagcctccagacatacgtgacccagcagctgatcagagccgccgagattagagcctctgccaatctggccgccaccaagatgtctgagtgtgtgctgggccagagcaagagagtggacttttgcggcaagggctaccacctgatgagcttccctcagtctgcccctcacggcgtggtgtttctgcacgtgacatatgtgcccgctcaagagaagaatttcaccaccgctccagccatctgccacgacggcaaagcccactttcctagagaaggcgtgttcgtgtccaacggcacccattggttcgtgacacagcggaacttctacgagccccagatcatcaccaccgacaacaccttcgtgtctggcaactgcgacgtcgtgatcggcattgtgaacaataccgtgtacgaccctctgcagcccgagctggacagcttcaaagaggaactggacaagtactttaagaaccacacaagccccgacgtggacctgggcgatatcagcggaatcaatgccagcgtcgtgaacatccagaaagagatcgaccggctgaacgaggtggccaagaatctgaacgagagcctgatcgacctgcaagaactggggaagtacgagcagtacatcaagtggccctggtacatctggctgggctttatcgccggactgattgccatcgtgatggtcacaatcatgctgtgttgcatgaccagctgctgtagctgcctgaagggctgttgtagctgtggcagctgctgcaagttcgacgaggacgattctgagcccgtgctgaagggcgtgaaactgcactacacatgatgactcgagctggtactgcatgcacgcaatgctagctgcccctttcccgtcctgggtaccccgagtctcccccgacctcgggtcccaggtatgctcccacctccacctgccccactcaccacctctgctagttccagacacctcccaagcacgcagcaatgcagctcaaaacgcttagcctagccacacccccacgggaaacagcagtgattaacctttagcaataaacgaaagtttaactaagctatactaaccccagggttggtcaatttcgtgccagccacaccctggagctagcaaaaaaaaaaaaaaaaaaaaaaaaaaaaaagcatatgactaaaaaaaaaaaaaaaaaaaaaaaaaaaaaaaaaaaaaaaaaaaaaaaaaaaaaaaaaaaaaaaaaaaaaa

SEQ ID NO: 73 - DNA, 4268 bp, synthetic construct
  source 1..4268: mol_type = other DNA
agaataaactagtattcttctggtccccacagactcagagagaacccgccaccatgttcgtgttcctggtgctgctgcctctggtgtccagccagtgtgtgaacctgatcaccagaacacagtcatacaccaacagctttaccagaggcgtgtactaccccgacaaggtgttcagatccagcgtgctgcactctacccaggacctgttcctgcctttcttcagcaacgtgacctggttccacgccatctccggcaccaatggcaccaagagattcgacaaccccgtgctgcccttcaacgacggggtgtactttgccagcaccgagaagtccaacatcatcagaggctggatcttcggcaccacactggacagcaagacccagagcctgctgatcgtgaacaacgccaccaacgtggtcatcaaagtgtgcgagttccagttctgcaacgaccccttcctggacgtctactaccacaagaacaacaagagctggatggaaagcgagttccgggtgtacagcagcgccaacaactgcaccttcgagtacgtgtcccagcctttcctgatggacctggaaggcaagcagggcaacttcaagaacctgcgcgagttcgtgtttaagaacatcgacggctacttcaagatctacagcaagcacacccctatcaacctcggccgggatctgcctcagggcttctctgctctggaacccctggtggatctgcccatcggcatcaacatcacccggtttcagacactgctggccctgcacagaagctacctgacacctggcgatagcagcagcggatggacagctggtgccgccgcttactatgtgggctacctgcagcctagaaccttcctgctgaagtacaacgagaacggcaccatcaccgacgccgtggattgtgctctggatcctctgagcgagacaaagtgcaccctgaagtccttcaccgtggaaaagggcatctaccagaccagcaacttccgggtgcagcccaccgaatccatcgtgcggttccccaatatcaccaatctgtgccccttcgacgaggtgttcaatgccaccagattcgcctctgtgtacgcctggaaccggaagcggatcagcaattgcgtggccgactactccgtgctgtacaacttcgcccccttcttcgcattcaagtgctacggcgtgtcccctaccaagctgaacgacctgtgcttcacaaacgtgtacgccgacagcttcgtgatccggggaaacgaagtgcggcagattgcccctggacagacaggcaacatcgccgactacaactacaagctgcccgacgacttcaccggctgtgtgattgcctggaacagcaacaagctggactccaaagtcggcggcaactacaattacaggtaccggctgttccggaagtccaatctgaagcccttcgagcgggacatctccaccgagatctatcaggccggcaacaagccttgtaacggcgtggcaggcgtgaactgctacttcccactgcagtcctacggctttaggcccacatacggcgtgggccaccagccctacagagtggtggtgctgagcttcgaactgctgcatgcccctgccacagtgtgcggccctaagaaaagcaccaatctcgtgaagaacaaatgcgtgaacttcaacttcaacggcctgaccggcaccggcgtgctgacagagagcaacaagaagttcctgccattccagcagtttggccgggatatcgccgataccacagacgccgttagagatccccagacactggaaatcctggacatcaccccttgcagcttcggcggagtgtctgtgatcacccctggcaccaacaccagcaatcaggtggcagtgctgtaccagggcgtgaactgtaccgaagtgcccgtggccattcacgccgatcagctgacacctacatggcgggtgtactccaccggcagcaatgtgtttcagaccagagccggctgtctgatcggagccgagtacgtgaacaatagctacgagtgcgacatccccatcggcgctggaatctgcgccagctaccagacacagacaaagagccaccggagagccagaagcgtggccagccagagcatcattgcctacacaatgtctctgggcgccgagaacagcgtggcctactccaacaactctatcgctatccccaccaacttcaccatcagcgtgaccacagagatcctgcctgtgtccatgaccaagaccagcgtggactgcaccatgtacatctgcggcgattccaccgagtgctccaacctgctgctgcagtacggcagcttctgcacccagctgaaaagagccctgacagggatcgccgtggaacaggacaagaacacccaagaggtgttcgcccaagtgaagcagatctacaagacccctcctatcaagtacttcggcggcttcaatttcagccagattctgcccgatcctagcaagcccagcaagcggagcttcatcgaggacctgctgttcaacaaagtgacactggccgacgccggcttcatcaagcagtatggcgattgtctgggcgacattgccgccagggatctgatttgcgcccagaagtttaacggactgacagtgctgcctcctctgctgaccgatgagatgatcgcccagtacacatctgccctgctggccggcacaatcacaagcggctggacatttggagcaggcgccgctctgcagatcccctttgctatgcagatggcctaccggttcaacggcatcggagtgacccagaatgtgctgtacgagaaccagaagctgatcgccaaccagttcaacagcgccatcggcaagatccaggacagcctgagcagcacagcaagcgccctgggaaagctgcaggacgtggtcaaccacaatgcccaggcactgaacaccctggtcaagcagctgtcctccaagttcggcgccatcagctctgtgctgaacgatatcctgagcagactggaccctcctgaggccgaggtgcagatcgacagactgatcacaggcagactgcagagcctccagacatacgtgacccagcagctgatcagagccgccgagattagagcctctgccaatctggccgccaccaagatgtctgagtgtgtgctgggccagagcaagagagtggacttttgcggcaagggctaccacctgatgagcttccctcagtctgcccctcacggcgtggtgtttctgcacgtgacatatgtgcccgctcaagagaagaatttcaccaccgctccagccatctgccacgacggcaaagcccactttcctagagaaggcgtgttcgtgtccaacggcacccattggttcgtgacacagcggaacttctacgagccccagatcatcaccaccgacaacaccttcgtgtctggcaactgcgacgtcgtgatcggcattgtgaacaataccgtgtacgaccctctgcagcccgagctggacagcttcaaagaggaactggacaagtactttaagaaccacacaagccccgacgtggacctgggcgatatcagcggaatcaatgccagcgtcgtgaacatccagaaagagatcgaccggctgaacgaggtggccaagaatctgaacgagagcctgatcgacctgcaagaactggggaagtacgagcagtacatcaagtggccctggtacatctggctgggctttatcgccggactgattgccatcgtgatggtcacaatcatgctgtgttgcatgaccagctgctgtagctgcctgaagggctgttgtagctgtggcagctgctgcaagttcgacgaggacgattctgagcccgtgctgaagggcgtgaaactgcactacacatgatgactcgagctggtactgcatgcacgcaatgctagctgcccctttcccgtcctgggtaccccgagtctcccccgacctcgggtcccaggtatgctcccacctccacctgccccactcaccacctctgctagttccagacacctcccaagcacgcagcaatgcagctcaaaacgcttagcctagccacacccccacgggaaacagcagtgattaacctttagcaataaacgaaagtttaactaagctatactaaccccagggttggtcaatttcgtgccagccacaccctggagctagcaaaaaaaaaaaaaaaaaaaaaaaaaaaaaagcatatgactaaaaaaaaaaaaaaaaaaaaaaaaaaaaaaaaaaaaaaaaaaaaaaaaaaaaaaaaaaaaaaaaaaaaaa

SEQ ID NO: 74 - protein, 1268 aa, synthetic construct
MFVFLVLLPLVSSQCVNLITRTQSYTNSFTRGVYYPDKVFRSSVLHSTQDLFLPFFSNVTWFHAISGTNGTKRFDNPVLPFNDGVYFASTEKSNIIRGWIFGTTLDSKTQSLLIVNNATNVVIKVCEFQFCNDPFLDVYYHKNNKSWMESEFRVYSSANNCTFEYVSQPFLMDLEGKQGNFKNLREFVFKNIDGYFKIYSKHTPINLGRDLPQGFSALEPLVDLPIGINITRFQTLLALHRSYLTPGDSSSGWTAGAAAYYVGYLQPRTFLLKYNENGTITDAVDCALDPLSETKCTLKSFTVEKGIYQTSNFRVQPTESIVRFPNITNLCPFDEVFNATRFASVYAWNRKRISNCVADYSVLYNFAPFFAFKCYGVSPTKLNDLCFTNVYADSFVIRGNEVSQIAPGQTGNIADYNYKLPDDFTGCVIAWNSNKLDSKVGGNYNYRYRLFRKSNLKPFERDISTEIYQAGNKPCNGVAGVNCYFPLQSYGFRPTYGVGHQPYRVVVLSFELLHAPATVCGPKKSTNLVKNKCVNFNFNGLTGTGVLTESNKKFLPFQQFGRDIADTTDAVRDPQTLEILDITPCSFGGVSVITPGTNTSNQVAVLYQGVNCTEVPVAIHADQLTPTWRVYSTGSNVFQTRAGCLIGAEYVNNSYECDIPIGAGICASYQTQTKSHRRARSVASQSIIAYTMSLGAENSVAYSNNSIAIPTNFTISVTTEILPVSMTKTSVDCTMYICGDSTECSNLLLQYGSFCTQLKRALTGIAVEQDKNTQEVFAQVKQIYKTPPIKYFGGFNFSQILPDPSKPSKRSFIEDLLFNKVTLADAGFIKQYGDCLGDIAARDLICAQKFNGLTVLPPLLTDEMIAQYTSALLAGTITSGWTFGAGAALQIPFAMQMAYRFNGIGVTQNVLYENQKLIANQFNSAIGKIQDSLSSTASALGKLQDVVNHNAQALNTLVKQLSSKFGAISSVLNDILSRLDPPEAEVQIDRLITGRLQSLQTYVTQQLIRAAEIRASANLAATKMSECVLGQSKRVDFCGKGYHLMSFPQSAPHGVVFLHVTYVPAQEKNFTTAPAICHDGKAHFPREGVFVSNGTHWFVTQRNFYEPQIITTDNTFVSGNCDVVIGIVNNTVYDPLQPELDSFKEELDKYFKNHTSPDVDLGDISGINASVVNIQKEIDRLNEVAKNLNESLIDLQELGKYEQYIKWPWYIWLGFIAGLIAIVMVTIMLCCMTSCCSCLKGCCSCGSCCKFDEDDSEPVLKGVKLHYT

SEQ ID NO: 75 - RNA, 3810 nt, synthetic construct
  source 1..3810: mol_type = other RNA
atgttcgtgttcctggtgctgctgcctctggtgtccagccagtgtgtgaacctgatcaccagaacacagagctacaccaacagctttaccagaggcgtgtactaccccgacaaggtgttcagatccagcgtgctgcactctacccaggacctgttcctgcctttcttcagcaacgtgacctggttccacgccatctccggcaccaatggcaccaagagattcgacaaccccgtgctgcccttcaacgacggggtgtactttgccagcaccgagaagtccaacatcatcagaggctggatcttcggcaccacactggacagcaagacccagagcctgctgatcgtgaacaacgccaccaacgtggtcatcaaagtgtgcgagttccagttctgcaacgaccccttcctggacgtgtactaccacaagaacaacaagagctggatggaaagcgagttccgggtgtacagcagcgccaacaactgcaccttcgagtacgtgtcccagcctttcctgatggacctggaaggcaagcagggcaacttcaagaacctgcgcgagttcgtgtttaagaacatcgacggctacttcaagatctacagcaagcacacccctatcaacctcggccgggatctgcctcagggcttctctgctctggaacccctggtggatctgcccatcggcatcaacatcacccggtttcagacactgctggccctgcacagaagctacctgacacctggcgatagcagcagcggatggacagctggtgccgccgcttactatgtgggctacctgcagcctagaaccttcctgctgaagtacaacgagaacggcaccatcaccgacgccgtggattgtgctctggatcctctgagcgagacaaagtgcaccctgaagtccttcaccgtggaaaagggcatctaccagaccagcaacttccgggtgcagcccaccgaatccatcgtgcggttccccaatatcaccaatctgtgccccttcgacgaggtgttcaatgccaccagattcgcctctgtgtacgcctggaaccggaagcggatcagcaattgcgtggccgactactccgtgctgtacaacttcgcccccttcttcgccttcaagtgctacggcgtgtcccctaccaagctgaacgacctgtgcttcacaaacgtgtacgccgacagcttcgtgatccggggaaacgaagtgagccagattgcccctggacagacaggcaacatcgccgactacaactacaagctgcccgacgacttcaccggctgtgtgattgcctggaacagcaacaagctggactccaaagtcggcggcaactacaattacaggtaccggctgttccggaagtccaatctgaagcccttcgagcgggacatctccaccgagatctatcaggccggcaacaagccttgtaacggcgtggccggcgtgaactgctacttcccactgcagtcctacggctttaggcccacatatggcgtgggccatcagccctacagagtggtggtgctgagcttcgaactgctgcatgcccctgccacagtgtgcggccctaagaaaagcaccaatctcgtgaagaacaaatgcgtgaacttcaacttcaacggcctgaccggcaccggcgtgctgacagagagcaacaagaagttcctgccattccagcagtttggccgggatatcgccgataccacagacgccgttagagatccccagacactggaaatcctggacatcaccccttgcagcttcggcggagtgtctgtgatcacccctggcaccaacaccagcaatcaggtggcagtgctgtaccagggcgtgaactgtaccgaagtgcccgtggccattcacgccgatcagctgacacctacatggcgggtgtactccaccggcagcaatgtgtttcagaccagagccggctgtctgatcggagccgagtacgtgaacaatagctacgagtgcgacatccccatcggcgctggaatctgcgccagctaccagacacagacaaagagccaccggagagccagaagcgtggccagccagagcatcattgcctacacaatgtctctgggcgccgagaacagcgtggcctactccaacaactctatcgctatccccaccaacttcaccatcagcgtgaccacagagatcctgcctgtgtccatgaccaagaccagcgtggactgcaccatgtacatctgcggcgattccaccgagtgctccaacctgctgctgcagtacggcagcttctgcacccagctgaagagagccctgacagggatcgccgtggaacaggacaagaacacccaagaggtgttcgcccaagtgaagcagatctacaagacccctcctatcaagtacttcggcggcttcaatttcagccagattctgcccgatcctagcaagcccagcaagcggagcttcatcgaggacctgctgttcaacaaagtgacactggccgacgccggcttcatcaagcagtatggcgattgtctgggcgacattgccgccagggatctgatttgcgcccagaagtttaacggactgacagtgctgcctcctctgctgaccgatgagatgatcgcccagtacacatctgccctgctggccggcacaatcacaagcggctggacatttggagcaggcgccgctctgcagatcccctttgctatgcagatggcctaccggttcaacggcatcggagtgacccagaatgtgctgtacgagaaccagaagctgatcgccaaccagttcaacagcgccatcggcaagatccaggacagcctgagcagcacagcaagcgccctgggaaagctgcaggacgtggtcaaccacaatgcccaggcactgaacaccctggtcaagcagctgtcctccaagttcggcgccatcagctctgtgctgaacgatatcctgagcagactggaccctcctgaggccgaggtgcagatcgacagactgatcacaggcagactgcagagcctccagacatacgtgacccagcagctgatcagagccgccgagattagagcctctgccaatctggccgccaccaagatgtctgagtgtgtgctgggccagagcaagagagtggacttttgcggcaagggctaccacctgatgagcttccctcagtctgcccctcacggcgtggtgtttctgcacgtgacatatgtgcccgctcaagagaagaatttcaccaccgctccagccatctgccacgacggcaaagcccactttcctagagaaggcgtgttcgtgtccaacggcacccattggttcgtgacacagcggaacttctacgagccccagatcatcaccaccgacaacaccttcgtgtctggcaactgcgacgtcgtgatcggcattgtgaacaataccgtgtacgaccctctgcagcccgagctggacagcttcaaagaggaactggacaagtactttaagaaccacacaagccccgacgtggacctgggcgatatcagcggaatcaatgccagcgtcgtgaacatccagaaagagatcgaccggctgaacgaggtggccaagaatctgaacgagagcctgatcgacctgcaagaactggggaagtacgagcagtacatcaagtggccctggtacatctggctgggctttatcgccggactgattgccatcgtgatggtcacaatcatgctgtgttgcatgaccagctgctgtagctgcctgaagggctgttgtagctgtggcagctgctgcaagttcgacgaggacgattctgagcccgtgctgaagggcgtgaaactgcactacacatgatga

SEQ ID NO: 76 - DNA, 3810 bp, synthetic construct
  source 1..3810: mol_type = other DNA
atgttcgtgttcctggtgctgctgcctctggtgtccagccagtgtgtgaacctgatcaccagaacacagagctacaccaacagctttaccagaggcgtgtactaccccgacaaggtgttcagatccagcgtgctgcactctacccaggacctgttcctgcctttcttcagcaacgtgacctggttccacgccatctccggcaccaatggcaccaagagattcgacaaccccgtgctgcccttcaacgacggggtgtactttgccagcaccgagaagtccaacatcatcagaggctggatcttcggcaccacactggacagcaagacccagagcctgctgatcgtgaacaacgccaccaacgtggtcatcaaagtgtgcgagttccagttctgcaacgaccccttcctggacgtgtactaccacaagaacaacaagagctggatggaaagcgagttccgggtgtacagcagcgccaacaactgcaccttcgagtacgtgtcccagcctttcctgatggacctggaaggcaagcagggcaacttcaagaacctgcgcgagttcgtgtttaagaacatcgacggctacttcaagatctacagcaagcacacccctatcaacctcggccgggatctgcctcagggcttctctgctctggaacccctggtggatctgcccatcggcatcaacatcacccggtttcagacactgctggccctgcacagaagctacctgacacctggcgatagcagcagcggatggacagctggtgccgccgcttactatgtgggctacctgcagcctagaaccttcctgctgaagtacaacgagaacggcaccatcaccgacgccgtggattgtgctctggatcctctgagcgagacaaagtgcaccctgaagtccttcaccgtggaaaagggcatctaccagaccagcaacttccgggtgcagcccaccgaatccatcgtgcggttccccaatatcaccaatctgtgccccttcgacgaggtgttcaatgccaccagattcgcctctgtgtacgcctggaaccggaagcggatcagcaattgcgtggccgactactccgtgctgtacaacttcgcccccttcttcgccttcaagtgctacggcgtgtcccctaccaagctgaacgacctgtgcttcacaaacgtgtacgccgacagcttcgtgatccggggaaacgaagtgagccagattgcccctggacagacaggcaacatcgccgactacaactacaagctgcccgacgacttcaccggctgtgtgattgcctggaacagcaacaagctggactccaaagtcggcggcaactacaattacaggtaccggctgttccggaagtccaatctgaagcccttcgagcgggacatctccaccgagatctatcaggccggcaacaagccttgtaacggcgtggccggcgtgaactgctacttcccactgcagtcctacggctttaggcccacatatggcgtgggccatcagccctacagagtggtggtgctgagcttcgaactgctgcatgcccctgccacagtgtgcggccctaagaaaagcaccaatctcgtgaagaacaaatgcgtgaacttcaacttcaacggcctgaccggcaccggcgtgctgacagagagcaacaagaagttcctgccattccagcagtttggccgggatatcgccgataccacagacgccgttagagatccccagacactggaaatcctggacatcaccccttgcagcttcggcggagtgtctgtgatcacccctggcaccaacaccagcaatcaggtggcagtgctgtaccagggcgtgaactgtaccgaagtgcccgtggccattcacgccgatcagctgacacctacatggcgggtgtactccaccggcagcaatgtgtttcagaccagagccggctgtctgatcggagccgagtacgtgaacaatagctacgagtgcgacatccccatcggcgctggaatctgcgccagctaccagacacagacaaagagccaccggagagccagaagcgtggccagccagagcatcattgcctacacaatgtctctgggcgccgagaacagcgtggcctactccaacaactctatcgctatccccaccaacttcaccatcagcgtgaccacagagatcctgcctgtgtccatgaccaagaccagcgtggactgcaccatgtacatctgcggcgattccaccgagtgctccaacctgctgctgcagtacggcagcttctgcacccagctgaagagagccctgacagggatcgccgtggaacaggacaagaacacccaagaggtgttcgcccaagtgaagcagatctacaagacccctcctatcaagtacttcggcggcttcaatttcagccagattctgcccgatcctagcaagcccagcaagcggagcttcatcgaggacctgctgttcaacaaagtgacactggccgacgccggcttcatcaagcagtatggcgattgtctgggcgacattgccgccagggatctgatttgcgcccagaagtttaacggactgacagtgctgcctcctctgctgaccgatgagatgatcgcccagtacacatctgccctgctggccggcacaatcacaagcggctggacatttggagcaggcgccgctctgcagatcccctttgctatgcagatggcctaccggttcaacggcatcggagtgacccagaatgtgctgtacgagaaccagaagctgatcgccaaccagttcaacagcgccatcggcaagatccaggacagcctgagcagcacagcaagcgccctgggaaagctgcaggacgtggtcaaccacaatgcccaggcactgaacaccctggtcaagcagctgtcctccaagttcggcgccatcagctctgtgctgaacgatatcctgagcagactggaccctcctgaggccgaggtgcagatcgacagactgatcacaggcagactgcagagcctccagacatacgtgacccagcagctgatcagagccgccgagattagagcctctgccaatctggccgccaccaagatgtctgagtgtgtgctgggccagagcaagagagtggacttttgcggcaagggctaccacctgatgagcttccctcagtctgcccctcacggcgtggtgtttctgcacgtgacatatgtgcccgctcaagagaagaatttcaccaccgctccagccatctgccacgacggcaaagcccactttcctagagaaggcgtgttcgtgtccaacggcacccattggttcgtgacacagcggaacttctacgagccccagatcatcaccaccgacaacaccttcgtgtctggcaactgcgacgtcgtgatcggcattgtgaacaataccgtgtacgaccctctgcagcccgagctggacagcttcaaagaggaactggacaagtactttaagaaccacacaagccccgacgtggacctgggcgatatcagcggaatcaatgccagcgtcgtgaacatccagaaagagatcgaccggctgaacgaggtggccaagaatctgaacgagagcctgatcgacctgcaagaactggggaagtacgagcagtacatcaagtggccctggtacatctggctgggctttatcgccggactgattgccatcgtgatggtcacaatcatgctgtgttgcatgaccagctgctgtagctgcctgaagggctgttgtagctgtggcagctgctgcaagttcgacgaggacgattctgagcccgtgctgaagggcgtgaaactgcactacacatgatga

SEQ ID NO: 77 - protein, 1268 aa, synthetic construct; identical to SEQ ID NO: 69

SEQ ID NO: 78 - RNA, 3810 nt, synthetic construct; identical to SEQ ID NO: 70
  source 1..3810: mol_type = other RNA

SEQ ID NO: 79 - DNA, 3810 bp, synthetic construct; identical to SEQ ID NO: 71
  source 1..3810: mol_type = other DNA

SEQ ID NO: 80 - protein, 1270 aa, synthetic construct
MFVFLVLLPLVSSQCVNLITRTQSYTNSFTRGVYYPDKVFRSSVLHSTQDLFLPFFSNVTWFHAIHVSGTNGTKRFDNPVLPFNDGVYFASTEKSNIIRGWIFGTTLDSKTQSLLIVNNATNVVIKVCEFQFCNDPFLDVYYHENNKSRMESELRVYSSANNCTFEYVSQPFLMDLEGKQGNFKNLREFVFKNIDGYFKIYSKHTPVNLGRDLPQGFSALEPLVDLPIGINITRFQTLLALHRSYLTPGDSSSSWTAGAAAYYVGYLQPRTFLLKYNENGTITDAVDCALDPLSETKCTLKSFTVEKGIYQTSNFRVQPTESIVRFPNITNLCPFHEVFNATRFASVYAWNRKRISNCVADYSVLYNFAPFFAFKCYGVSPTKLNDLCFTNVYADSFVIRGNEVSQIAPGQTGNIADYNYKLPDDFTGCVIAWNSNKLDSKVSGNYNYLYRLFRKSKLKPFERDISTEIYQAGNKPCNGVAGFNCYFPLQSYGFRPTYGVGHQPYRVVVLSFELLHAPATVCGPKKSTNLVKNKCVNFNFNGLTGTGVLTESNKKFLPFQQFGRDIADTTDAVRDPQTLEILDITPCSFGGVSVITPGTNTSNQVAVLYQGVNCTEVPVAIHADQLTPTWRVYSTGSNVFQTRAGCLIGAEYVNNSYECDIPIGAGICASYQTQTKSHRRARSVASQSIIAYTMSLGAENSVAYSNNSIAIPTNFTISVTTEILPVSMTKTSVDCTMYICGDSTECSNLLLQYGSFCTQLKRALTGIAVEQDKNTQEVFAQVKQIYKTPPIKYFGGFNFSQILPDPSKPSKRSFIEDLLFNKVTLADAGFIKQYGDCLGDIAARDLICAQKFNGLTVLPPLLTDEMIAQYTSALLAGTITSGWTFGAGAALQIPFAMQMAYRFNGIGVTQNVLYENQKLIANQFNSAIGKIQDSLSSTASALGKLQDVVNHNAQALNTLVKQLSSKFGAISSVLNDILSRLDPPEAEVQIDRLITGRLQSLQTYVTQQLIRAAEIRASANLAATKMSECVLGQSKRVDFCGKGYHLMSFPQSAPHGVVFLHVTYVPAQEKNFTTAPAICHDGKAHFPREGVFVSNGTHWFVTQRNFYEPQIITTDNTFVSGNCDVVIGIVNNTVYDPLQPELDSFKEELDKYFKNHTSPDVDLGDISGINASVVNIQKEIDRLNEVAKNLNESLIDLQELGKYEQYIKWPWYIWLGFIAGLIAIVMVTIMLCCMTSCCSCLKGCCSCGSCCKFDEDDSEPVLKGVKLHYT

SEQ ID NO: 81 - RNA, 3816 nt, synthetic construct
  source 1..3816: mol_type = other RNA
atgttcgtgttcctggtgctgctgcctctggtgtccagccagtgtgtgaacctgatcaccagaacacagtcatacaccaacagctttaccagaggcgtgtactaccccgacaaggtgttcagatccagcgtgctgcactctacccaggacctgttcctgcctttcttcagcaacgtgacctggttccacgccatccacgtgtccggcaccaatggcaccaagagattcgacaaccccgtgctgcccttcaacgacggggtgtactttgccagcaccgagaagtccaacatcatcagaggctggatcttcggcaccacactggacagcaagacccagagcctgctgatcgtgaacaacgccaccaacgtggtcatcaaagtgtgcgagttccagttctgcaacgaccccttcctggacgtctactaccacgagaacaacaagagcaggatggaaagcgagctccgggtgtacagcagcgccaacaactgcaccttcgagtacgtgtcccagcctttcctgatggacctggaaggcaagcagggcaacttcaagaacctgcgcgagttcgtgtttaagaacatcgacggctacttcaagatctacagcaagcacacccctgtgaacctcggccgggatctgcctcagggcttctctgctctggaacccctggtggatctgcccatcggcatcaacatcacccggtttcagacactgctggccctgcacagaagctacctgacacctggcgatagcagcagcagctggacagctggtgccgccgcttactatgtgggctacctgcagcctagaaccttcctgctgaagtacaacgagaacggcaccatcaccgacgccgtggattgtgctctggatcctctgagcgagacaaagtgcaccctgaagtccttcaccgtggaaaagggcatctaccagaccagcaacttccgggtgcagcccaccgaatccatcgtgcggttccccaatatcaccaatctgtgccccttccacgaggtgttcaatgccaccagattcgcctctgtgtacgcctggaaccggaagcggatcagcaattgcgtggccgactactccgtgctgtacaacttcgcccccttcttcgcattcaagtgctacggcgtgtcccctaccaagctgaacgacctgtgcttcacaaacgtgtacgccgacagcttcgtgatccggggaaacgaagtgtcacagattgcccctggacagacaggcaacatcgccgactacaactacaagctgcccgacgacttcaccggctgtgtgattgcctggaacagcaacaagctggactccaaagtcagcggcaactacaattacctgtaccggctgttccggaagtccaagctgaagcccttcgagcgggacatctccaccgagatctatcaggccggcaacaagccttgtaacggcgtggcaggcttcaactgctacttcccactgcagtcctacggctttaggcccacatacggcgtgggccaccagccctacagagtggtggtgctgagcttcgaactgctgcatgcccctgccacagtgtgcggccctaagaaaagcaccaatctcgtgaagaacaaatgcgtgaacttcaacttcaacggcctgaccggcaccggcgtgctgacagagagcaacaagaagttcctgccattccagcagtttggccgggatatcgccgataccacagacgccgttagagatccccagacactggaaatcctggacatcaccccttgcagcttcggcggagtgtctgtgatcacccctggcaccaacaccagcaatcaggtggcagtgctgtaccagggcgtgaactgtaccgaagtgcccgtggccattcacgccgatcagctgacacctacatggcgggtgtactccaccggcagcaatgtgtttcagaccagagccggctgtctgatcggagccgagtacgtgaacaatagctacgagtgcgacatccccatcggcgctggaatctgcgccagctaccagacacagacaaagagccaccggagagccagaagcgtggccagccagagcatcattgcctacacaatgtctctgggcgccgagaacagcgtggcctactccaacaactctatcgctatccccaccaacttcaccatcagcgtgaccacagagatcctgcctgtgtccatgaccaagaccagcgtggactgcaccatgtacatctgcggcgattccaccgagtgctccaacctgctgctgcagtacggcagcttctgcacccagctgaaaagagccctgacagggatcgccgtggaacaggacaagaacacccaagaggtgttcgcccaagtgaagcagatctacaagacccctcctatcaagtacttcggcggcttcaatttcagccagattctgcccgatcctagcaagcccagcaagcggagcttcatcgaggacctgctgttcaacaaagtgacactggccgacgccggcttcatcaagcagtatggcgattgtctgggcgacattgccgccagggatctgatttgcgcccagaagtttaacggactgacagtgctgcctcctctgctgaccgatgagatgatcgcccagtacacatctgccctgctggccggcacaatcacaagcggctggacatttggagcaggcgccgctctgcagatcccctttgctatgcagatggcctaccggttcaacggcatcggagtgacccagaatgtgctgtacgagaaccagaagctgatcgccaaccagttcaacagcgccatcggcaagatccaggacagcctgagcagcacagcaagcgccctgggaaagctgcaggacgtggtcaaccacaatgcccaggcactgaacaccctggtcaagcagctgtcctccaagttcggcgccatcagctctgtgctgaacgatatcctgagcagactggaccctcctgaggccgaggtgcagatcgacagactgatcacaggcagactgcagagcctccagacatacgtgacccagcagctgatcagagccgccgagattagagcctctgccaatctggccgccaccaagatgtctgagtgtgtgctgggccagagcaagagagtggacttttgcggcaagggctaccacctgatgagcttccctcagtctgcccctcacggcgtggtgtttctgcacgtgacatatgtgcccgctcaagagaagaatttcaccaccgctccagccatctgccacgacggcaaagcccactttcctagagaaggcgtgttcgtgtccaacggcacccattggttcgtgacacagcggaacttctacgagccccagatcatcaccaccgacaacaccttcgtgtctggcaactgcgacgtcgtgatcggcattgtgaacaataccgtgtacgaccctctgcagcccgagctggacagcttcaaagaggaactggacaagtactttaagaaccacacaagccccgacgtggacctgggcgatatcagcggaatcaatgccagcgtcgtgaacatccagaaagagatcgaccggctgaacgaggtggccaagaatctgaacgagagcctgatcgacctgcaagaactggggaagtacgagcagtacatcaagtggccctggtacatctggctgggctttatcgccggactgattgccatcgtgatggtcacaatcatgctgtgttgcatgaccagctgctgtagctgcctgaagggctgttgtagctgtggcagctgctgcaagttcgacgaggacgattctgagcccgtgctgaagggcgtgaaactgcactacacatgatga

SEQ ID NO: 82 - DNA, 3816 bp, synthetic construct
  source 1..3816: mol_type = other DNA
atgttcgtgttcctggtgctgctgcctctggtgtccagccagtgtgtgaacctgatcaccagaacacagtcatacaccaacagctttaccagaggcgtgtactaccccgacaaggtgttcagatccagcgtgctgcactctacccaggacctgttcctgcctttcttcagcaacgtgacctggttccacgccatccacgtgtccggcaccaatggcaccaagagattcgacaaccccgtgctgcccttcaacgacggggtgtactttgccagcaccgagaagtccaacatcatcagaggctggatcttcggcaccacactggacagcaagacccagagcctgctgatcgtgaacaacgccaccaacgtggtcatcaaagtgtgcgagttccagttctgcaacgaccccttcctggacgtctactaccacgagaacaacaagagcaggatggaaagcgagctccgggtgtacagcagcgccaacaactgcaccttcgagtacgtgtcccagcctttcctgatggacctggaaggcaagcagggcaacttcaagaacctgcgcgagttcgtgtttaagaacatcgacggctacttcaagatctacagcaagcacacccctgtgaacctcggccgggatctgcctcagggcttctctgctctggaacccctggtggatctgcccatcggcatcaacatcacccggtttcagacactgctggccctgcacagaagctacctgacacctggcgatagcagcagcagctggacagctggtgccgccgcttactatgtgggctacctgcagcctagaaccttcctgctgaagtacaacgagaacggcaccatcaccgacgccgtggattgtgctctggatcctctgagcgagacaaagtgcaccctgaagtccttcaccgtggaaaagggcatctaccagaccagcaacttccgggtgcagcccaccgaatccatcgtgcggttccccaatatcaccaatctgtgccccttccacgaggtgttcaatgccaccagattcgcctctgtgtacgcctggaaccggaagcggatcagcaattgcgtggccgactactccgtgctgtacaacttcgcccccttcttcgcattcaagtgctacggcgtgtcccctaccaagctgaacgacctgtgcttcacaaacgtgtacgccgacagcttcgtgatccggggaaacgaagtgtcacagattgcccctggacagacaggcaacatcgccgactacaactacaagctgcccgacgacttcaccggctgtgtgattgcctggaacagcaacaagctggactccaaagtcagcggcaactacaattacctgtaccggctgttccggaagtccaagctgaagcccttcgagcgggacatctccaccgagatctatcaggccggcaacaagccttgtaacggcgtggcaggcttcaactgctacttcccactgcagtcctacggctttaggcccacatacggcgtgggccaccagccctacagagtggtggtgctgagcttcgaactgctgcatgcccctgccacagtgtgcggccctaagaaaagcaccaatctcgtgaagaacaaatgcgtgaacttcaacttcaacggcctgaccggcaccggcgtgctgacagagagcaacaagaagttcctgccattccagcagtttggccgggatatcgccgataccacagacgccgttagagatccccagacactggaaatcctggacatcaccccttgcagcttcggcggagtgtctgtgatcacccctggcaccaacaccagcaatcaggtggcagtgctgtaccagggcgtgaactgtaccgaagtgcccgtggccattcacgccgatcagctgacacctacatggcgggtgtactccaccggcagcaatgtgtttcagaccagagccggctgtctgatcggagccgagtacgtgaacaatagctacgagtgcgacatccccatcggcgctggaatctgcgccagctaccagacacagacaaagagccaccggagagccagaagcgtggccagccagagcatcattgcctacacaatgtctctgggcgccgagaacagcgtggcctactccaacaactctatcgctatccccaccaacttcaccatcagcgtgaccacagagatcctgcctgtgtccatgaccaagaccagcgtggactgcaccatgtacatctgcggcgattccaccgagtgctccaacctgctgctgcagtacggcagcttctgcacccagctgaaaagagccctgacagggatcgccgtggaacaggacaagaacacccaagaggtgttcgcccaagtgaagcagatctacaagacccctcctatcaagtacttcggcggcttcaatttcagccagattctgcccgatcctagcaagcccagcaagcggagcttcatcgaggacctgctgttcaacaaagtgacactggccgacgccggcttcatcaagcagtatggcgattgtctgggcgacattgccgccagggatctgatttgcgcccagaagtttaacggactgacagtgctgcctcctctgctgaccgatgagatgatcgcccagtacacatctgccctgctggccggcacaatcacaagcggctggacatttggagcaggcgccgctctgcagatcccctttgctatgcagatggcctaccggttcaacggcatcggagtgacccagaatgtgctgtacgagaaccagaagctgatcgccaaccagttcaacagcgccatcggcaagatccaggacagcctgagcagcacagcaagcgccctgggaaagctgcaggacgtggtcaaccacaatgcccaggcactgaacaccctggtcaagcagctgtcctccaagttcggcgccatcagctctgtgctgaacgatatcctgagcagactggaccctcctgaggccgaggtgcagatcgacagactgatcacaggcagactgcagagcctccagacatacgtgacccagcagctgatcagagccgccgagattagagcctctgccaatctggccgccaccaagatgtctgagtgtgtgctgggccagagcaagagagtggacttttgcggcaagggctaccacctgatgagcttccctcagtctgcccctcacggcgtggtgtttctgcacgtgacatatgtgcccgctcaagagaagaatttcaccaccgctccagccatctgccacgacggcaaagcccactttcctagagaaggcgtgttcgtgtccaacggcacccattggttcgtgacacagcggaacttctacgagccccagatcatcaccaccgacaacaccttcgtgtctggcaactgcgacgtcgtgatcggcattgtgaacaataccgtgtacgaccctctgcagcccgagctggacagcttcaaagaggaactggacaagtactttaagaaccacacaagccccgacgtggacctgggcgatatcagcggaatcaatgccagcgtcgtgaacatccagaaagagatcgaccggctgaacgaggtggccaagaatctgaacgagagcctgatcgacctgcaagaactggggaagtacgagcagtacatcaagtggccctggtacatctggctgggctttatcgccggactgattgccatcgtgatggtcacaatcatgctgtgttgcatgaccagctgctgtagctgcctgaagggctgttgtagctgtggcagctgctgcaagttcgacgaggacgattctgagcccgtgctgaagggcgtgaaactgcactacacatgatga

SEQ ID NO: 83 - RNA, 4273 nt, synthetic construct
  source 1..4273: mol_type = other RNA
agaataaactagtattcttctggtccccacagactcagagagaacccgccaccatgttcgtgttcctggtgctgctgcctctggtgtccagccagtgtgtgaacctgatcaccagaacacagtcatacaccaacagctttaccagaggcgtgtactaccccgacaaggtgttcagatccagcgtgctgcactctacccaggacctgttcctgcctttcttcagcaacgtgacctggttccacgccatccacgtgtccggcaccaatggcaccaagagattcgacaaccccgtgctgcccttcaacgacggggtgtactttgccagcaccgagaagtccaacatcatcagaggctggatcttcggcaccacactggacagcaagacccagagcctgctgatcgtgaacaacgccaccaacgtggtcatcaaagtgtgcgagttccagttctgcaacgaccccttcctggacgtctactaccacgagaacaacaagagcaggatggaaagcgagctccgggtgtacagcagcgccaacaactgcaccttcgagtacgtgtcccagcctttcctgatggacctggaaggcaagcagggcaacttcaagaacctgcgcgagttcgtgtttaagaacatcgacggctacttcaagatctacagcaagcacacccctgtgaacctcggccgggatctgcctcagggcttctctgctctggaacccctggtggatctgcccatcggcatcaacatcacccggtttcagacactgctggccctgcacagaagctacctgacacctggcgatagcagcagcagctggacagctggtgccgccgcttactatgtgggctacctgcagcctagaaccttcctgctgaagtacaacgagaacggcaccatcaccgacgccgtggattgtgctctggatcctctgagcgagacaaagtgcaccctgaagtccttcaccgtggaaaagggcatctaccagaccagcaacttccgggtgcagcccaccgaatccatcgtgcggttccccaatatcaccaatctgtgccccttccacgaggtgttcaatgccaccagattcgcctctgtgtacgcctggaaccggaagcggatcagcaattgcgtggccgactactccgtgctgtacaacttcgcccccttcttcgcattcaagtgctacggcgtgtcccctaccaagctgaacgacctgtgcttcacaaacgtgtacgccgacagcttcgtgatccggggaaacgaagtgtcacagattgcccctggacagacaggcaacatcgccgactacaactacaagctgcccgacgacttcaccggctgtgtgattgcctggaacagcaacaagctggactccaaagtcagcggcaactacaattacctgtaccggctgttccggaagtccaagctgaagcccttcgagcgggacatctccaccgagatctatcaggccggcaacaagccttgtaacggcgtggcaggcttcaactgctacttcccactgcagtcctacggctttaggcccacatacggcgtgggccaccagccctacagagtggtggtgctgagcttcgaactgctgcatgcccctgccacagtgtgcggccctaagaaaagcaccaatctcgtgaagaacaaatgcgtgaacttcaacttcaacggcctgaccggcaccggcgtgctgacagagagcaacaagaagttcctgccattccagcagtttggccgggatatcgccgataccacagacgccgttagagatccccagacactggaaatcctggacatcaccccttgcagcttcggcggagtgtctgtgatcacccctggcaccaacaccagcaatcaggtggcagtgctgtaccagggcgtgaactgtaccgaagtgcccgtggccattcacgccgatcagctgacacctacatggcgggtgtactccaccggcagcaatgtgtttcagaccagagccggctgtctgatcggagccgagtacgtgaacaatagctacgagtgcgacatccccatcggcgctggaatctgcgccagctaccagacacagacaaagagccaccggagagccagaagcgtggccagccagagcatcattgcctacacaatgtctctgggcgccgagaacagcgtggcctactccaacaactctatcgctatccccaccaacttcaccatcagcgtgaccacagagatcctgcctgtgtccatgaccaagaccagcgtggactgcaccatgtacatctgcggcgattccaccgagtgctccaacctgctgctgcagtacggcagcttctgcacccagctgaaaagagccctgacagggatcgccgtggaacaggacaagaacacccaagaggtgttcgcccaagtgaagcagatctacaagacccctcctatcaagtacttcggcggcttcaatttcagccagattctgcccgatcctagcaagcccagcaagcggagcttcatcgaggacctgctgttcaacaaagtgacactggccgacgccggcttcatcaagcagtatggcgattgtctgggcgacattgccgccagggatctgatttgcgcccagaagtttaacggactgacagtgctgcctcctctgctgaccgatgagatgatcgcccagtacacatctgccctgctggccggcacaatcacaagcggctggacatttggagcaggcgccgctctgcagatcccctttgctatgcagatggcctaccggttcaacggcatcggagtgacccagaatgtgctgtacgagaaccagaagctgatcgccaaccagttcaacagcgccatcggcaagatccaggacagcctgagcagcacagcaagcgccctgggaaagctgcaggacgtggtcaaccacaatgcccaggcactgaacaccctggtcaagcagctgtcctccaagttcggcgccatcagctctgtgctgaacgatatcctgagcagactggaccctcctgaggccgaggtgcagatcgacagactgatcacaggcagactgcagagcctccagacatacgtgacccagcagctgatcagagccgccgagattagagcctctgccaatctggccgccaccaagatgtctgagtgtgtgctgggccagagcaagagagtggacttttgcggcaagggctaccacctgatgagcttccctcagtctgcccctcacggcgtggtgtttctgcacgtgacatatgtgcccgctcaagagaagaatttcaccaccgctccagccatctgccacgacggcaaagcccactttcctagagaaggcgtgttcgtgtccaacggcacccattggttcgtgacacagcggaacttctacgagccccagatcatcaccaccgacaacaccttcgtgtctggcaactgcgacgtcgtgatcggcattgtgaacaataccgtgtacgaccctctgcagcccgagctggacagcttcaaagaggaactggacaagtactttaagaaccacacaagccccgacgtggacctgggcgatatcagcggaatcaatgccagcgtcgtgaacatccagaaagagatcgaccggctgaacgaggtggccaagaatctgaacgagagcctgatcgacctgcaagaactggggaagtacgagcagtacatcaagtggccctggtacatctggctgggctttatcgccggactgattgccatcgtgatggtcacaatcatgctgtgttgcatgaccagctgctgtagctgcctgaagggctgttgtagctgtggcagctgctgcaagttcgacgaggacgattctgagcccgtgctgaagggcgtgaaactgcactacacatgatgactcgagctggtactgcatgcacgcaatgctagctgcccctttcccgtcctgggtaccccgagtctcccccgacctcgggtcccaggtatgctcccacctccacctgccccactcaccacctctgctagttccagacacctcccaagcacgcagcaatgcagctcaaaacgcttagcctagccacacccccacgggaaacagcagtgattaacctttagcaataaacgaaagtttaactaagctatactaaccccagggttggtcaatttcgtgccagccacaccctggagctagcaaaaaaaaaaaaaaaaaaaaaaaaaaaaaagcatatgactaaaaaaaaaaaaaaaaaaaaaaaaaaaaaaaaaaaaaaaaaaaaaaaaaaaaaaaaaaaaaaaaaaaaa

SEQ ID NO: 84 - DNA, 4273 bp, synthetic construct
  source 1..4273: mol_type = other DNA
agaataaactagtattcttctggtccccacagactcagagagaacccgccaccatgttcgtgttcctggtgctgctgcctctggtgtccagccagtgtgtgaacctgatcaccagaacacagtcatacaccaacagctttaccagaggcgtgtactaccccgacaaggtgttcagatccagcgtgctgcactctacccaggacctgttcctgcctttcttcagcaacgtgacctggttccacgccatccacgtgtccggcaccaatggcaccaagagattcgacaaccccgtgctgcccttcaacgacggggtgtactttgccagcaccgagaagtccaacatcatcagaggctggatcttcggcaccacactggacagcaagacccagagcctgctgatcgtgaacaacgccaccaacgtggtcatcaaagtgtgcgagttccagttctgcaacgaccccttcctggacgtctactaccacgagaacaacaagagcaggatggaaagcgagctccgggtgtacagcagcgccaacaactgcaccttcgagtacgtgtcccagcctttcctgatggacctggaaggcaagcagggcaacttcaagaacctgcgcgagttcgtgtttaagaacatcgacggctacttcaagatctacagcaagcacacccctgtgaacctcggccgggatctgcctcagggcttctctgctctggaacccctggtggatctgcccatcggcatcaacatcacccggtttcagacactgctggccctgcacagaagctacctgacacctggcgatagcagcagcagctggacagctggtgccgccgcttactatgtgggctacctgcagcctagaaccttcctgctgaagtacaacgagaacggcaccatcaccgacgccgtggattgtgctctggatcctctgagcgagacaaagtgcaccctgaagtccttcaccgtggaaaagggcatctaccagaccagcaacttccgggtgcagcccaccgaatccatcgtgcggttccccaatatcaccaatctgtgccccttccacgaggtgttcaatgccaccagattcgcctctgtgtacgcctggaaccggaagcggatcagcaattgcgtggccgactactccgtgctgtacaacttcgcccccttcttcgcattcaagtgctacggcgtgtcccctaccaagctgaacgacctgtgcttcacaaacgtgtacgccgacagcttcgtgatccggggaaacgaagtgtcacagattgcccctggacagacaggcaacatcgccgactacaactacaagctgcccgacgacttcaccggctgtgtgattgcctggaacagcaacaagctggactccaaagtcagcggcaactacaattacctgtaccggctgttccggaagtccaagctgaagcccttcgagcgggacatctccaccgagatctatcaggccggcaacaagccttgtaacggcgtggcaggcttcaactgctacttcccactgcagtcctacggctttaggcccacatacggcgtgggccaccagccctacagagtggtggtgctgagcttcgaactgctgcatgcccctgccacagtgtgcggccctaagaaaagcaccaatctcgtgaagaacaaatgcgtgaacttcaacttcaacggcctgaccggcaccggcgtgctgacagagagcaacaagaagttcctgccattccagcagtttggccgggatatcgccgataccacagacgccgttagagatccccagacactggaaatcctggacatcaccccttgcagcttcggcggagtgtctgtgatcacccctggcaccaacaccagcaatcaggtggcagtgctgtaccagggcgtgaactgtaccgaagtgcccgtggccattcacgccgatcagctgacacctacatggcgggtgtactccaccggcagcaatgtgtttcagaccagagccggctgtctgatcggagccgagtacgtgaacaatagctacgagtgcgacatccccatcggcgctggaatctgcgccagctaccagacacagacaaagagccaccggagagccagaagcgtggccagccagagcatcattgcctacacaatgtctctgggcgccgagaacagcgtggcctactccaacaactctatcgctatccccaccaacttcaccatcagcgtgaccacagagatcctgcctgtgtccatgaccaagaccagcgtggactgcaccatgtacatctgcggcgattccaccgagtgctccaacctgctgctgcagtacggcagcttctgcacccagctgaaaagagccctgacagggatcgccgtggaacaggacaagaacacccaagaggtgttcgcccaagtgaagcagatctacaagacccctcctatcaagtacttcggcggcttcaatttcagccagattctgcccgatcctagcaagcccagcaagcggagcttcatcgaggacctgctgttcaacaaagtgacactggccgacgccggcttcatcaagcagtatggcgattgtctgggcgacattgccgccagggatctgatttgcgcccagaagtttaacggactgacagtgctgcctcctctgctgaccgatgagatgatcgcccagtacacatctgccctgctggccggcacaatcacaagcggctggacatttggagcaggcgccgctctgcagatcccctttgctatgcagatggcctaccggttcaacggcatcggagtgacccagaatgtgctgtacgagaaccagaagctgatcgccaaccagttcaacagcgccatcggcaagatccaggacagcctgagcagcacagcaagcgccctgggaaagctgcaggacgtggtcaaccacaatgcccaggcactgaacaccctggtcaagcagctgtcctccaagttcggcgccatcagctctgtgctgaacgatatcctgagcagactggaccctcctgaggccgaggtgcagatcgacagactgatcacaggcagactgcagagcctccagacatacgtgacccagcagctgatcagagccgccgagattagagcctctgccaatctggccgccaccaagatgtctgagtgtgtgctgggccagagcaagagagtggacttttgcggcaagggctaccacctgatgagcttccctcagtctgcccctcacggcgtggtgtttctgcacgtgacatatgtgcccgctcaagagaagaatttcaccaccgctccagccatctgccacgacggcaaagcccactttcctagagaaggcgtgttcgtgtccaacggcacccattggttcgtgacacagcggaacttctacgagccccagatcatcaccaccgacaacaccttcgtgtctggcaactgcgacgtcgtgatcggcattgtgaacaataccgtgtacgaccctctgcagcccgagctggacagcttcaaagaggaactggacaagtactttaagaaccacacaagccccgacgtggacctgggcgatatcagcggaatcaatgccagcgtcgtgaacatccagaaagagatcgaccggctgaacgaggtggccaagaatctgaacgagagcctgatcgacctgcaagaactggggaagtacgagcagtacatcaagtggccctggtacatctggctgggctttatcgccggactgattgccatcgtgatggtcacaatcatgctgtgttgcatgaccagctgctgtagctgcctgaagggctgttgtagctgtggcagctgctgcaagttcgacgaggacgattctgagcccgtgctgaagggcgtgaaactgcactacacatgatgactcgagctggtactgcatgcacgcaatgctagctgcccctttcccgtcctgggtaccccgagtctcccccgacctcgggtcccaggtatgctcccacctccacctgccccactcaccacctctgctagttccagacacctcccaagcacgcagcaatgcagctcaaaacgcttagcctagccacacccccacgggaaacagcagtgattaacctttagcaataaacgaaagtttaactaagctatactaaccccagggttggtcaatttcgtgccagccacaccctggagctagcaaaaaaaaaaaaaaaaaaaaaaaaaaaaaagcatatgactaaaaaaaaaaaaaaaaaaaaaaaaaaaaaaaaaaaaaaaaaaaaaaaaaaaaaaaaaaaaaaaaaaaaa

SEQ ID NO: 85 - protein, 1270 aa, synthetic construct
MFVFLVLLPLVSSQCVNLITRTQSYTNSFTRGVYYPDKVFRSSVLHSTQDLFLPFFSNVTWFHAIHVSGTNGTKRFDNPVLPFNDGVYFASTEKSNIIRGWIFGTTLDSKTQSLLIVNNATNVVIKVCEFQFCNDPFLDVYYHENNKSRMESELRVYSSANNCTFEYVSQPFLMDLEGKQGNFKNLREFVFKNIDGYFKIYSKHTPVNLGRDLPQGFSALEPLVDLPIGINITRFQTLLALHRSYLTPGDSSSSWTAGAAAYYVGYLQPRTFLLKYNENGTITDAVDCALDPLSETKCTLKSFTVEKGIYQTSNFRVQPTESIVRFPNITNLCPFHEVFNATTFASVYAWNRKRISNCVADYSVLYNFAPFFAFKCYGVSPTKLNDLCFTNVYADSFVIRGNEVSQIAPGQTGNIADYNYKLPDDFTGCVIAWNSNKLDSKVSGNYNYLYRLFRKSKLKPFERDISTEIYQAGNKPCNGVAGSNCYFPLQSYGFRPTYGVGHQPYRVVVLSFELLHAPATVCGPKKSTNLVKNKCVNFNFNGLTGTGVLTESNKKFLPFQQFGRDIADTTDAVRDPQTLEILDITPCSFGGVSVITPGTNTSNQVAVLYQGVNCTEVPVAIHADQLTPTWRVYSTGSNVFQTRAGCLIGAEYVNNSYECDIPIGAGICASYQTQTKSHRRARSVASQSIIAYTMSLGAENSVAYSNNSIAIPTNFTISVTTEILPVSMTKTSVDCTMYICGDSTECSNLLLQYGSFCTQLKRALTGIAVEQDKNTQEVFAQVKQIYKTPPIKYFGGFNFSQILPDPSKPSKRSFIEDLLFNKVTLADAGFIKQYGDCLGDIAARDLICAQKFNGLTVLPPLLTDEMIAQYTSALLAGTITSGWTFGAGAALQIPFAMQMAYRFNGIGVTQNVLYENQKLIANQFNSAIGKIQDSLSSTASALGKLQDVVNHNAQALNTLVKQLSSKFGAISSVLNDILSRLDPPEAEVQIDRLITGRLQSLQTYVTQQLIRAAEIRASANLAATKMSECVLGQSKRVDFCGKGYHLMSFPQSAPHGVVFLHVTYVPAQEKNFTTAPAICHDGKAHFPREGVFVSNGTHWFVTQRNFYEPQIITTDNTFVSGNCDVVIGIVNNTVYDPLQPELDSFKEELDKYFKNHTSPDVDLGDISGINASVVNIQKEIDRLNEVAKNLNESLINLQELGKYEQYIKWPWYIWLGFIAGLIAIVMVTIMLCCMTSCCSCLKGCCSCGSCCKFDEDDSEPVLKGVKLHYT

SEQ ID NO: 86 - RNA, 3816 nt, synthetic construct
  source 1..3816: mol_type = other RNA
atgttcgtgttcctggtgctgctgcctctggtgtccagccagtgtgtgaacctgatcaccagaacacagtcatacaccaacagctttaccagaggcgtgtactaccccgacaaggtgttcagatccagcgtgctgcactctacccaggacctgttcctgcctttcttcagcaacgtgacctggttccacgccatccacgtgtccggcaccaatggcaccaagagattcgacaaccccgtgctgcccttcaacgacggggtgtactttgccagcaccgagaagtccaacatcatcagaggctggatcttcggcaccacactggacagcaagacccagagcctgctgatcgtgaacaacgccaccaacgtggtcatcaaagtgtgcgagttccagttctgcaacgaccccttcctggacgtctactaccacgagaacaacaagagcaggatggaaagcgagctccgggtgtacagcagcgccaacaactgcaccttcgagtacgtgtcccagcctttcctgatggacctggaaggcaagcagggcaacttcaagaacctgcgcgagttcgtgtttaagaacatcgacggctacttcaagatctacagcaagcacacccctgtgaacctcggccgggatctgcctcagggcttctctgctctggaacccctggtggatctgcccatcggcatcaacatcacccggtttcagacactgctggccctgcacagaagctacctgacacctggcgatagcagcagcagctggacagctggtgccgccgcttactatgtgggctacctgcagcctagaaccttcctgctgaagtacaacgagaacggcaccatcaccgacgccgtggattgtgctctggatcctctgagcgagacaaagtgcaccctgaagtccttcaccgtggaaaagggcatctaccagaccagcaacttccgggtgcagcccaccgaatccatcgtgcggttccccaatatcaccaatctgtgccccttccacgaggtgttcaatgccaccaccttcgcctctgtgtacgcctggaaccggaagcggatcagcaattgcgtggccgactactccgtgctgtacaacttcgcccccttcttcgcattcaagtgctacggcgtgtcccctaccaagctgaacgacctgtgcttcacaaacgtgtacgccgacagcttcgtgatccggggaaacgaagtgtcacagattgcccctggacagacaggcaacatcgccgactacaactacaagctgcccgacgacttcaccggctgtgtgattgcctggaacagcaacaagctggactccaaagtcagcggcaactacaattacctgtaccggctgttccggaagtccaagctgaagcccttcgagcgggacatctccaccgagatctatcaggccggcaacaagccttgtaacggcgtggcaggcagcaactgctacttcccactgcagtcctacggctttaggcccacatacggcgtgggccaccagccctacagagtggtggtgctgagcttcgaactgctgcatgcccctgccacagtgtgcggccctaagaaaagcaccaatctcgtgaagaacaaatgcgtgaacttcaacttcaacggcctgaccggcaccggcgtgctgacagagagcaacaagaagttcctgccattccagcagtttggccgggatatcgccgataccacagacgccgttagagatccccagacactggaaatcctggacatcaccccttgcagcttcggcggagtgtctgtgatcacccctggcaccaacaccagcaatcaggtggcagtgctgtaccagggcgtgaactgtaccgaagtgcccgtggccattcacgccgatcagctgacacctacatggcgggtgtactccaccggcagcaatgtgtttcagaccagagccggctgtctgatcggagccgagtacgtgaacaatagctacgagtgcgacatccccatcggcgctggaatctgcgccagctaccagacacagacaaagagccaccggagagccagaagcgtggccagccagagcatcattgcctacacaatgtctctgggcgccgagaacagcgtggcctactccaacaactctatcgctatccccaccaacttcaccatcagcgtgaccacagagatcctgcctgtgtccatgaccaagaccagcgtggactgcaccatgtacatctgcggcgattccaccgagtgctccaacctgctgctgcagtacggcagcttctgcacccagctgaaaagagccctgacagggatcgccgtggaacaggacaagaacacccaagaggtgttcgcccaagtgaagcagatctacaagacccctcctatcaagtacttcggcggcttcaatttcagccagattctgcccgatcctagcaagcccagcaagcggagcttcatcgaggacctgctgttcaacaaagtgacactggccgacgccggcttcatcaagcagtatggcgattgtctgggcgacattgccgccagggatctgatttgcgcccagaagtttaacggactgacagtgctgcctcctctgctgaccgatgagatgatcgcccagtacacatctgccctgctggccggcacaatcacaagcggctggacatttggagcaggcgccgctctgcagatcccctttgctatgcagatggcctaccggttcaacggcatcggagtgacccagaatgtgctgtacgagaaccagaagctgatcgccaaccagttcaacagcgccatcggcaagatccaggacagcctgagcagcacagcaagcgccctgggaaagctgcaggacgtggtcaaccacaatgcccaggcactgaacaccctggtcaagcagctgtcctccaagttcggcgccatcagctctgtgctgaacgatatcctgagcagactggaccctcctgaggccgaggtgcagatcgacagactgatcacaggcagactgcagagcctccagacatacgtgacccagcagctgatcagagccgccgagattagagcctctgccaatctggccgccaccaagatgtctgagtgtgtgctgggccagagcaagagagtggacttttgcggcaagggctaccacctgatgagcttccctcagtctgcccctcacggcgtggtgtttctgcacgtgacatatgtgcccgctcaagagaagaatttcaccaccgctccagccatctgccacgacggcaaagcccactttcctagagaaggcgtgttcgtgtccaacggcacccattggttcgtgacacagcggaacttctacgagccccagatcatcaccaccgacaacaccttcgtgtctggcaactgcgacgtcgtgatcggcattgtgaacaataccgtgtacgaccctctgcagcccgagctggacagcttcaaagaggaactggacaagtactttaagaaccacacaagccccgacgtggacctgggcgatatcagcggaatcaatgccagcgtcgtgaacatccagaaagagatcgaccggctgaacgaggtggccaagaatctgaacgagagcctgatcaacctgcaagaactggggaagtacgagcagtacatcaagtggccctggtacatctggctgggctttatcgccggactgattgccatcgtgatggtcacaatcatgctgtgttgcatgaccagctgctgtagctgcctgaagggctgttgtagctgtggcagctgctgcaagttcgacgaggacgattctgagcccgtgctgaagggcgtgaaactgcactacacatgatga

SEQ ID NO: 87 - DNA, 3816 bp, synthetic construct
  source 1..3816: mol_type = other DNA
atgttcgtgttcctggtgctgctgcctctggtgtccagccagtgtgtgaacctgatcaccagaacacagtcatacaccaacagctttaccagaggcgtgtactaccccgacaaggtgttcagatccagcgtgctgcactctacccaggacctgttcctgcctttcttcagcaacgtgacctggttccacgccatccacgtgtccggcaccaatggcaccaagagattcgacaaccccgtgctgcccttcaacgacggggtgtactttgccagcaccgagaagtccaacatcatcagaggctggatcttcggcaccacactggacagcaagacccagagcctgctgatcgtgaacaacgccaccaacgtggtcatcaaagtgtgcgagttccagttctgcaacgaccccttcctggacgtctactaccacgagaacaacaagagcaggatggaaagcgagctccgggtgtacagcagcgccaacaactgcaccttcgagtacgtgtcccagcctttcctgatggacctggaaggcaagcagggcaacttcaagaacctgcgcgagttcgtgtttaagaacatcgacggctacttcaagatctacagcaagcacacccctgtgaacctcggccgggatctgcctcagggcttctctgctctggaacccctggtggatctgcccatcggcatcaacatcacccggtttcagacactgctggccctgcacagaagctacctgacacctggcgatagcagcagcagctggacagctggtgccgccgcttactatgtgggctacctgcagcctagaaccttcctgctgaagtacaacgagaacggcaccatcaccgacgccgtggattgtgctctggatcctctgagcgagacaaagtgcaccctgaagtccttcaccgtggaaaagggcatctaccagaccagcaacttccgggtgcagcccaccgaatccatcgtgcggttccccaatatcaccaatctgtgccccttccacgaggtgttcaatgccaccaccttcgcctctgtgtacgcctggaaccggaagcggatcagcaattgcgtggccgactactccgtgctgtacaacttcgcccccttcttcgcattcaagtgctacggcgtgtcccctaccaagctgaacgacctgtgcttcacaaacgtgtacgccgacagcttcgtgatccggggaaacgaagtgtcacagattgcccctggacagacaggcaacatcgccgactacaactacaagctgcccgacgacttcaccggctgtgtgattgcctggaacagcaacaagctggactccaaagtcagcggcaactacaattacctgtaccggctgttccggaagtccaagctgaagcccttcgagcgggacatctccaccgagatctatcaggccggcaacaagccttgtaacggcgtggcaggcagcaactgctacttcccactgcagtcctacggctttaggcccacatacggcgtgggccaccagccctacagagtggtggtgctgagcttcgaactgctgcatgcccctgccacagtgtgcggccctaagaaaagcaccaatctcgtgaagaacaaatgcgtgaacttcaacttcaacggcctgaccggcaccggcgtgctgacagagagcaacaagaagttcctgccattccagcagtttggccgggatatcgccgataccacagacgccgttagagatccccagacactggaaatcctggacatcaccccttgcagcttcggcggagtgtctgtgatcacccctggcaccaacaccagcaatcaggtggcagtgctgtaccagggcgtgaactgtaccgaagtgcccgtggccattcacgccgatcagctgacacctacatggcgggtgtactccaccggcagcaatgtgtttcagaccagagccggctgtctgatcggagccgagtacgtgaacaatagctacgagtgcgacatccccatcggcgctggaatctgcgccagctaccagacacagacaaagagccaccggagagccagaagcgtggccagccagagcatcattgcctacacaatgtctctgggcgccgagaacagcgtggcctactccaacaactctatcgctatccccaccaacttcaccatcagcgtgaccacagagatcctgcctgtgtccatgaccaagaccagcgtggactgcaccatgtacatctgcggcgattccaccgagtgctccaacctgctgctgcagtacggcagcttctgcacccagctgaaaagagccctgacagggatcgccgtggaacaggacaagaacacccaagaggtgttcgcccaagtgaagcagatctacaagacccctcctatcaagtacttcggcggcttcaatttcagccagattctgcccgatcctagcaagcccagcaagcggagcttcatcgaggacctgctgttcaacaaagtgacactggccgacgccggcttcatcaagcagtatggcgattgtctgggcgacattgccgccagggatctgatttgcgcccagaagtttaacggactgacagtgctgcctcctctgctgaccgatgagatgatcgcccagtacacatctgccctgctggccggcacaatcacaagcggctggacatttggagcaggcgccgctctgcagatcccctttgctatgcagatggcctaccggttcaacggcatcggagtgacccagaatgtgctgtacgagaaccagaagctgatcgccaaccagttcaacagcgccatcggcaagatccaggacagcctgagcagcacagcaagcgccctgggaaagctgcaggacgtggtcaaccacaatgcccaggcactgaacaccctggtcaagcagctgtcctccaagttcggcgccatcagctctgtgctgaacgatatcctgagcagactggaccctcctgaggccgaggtgcagatcgacagactgatcacaggcagactgcagagcctccagacatacgtgacccagcagctgatcagagccgccgagattagagcctctgccaatctggccgccaccaagatgtctgagtgtgtgctgggccagagcaagagagtggacttttgcggcaagggctaccacctgatgagcttccctcagtctgcccctcacggcgtggtgtttctgcacgtgacatatgtgcccgctcaagagaagaatttcaccaccgctccagccatctgccacgacggcaaagcccactttcctagagaaggcgtgttcgtgtccaacggcacccattggttcgtgacacagcggaacttctacgagccccagatcatcaccaccgacaacaccttcgtgtctggcaactgcgacgtcgtgatcggcattgtgaacaataccgtgtacgaccctctgcagcccgagctggacagcttcaaagaggaactggacaagtactttaagaaccacacaagccccgacgtggacctgggcgatatcagcggaatcaatgccagcgtcgtgaacatccagaaagagatcgaccggctgaacgaggtggccaagaatctgaacgagagcctgatcaacctgcaagaactggggaagtacgagcagtacatcaagtggccctggtacatctggctgggctttatcgccggactgattgccatcgtgatggtcacaatcatgctgtgttgcatgaccagctgctgtagctgcctgaagggctgttgtagctgtggcagctgctgcaagttcgacgaggacgattctgagcccgtgctgaagggcgtgaaactgcactacacatgatga

SEQ ID NO: 88 - RNA, 4273 nt, synthetic construct
  source 1..4273: mol_type = other RNA
agaataaactagtattcttctggtccccacagactcagagagaacccgccaccatgttcgtgttcctggtgctgctgcctctggtgtccagccagtgtgtgaacctgatcaccagaacacagtcatacaccaacagctttaccagaggcgtgtactaccccgacaaggtgttcagatccagcgtgctgcactctacccaggacctgttcctgcctttcttcagcaacgtgacctggttccacgccatccacgtgtccggcaccaatggcaccaagagattcgacaaccccgtgctgcccttcaacgacggggtgtactttgccagcaccgagaagtccaacatcatcagaggctggatcttcggcaccacactggacagcaagacccagagcctgctgatcgtgaacaacgccaccaacgtggtcatcaaagtgtgcgagttccagttctgcaacgaccccttcctggacgtctactaccacgagaacaacaagagcaggatggaaagcgagctccgggtgtacagcagcgccaacaactgcaccttcgagtacgtgtcccagcctttcctgatggacctggaaggcaagcagggcaacttcaagaacctgcgcgagttcgtgtttaagaacatcgacggctacttcaagatctacagcaagcacacccctgtgaacctcggccgggatctgcctcagggcttctctgctctggaacccctggtggatctgcccatcggcatcaacatcacccggtttcagacactgctggccctgcacagaagctacctgacacctggcgatagcagcagcagctggacagctggtgccgccgcttactatgtgggctacctgcagcctagaaccttcctgctgaagtacaacgagaacggcaccatcaccgacgccgtggattgtgctctggatcctctgagcgagacaaagtgcaccctgaagtccttcaccgtggaaaagggcatctaccagaccagcaacttccgggtgcagcccaccgaatccatcgtgcggttccccaatatcaccaatctgtgccccttccacgaggtgttcaatgccaccaccttcgcctctgtgtacgcctggaaccggaagcggatcagcaattgcgtggccgactactccgtgctgtacaacttcgcccccttcttcgcattcaagtgctacggcgtgtcccctaccaagctgaacgacctgtgcttcacaaacgtgtacgccgacagcttcgtgatccggggaaacgaagtgtcacagattgcccctggacagacaggcaacatcgccgactacaactacaagctgcccgacgacttcaccggctgtgtgattgcctggaacagcaacaagctggactccaaagtcagcggcaactacaattacctgtaccggctgttccggaagtccaagctgaagcccttcgagcgggacatctccaccgagatctatcaggccggcaacaagccttgtaacggcgtggcaggcagcaactgctacttcccactgcagtcctacggctttaggcccacatacggcgtgggccaccagccctacagagtggtggtgctgagcttcgaactgctgcatgcccctgccacagtgtgcggccctaagaaaagcaccaatctcgtgaagaacaaatgcgtgaacttcaacttcaacggcctgaccggcaccggcgtgctgacagagagcaacaagaagttcctgccattccagcagtttggccgggatatcgccgataccacagacgccgttagagatccccagacactggaaatcctggacatcaccccttgcagcttcggcggagtgtctgtgatcacccctggcaccaacaccagcaatcaggtggcagtgctgtaccagggcgtgaactgtaccgaagtgcccgtggccattcacgccgatcagctgacacctacatggcgggtgtactccaccggcagcaatgtgtttcagaccagagccggctgtctgatcggagccgagtacgtgaacaatagctacgagtgcgacatccccatcggcgctggaatctgcgccagctaccagacacagacaaagagccaccggagagccagaagcgtggccagccagagcatcattgcctacacaatgtctctgggcgccgagaacagcgtggcctactccaacaactctatcgctatccccaccaacttcaccatcagcgtgaccacagagatcctgcctgtgtccatgaccaagaccagcgtggactgcaccatgtacatctgcggcgattccaccgagtgctccaacctgctgctgcagtacggcagcttctgcacccagctgaaaagagccctgacagggatcgccgtggaacaggacaagaacacccaagaggtgttcgcccaagtgaagcagatctacaagacccctcctatcaagtacttcggcggcttcaatttcagccagattctgcccgatcctagcaagcccagcaagcggagcttcatcgaggacctgctgttcaacaaagtgacactggccgacgccggcttcatcaagcagtatggcgattgtctgggcgacattgccgccagggatctgatttgcgcccagaagtttaacggactgacagtgctgcctcctctgctgaccgatgagatgatcgcccagtacacatctgccctgctggccggcacaatcacaagcggctggacatttggagcaggcgccgctctgcagatcccctttgctatgcagatggcctaccggttcaacggcatcggagtgacccagaatgtgctgtacgagaaccagaagctgatcgccaaccagttcaacagcgccatcggcaagatccaggacagcctgagcagcacagcaagcgccctgggaaagctgcaggacgtggtcaaccacaatgcccaggcactgaacaccctggtcaagcagctgtcctccaagttcggcgccatcagctctgtgctgaacgatatcctgagcagactggaccctcctgaggccgaggtgcagatcgacagactgatcacaggcagactgcagagcctccagacatacgtgacccagcagctgatcagagccgccgagattagagcctctgccaatctggccgccaccaagatgtctgagtgtgtgctgggccagagcaagagagtggacttttgcggcaagggctaccacctgatgagcttccctcagtctgcccctcacggcgtggtgtttctgcacgtgacatatgtgcccgctcaagagaagaatttcaccaccgctccagccatctgccacgacggcaaagcccactttcctagagaaggcgtgttcgtgtccaacggcacccattggttcgtgacacagcggaacttctacgagccccagatcatcaccaccgacaacaccttcgtgtctggcaactgcgacgtcgtgatcggcattgtgaacaataccgtgtacgaccctctgcagcccgagctggacagcttcaaagaggaactggacaagtactttaagaaccacacaagccccgacgtggacctgggcgatatcagcggaatcaatgccagcgtcgtgaacatccagaaagagatcgaccggctgaacgaggtggccaagaatctgaacgagagcctgatcaacctgcaagaactggggaagtacgagcagtacatcaagtggccctggtacatctggctgggctttatcgccggactgattgccatcgtgatggtcacaatcatgctgtgttgcatgaccagctgctgtagctgcctgaagggctgttgtagctgtggcagctgctgcaagttcgacgaggacgattctgagcccgtgctgaagggcgtgaaactgcactacacatgatgactcgagctggtactgcatgcacgcaatgctagctgcccctttcccgtcctgggtaccccgagtctcccccgacctcgggtcccaggtatgctcccacctccacctgccccactcaccacctctgctagttccagacacctcccaagcacgcagcaatgcagctcaaaacgcttagcctagccacacccccacgggaaacagcagtgattaacctttagcaataaacgaaagtttaactaagctatactaaccccagggttggtcaatttcgtgccagccacaccctggagctagcaaaaaaaaaaaaaaaaaaaaaaaaaaaaaagcatatgactaaaaaaaaaaaaaaaaaaaaaaaaaaaaaaaaaaaaaaaaaaaaaaaaaaaaaaaaaaaaaaaaaaaaa

SEQ ID NO: 89 - DNA, 4273 bp, synthetic construct
  source 1..4273: mol_type = other DNA
agaataaactagtattcttctggtccccacagactcagagagaacccgccaccatgttcgtgttcctggtgctgctgcctctggtgtccagccagtgtgtgaacctgatcaccagaacacagtcatacaccaacagctttaccagaggcgtgtactaccccgacaaggtgttcagatccagcgtgctgcactctacccaggacctgttcctgcctttcttcagcaacgtgacctggttccacgccatccacgtgtccggcaccaatggcaccaagagattcgacaaccccgtgctgcccttcaacgacggggtgtactttgccagcaccgagaagtccaacatcatcagaggctggatcttcggcaccacactggacagcaagacccagagcctgctgatcgtgaacaacgccaccaacgtggtcatcaaagtgtgcgagttccagttctgcaacgaccccttcctggacgtctactaccacgagaacaacaagagcaggatggaaagcgagctccgggtgtacagcagcgccaacaactgcaccttcgagtacgtgtcccagcctttcctgatggacctggaaggcaagcagggcaacttcaagaacctgcgcgagttcgtgtttaagaacatcgacggctacttcaagatctacagcaagcacacccctgtgaacctcggccgggatctgcctcagggcttctctgctctggaacccctggtggatctgcccatcggcatcaacatcacccggtttcagacactgctggccctgcacagaagctacctgacacctggcgatagcagcagcagctggacagctggtgccgccgcttactatgtgggctacctgcagcctagaaccttcctgctgaagtacaacgagaacggcaccatcaccgacgccgtggattgtgctctggatcctctgagcgagacaaagtgcaccctgaagtccttcaccgtggaaaagggcatctaccagaccagcaacttccgggtgcagcccaccgaatccatcgtgcggttccccaatatcaccaatctgtgccccttccacgaggtgttcaatgccaccaccttcgcctctgtgtacgcctggaaccggaagcggatcagcaattgcgtggccgactactccgtgctgtacaacttcgcccccttcttcgcattcaagtgctacggcgtgtcccctaccaagctgaacgacctgtgcttcacaaacgtgtacgccgacagcttcgtgatccggggaaacgaagtgtcacagattgcccctggacagacaggcaacatcgccgactacaactacaagctgcccgacgacttcaccggctgtgtgattgcctggaacagcaacaagctggactccaaagtcagcggcaactacaattacctgtaccggctgttccggaagtccaagctgaagcccttcgagcgggacatctccaccgagatctatcaggccggcaacaagccttgtaacggcgtggcaggcagcaactgctacttcccactgcagtcctacggctttaggcccacatacggcgtgggccaccagccctacagagtggtggtgctgagcttcgaactgctgcatgcccctgccacagtgtgcggccctaagaaaagcaccaatctcgtgaagaacaaatgcgtgaacttcaacttcaacggcctgaccggcaccggcgtgctgacagagagcaacaagaagttcctgccattccagcagtttggccgggatatcgccgataccacagacgccgttagagatccccagacactggaaatcctggacatcaccccttgcagcttcggcggagtgtctgtgatcacccctggcaccaacaccagcaatcaggtggcagtgctgtaccagggcgtgaactgtaccgaagtgcccgtggccattcacgccgatcagctgacacctacatggcgggtgtactccaccggcagcaatgtgtttcagaccagagccggctgtctgatcggagccgagtacgtgaacaatagctacgagtgcgacatccccatcggcgctggaatctgcgccagctaccagacacagacaaagagccaccggagagccagaagcgtggccagccagagcatcattgcctacacaatgtctctgggcgccgagaacagcgtggcctactccaacaactctatcgctatccccaccaacttcaccatcagcgtgaccacagagatcctgcctgtgtccatgaccaagaccagcgtggactgcaccatgtacatctgcggcgattccaccgagtgctccaacctgctgctgcagtacggcagcttctgcacccagctgaaaagagccctgacagggatcgccgtggaacaggacaagaacacccaagaggtgttcgcccaagtgaagcagatctacaagacccctcctatcaagtacttcggcggcttcaatttcagccagattctgcccgatcctagcaagcccagcaagcggagcttcatcgaggacctgctgttcaacaaagtgacactggccgacgccggcttcatcaagcagtatggcgattgtctgggcgacattgccgccagggatctgatttgcgcccagaagtttaacggactgacagtgctgcctcctctgctgaccgatgagatgatcgcccagtacacatctgccctgctggccggcacaatcacaagcggctggacatttggagcaggcgccgctctgcagatcccctttgctatgcagatggcctaccggttcaacggcatcggagtgacccagaatgtgctgtacgagaaccagaagctgatcgccaaccagttcaacagcgccatcggcaagatccaggacagcctgagcagcacagcaagcgccctgggaaagctgcaggacgtggtcaaccacaatgcccaggcactgaacaccctggtcaagcagctgtcctccaagttcggcgccatcagctctgtgctgaacgatatcctgagcagactggaccctcctgaggccgaggtgcagatcgacagactgatcacaggcagactgcagagcctccagacatacgtgacccagcagctgatcagagccgccgagattagagcctctgccaatctggccgccaccaagatgtctgagtgtgtgctgggccagagcaagagagtggacttttgcggcaagggctaccacctgatgagcttccctcagtctgcccctcacggcgtggtgtttctgcacgtgacatatgtgcccgctcaagagaagaatttcaccaccgctccagccatctgccacgacggcaaagcccactttcctagagaaggcgtgttcgtgtccaacggcacccattggttcgtgacacagcggaacttctacgagccccagatcatcaccaccgacaacaccttcgtgtctggcaactgcgacgtcgtgatcggcattgtgaacaataccgtgtacgaccctctgcagcccgagctggacagcttcaaagaggaactggacaagtactttaagaaccacacaagccccgacgtggacctgggcgatatcagcggaatcaatgccagcgtcgtgaacatccagaaagagatcgaccggctgaacgaggtggccaagaatctgaacgagagcctgatcaacctgcaagaactggggaagtacgagcagtacatcaagtggccctggtacatctggctgggctttatcgccggactgattgccatcgtgatggtcacaatcatgctgtgttgcatgaccagctgctgtagctgcctgaagggctgttgtagctgtggcagctgctgcaagttcgacgaggacgattctgagcccgtgctgaagggcgtgaaactgcactacacatgatgactcgagctggtactgcatgcacgcaatgctagctgcccctttcccgtcctgggtaccccgagtctcccccgacctcgggtcccaggtatgctcccacctccacctgccccactcaccacctctgctagttccagacacctcccaagcacgcagcaatgcagctcaaaacgcttagcctagccacacccccacgggaaacagcagtgattaacctttagcaataaacgaaagtttaactaagctatactaaccccagggttggtcaatttcgtgccagccacaccctggagctagcaaaaaaaaaaaaaaaaaaaaaaaaaaaaaagcatatgactaaaaaaaaaaaaaaaaaaaaaaaaaaaaaaaaaaaaaaaaaaaaaaaaaaaaaaaaaaaaaaaaaaaaa

SEQ ID NO: 90 - protein, 1268 aa, synthetic construct
MFVFLVLLPLVSSQCVNLITRTQSYTNSFTRGVYYPDKVFRSSVLHSTQDLFLPFFSNVTWFHAISGTNGTKRFDNPVLPFNDGVYFASTEKSNIIRGWIFGTTLDSKTQSLLIVNNATNVVIKVCEFQFCNDPFLDVYYHKNNKSWMESEFRVYSSANNCTFEYVSQPFLMDLEGKQGNFKNLREFVFKNIDGYFKIYSKHTPINLGRDLPQGFSALEPLVDLPIGINITRFQTLLALHRSYLTPGDSSSGWTAGAAAYYVGYLQPRTFLLKYNENGTITDAVDCALDPLSETKCTLKSFTVEKGIYQTSNFRVQPTESIVRFPNITNLCPFDEVFNATTFASVYAWNRKRISNCVADYSVLYNFAPFFAFKCYGVSPTKLNDLCFTNVYADSFVIRGNEVRQIAPGQTGNIADYNYKLPDDFTGCVIAWNSNKLDSKVGGNYNYRYRLFRKSNLKPFERDISTEIYQAGNKPCNGVAGVNCYFPLQSYGFRPTYGVGHQPYRVVVLSFELLHAPATVCGPKKSTNLVKNKCVNFNFNGLTGTGVLTESNKKFLPFQQFGRDIADTTDAVRDPQTLEILDITPCSFGGVSVITPGTNTSNQVAVLYQGVNCTEVPVAIHADQLTPTWRVYSTGSNVFQTRAGCLIGAEYVNNSYECDIPIGAGICASYQTQTKSHRRARSVASQSIIAYTMSLGAENSVAYSNNSIAIPTNFTISVTTEILPVSMTKTSVDCTMYICGDSTECSNLLLQYGSFCTQLKRALTGIAVEQDKNTQEVFAQVKQIYKTPPIKYFGGFNFSQILPDPSKPSKRSFIEDLLFNKVTLADAGFIKQYGDCLGDIAARDLICAQKFNGLTVLPPLLTDEMIAQYTSALLAGTITSGWTFGAGAALQIPFAMQMAYRFNGIGVTQNVLYENQKLIANQFNSAIGKIQDSLSSTASALGKLQDVVNHNAQALNTLVKQLSSKFGAISSVLNDILSRLDPPEAEVQIDRLITGRLQSLQTYVTQQLIRAAEIRASANLAATKMSECVLGQSKRVDFCGKGYHLMSFPQSAPHGVVFLHVTYVPAQEKNFTTAPAICHDGKAHFPREGVFVSNGTHWFVTQRNFYEPQIITTDNTFVSGNCDVVIGIVNNTVYDPLQPELDSFKEELDKYFKNHTSPDVDLGDISGINASVVNIQKEIDRLNEVAKNLNESLIDLQELGKYEQYIKWPWYIWLGFIAGLIAIVMVTIMLCCMTSCCSCLKGCCSCGSCCKFDEDDSEPVLKGVKLHYT

SEQ ID NO: 91 - RNA, 3810 nt, synthetic construct
  source 1..3810: mol_type = other RNA
atgttcgtgttcctggtgctgctgcctctggtgtccagccagtgtgtgaacctgatcaccagaacacagtcatacaccaacagctttaccagaggcgtgtactaccccgacaaggtgttcagatccagcgtgctgcactctacccaggacctgttcctgcctttcttcagcaacgtgacctggttccacgccatctccggcaccaatggcaccaagagattcgacaaccccgtgctgcccttcaacgacggggtgtactttgccagcaccgagaagtccaacatcatcagaggctggatcttcggcaccacactggacagcaagacccagagcctgctgatcgtgaacaacgccaccaacgtggtcatcaaagtgtgcgagttccagttctgcaacgaccccttcctggacgtctactaccacaagaacaacaagagctggatggaaagcgagttccgggtgtacagcagcgccaacaactgcaccttcgagtacgtgtcccagcctttcctgatggacctggaaggcaagcagggcaacttcaagaacctgcgcgagttcgtgtttaagaacatcgacggctacttcaagatctacagcaagcacacccctatcaacctcggccgggatctgcctcagggcttctctgctctggaacccctggtggatctgcccatcggcatcaacatcacccggtttcagacactgctggccctgcacagaagctacctgacacctggcgatagcagcagcggatggacagctggtgccgccgcttactatgtgggctacctgcagcctagaaccttcctgctgaagtacaacgagaacggcaccatcaccgacgccgtggattgtgctctggatcctctgagcgagacaaagtgcaccctgaagtccttcaccgtggaaaagggcatctaccagaccagcaacttccgggtgcagcccaccgaatccatcgtgcggttccccaatatcaccaatctgtgccccttcgacgaggtgttcaatgccaccaccttcgcctctgtgtacgcctggaaccggaagcggatcagcaattgcgtggccgactactccgtgctgtacaacttcgcccccttcttcgcattcaagtgctacggcgtgtcccctaccaagctgaacgacctgtgcttcacaaacgtgtacgccgacagcttcgtgatccggggaaacgaagtgcggcagattgcccctggacagacaggcaacatcgccgactacaactacaagctgcccgacgacttcaccggctgtgtgattgcctggaacagcaacaagctggactccaaagtcggcggcaactacaattacaggtaccggctgttccggaagtccaatctgaagcccttcgagcgggacatctccaccgagatctatcaggccggcaacaagccttgtaacggcgtggcaggcgtgaactgctacttcccactgcagtcctacggctttaggcccacatacggcgtgggccaccagccctacagagtggtggtgctgagcttcgaactgctgcatgcccctgccacagtgtgcggccctaagaaaagcaccaatctcgtgaagaacaaatgcgtgaacttcaacttcaacggcctgaccggcaccggcgtgctgacagagagcaacaagaagttcctgccattccagcagtttggccgggatatcgccgataccacagacgccgttagagatccccagacactggaaatcctggacatcaccccttgcagcttcggcggagtgtctgtgatcacccctggcaccaacaccagcaatcaggtggcagtgctgtaccagggcgtgaactgtaccgaagtgcccgtggccattcacgccgatcagctgacacctacatggcgggtgtactccaccggcagcaatgtgtttcagaccagagccggctgtctgatcggagccgagtacgtgaacaatagctacgagtgcgacatccccatcggcgctggaatctgcgccagctaccagacacagacaaagagccaccggagagccagaagcgtggccagccagagcatcattgcctacacaatgtctctgggcgccgagaacagcgtggcctactccaacaactctatcgctatccccaccaacttcaccatcagcgtgaccacagagatcctgcctgtgtccatgaccaagaccagcgtggactgcaccatgtacatctgcggcgattccaccgagtgctccaacctgctgctgcagtacggcagcttctgcacccagctgaaaagagccctgacagggatcgccgtggaacaggacaagaacacccaagaggtgttcgcccaagtgaagcagatctacaagacccctcctatcaagtacttcggcggcttcaatttcagccagattctgcccgatcctagcaagcccagcaagcggagcttcatcgaggacctgctgttcaacaaagtgacactggccgacgccggcttcatcaagcagtatggcgattgtctgggcgacattgccgccagggatctgatttgcgcccagaagtttaacggactgacagtgctgcctcctctgctgaccgatgagatgatcgcccagtacacatctgccctgctggccggcacaatcacaagcggctggacatttggagcaggcgccgctctgcagatcccctttgctatgcagatggcctaccggttcaacggcatcggagtgacccagaatgtgctgtacgagaaccagaagctgatcgccaaccagttcaacagcgccatcggcaagatccaggacagcctgagcagcacagcaagcgccctgggaaagctgcaggacgtggtcaaccacaatgcccaggcactgaacaccctggtcaagcagctgtcctccaagttcggcgccatcagctctgtgctgaacgatatcctgagcagactggaccctcctgaggccgaggtgcagatcgacagactgatcacaggcagactgcagagcctccagacatacgtgacccagcagctgatcagagccgccgagattagagcctctgccaatctggccgccaccaagatgtctgagtgtgtgctgggccagagcaagagagtggacttttgcggcaagggctaccacctgatgagcttccctcagtctgcccctcacggcgtggtgtttctgcacgtgacatatgtgcccgctcaagagaagaatttcaccaccgctccagccatctgccacgacggcaaagcccactttcctagagaaggcgtgttcgtgtccaacggcacccattggttcgtgacacagcggaacttctacgagccccagatcatcaccaccgacaacaccttcgtgtctggcaactgcgacgtcgtgatcggcattgtgaacaataccgtgtacgaccctctgcagcccgagctggacagcttcaaagaggaactggacaagtactttaagaaccacacaagccccgacgtggacctgggcgatatcagcggaatcaatgccagcgtcgtgaacatccagaaagagatcgaccggctgaacgaggtggccaagaatctgaacgagagcctgatcgacctgcaagaactggggaagtacgagcagtacatcaagtggccctggtacatctggctgggctttatcgccggactgattgccatcgtgatggtcacaatcatgctgtgttgcatgaccagctgctgtagctgcctgaagggctgttgtagctgtggcagctgctgcaagttcgacgaggacgattctgagcccgtgctgaagggcgtgaaactgcactacacatgatga

SEQ ID NO: 92 - DNA, 3810 bp, synthetic construct
  source 1..3810: mol_type = other DNA
atgttcgtgttcctggtgctgctgcctctggtgtccagccagtgtgtgaacctgatcaccagaacacagtcatacaccaacagctttaccagaggcgtgtactaccccgacaaggtgttcagatccagcgtgctgcactctacccaggacctgttcctgcctttcttcagcaacgtgacctggttccacgccatctccggcaccaatggcaccaagagattcgacaaccccgtgctgcccttcaacgacggggtgtactttgccagcaccgagaagtccaacatcatcagaggctggatcttcggcaccacactggacagcaagacccagagcctgctgatcgtgaacaacgccaccaacgtggtcatcaaagtgtgcgagttccagttctgcaacgaccccttcctggacgtctactaccacaagaacaacaagagctggatggaaagcgagttccgggtgtacagcagcgccaacaactgcaccttcgagtacgtgtcccagcctttcctgatggacctggaaggcaagcagggcaacttcaagaacctgcgcgagttcgtgtttaagaacatcgacggctacttcaagatctacagcaagcacacccctatcaacctcggccgggatctgcctcagggcttctctgctctggaacccctggtggatctgcccatcggcatcaacatcacccggtttcagacactgctggccctgcacagaagctacctgacacctggcgatagcagcagcggatggacagctggtgccgccgcttactatgtgggctacctgcagcctagaaccttcctgctgaagtacaacgagaacggcaccatcaccgacgccgtggattgtgctctggatcctctgagcgagacaaagtgcaccctgaagtccttcaccgtggaaaagggcatctaccagaccagcaacttccgggtgcagcccaccgaatccatcgtgcggttccccaatatcaccaatctgtgccccttcgacgaggtgttcaatgccaccaccttcgcctctgtgtacgcctggaaccggaagcggatcagcaattgcgtggccgactactccgtgctgtacaacttcgcccccttcttcgcattcaagtgctacggcgtgtcccctaccaagctgaacgacctgtgcttcacaaacgtgtacgccgacagcttcgtgatccggggaaacgaagtgcggcagattgcccctggacagacaggcaacatcgccgactacaactacaagctgcccgacgacttcaccggctgtgtgattgcctggaacagcaacaagctggactccaaagtcggcggcaactacaattacaggtaccggctgttccggaagtccaatctgaagcccttcgagcgggacatctccaccgagatctatcaggccggcaacaagccttgtaacggcgtggcaggcgtgaactgctacttcccactgcagtcctacggctttaggcccacatacggcgtgggccaccagccctacagagtggtggtgctgagcttcgaactgctgcatgcccctgccacagtgtgcggccctaagaaaagcaccaatctcgtgaagaacaaatgcgtgaacttcaacttcaacggcctgaccggcaccggcgtgctgacagagagcaacaagaagttcctgccattccagcagtttggccgggatatcgccgataccacagacgccgttagagatccccagacactggaaatcctggacatcaccccttgcagcttcggcggagtgtctgtgatcacccctggcaccaacaccagcaatcaggtggcagtgctgtaccagggcgtgaactgtaccgaagtgcccgtggccattcacgccgatcagctgacacctacatggcgggtgtactccaccggcagcaatgtgtttcagaccagagccggctgtctgatcggagccgagtacgtgaacaatagctacgagtgcgacatccccatcggcgctggaatctgcgccagctaccagacacagacaaagagccaccggagagccagaagcgtggccagccagagcatcattgcctacacaatgtctctgggcgccgagaacagcgtggcctactccaacaactctatcgctatccccaccaacttcaccatcagcgtgaccacagagatcctgcctgtgtccatgaccaagaccagcgtggactgcaccatgtacatctgcggcgattccaccgagtgctccaacctgctgctgcagtacggcagcttctgcacccagctgaaaagagccctgacagggatcgccgtggaacaggacaagaacacccaagaggtgttcgcccaagtgaagcagatctacaagacccctcctatcaagtacttcggcggcttcaatttcagccagattctgcccgatcctagcaagcccagcaagcggagcttcatcgaggacctgctgttcaacaaagtgacactggccgacgccggcttcatcaagcagtatggcgattgtctgggcgacattgccgccagggatctgatttgcgcccagaagtttaacggactgacagtgctgcctcctctgctgaccgatgagatgatcgcccagtacacatctgccctgctggccggcacaatcacaagcggctggacatttggagcaggcgccgctctgcagatcccctttgctatgcagatggcctaccggttcaacggcatcggagtgacccagaatgtgctgtacgagaaccagaagctgatcgccaaccagttcaacagcgccatcggcaagatccaggacagcctgagcagcacagcaagcgccctgggaaagctgcaggacgtggtcaaccacaatgcccaggcactgaacaccctggtcaagcagctgtcctccaagttcggcgccatcagctctgtgctgaacgatatcctgagcagactggaccctcctgaggccgaggtgcagatcgacagactgatcacaggcagactgcagagcctccagacatacgtgacccagcagctgatcagagccgccgagattagagcctctgccaatctggccgccaccaagatgtctgagtgtgtgctgggccagagcaagagagtggacttttgcggcaagggctaccacctgatgagcttccctcagtctgcccctcacggcgtggtgtttctgcacgtgacatatgtgcccgctcaagagaagaatttcaccaccgctccagccatctgccacgacggcaaagcccactttcctagagaaggcgtgttcgtgtccaacggcacccattggttcgtgacacagcggaacttctacgagccccagatcatcaccaccgacaacaccttcgtgtctggcaactgcgacgtcgtgatcggcattgtgaacaataccgtgtacgaccctctgcagcccgagctggacagcttcaaagaggaactggacaagtactttaagaaccacacaagccccgacgtggacctgggcgatatcagcggaatcaatgccagcgtcgtgaacatccagaaagagatcgaccggctgaacgaggtggccaagaatctgaacgagagcctgatcgacctgcaagaactggggaagtacgagcagtacatcaagtggccctggtacatctggctgggctttatcgccggactgattgccatcgtgatggtcacaatcatgctgtgttgcatgaccagctgctgtagctgcctgaagggctgttgtagctgtggcagctgctgcaagttcgacgaggacgattctgagcccgtgctgaagggcgtgaaactgcactacacatgatga

SEQ ID NO: 93 - RNA, 4267 nt, synthetic construct
  source 1..4267: mol_type = other RNA
agaataaactagtattcttctggtccccacagactcagagagaacccgccaccatgttcgtgttcctggtgctgctgcctctggtgtccagccagtgtgtgaacctgatcaccagaacacagtcatacaccaacagctttaccagaggcgtgtactaccccgacaaggtgttcagatccagcgtgctgcactctacccaggacctgttcctgcctttcttcagcaacgtgacctggttccacgccatctccggcaccaatggcaccaagagattcgacaaccccgtgctgcccttcaacgacggggtgtactttgccagcaccgagaagtccaacatcatcagaggctggatcttcggcaccacactggacagcaagacccagagcctgctgatcgtgaacaacgccaccaacgtggtcatcaaagtgtgcgagttccagttctgcaacgaccccttcctggacgtctactaccacaagaacaacaagagctggatggaaagcgagttccgggtgtacagcagcgccaacaactgcaccttcgagtacgtgtcccagcctttcctgatggacctggaaggcaagcagggcaacttcaagaacctgcgcgagttcgtgtttaagaacatcgacggctacttcaagatctacagcaagcacacccctatcaacctcggccgggatctgcctcagggcttctctgctctggaacccctggtggatctgcccatcggcatcaacatcacccggtttcagacactgctggccctgcacagaagctacctgacacctggcgatagcagcagcggatggacagctggtgccgccgcttactatgtgggctacctgcagcctagaaccttcctgctgaagtacaacgagaacggcaccatcaccgacgccgtggattgtgctctggatcctctgagcgagacaaagtgcaccctgaagtccttcaccgtggaaaagggcatctaccagaccagcaacttccgggtgcagcccaccgaatccatcgtgcggttccccaatatcaccaatctgtgccccttcgacgaggtgttcaatgccaccaccttcgcctctgtgtacgcctggaaccggaagcggatcagcaattgcgtggccgactactccgtgctgtacaacttcgcccccttcttcgcattcaagtgctacggcgtgtcccctaccaagctgaacgacctgtgcttcacaaacgtgtacgccgacagcttcgtgatccggggaaacgaagtgcggcagattgcccctggacagacaggcaacatcgccgactacaactacaagctgcccgacgacttcaccggctgtgtgattgcctggaacagcaacaagctggactccaaagtcggcggcaactacaattacaggtaccggctgttccggaagtccaatctgaagcccttcgagcgggacatctccaccgagatctatcaggccggcaacaagccttgtaacggcgtggcaggcgtgaactgctacttcccactgcagtcctacggctttaggcccacatacggcgtgggccaccagccctacagagtggtggtgctgagcttcgaactgctgcatgcccctgccacagtgtgcggccctaagaaaagcaccaatctcgtgaagaacaaatgcgtgaacttcaacttcaacggcctgaccggcaccggcgtgctgacagagagcaacaagaagttcctgccattccagcagtttggccgggatatcgccgataccacagacgccgttagagatccccagacactggaaatcctggacatcaccccttgcagcttcggcggagtgtctgtgatcacccctggcaccaacaccagcaatcaggtggcagtgctgtaccagggcgtgaactgtaccgaagtgcccgtggccattcacgccgatcagctgacacctacatggcgggtgtactccaccggcagcaatgtgtttcagaccagagccggctgtctgatcggagccgagtacgtgaacaatagctacgagtgcgacatccccatcggcgctggaatctgcgccagctaccagacacagacaaagagccaccggagagccagaagcgtggccagccagagcatcattgcctacacaatgtctctgggcgccgagaacagcgtggcctactccaacaactctatcgctatccccaccaacttcaccatcagcgtgaccacagagatcctgcctgtgtccatgaccaagaccagcgtggactgcaccatgtacatctgcggcgattccaccgagtgctccaacctgctgctgcagtacggcagcttctgcacccagctgaaaagagccctgacagggatcgccgtggaacaggacaagaacacccaagaggtgttcgcccaagtgaagcagatctacaagacccctcctatcaagtacttcggcggcttcaatttcagccagattctgcccgatcctagcaagcccagcaagcggagcttcatcgaggacctgctgttcaacaaagtgacactggccgacgccggcttcatcaagcagtatggcgattgtctgggcgacattgccgccagggatctgatttgcgcccagaagtttaacggactgacagtgctgcctcctctgctgaccgatgagatgatcgcccagtacacatctgccctgctggccggcacaatcacaagcggctggacatttggagcaggcgccgctctgcagatcccctttgctatgcagatggcctaccggttcaacggcatcggagtgacccagaatgtgctgtacgagaaccagaagctgatcgccaaccagttcaacagcgccatcggcaagatccaggacagcctgagcagcacagcaagcgccctgggaaagctgcaggacgtggtcaaccacaatgcccaggcactgaacaccctggtcaagcagctgtcctccaagttcggcgccatcagctctgtgctgaacgatatcctgagcagactggaccctcctgaggccgaggtgcagatcgacagactgatcacaggcagactgcagagcctccagacatacgtgacccagcagctgatcagagccgccgagattagagcctctgccaatctggccgccaccaagatgtctgagtgtgtgctgggccagagcaagagagtggacttttgcggcaagggctaccacctgatgagcttccctcagtctgcccctcacggcgtggtgtttctgcacgtgacatatgtgcccgctcaagagaagaatttcaccaccgctccagccatctgccacgacggcaaagcccactttcctagagaaggcgtgttcgtgtccaacggcacccattggttcgtgacacagcggaacttctacgagccccagatcatcaccaccgacaacaccttcgtgtctggcaactgcgacgtcgtgatcggcattgtgaacaataccgtgtacgaccctctgcagcccgagctggacagcttcaaagaggaactggacaagtactttaagaaccacacaagccccgacgtggacctgggcgatatcagcggaatcaatgccagcgtcgtgaacatccagaaagagatcgaccggctgaacgaggtggccaagaatctgaacgagagcctgatcgacctgcaagaactggggaagtacgagcagtacatcaagtggccctggtacatctggctgggctttatcgccggactgattgccatcgtgatggtcacaatcatgctgtgttgcatgaccagctgctgtagctgcctgaagggctgttgtagctgtggcagctgctgcaagttcgacgaggacgattctgagcccgtgctgaagggcgtgaaactgcactacacatgatgactcgagctggtactgcatgcacgcaatgctagctgcccctttcccgtcctgggtaccccgagtctcccccgacctcgggtcccaggtatgctcccacctccacctgccccactcaccacctctgctagttccagacacctcccaagcacgcagcaatgcagctcaaaacgcttagcctagccacacccccacgggaaacagcagtgattaacctttagcaataaacgaaagtttaactaagctatactaaccccagggttggtcaatttcgtgccagccacaccctggagctagcaaaaaaaaaaaaaaaaaaaaaaaaaaaaaagcatatgactaaaaaaaaaaaaaaaaaaaaaaaaaaaaaaaaaaaaaaaaaaaaaaaaaaaaaaaaaaaaaaaaaaaaa

SEQ ID NO: 94 - DNA, 4267 bp, synthetic construct
  source 1..4267: mol_type = other DNA
agaataaactagtattcttctggtccccacagactcagagagaacccgccaccatgttcgtgttcctggtgctgctgcctctggtgtccagccagtgtgtgaacctgatcaccagaacacagtcatacaccaacagctttaccagaggcgtgtactaccccgacaaggtgttcagatccagcgtgctgcactctacccaggacctgttcctgcctttcttcagcaacgtgacctggttccacgccatctccggcaccaatggcaccaagagattcgacaaccccgtgctgcccttcaacgacggggtgtactttgccagcaccgagaagtccaacatcatcagaggctggatcttcggcaccacactggacagcaagacccagagcctgctgatcgtgaacaacgccaccaacgtggtcatcaaagtgtgcgagttccagttctgcaacgaccccttcctggacgtctactaccacaagaacaacaagagctggatggaaagcgagttccgggtgtacagcagcgccaacaactgcaccttcgagtacgtgtcccagcctttcctgatggacctggaaggcaagcagggcaacttcaagaacctgcgcgagttcgtgtttaagaacatcgacggctacttcaagatctacagcaagcacacccctatcaacctcggccgggatctgcctcagggcttctctgctctggaacccctggtggatctgcccatcggcatcaacatcacccggtttcagacactgctggccctgcacagaagctacctgacacctggcgatagcagcagcggatggacagctggtgccgccgcttactatgtgggctacctgcagcctagaaccttcctgctgaagtacaacgagaacggcaccatcaccgacgccgtggattgtgctctggatcctctgagcgagacaaagtgcaccctgaagtccttcaccgtggaaaagggcatctaccagaccagcaacttccgggtgcagcccaccgaatccatcgtgcggttccccaatatcaccaatctgtgccccttcgacgaggtgttcaatgccaccaccttcgcctctgtgtacgcctggaaccggaagcggatcagcaattgcgtggccgactactccgtgctgtacaacttcgcccccttcttcgcattcaagtgctacggcgtgtcccctaccaagctgaacgacctgtgcttcacaaacgtgtacgccgacagcttcgtgatccggggaaacgaagtgcggcagattgcccctggacagacaggcaacatcgccgactacaactacaagctgcccgacgacttcaccggctgtgtgattgcctggaacagcaacaagctggactccaaagtcggcggcaactacaattacaggtaccggctgttccggaagtccaatctgaagcccttcgagcgggacatctccaccgagatctatcaggccggcaacaagccttgtaacggcgtggcaggcgtgaactgctacttcccactgcagtcctacggctttaggcccacatacggcgtgggccaccagccctacagagtggtggtgctgagcttcgaactgctgcatgcccctgccacagtgtgcggccctaagaaaagcaccaatctcgtgaagaacaaatgcgtgaacttcaacttcaacggcctgaccggcaccggcgtgctgacagagagcaacaagaagttcctgccattccagcagtttggccgggatatcgccgataccacagacgccgttagagatccccagacactggaaatcctggacatcaccccttgcagcttcggcggagtgtctgtgatcacccctggcaccaacaccagcaatcaggtggcagtgctgtaccagggcgtgaactgtaccgaagtgcccgtggccattcacgccgatcagctgacacctacatggcgggtgtactccaccggcagcaatgtgtttcagaccagagccggctgtctgatcggagccgagtacgtgaacaatagctacgagtgcgacatccccatcggcgctggaatctgcgccagctaccagacacagacaaagagccaccggagagccagaagcgtggccagccagagcatcattgcctacacaatgtctctgggcgccgagaacagcgtggcctactccaacaactctatcgctatccccaccaacttcaccatcagcgtgaccacagagatcctgcctgtgtccatgaccaagaccagcgtggactgcaccatgtacatctgcggcgattccaccgagtgctccaacctgctgctgcagtacggcagcttctgcacccagctgaaaagagccctgacagggatcgccgtggaacaggacaagaacacccaagaggtgttcgcccaagtgaagcagatctacaagacccctcctatcaagtacttcggcggcttcaatttcagccagattctgcccgatcctagcaagcccagcaagcggagcttcatcgaggacctgctgttcaacaaagtgacactggccgacgccggcttcatcaagcagtatggcgattgtctgggcgacattgccgccagggatctgatttgcgcccagaagtttaacggactgacagtgctgcctcctctgctgaccgatgagatgatcgcccagtacacatctgccctgctggccggcacaatcacaagcggctggacatttggagcaggcgccgctctgcagatcccctttgctatgcagatggcctaccggttcaacggcatcggagtgacccagaatgtgctgtacgagaaccagaagctgatcgccaaccagttcaacagcgccatcggcaagatccaggacagcctgagcagcacagcaagcgccctgggaaagctgcaggacgtggtcaaccacaatgcccaggcactgaacaccctggtcaagcagctgtcctccaagttcggcgccatcagctctgtgctgaacgatatcctgagcagactggaccctcctgaggccgaggtgcagatcgacagactgatcacaggcagactgcagagcctccagacatacgtgacccagcagctgatcagagccgccgagattagagcctctgccaatctggccgccaccaagatgtctgagtgtgtgctgggccagagcaagagagtggacttttgcggcaagggctaccacctgatgagcttccctcagtctgcccctcacggcgtggtgtttctgcacgtgacatatgtgcccgctcaagagaagaatttcaccaccgctccagccatctgccacgacggcaaagcccactttcctagagaaggcgtgttcgtgtccaacggcacccattggttcgtgacacagcggaacttctacgagccccagatcatcaccaccgacaacaccttcgtgtctggcaactgcgacgtcgtgatcggcattgtgaacaataccgtgtacgaccctctgcagcccgagctggacagcttcaaagaggaactggacaagtactttaagaaccacacaagccccgacgtggacctgggcgatatcagcggaatcaatgccagcgtcgtgaacatccagaaagagatcgaccggctgaacgaggtggccaagaatctgaacgagagcctgatcgacctgcaagaactggggaagtacgagcagtacatcaagtggccctggtacatctggctgggctttatcgccggactgattgccatcgtgatggtcacaatcatgctgtgttgcatgaccagctgctgtagctgcctgaagggctgttgtagctgtggcagctgctgcaagttcgacgaggacgattctgagcccgtgctgaagggcgtgaaactgcactacacatgatgactcgagctggtactgcatgcacgcaatgctagctgcccctttcccgtcctgggtaccccgagtctcccccgacctcgggtcccaggtatgctcccacctccacctgccccactcaccacctctgctagttccagacacctcccaagcacgcagcaatgcagctcaaaacgcttagcctagccacacccccacgggaaacagcagtgattaacctttagcaataaacgaaagtttaactaagctatactaaccccagggttggtcaatttcgtgccagccacaccctggagctagcaaaaaaaaaaaaaaaaaaaaaaaaaaaaaagcatatgactaaaaaaaaaaaaaaaaaaaaaaaaaaaaaaaaaaaaaaaaaaaaaaaaaaaaaaaaaaaaaaaaaaaaa

SEQ ID NO: 95 - protein, 1269 aa, synthetic construct
MFVFLVLLPLVSSQCVNLITRTQSYTNSFTRGVYYPDKVFRSSVLHSTQDLFLPFFSNVTWFHAIHVSGTNGTKRFDNPALPFNDGVYFASTEKSNIIRGWIFGTTLDSKTQSLLIVNNATNVVIKVCEFQFCNDPFLDVYQKNNKSWMESEFRVYSSANNCTFEYVSQPFLMDLEGKEGNFKNLREFVFKNIDGYFKIYSKHTPINLERDLPQGFSALEPLVDLPIGINITRFQTLLALHRSYLTPGDSSSGWTAGAAAYYVGYLQPRTFLLKYNENGTITDAVDCALDPLSETKCTLKSFTVEKGIYQTSNFRVQPTESIVRFPNITNLCPFHEVFNATTFASVYAWNRKRISNCVADYSVIYNFAPFFAFKCYGVSPTKLNDLCFTNVYADSFVIRGNEVSQIAPGQTGNIADYNYKLPDDFTGCVIAWNSNKLDSKPSGNYNYLYRLFRKSKLKPFERDISTEIYQAGNKPCNGVAGSNCYSPLQSYGFRPTYGVGHQPYRVVVLSFELLHAPATVCGPKKSTNLVKNKCVNFNFNGLTGTGVLTESNKKFLPFQQFGRDIADTTDAVRDPQTLEILDITPCSFGGVSVITPGTNTSNQVAVLYQGVNCTEVPVAIHADQLTPTWRVYSTGSNVFQTRAGCLIGAEYVNNSYECDIPIGAGICASYQTQTKSHRRARSVASQSIIAYTMSLGAENSVAYSNNSIAIPTNFTISVTTEILPVSMTKTSVDCTMYICGDSTECSNLLLQYGSFCTQLKRALTGIAVEQDKNTQEVFAQVKQIYKTPPIKYFGGFNFSQILPDPSKPSKRSFIEDLLFNKVTLADAGFIKQYGDCLGDIAARDLICAQKFNGLTVLPPLLTDEMIAQYTSALLAGTITSGWTFGAGAALQIPFAMQMAYRFNGIGVTQNVLYENQKLIANQFNSAIGKIQDSLSSTASALGKLQDVVNHNAQALNTLVKQLSSKFGAISSVLNDILSRLDPPEAEVQIDRLITGRLQSLQTYVTQQLIRAAEIRASANLAATKMSECVLGQSKRVDFCGKGYHLMSFPQSAPHGVVFLHVTYVPAQEKNFTTAPAICHDGKAHFPREGVFVSNGTHWFVTQRNFYEPQIITTDNTFVSGNCDVVIGIVNNTVYDPLQPELDSFKEELDKYFKNHTSPDVDLGDISGINASVVNIQKEIDRLNEVAKNLNESLIDLQELGKYEQYIKWPWYIWLGFIAGLIAIVMVTIMLCCMTSCCSCLKGCCSCGSCCKFDEDDSEPVLKGVKLHYT

SEQ ID NO: 96 - RNA, 3813 nt, synthetic construct
  source 1..3813: mol_type = other RNA
atgttcgtgttcctggtgctgctgcctctggtgtccagccagtgtgtgaacctgatcaccagaacacagtcatacaccaacagctttaccagaggcgtgtactaccccgacaaggtgttcagatccagcgtgctgcactctacccaggacctgttcctgcctttcttcagcaacgtgacctggttccacgccatccacgtgtccggcaccaatggcaccaagagattcgacaaccccgccctgcccttcaacgacggggtgtactttgccagcaccgagaagtccaacatcatcagaggctggatcttcggcaccacactggacagcaagacccagagcctgctgatcgtgaacaacgccaccaacgtggtcatcaaagtgtgcgagttccagttctgcaacgaccccttcctggacgtctaccagaagaacaacaagagctggatggaaagcgagttccgggtgtacagcagcgccaacaactgcaccttcgagtacgtgtcccagcctttcctgatggacctggaaggcaaggagggcaacttcaagaacctgcgcgagttcgtgtttaagaacatcgacggctacttcaagatctacagcaagcacacccctatcaacctcgagcgggatctgcctcagggcttctctgctctggaacccctggtggatctgcccatcggcatcaacatcacccggtttcagacactgctggccctgcacagaagctacctgacacctggcgatagcagcagcggatggacagctggtgccgccgcttactatgtgggctacctgcagcctagaaccttcctgctgaagtacaacgagaacggcaccatcaccgacgccgtggattgtgctctggatcctctgagcgagacaaagtgcaccctgaagtccttcaccgtggaaaagggcatctaccagaccagcaacttccgggtgcagcccaccgaatccatcgtgcggttccccaatatcaccaatctgtgccccttccacgaggtgttcaatgccaccaccttcgcctctgtgtacgcctggaaccggaagcggatcagcaattgcgtggccgactactccgtgatctacaacttcgcccccttcttcgcattcaagtgctacggcgtgtcccctaccaagctgaacgacctgtgcttcacaaacgtgtacgccgacagcttcgtgatccggggaaacgaagtgtcacagattgcccctggacagacaggcaacatcgccgactacaactacaagctgcccgacgacttcaccggctgtgtgattgcctggaacagcaacaagctggactccaaacccagcggcaactacaattacctgtaccggctgttccggaagtccaagctgaagcccttcgagcgggacatctccaccgagatctatcaggccggcaacaagccttgtaacggcgtggcaggcagcaactgctacagcccactgcagtcctacggctttaggcccacatacggcgtgggccaccagccctacagagtggtggtgctgagcttcgaactgctgcatgcccctgccacagtgtgcggccctaagaaaagcaccaatctcgtgaagaacaaatgcgtgaacttcaacttcaacggcctgaccggcaccggcgtgctgacagagagcaacaagaagttcctgccattccagcagtttggccgggatatcgccgataccacagacgccgttagagatccccagacactggaaatcctggacatcaccccttgcagcttcggcggagtgtctgtgatcacccctggcaccaacaccagcaatcaggtggcagtgctgtaccagggcgtgaactgtaccgaagtgcccgtggccattcacgccgatcagctgacacctacatggcgggtgtactccaccggcagcaatgtgtttcagaccagagccggctgtctgatcggagccgagtacgtgaacaatagctacgagtgcgacatccccatcggcgctggaatctgcgccagctaccagacacagacaaagagccaccggagagccagaagcgtggccagccagagcatcattgcctacacaatgtctctgggcgccgagaacagcgtggcctactccaacaactctatcgctatccccaccaacttcaccatcagcgtgaccacagagatcctgcctgtgtccatgaccaagaccagcgtggactgcaccatgtacatctgcggcgattccaccgagtgctccaacctgctgctgcagtacggcagcttctgcacccagctgaaaagagccctgacagggatcgccgtggaacaggacaagaacacccaagaggtgttcgcccaagtgaagcagatctacaagacccctcctatcaagtacttcggcggcttcaatttcagccagattctgcccgatcctagcaagcccagcaagcggagcttcatcgaggacctgctgttcaacaaagtgacactggccgacgccggcttcatcaagcagtatggcgattgtctgggcgacattgccgccagggatctgatttgcgcccagaagtttaacggactgacagtgctgcctcctctgctgaccgatgagatgatcgcccagtacacatctgccctgctggccggcacaatcacaagcggctggacatttggagcaggcgccgctctgcagatcccctttgctatgcagatggcctaccggttcaacggcatcggagtgacccagaatgtgctgtacgagaaccagaagctgatcgccaaccagttcaacagcgccatcggcaagatccaggacagcctgagcagcacagcaagcgccctgggaaagctgcaggacgtggtcaaccacaatgcccaggcactgaacaccctggtcaagcagctgtcctccaagttcggcgccatcagctctgtgctgaacgatatcctgagcagactggaccctcctgaggccgaggtgcagatcgacagactgatcacaggcagactgcagagcctccagacatacgtgacccagcagctgatcagagccgccgagattagagcctctgccaatctggccgccaccaagatgtctgagtgtgtgctgggccagagcaagagagtggacttttgcggcaagggctaccacctgatgagcttccctcagtctgcccctcacggcgtggtgtttctgcacgtgacatatgtgcccgctcaagagaagaatttcaccaccgctccagccatctgccacgacggcaaagcccactttcctagagaaggcgtgttcgtgtccaacggcacccattggttcgtgacacagcggaacttctacgagccccagatcatcaccaccgacaacaccttcgtgtctggcaactgcgacgtcgtgatcggcattgtgaacaataccgtgtacgaccctctgcagcccgagctggacagcttcaaagaggaactggacaagtactttaagaaccacacaagccccgacgtggacctgggcgatatcagcggaatcaatgccagcgtcgtgaacatccagaaagagatcgaccggctgaacgaggtggccaagaatctgaacgagagcctgatcgacctgcaagaactggggaagtacgagcagtacatcaagtggccctggtacatctggctgggctttatcgccggactgattgccatcgtgatggtcacaatcatgctgtgttgcatgaccagctgctgtagctgcctgaagggctgttgtagctgtggcagctgctgcaagttcgacgaggacgattctgagcccgtgctgaagggcgtgaaactgcactacacatgatga

SEQ ID NO: 97 - DNA, 3813 bp, synthetic construct
  source 1..3813: mol_type = other DNA
atgttcgtgttcctggtgctgctgcctctggtgtccagccagtgtgtgaacctgatcaccagaacacagtcatacaccaacagctttaccagaggcgtgtactaccccgacaaggtgttcagatccagcgtgctgcactctacccaggacctgttcctgcctttcttcagcaacgtgacctggttccacgccatccacgtgtccggcaccaatggcaccaagagattcgacaaccccgccctgcccttcaacgacggggtgtactttgccagcaccgagaagtccaacatcatcagaggctggatcttcggcaccacactggacagcaagacccagagcctgctgatcgtgaacaacgccaccaacgtggtcatcaaagtgtgcgagttccagttctgcaacgaccccttcctggacgtctaccagaagaacaacaagagctggatggaaagcgagttccgggtgtacagcagcgccaacaactgcaccttcgagtacgtgtcccagcctttcctgatggacctggaaggcaaggagggcaacttcaagaacctgcgcgagttcgtgtttaagaacatcgacggctacttcaagatctacagcaagcacacccctatcaacctcgagcgggatctgcctcagggcttctctgctctggaacccctggtggatctgcccatcggcatcaacatcacccggtttcagacactgctggccctgcacagaagctacctgacacctggcgatagcagcagcggatggacagctggtgccgccgcttactatgtgggctacctgcagcctagaaccttcctgctgaagtacaacgagaacggcaccatcaccgacgccgtggattgtgctctggatcctctgagcgagacaaagtgcaccctgaagtccttcaccgtggaaaagggcatctaccagaccagcaacttccgggtgcagcccaccgaatccatcgtgcggttccccaatatcaccaatctgtgccccttccacgaggtgttcaatgccaccaccttcgcctctgtgtacgcctggaaccggaagcggatcagcaattgcgtggccgactactccgtgatctacaacttcgcccccttcttcgcattcaagtgctacggcgtgtcccctaccaagctgaacgacctgtgcttcacaaacgtgtacgccgacagcttcgtgatccggggaaacgaagtgtcacagattgcccctggacagacaggcaacatcgccgactacaactacaagctgcccgacgacttcaccggctgtgtgattgcctggaacagcaacaagctggactccaaacccagcggcaactacaattacctgtaccggctgttccggaagtccaagctgaagcccttcgagcgggacatctccaccgagatctatcaggccggcaacaagccttgtaacggcgtggcaggcagcaactgctacagcccactgcagtcctacggctttaggcccacatacggcgtgggccaccagccctacagagtggtggtgctgagcttcgaactgctgcatgcccctgccacagtgtgcggccctaagaaaagcaccaatctcgtgaagaacaaatgcgtgaacttcaacttcaacggcctgaccggcaccggcgtgctgacagagagcaacaagaagttcctgccattccagcagtttggccgggatatcgccgataccacagacgccgttagagatccccagacactggaaatcctggacatcaccccttgcagcttcggcggagtgtctgtgatcacccctggcaccaacaccagcaatcaggtggcagtgctgtaccagggcgtgaactgtaccgaagtgcccgtggccattcacgccgatcagctgacacctacatggcgggtgtactccaccggcagcaatgtgtttcagaccagagccggctgtctgatcggagccgagtacgtgaacaatagctacgagtgcgacatccccatcggcgctggaatctgcgccagctaccagacacagacaaagagccaccggagagccagaagcgtggccagccagagcatcattgcctacacaatgtctctgggcgccgagaacagcgtggcctactccaacaactctatcgctatccccaccaacttcaccatcagcgtgaccacagagatcctgcctgtgtccatgaccaagaccagcgtggactgcaccatgtacatctgcggcgattccaccgagtgctccaacctgctgctgcagtacggcagcttctgcacccagctgaaaagagccctgacagggatcgccgtggaacaggacaagaacacccaagaggtgttcgcccaagtgaagcagatctacaagacccctcctatcaagtacttcggcggcttcaatttcagccagattctgcccgatcctagcaagcccagcaagcggagcttcatcgaggacctgctgttcaacaaagtgacactggccgacgccggcttcatcaagcagtatggcgattgtctgggcgacattgccgccagggatctgatttgcgcccagaagtttaacggactgacagtgctgcctcctctgctgaccgatgagatgatcgcccagtacacatctgccctgctggccggcacaatcacaagcggctggacatttggagcaggcgccgctctgcagatcccctttgctatgcagatggcctaccggttcaacggcatcggagtgacccagaatgtgctgtacgagaaccagaagctgatcgccaaccagttcaacagcgccatcggcaagatccaggacagcctgagcagcacagcaagcgccctgggaaagctgcaggacgtggtcaaccacaatgcccaggcactgaacaccctggtcaagcagctgtcctccaagttcggcgccatcagctctgtgctgaacgatatcctgagcagactggaccctcctgaggccgaggtgcagatcgacagactgatcacaggcagactgcagagcctccagacatacgtgacccagcagctgatcagagccgccgagattagagcctctgccaatctggccgccaccaagatgtctgagtgtgtgctgggccagagcaagagagtggacttttgcggcaagggctaccacctgatgagcttccctcagtctgcccctcacggcgtggtgtttctgcacgtgacatatgtgcccgctcaagagaagaatttcaccaccgctccagccatctgccacgacggcaaagcccactttcctagagaaggcgtgttcgtgtccaacggcacccattggttcgtgacacagcggaacttctacgagccccagatcatcaccaccgacaacaccttcgtgtctggcaactgcgacgtcgtgatcggcattgtgaacaataccgtgtacgaccctctgcagcccgagctggacagcttcaaagaggaactggacaagtactttaagaaccacacaagccccgacgtggacctgggcgatatcagcggaatcaatgccagcgtcgtgaacatccagaaagagatcgaccggctgaacgaggtggccaagaatctgaacgagagcctgatcgacctgcaagaactggggaagtacgagcagtacatcaagtggccctggtacatctggctgggctttatcgccggactgattgccatcgtgatggtcacaatcatgctgtgttgcatgaccagctgctgtagctgcctgaagggctgttgtagctgtggcagctgctgcaagttcgacgaggacgattctgagcccgtgctgaagggcgtgaaactgcactacacatgatga

SEQ ID NO: 98 - RNA, 4270 nt, synthetic construct
  source 1..4270: mol_type = other RNA
agaataaactagtattcttctggtccccacagactcagagagaacccgccaccatgttcgtgttcctggtgctgctgcctctggtgtccagccagtgtgtgaacctgatcaccagaacacagtcatacaccaacagctttaccagaggcgtgtactaccccgacaaggtgttcagatccagcgtgctgcactctacccaggacctgttcctgcctttcttcagcaacgtgacctggttccacgccatccacgtgtccggcaccaatggcaccaagagattcgacaaccccgccctgcccttcaacgacggggtgtactttgccagcaccgagaagtccaacatcatcagaggctggatcttcggcaccacactggacagcaagacccagagcctgctgatcgtgaacaacgccaccaacgtggtcatcaaagtgtgcgagttccagttctgcaacgaccccttcctggacgtctaccagaagaacaacaagagctggatggaaagcgagttccgggtgtacagcagcgccaacaactgcaccttcgagtacgtgtcccagcctttcctgatggacctggaaggcaaggagggcaacttcaagaacctgcgcgagttcgtgtttaagaacatcgacggctacttcaagatctacagcaagcacacccctatcaacctcgagcgggatctgcctcagggcttctctgctctggaacccctggtggatctgcccatcggcatcaacatcacccggtttcagacactgctggccctgcacagaagctacctgacacctggcgatagcagcagcggatggacagctggtgccgccgcttactatgtgggctacctgcagcctagaaccttcctgctgaagtacaacgagaacggcaccatcaccgacgccgtggattgtgctctggatcctctgagcgagacaaagtgcaccctgaagtccttcaccgtggaaaagggcatctaccagaccagcaacttccgggtgcagcccaccgaatccatcgtgcggttccccaatatcaccaatctgtgccccttccacgaggtgttcaatgccaccaccttcgcctctgtgtacgcctggaaccggaagcggatcagcaattgcgtggccgactactccgtgatctacaacttcgcccccttcttcgcattcaagtgctacggcgtgtcccctaccaagctgaacgacctgtgcttcacaaacgtgtacgccgacagcttcgtgatccggggaaacgaagtgtcacagattgcccctggacagacaggcaacatcgccgactacaactacaagctgcccgacgacttcaccggctgtgtgattgcctggaacagcaacaagctggactccaaacccagcggcaactacaattacctgtaccggctgttccggaagtccaagctgaagcccttcgagcgggacatctccaccgagatctatcaggccggcaacaagccttgtaacggcgtggcaggcagcaactgctacagcccactgcagtcctacggctttaggcccacatacggcgtgggccaccagccctacagagtggtggtgctgagcttcgaactgctgcatgcccctgccacagtgtgcggccctaagaaaagcaccaatctcgtgaagaacaaatgcgtgaacttcaacttcaacggcctgaccggcaccggcgtgctgacagagagcaacaagaagttcctgccattccagcagtttggccgggatatcgccgataccacagacgccgttagagatccccagacactggaaatcctggacatcaccccttgcagcttcggcggagtgtctgtgatcacccctggcaccaacaccagcaatcaggtggcagtgctgtaccagggcgtgaactgtaccgaagtgcccgtggccattcacgccgatcagctgacacctacatggcgggtgtactccaccggcagcaatgtgtttcagaccagagccggctgtctgatcggagccgagtacgtgaacaatagctacgagtgcgacatccccatcggcgctggaatctgcgccagctaccagacacagacaaagagccaccggagagccagaagcgtggccagccagagcatcattgcctacacaatgtctctgggcgccgagaacagcgtggcctactccaacaactctatcgctatccccaccaacttcaccatcagcgtgaccacagagatcctgcctgtgtccatgaccaagaccagcgtggactgcaccatgtacatctgcggcgattccaccgagtgctccaacctgctgctgcagtacggcagcttctgcacccagctgaaaagagccctgacagggatcgccgtggaacaggacaagaacacccaagaggtgttcgcccaagtgaagcagatctacaagacccctcctatcaagtacttcggcggcttcaatttcagccagattctgcccgatcctagcaagcccagcaagcggagcttcatcgaggacctgctgttcaacaaagtgacactggccgacgccggcttcatcaagcagtatggcgattgtctgggcgacattgccgccagggatctgatttgcgcccagaagtttaacggactgacagtgctgcctcctctgctgaccgatgagatgatcgcccagtacacatctgccctgctggccggcacaatcacaagcggctggacatttggagcaggcgccgctctgcagatcccctttgctatgcagatggcctaccggttcaacggcatcggagtgacccagaatgtgctgtacgagaaccagaagctgatcgccaaccagttcaacagcgccatcggcaagatccaggacagcctgagcagcacagcaagcgccctgggaaagctgcaggacgtggtcaaccacaatgcccaggcactgaacaccctggtcaagcagctgtcctccaagttcggcgccatcagctctgtgctgaacgatatcctgagcagactggaccctcctgaggccgaggtgcagatcgacagactgatcacaggcagactgcagagcctccagacatacgtgacccagcagctgatcagagccgccgagattagagcctctgccaatctggccgccaccaagatgtctgagtgtgtgctgggccagagcaagagagtggacttttgcggcaagggctaccacctgatgagcttccctcagtctgcccctcacggcgtggtgtttctgcacgtgacatatgtgcccgctcaagagaagaatttcaccaccgctccagccatctgccacgacggcaaagcccactttcctagagaaggcgtgttcgtgtccaacggcacccattggttcgtgacacagcggaacttctacgagccccagatcatcaccaccgacaacaccttcgtgtctggcaactgcgacgtcgtgatcggcattgtgaacaataccgtgtacgaccctctgcagcccgagctggacagcttcaaagaggaactggacaagtactttaagaaccacacaagccccgacgtggacctgggcgatatcagcggaatcaatgccagcgtcgtgaacatccagaaagagatcgaccggctgaacgaggtggccaagaatctgaacgagagcctgatcgacctgcaagaactggggaagtacgagcagtacatcaagtggccctggtacatctggctgggctttatcgccggactgattgccatcgtgatggtcacaatcatgctgtgttgcatgaccagctgctgtagctgcctgaagggctgttgtagctgtggcagctgctgcaagttcgacgaggacgattctgagcccgtgctgaagggcgtgaaactgcactacacatgatgactcgagctggtactgcatgcacgcaatgctagctgcccctttcccgtcctgggtaccccgagtctcccccgacctcgggtcccaggtatgctcccacctccacctgccccactcaccacctctgctagttccagacacctcccaagcacgcagcaatgcagctcaaaacgcttagcctagccacacccccacgggaaacagcagtgattaacctttagcaataaacgaaagtttaactaagctatactaaccccagggttggtcaatttcgtgccagccacaccctggagctagcaaaaaaaaaaaaaaaaaaaaaaaaaaaaaagcatatgactaaaaaaaaaaaaaaaaaaaaaaaaaaaaaaaaaaaaaaaaaaaaaaaaaaaaaaaaaaaaaaaaaaaaa

SEQ ID NO: 99 - DNA, 4270 bp, synthetic construct
  source 1..4270: mol_type = other DNA
agaataaactagtattcttctggtccccacagactcagagagaacccgccaccatgttcgtgttcctggtgctgctgcctctggtgtccagccagtgtgtgaacctgatcaccagaacacagtcatacaccaacagctttaccagaggcgtgtactaccccgacaaggtgttcagatccagcgtgctgcactctacccaggacctgttcctgcctttcttcagcaacgtgacctggttccacgccatccacgtgtccggcaccaatggcaccaagagattcgacaaccccgccctgcccttcaacgacggggtgtactttgccagcaccgagaagtccaacatcatcagaggctggatcttcggcaccacactggacagcaagacccagagcctgctgatcgtgaacaacgccaccaacgtggtcatcaaagtgtgcgagttccagttctgcaacgaccccttcctggacgtctaccagaagaacaacaagagctggatggaaagcgagttccgggtgtacagcagcgccaacaactgcaccttcgagtacgtgtcccagcctttcctgatggacctggaaggcaaggagggcaacttcaagaacctgcgcgagttcgtgtttaagaacatcgacggctacttcaagatctacagcaagcacacccctatcaacctcgagcgggatctgcctcagggcttctctgctctggaacccctggtggatctgcccatcggcatcaacatcacccggtttcagacactgctggccctgcacagaagctacctgacacctggcgatagcagcagcggatggacagctggtgccgccgcttactatgtgggctacctgcagcctagaaccttcctgctgaagtacaacgagaacggcaccatcaccgacgccgtggattgtgctctggatcctctgagcgagacaaagtgcaccctgaagtccttcaccgtggaaaagggcatctaccagaccagcaacttccgggtgcagcccaccgaatccatcgtgcggttccccaatatcaccaatctgtgccccttccacgaggtgttcaatgccaccaccttcgcctctgtgtacgcctggaaccggaagcggatcagcaattgcgtggccgactactccgtgatctacaacttcgcccccttcttcgcattcaagtgctacggcgtgtcccctaccaagctgaacgacctgtgcttcacaaacgtgtacgccgacagcttcgtgatccggggaaacgaagtgtcacagattgcccctggacagacaggcaacatcgccgactacaactacaagctgcccgacgacttcaccggctgtgtgattgcctggaacagcaacaagctggactccaaacccagcggcaactacaattacctgtaccggctgttccggaagtccaagctgaagcccttcgagcgggacatctccaccgagatctatcaggccggcaacaagccttgtaacggcgtggcaggcagcaactgctacagcccactgcagtcctacggctttaggcccacatacggcgtgggccaccagccctacagagtggtggtgctgagcttcgaactgctgcatgcccctgccacagtgtgcggccctaagaaaagcaccaatctcgtgaagaacaaatgcgtgaacttcaacttcaacggcctgaccggcaccggcgtgctgacagagagcaacaagaagttcctgccattccagcagtttggccgggatatcgccgataccacagacgccgttagagatccccagacactggaaatcctggacatcaccccttgcagcttcggcggagtgtctgtgatcacccctggcaccaacaccagcaatcaggtggcagtgctgtaccagggcgtgaactgtaccgaagtgcccgtggccattcacgccgatcagctgacacctacatggcgggtgtactccaccggcagcaatgtgtttcagaccagagccggctgtctgatcggagccgagtacgtgaacaatagctacgagtgcgacatccccatcggcgctggaatctgcgccagctaccagacacagacaaagagccaccggagagccagaagcgtggccagccagagcatcattgcctacacaatgtctctgggcgccgagaacagcgtggcctactccaacaactctatcgctatccccaccaacttcaccatcagcgtgaccacagagatcctgcctgtgtccatgaccaagaccagcgtggactgcaccatgtacatctgcggcgattccaccgagtgctccaacctgctgctgcagtacggcagcttctgcacccagctgaaaagagccctgacagggatcgccgtggaacaggacaagaacacccaagaggtgttcgcccaagtgaagcagatctacaagacccctcctatcaagtacttcggcggcttcaatttcagccagattctgcccgatcctagcaagcccagcaagcggagcttcatcgaggacctgctgttcaacaaagtgacactggccgacgccggcttcatcaagcagtatggcgattgtctgggcgacattgccgccagggatctgatttgcgcccagaagtttaacggactgacagtgctgcctcctctgctgaccgatgagatgatcgcccagtacacatctgccctgctggccggcacaatcacaagcggctggacatttggagcaggcgccgctctgcagatcccctttgctatgcagatggcctaccggttcaacggcatcggagtgacccagaatgtgctgtacgagaaccagaagctgatcgccaaccagttcaacagcgccatcggcaagatccaggacagcctgagcagcacagcaagcgccctgggaaagctgcaggacgtggtcaaccacaatgcccaggcactgaacaccctggtcaagcagctgtcctccaagttcggcgccatcagctctgtgctgaacgatatcctgagcagactggaccctcctgaggccgaggtgcagatcgacagactgatcacaggcagactgcagagcctccagacatacgtgacccagcagctgatcagagccgccgagattagagcctctgccaatctggccgccaccaagatgtctgagtgtgtgctgggccagagcaagagagtggacttttgcggcaagggctaccacctgatgagcttccctcagtctgcccctcacggcgtggtgtttctgcacgtgacatatgtgcccgctcaagagaagaatttcaccaccgctccagccatctgccacgacggcaaagcccactttcctagagaaggcgtgttcgtgtccaacggcacccattggttcgtgacacagcggaacttctacgagccccagatcatcaccaccgacaacaccttcgtgtctggcaactgcgacgtcgtgatcggcattgtgaacaataccgtgtacgaccctctgcagcccgagctggacagcttcaaagaggaactggacaagtactttaagaaccacacaagccccgacgtggacctgggcgatatcagcggaatcaatgccagcgtcgtgaacatccagaaagagatcgaccggctgaacgaggtggccaagaatctgaacgagagcctgatcgacctgcaagaactggggaagtacgagcagtacatcaagtggccctggtacatctggctgggctttatcgccggactgattgccatcgtgatggtcacaatcatgctgtgttgcatgaccagctgctgtagctgcctgaagggctgttgtagctgtggcagctgctgcaagttcgacgaggacgattctgagcccgtgctgaagggcgtgaaactgcactacacatgatgactcgagctggtactgcatgcacgcaatgctagctgcccctttcccgtcctgggtaccccgagtctcccccgacctcgggtcccaggtatgctcccacctccacctgccccactcaccacctctgctagttccagacacctcccaagcacgcagcaatgcagctcaaaacgcttagcctagccacacccccacgggaaacagcagtgattaacctttagcaataaacgaaagtttaactaagctatactaaccccagggttggtcaatttcgtgccagccacaccctggagctagcaaaaaaaaaaaaaaaaaaaaaaaaaaaaaagcatatgactaaaaaaaaaaaaaaaaaaaaaaaaaaaaaaaaaaaaaaaaaaaaaaaaaaaaaaaaaaaaaaaaaaaaa

SEQ ID NO: 100 - protein, 1268 aa, synthetic construct
MFVFLVLLPLVSSQCVNLITRTQSYTNSFTRGVYYPDKVFRSSVLHSTQDLFLPFFSNVTWFHAISGTNGTKRFDNPVLPFNDGVYFASTEKSNIIRGWIFGTTLDSKTQSLLIVNNATNVVIKVCEFQFCNDPFLDVYYHKNNKSWMESEFRVYSSANNCTFEYVSQPFLMDLEGKQGNFKNLREFVFKNIDGYFKIYSKHTPINLGRDLPQGFSALEPLVDLPIGINITRFQTLLALHRSYLTPGDSSSGWTAGAAAYYVGYLQPRTFLLKYNENGTITDAVDCALDPLSETKCTLKSFTVEKGIYQTSNFRVQPTESIVRFPNITNLCPFDEVFNATTFASVYAWNRKRISNCVADYSVLYNFAPFFAFKCYGVSPTKLNDLCFTNVYADSFVIRGNEVSQIAPGQTGNIADYNYKLPDDFTGCVIAWNSNKLDSTVGGNYNYRYRLFRKSKLKPFERDISTEIYQAGNKPCNGVAGVNCYFPLQSYGFRPTYGVGHQPYRVVVLSFELLHAPATVCGPKKSTNLVKNKCVNFNFNGLTGTGVLTESNKKFLPFQQFGRDIADTTDAVRDPQTLEILDITPCSFGGVSVITPGTNTSNQVAVLYQGVNCTEVPVAIHADQLTPTWRVYSTGSNVFQTRAGCLIGAEYVNNSYECDIPIGAGICASYQTQTKSHRRARSVASQSIIAYTMSLGAENSVAYSNNSIAIPTNFTISVTTEILPVSMTKTSVDCTMYICGDSTECSNLLLQYGSFCTQLKRALTGIAVEQDKNTQEVFAQVKQIYKTPPIKYFGGFNFSQILPDPSKPSKRSFIEDLLFNKVTLADAGFIKQYGDCLGDIAARDLICAQKFNGLTVLPPLLTDEMIAQYTSALLAGTITSGWTFGAGAALQIPFAMQMAYRFNGIGVTQNVLYENQKLIANQFNSAIGKIQDSLSSTASALGKLQDVVNHNAQALNTLVKQLSSKFGAISSVLNDILSRLDPPEAEVQIDRLITGRLQSLQTYVTQQLIRAAEIRASANLAATKMSECVLGQSKRVDFCGKGYHLMSFPQSAPHGVVFLHVTYVPAQEKNFTTAPAICHDGKAHFPREGVFVSNGTHWFVTQRNFYEPQIITTDNTFVSGNCDVVIGIVNNTVYDPLQPELDSFKEELDKYFKNHTSPDVDLGDISGINASVVNIQKEIDRLNEVAKNLNESLIDLQELGKYEQYIKWPWYIWLGFIAGLIAIVMVTIMLCCMTSCCSCLKGCCSCGSCCKFDEDDSEPVLKGVKLHYT

SEQ ID NO: 101 - RNA, 3810 nt, synthetic construct
  source 1..3810: mol_type = other RNA
atgttcgtgttcctggtgctgctgcctctggtgtccagccagtgtgtgaacctgatcaccagaacacagtcatacaccaacagctttaccagaggcgtgtactaccccgacaaggtgttcagatccagcgtgctgcactctacccaggacctgttcctgcctttcttcagcaacgtgacctggttccacgccatctccggcaccaatggcaccaagagattcgacaaccccgtgctgcccttcaacgacggggtgtactttgccagcaccgagaagtccaacatcatcagaggctggatcttcggcaccacactggacagcaagacccagagcctgctgatcgtgaacaacgccaccaacgtggtcatcaaagtgtgcgagttccagttctgcaacgaccccttcctggacgtctactaccacaagaacaacaagagctggatggaaagcgagttccgggtgtacagcagcgccaacaactgcaccttcgagtacgtgtcccagcctttcctgatggacctggaaggcaagcagggcaacttcaagaacctgcgcgagttcgtgtttaagaacatcgacggctacttcaagatctacagcaagcacacccctatcaacctcggccgggatctgcctcagggcttctctgctctggaacccctggtggatctgcccatcggcatcaacatcacccggtttcagacactgctggccctgcacagaagctacctgacacctggcgatagcagcagcggatggacagctggtgccgccgcttactatgtgggctacctgcagcctagaaccttcctgctgaagtacaacgagaacggcaccatcaccgacgccgtggattgtgctctggatcctctgagcgagacaaagtgcaccctgaagtccttcaccgtggaaaagggcatctaccagaccagcaacttccgggtgcagcccaccgaatccatcgtgcggttccccaatatcaccaatctgtgccccttcgacgaggtgttcaatgccaccaccttcgcctctgtgtacgcctggaaccggaagcggatcagcaattgcgtggccgactactccgtgctgtacaacttcgcccccttcttcgcattcaagtgctacggcgtgtcccctaccaagctgaacgacctgtgcttcacaaacgtgtacgccgacagcttcgtgatccggggaaacgaagtgtcacagattgcccctggacagacaggcaacatcgccgactacaactacaagctgcccgacgacttcaccggctgtgtgattgcctggaacagcaacaagctggactccaccgtcggcggcaactacaattacaggtaccggctgttccggaagtccaagctgaagcccttcgagcgggacatctccaccgagatctatcaggccggcaacaagccttgtaacggcgtggcaggcgtgaactgctacttcccactgcagtcctacggctttaggcccacatacggcgtgggccaccagccctacagagtggtggtgctgagcttcgaactgctgcatgcccctgccacagtgtgcggccctaagaaaagcaccaatctcgtgaagaacaaatgcgtgaacttcaacttcaacggcctgaccggcaccggcgtgctgacagagagcaacaagaagttcctgccattccagcagtttggccgggatatcgccgataccacagacgccgttagagatccccagacactggaaatcctggacatcaccccttgcagcttcggcggagtgtctgtgatcacccctggcaccaacaccagcaatcaggtggcagtgctgtaccagggcgtgaactgtaccgaagtgcccgtggccattcacgccgatcagctgacacctacatggcgggtgtactccaccggcagcaatgtgtttcagaccagagccggctgtctgatcggagccgagtacgtgaacaatagctacgagtgcgacatccccatcggcgctggaatctgcgccagctaccagacacagacaaagagccaccggagagccagaagcgtggccagccagagcatcattgcctacacaatgtctctgggcgccgagaacagcgtggcctactccaacaactctatcgctatccccaccaacttcaccatcagcgtgaccacagagatcctgcctgtgtccatgaccaagaccagcgtggactgcaccatgtacatctgcggcgattccaccgagtgctccaacctgctgctgcagtacggcagcttctgcacccagctgaaaagagccctgacagggatcgccgtggaacaggacaagaacacccaagaggtgttcgcccaagtgaagcagatctacaagacccctcctatcaagtacttcggcggcttcaatttcagccagattctgcccgatcctagcaagcccagcaagcggagcttcatcgaggacctgctgttcaacaaagtgacactggccgacgccggcttcatcaagcagtatggcgattgtctgggcgacattgccgccagggatctgatttgcgcccagaagtttaacggactgacagtgctgcctcctctgctgaccgatgagatgatcgcccagtacacatctgccctgctggccggcacaatcacaagcggctggacatttggagcaggcgccgctctgcagatcccctttgctatgcagatggcctaccggttcaacggcatcggagtgacccagaatgtgctgtacgagaaccagaagctgatcgccaaccagttcaacagcgccatcggcaagatccaggacagcctgagcagcacagcaagcgccctgggaaagctgcaggacgtggtcaaccacaatgcccaggcactgaacaccctggtcaagcagctgtcctccaagttcggcgccatcagctctgtgctgaacgatatcctgagcagactggaccctcctgaggccgaggtgcagatcgacagactgatcacaggcagactgcagagcctccagacatacgtgacccagcagctgatcagagccgccgagattagagcctctgccaatctggccgccaccaagatgtctgagtgtgtgctgggccagagcaagagagtggacttttgcggcaagggctaccacctgatgagcttccctcagtctgcccctcacggcgtggtgtttctgcacgtgacatatgtgcccgctcaagagaagaatttcaccaccgctccagccatctgccacgacggcaaagcccactttcctagagaaggcgtgttcgtgtccaacggcacccattggttcgtgacacagcggaacttctacgagccccagatcatcaccaccgacaacaccttcgtgtctggcaactgcgacgtcgtgatcggcattgtgaacaataccgtgtacgaccctctgcagcccgagctggacagcttcaaagaggaactggacaagtactttaagaaccacacaagccccgacgtggacctgggcgatatcagcggaatcaatgccagcgtcgtgaacatccagaaagagatcgaccggctgaacgaggtggccaagaatctgaacgagagcctgatcgacctgcaagaactggggaagtacgagcagtacatcaagtggccctggtacatctggctgggctttatcgccggactgattgccatcgtgatggtcacaatcatgctgtgttgcatgaccagctgctgtagctgcctgaagggctgttgtagctgtggcagctgctgcaagttcgacgaggacgattctgagcccgtgctgaagggcgtgaaactgcactacacatgatga

SEQ ID NO: 102 - DNA, 3810 bp, synthetic construct
  source 1..3810: mol_type = other DNA
atgttcgtgttcctggtgctgctgcctctggtgtccagccagtgtgtgaacctgatcaccagaacacagtcatacaccaacagctttaccagaggcgtgtactaccccgacaaggtgttcagatccagcgtgctgcactctacccaggacctgttcctgcctttcttcagcaacgtgacctggttccacgccatctccggcaccaatggcaccaagagattcgacaaccccgtgctgcccttcaacgacggggtgtactttgccagcaccgagaagtccaacatcatcagaggctggatcttcggcaccacactggacagcaagacccagagcctgctgatcgtgaacaacgccaccaacgtggtcatcaaagtgtgcgagttccagttctgcaacgaccccttcctggacgtctactaccacaagaacaacaagagctggatggaaagcgagttccgggtgtacagcagcgccaacaactgcaccttcgagtacgtgtcccagcctttcctgatggacctggaaggcaagcagggcaacttcaagaacctgcgcgagttcgtgtttaagaacatcgacggctacttcaagatctacagcaagcacacccctatcaacctcggccgggatctgcctcagggcttctctgctctggaacccctggtggatctgcccatcggcatcaacatcacccggtttcagacactgctggccctgcacagaagctacctgacacctggcgatagcagcagcggatggacagctggtgccgccgcttactatgtgggctacctgcagcctagaaccttcctgctgaagtacaacgagaacggcaccatcaccgacgccgtggattgtgctctggatcctctgagcgagacaaagtgcaccctgaagtccttcaccgtggaaaagggcatctaccagaccagcaacttccgggtgcagcccaccgaatccatcgtgcggttccccaatatcaccaatctgtgccccttcgacgaggtgttcaatgccaccaccttcgcctctgtgtacgcctggaaccggaagcggatcagcaattgcgtggccgactactccgtgctgtacaacttcgcccccttcttcgcattcaagtgctacggcgtgtcccctaccaagctgaacgacctgtgcttcacaaacgtgtacgccgacagcttcgtgatccggggaaacgaagtgtcacagattgcccctggacagacaggcaacatcgccgactacaactacaagctgcccgacgacttcaccggctgtgtgattgcctggaacagcaacaagctggactccaccgtcggcggcaactacaattacaggtaccggctgttccggaagtccaagctgaagcccttcgagcgggacatctccaccgagatctatcaggccggcaacaagccttgtaacggcgtggcaggcgtgaactgctacttcccactgcagtcctacggctttaggcccacatacggcgtgggccaccagccctacagagtggtggtgctgagcttcgaactgctgcatgcccctgccacagtgtgcggccctaagaaaagcaccaatctcgtgaagaacaaatgcgtgaacttcaacttcaacggcctgaccggcaccggcgtgctgacagagagcaacaagaagttcctgccattccagcagtttggccgggatatcgccgataccacagacgccgttagagatccccagacactggaaatcctggacatcaccccttgcagcttcggcggagtgtctgtgatcacccctggcaccaacaccagcaatcaggtggcagtgctgtaccagggcgtgaactgtaccgaagtgcccgtggccattcacgccgatcagctgacacctacatggcgggtgtactccaccggcagcaatgtgtttcagaccagagccggctgtctgatcggagccgagtacgtgaacaatagctacgagtgcgacatccccatcggcgctggaatctgcgccagctaccagacacagacaaagagccaccggagagccagaagcgtggccagccagagcatcattgcctacacaatgtctctgggcgccgagaacagcgtggcctactccaacaactctatcgctatccccaccaacttcaccatcagcgtgaccacagagatcctgcctgtgtccatgaccaagaccagcgtggactgcaccatgtacatctgcggcgattccaccgagtgctccaacctgctgctgcagtacggcagcttctgcacccagctgaaaagagccctgacagggatcgccgtggaacaggacaagaacacccaagaggtgttcgcccaagtgaagcagatctacaagacccctcctatcaagtacttcggcggcttcaatttcagccagattctgcccgatcctagcaagcccagcaagcggagcttcatcgaggacctgctgttcaacaaagtgacactggccgacgccggcttcatcaagcagtatggcgattgtctgggcgacattgccgccagggatctgatttgcgcccagaagtttaacggactgacagtgctgcctcctctgctgaccgatgagatgatcgcccagtacacatctgccctgctggccggcacaatcacaagcggctggacatttggagcaggcgccgctctgcagatcccctttgctatgcagatggcctaccggttcaacggcatcggagtgacccagaatgtgctgtacgagaaccagaagctgatcgccaaccagttcaacagcgccatcggcaagatccaggacagcctgagcagcacagcaagcgccctgggaaagctgcaggacgtggtcaaccacaatgcccaggcactgaacaccctggtcaagcagctgtcctccaagttcggcgccatcagctctgtgctgaacgatatcctgagcagactggaccctcctgaggccgaggtgcagatcgacagactgatcacaggcagactgcagagcctccagacatacgtgacccagcagctgatcagagccgccgagattagagcctctgccaatctggccgccaccaagatgtctgagtgtgtgctgggccagagcaagagagtggacttttgcggcaagggctaccacctgatgagcttccctcagtctgcccctcacggcgtggtgtttctgcacgtgacatatgtgcccgctcaagagaagaatttcaccaccgctccagccatctgccacgacggcaaagcccactttcctagagaaggcgtgttcgtgtccaacggcacccattggttcgtgacacagcggaacttctacgagccccagatcatcaccaccgacaacaccttcgtgtctggcaactgcgacgtcgtgatcggcattgtgaacaataccgtgtacgaccctctgcagcccgagctggacagcttcaaagaggaactggacaagtactttaagaaccacacaagccccgacgtggacctgggcgatatcagcggaatcaatgccagcgtcgtgaacatccagaaagagatcgaccggctgaacgaggtggccaagaatctgaacgagagcctgatcgacctgcaagaactggggaagtacgagcagtacatcaagtggccctggtacatctggctgggctttatcgccggactgattgccatcgtgatggtcacaatcatgctgtgttgcatgaccagctgctgtagctgcctgaagggctgttgtagctgtggcagctgctgcaagttcgacgaggacgattctgagcccgtgctgaagggcgtgaaactgcactacacatgatga

SEQ ID NO: 103 - RNA, 4267 nt, synthetic construct
  source 1..4267: mol_type = other RNA
agaataaactagtattcttctggtccccacagactcagagagaacccgccaccatgttcgtgttcctggtgctgctgcctctggtgtccagccagtgtgtgaacctgatcaccagaacacagtcatacaccaacagctttaccagaggcgtgtactaccccgacaaggtgttcagatccagcgtgctgcactctacccaggacctgttcctgcctttcttcagcaacgtgacctggttccacgccatctccggcaccaatggcaccaagagattcgacaaccccgtgctgcccttcaacgacggggtgtactttgccagcaccgagaagtccaacatcatcagaggctggatcttcggcaccacactggacagcaagacccagagcctgctgatcgtgaacaacgccaccaacgtggtcatcaaagtgtgcgagttccagttctgcaacgaccccttcctggacgtctactaccacaagaacaacaagagctggatggaaagcgagttccgggtgtacagcagcgccaacaactgcaccttcgagtacgtgtcccagcctttcctgatggacctggaaggcaagcagggcaacttcaagaacctgcgcgagttcgtgtttaagaacatcgacggctacttcaagatctacagcaagcacacccctatcaacctcggccgggatctgcctcagggcttctctgctctggaacccctggtggatctgcccatcggcatcaacatcacccggtttcagacactgctggccctgcacagaagctacctgacacctggcgatagcagcagcggatggacagctggtgccgccgcttactatgtgggctacctgcagcctagaaccttcctgctgaagtacaacgagaacggcaccatcaccgacgccgtggattgtgctctggatcctctgagcgagacaaagtgcaccctgaagtccttcaccgtggaaaagggcatctaccagaccagcaacttccgggtgcagcccaccgaatccatcgtgcggttccccaatatcaccaatctgtgccccttcgacgaggtgttcaatgccaccaccttcgcctctgtgtacgcctggaaccggaagcggatcagcaattgcgtggccgactactccgtgctgtacaacttcgcccccttcttcgcattcaagtgctacggcgtgtcccctaccaagctgaacgacctgtgcttcacaaacgtgtacgccgacagcttcgtgatccggggaaacgaagtgtcacagattgcccctggacagacaggcaacatcgccgactacaactacaagctgcccgacgacttcaccggctgtgtgattgcctggaacagcaacaagctggactccaccgtcggcggcaactacaattacaggtaccggctgttccggaagtccaagctgaagcccttcgagcgggacatctccaccgagatctatcaggccggcaacaagccttgtaacggcgtggcaggcgtgaactgctacttcccactgcagtcctacggctttaggcccacatacggcgtgggccaccagccctacagagtggtggtgctgagcttcgaactgctgcatgcccctgccacagtgtgcggccctaagaaaagcaccaatctcgtgaagaacaaatgcgtgaacttcaacttcaacggcctgaccggcaccggcgtgctgacagagagcaacaagaagttcctgccattccagcagtttggccgggatatcgccgataccacagacgccgttagagatccccagacactggaaatcctggacatcaccccttgcagcttcggcggagtgtctgtgatcacccctggcaccaacaccagcaatcaggtggcagtgctgtaccagggcgtgaactgtaccgaagtgcccgtggccattcacgccgatcagctgacacctacatggcgggtgtactccaccggcagcaatgtgtttcagaccagagccggctgtctgatcggagccgagtacgtgaacaatagctacgagtgcgacatccccatcggcgctggaatctgcgccagctaccagacacagacaaagagccaccggagagccagaagcgtggccagccagagcatcattgcctacacaatgtctctgggcgccgagaacagcgtggcctactccaacaactctatcgctatccccaccaacttcaccatcagcgtgaccacagagatcctgcctgtgtccatgaccaagaccagcgtggactgcaccatgtacatctgcggcgattccaccgagtgctccaacctgctgctgcagtacggcagcttctgcacccagctgaaaagagccctgacagggatcgccgtggaacaggacaagaacacccaagaggtgttcgcccaagtgaagcagatctacaagacccctcctatcaagtacttcggcggcttcaatttcagccagattctgcccgatcctagcaagcccagcaagcggagcttcatcgaggacctgctgttcaacaaagtgacactggccgacgccggcttcatcaagcagtatggcgattgtctgggcgacattgccgccagggatctgatttgcgcccagaagtttaacggactgacagtgctgcctcctctgctgaccgatgagatgatcgcccagtacacatctgccctgctggccggcacaatcacaagcggctggacatttggagcaggcgccgctctgcagatcccctttgctatgcagatggcctaccggttcaacggcatcggagtgacccagaatgtgctgtacgagaaccagaagctgatcgccaaccagttcaacagcgccatcggcaagatccaggacagcctgagcagcacagcaagcgccctgggaaagctgcaggacgtggtcaaccacaatgcccaggcactgaacaccctggtcaagcagctgtcctccaagttcggcgccatcagctctgtgctgaacgatatcctgagcagactggaccctcctgaggccgaggtgcagatcgacagactgatcacaggcagactgcagagcctccagacatacgtgacccagcagctgatcagagccgccgagattagagcctctgccaatctggccgccaccaagatgtctgagtgtgtgctgggccagagcaagagagtggacttttgcggcaagggctaccacctgatgagcttccctcagtctgcccctcacggcgtggtgtttctgcacgtgacatatgtgcccgctcaagagaagaatttcaccaccgctccagccatctgccacgacggcaaagcccactttcctagagaaggcgtgttcgtgtccaacggcacccattggttcgtgacacagcggaacttctacgagccccagatcatcaccaccgacaacaccttcgtgtctggcaactgcgacgtcgtgatcggcattgtgaacaataccgtgtacgaccctctgcagcccgagctggacagcttcaaagaggaactggacaagtactttaagaaccacacaagccccgacgtggacctgggcgatatcagcggaatcaatgccagcgtcgtgaacatccagaaagagatcgaccggctgaacgaggtggccaagaatctgaacgagagcctgatcgacctgcaagaactggggaagtacgagcagtacatcaagtggccctggtacatctggctgggctttatcgccggactgattgccatcgtgatggtcacaatcatgctgtgttgcatgaccagctgctgtagctgcctgaagggctgttgtagctgtggcagctgctgcaagttcgacgaggacgattctgagcccgtgctgaagggcgtgaaactgcactacacatgatgactcgagctggtactgcatgcacgcaatgctagctgcccctttcccgtcctgggtaccccgagtctcccccgacctcgggtcccaggtatgctcccacctccacctgccccactcaccacctctgctagttccagacacctcccaagcacgcagcaatgcagctcaaaacgcttagcctagccacacccccacgggaaacagcagtgattaacctttagcaataaacgaaagtttaactaagctatactaaccccagggttggtcaatttcgtgccagccacaccctggagctagcaaaaaaaaaaaaaaaaaaaaaaaaaaaaaagcatatgactaaaaaaaaaaaaaaaaaaaaaaaaaaaaaaaaaaaaaaaaaaaaaaaaaaaaaaaaaaaaaaaaaaaaa

SEQ ID NO: 104 - DNA, 4267 bp, synthetic construct
  source 1..4267: mol_type = other DNA
agaataaactagtattcttctggtccccacagactcagagagaacccgccaccatgttcgtgttcctggtgctgctgcctctggtgtccagccagtgtgtgaacctgatcaccagaacacagtcatacaccaacagctttaccagaggcgtgtactaccccgacaaggtgttcagatccagcgtgctgcactctacccaggacctgttcctgcctttcttcagcaacgtgacctggttccacgccatctccggcaccaatggcaccaagagattcgacaaccccgtgctgcccttcaacgacggggtgtactttgccagcaccgagaagtccaacatcatcagaggctggatcttcggcaccacactggacagcaagacccagagcctgctgatcgtgaacaacgccaccaacgtggtcatcaaagtgtgcgagttccagttctgcaacgaccccttcctggacgtctactaccacaagaacaacaagagctggatggaaagcgagttccgggtgtacagcagcgccaacaactgcaccttcgagtacgtgtcccagcctttcctgatggacctggaaggcaagcagggcaacttcaagaacctgcgcgagttcgtgtttaagaacatcgacggctacttcaagatctacagcaagcacacccctatcaacctcggccgggatctgcctcagggcttctctgctctggaacccctggtggatctgcccatcggcatcaacatcacccggtttcagacactgctggccctgcacagaagctacctgacacctggcgatagcagcagcggatggacagctggtgccgccgcttactatgtgggctacctgcagcctagaaccttcctgctgaagtacaacgagaacggcaccatcaccgacgccgtggattgtgctctggatcctctgagcgagacaaagtgcaccctgaagtccttcaccgtggaaaagggcatctaccagaccagcaacttccgggtgcagcccaccgaatccatcgtgcggttccccaatatcaccaatctgtgccccttcgacgaggtgttcaatgccaccaccttcgcctctgtgtacgcctggaaccggaagcggatcagcaattgcgtggccgactactccgtgctgtacaacttcgcccccttcttcgcattcaagtgctacggcgtgtcccctaccaagctgaacgacctgtgcttcacaaacgtgtacgccgacagcttcgtgatccggggaaacgaagtgtcacagattgcccctggacagacaggcaacatcgccgactacaactacaagctgcccgacgacttcaccggctgtgtgattgcctggaacagcaacaagctggactccaccgtcggcggcaactacaattacaggtaccggctgttccggaagtccaagctgaagcccttcgagcgggacatctccaccgagatctatcaggccggcaacaagccttgtaacggcgtggcaggcgtgaactgctacttcccactgcagtcctacggctttaggcccacatacggcgtgggccaccagccctacagagtggtggtgctgagcttcgaactgctgcatgcccctgccacagtgtgcggccctaagaaaagcaccaatctcgtgaagaacaaatgcgtgaacttcaacttcaacggcctgaccggcaccggcgtgctgacagagagcaacaagaagttcctgccattccagcagtttggccgggatatcgccgataccacagacgccgttagagatccccagacactggaaatcctggacatcaccccttgcagcttcggcggagtgtctgtgatcacccctggcaccaacaccagcaatcaggtggcagtgctgtaccagggcgtgaactgtaccgaagtgcccgtggccattcacgccgatcagctgacacctacatggcgggtgtactccaccggcagcaatgtgtttcagaccagagccggctgtctgatcggagccgagtacgtgaacaatagctacgagtgcgacatccccatcggcgctggaatctgcgccagctaccagacacagacaaagagccaccggagagccagaagcgtggccagccagagcatcattgcctacacaatgtctctgggcgccgagaacagcgtggcctactccaacaactctatcgctatccccaccaacttcaccatcagcgtgaccacagagatcctgcctgtgtccatgaccaagaccagcgtggactgcaccatgtacatctgcggcgattccaccgagtgctccaacctgctgctgcagtacggcagcttctgcacccagctgaaaagagccctgacagggatcgccgtggaacaggacaagaacacccaagaggtgttcgcccaagtgaagcagatctacaagacccctcctatcaagtacttcggcggcttcaatttcagccagattctgcccgatcctagcaagcccagcaagcggagcttcatcgaggacctgctgttcaacaaagtgacactggccgacgccggcttcatcaagcagtatggcgattgtctgggcgacattgccgccagggatctgatttgcgcccagaagtttaacggactgacagtgctgcctcctctgctgaccgatgagatgatcgcccagtacacatctgccctgctggccggcacaatcacaagcggctggacatttggagcaggcgccgctctgcagatcccctttgctatgcagatggcctaccggttcaacggcatcggagtgacccagaatgtgctgtacgagaaccagaagctgatcgccaaccagttcaacagcgccatcggcaagatccaggacagcctgagcagcacagcaagcgccctgggaaagctgcaggacgtggtcaaccacaatgcccaggcactgaacaccctggtcaagcagctgtcctccaagttcggcgccatcagctctgtgctgaacgatatcctgagcagactggaccctcctgaggccgaggtgcagatcgacagactgatcacaggcagactgcagagcctccagacatacgtgacccagcagctgatcagagccgccgagattagagcctctgccaatctggccgccaccaagatgtctgagtgtgtgctgggccagagcaagagagtggacttttgcggcaagggctaccacctgatgagcttccctcagtctgcccctcacggcgtggtgtttctgcacgtgacatatgtgcccgctcaagagaagaatttcaccaccgctccagccatctgccacgacggcaaagcccactttcctagagaaggcgtgttcgtgtccaacggcacccattggttcgtgacacagcggaacttctacgagccccagatcatcaccaccgacaacaccttcgtgtctggcaactgcgacgtcgtgatcggcattgtgaacaataccgtgtacgaccctctgcagcccgagctggacagcttcaaagaggaactggacaagtactttaagaaccacacaagccccgacgtggacctgggcgatatcagcggaatcaatgccagcgtcgtgaacatccagaaagagatcgaccggctgaacgaggtggccaagaatctgaacgagagcctgatcgacctgcaagaactggggaagtacgagcagtacatcaagtggccctggtacatctggctgggctttatcgccggactgattgccatcgtgatggtcacaatcatgctgtgttgcatgaccagctgctgtagctgcctgaagggctgttgtagctgtggcagctgctgcaagttcgacgaggacgattctgagcccgtgctgaagggcgtgaaactgcactacacatgatgactcgagctggtactgcatgcacgcaatgctagctgcccctttcccgtcctgggtaccccgagtctcccccgacctcgggtcccaggtatgctcccacctccacctgccccactcaccacctctgctagttccagacacctcccaagcacgcagcaatgcagctcaaaacgcttagcctagccacacccccacgggaaacagcagtgattaacctttagcaataaacgaaagtttaactaagctatactaaccccagggttggtcaatttcgtgccagccacaccctggagctagcaaaaaaaaaaaaaaaaaaaaaaaaaaaaaagcatatgactaaaaaaaaaaaaaaaaaaaaaaaaaaaaaaaaaaaaaaaaaaaaaaaaaaaaaaaaaaaaaaaaaaaaa

SEQ ID NO: 105 - protein, 27 aa, synthetic construct
MGGAAARLGAVILFVVIVGLHGVRSKY

SEQ ID NO: 106 - protein, 25 aa, synthetic construct
MGRLTSGVGTAALLVVAVGLRVVCA

SEQ ID NO: 107 - protein, 28 aa, synthetic construct
MGRLTSGVGTAALLVVAVGLRVVCAKYA

SEQ ID NO: 108 - protein, 19 aa, synthetic construct
MFVFLVLLPLVSSQCVNLT

SEQ ID NO: 109 - protein, 21 aa, synthetic construct
MDWIWRILFLVGAATGAHSQM

SEQ ID NO: 110 - protein, 20 aa, synthetic construct
METPAQLLFLLLLWLPDTTG

SEQ ID NO: 111 - protein, 18 aa, synthetic construct
MDWTWILFLVAAATRVHS

SEQ ID NO: 112 - protein, 24 aa, synthetic construct
MLGSNSGQRVVFTILLLLVAPAYS

SEQ ID NO: 113 - protein, 17 aa, synthetic construct
MKCLLYLAFLFIGVNCA

SEQ ID NO: 114 - protein, 18 aa, synthetic construct
MDWTWILFLVAAATRVHS

SEQ ID NO: 115 - protein, 19 aa, synthetic construct
ETPAQLLFLLLLWLPDTTG

SEQ ID NO: 116 - protein, 24 aa, synthetic construct
MLGSNSGQRVVFTILLLLVAPAYS

SEQ ID NO: 117 - protein, 17 aa, synthetic construct
MKCLLYLAFLFIGVNCA

SEQ ID NO: 118 - protein, 15 aa, synthetic construct
MWLVSLAIVTACAGA

SEQ ID NO: 119 - protein, 15 aa, synthetic construct
MFVFLVLLPLVSSQC

SEQ ID NO: 120 - DNA, 81 bp, synthetic construct
  source 1..81: mol_type = other DNA
atggggggggctgccgccaggttgggggccgtgattttgtttgtcgtcatagtgggcctccatggggtccgcagcaaatat

SEQ ID NO: 121 - DNA, 81 bp, synthetic construct
  source 1..81: mol_type = other DNA
atgggaggagccgccgccagactgggagccgtgatcctgttcgtggtgatcgtgggactgcatggagtgagaagcaagtac

SEQ ID NO: 122 - DNA, 57 bp, synthetic construct
  source 1..57: mol_type = other DNA
atgtttgtgtttcttgtgctgctgcctcttgtgtcttctcagtgtgtgaatttgaca

SEQ ID NO: 123 - DNA, 63 bp, synthetic construct
  source 1..63: mol_type = other DNA
atggattggatttggagaatcctgttcctcgtgggagccgctacaggagcccactcccagatg

SEQ ID NO: 124 - protein, 5 aa, synthetic construct
YLYRL

SEQ ID NO: 125 - protein, 5 aa, synthetic construct
YRYRL

SEQ ID NO: 126 - protein, 5 aa, synthetic construct
AGSTP

SEQ ID NO: 127 - protein, 5 aa, synthetic construct
AGSKP

SEQ ID NO: 128 - protein, 5 aa, synthetic construct
AGNKP

SEQ ID NO: 129 - protein, 250 aa, synthetic construct
CTLKSFTVEKGIYQTSNFRVQPTESIVRFPNITNLCPFGEVFNATRFASVYAWNRKRISNCVADYSVLYNSASFSTFKCYGVSPTKLNDLCFTNVYADSFVIRGDEVRQIAPGQTGKIADYNYKLPDDFTGCVIAWNSNNLDSKVGGNYNYLYRLFRKSNLKPFERDISTEIYQAGSTPCNGVEGFNCYFPLQSYGFQPTNGVGYQPYRVVVLSFELLHAPATVCGPKKSTNLVKNKCVNFNFNGLTGTG

SEQ ID NO: 130 - protein, 250 aa, synthetic construct
CTLKSFTVEKGIYQTSNFRVQPTESIVRFPNITNLCPFGEVFNATRFASVYAWNRKRISNCVADYSVLYNSASFSTFKCYGVSPTKLNDLCFTNVYADSFVIRGDEVRQIAPGQTGKIADYNYKLPDDFTGCVIAWNSNNLDSKVGGNYNYLYRLFRKSNLKPFERDISTEIYQAGSTPCNGVEGFNCYFPLQSYGFQPTYGVGYQPYRVVVLSFELLHAPATVCGPKKSTNLVKNKCVNFNFNGLTGTG

SEQ ID NO: 131 - protein, 250 aa, synthetic construct
CTLKSFTVEKGIYQTSNFRVQPTESIVRFPNITNLCPFGEVFNATRFASVYAWNRKRISNCVADYSVLYNSASFSTFKCYGVSPTKLNDLCFTNVYADSFVIRGDEVRQIAPGQTGKIADYNYKLPDDFTGCVIAWNSNNLDSKVGGNYNYRYRLFRKSNLKPFERDISTEIYQAGSKPCNGVEGFNCYFPLQSYGFQPTNGVGYQPYRVVVLSFELLHAPATVCGPKKSTNLVKNKCVNFNFNGLTGTG

SEQ ID NO: 132 - protein, 250 aa, synthetic construct
CTLKSFTVEKGIYQTSNFRVQPTESIVRFPNITNLCPFDEVFNATRFASVYAWNRKRISNCVADYSVLYNLAPFFTFKCYGVSPTKLNDLCFTNVYADSFVIRGDEVRQIAPGQTGNIADYNYKLPDDFTGCVIAWNSNKLDSKVSGNYNYLYRLFRKSNLKPFERDISTEIYQAGNKPCNGVAGFNCYFPLRSYSFRPTYGVGHQPYRVVVLSFELLHAPATVCGPKKSTNLVKNKCVNFNFNGLKGTG

SEQ ID NO: 133 - protein, 250 aa, synthetic construct
CTLKSFTVEKGIYQTSNFRVQPTESIVRFPNITNLCPFDEVFNATRFASVYAWNRKRISNCVADYSVLYNFAPFFAFKCYGVSPTKLNDLCFTNVYADSFVIRGNEVSQIAPGQTGNIADYNYKLPDDFTGCVIAWNSNKLDSKVGGNYNYRYRLFRKSNLKPFERDISTEIYQAGNKPCNGVAGVNCYFPLQSYGFRPTYGVGHQPYRVVVLSFELLHAPATVCGPKKSTNLVKNKCVNFNFNGLTGTG

SEQ ID NO: 134 - protein, 9 aa, synthetic construct
GSPGSGSGS

SEQ ID NO: 135 - protein, 6 aa, synthetic construct
GSGSGS

SEQ ID NO: 136 - protein, 4 aa, synthetic construct
RRAR

SEQ ID NO: 137 - protein, 12 aa, synthetic construct
CGGAGAGCCAGA

SEQ ID NO: 138 - protein, 9 aa, synthetic construct
YLQPRTFLL

SEQ ID NO: 139 - protein, 9 aa, synthetic construct
RLQSLQTYV

SEQ ID NO: 140 - protein, 9 aa, synthetic construct
QYIKWPWYI

SEQ ID NO: 141 - protein, 9 aa, synthetic construct
NYNYLYRLF

SEQ ID NO: 142 - protein, 10 aa, synthetic construct
KWPWYIWLGF

SEQ ID NO: 143 - protein, 9 aa, synthetic construct
QPTESIVRF

SEQ ID NO: 144 - protein, 9 aa, synthetic construct
IPFAMQMAY

SEQ ID NO: 145 - protein, 9 aa, synthetic construct
LPFNDGVYF

SEQ ID NO: 146 - protein, 9 aa, synthetic construct
GVYFASTEK

SEQ ID NO: 147 - protein, 9 aa, synthetic construct
CVADYSVLY

SEQ ID NO: 148 - protein, 9 aa, synthetic construct
FQPTNGVGY

SEQ ID NO: 149 - protein, 9 aa, synthetic construct
GTHWFVTQR

SEQ ID NO: 150 - protein, 9 aa, synthetic construct
VYDPLQPEL

SEQ ID NO: 151 - protein, 9 aa, synthetic construct
KCYGVSPTK

SEQ ID NO: 152 - DNA, 3817 bp, synthetic construct
  source 1..3817: mol_type = other DNA
atgttcgtgttcctggtgctgctgcctctggtgtccagccagtgtgtgaacttcaccaccagaacacagctgcctccagcctacaccaacagctttaccagaggcgtgtactaccccgacaaggtgttcagatccagcgtgctgcactctacccaggacctgttcctgcctttcttcagcaacgtgacctggttccacgccatccacgtgtccggcaccaatggcaccaagagattcgccaaccccgtgctgcccttcaacgacggggtgtactttgccagcaccgagaagtccaacatcatcagaggctggatcttcggcaccacactggacagcaagacccagagcctgctgatcgtgaacaacgccaccaacgtggtcatcaaagtgtgcgagttccagttctgcaacgaccccttcctgggcgtctactaccacaagaacaacaagagctggatggaaagcgagttccgggtgtacagcagcgccaacaactgcaccttcgagtacgtgtcccagcctttcctgatggacctggaaggcaagcagggcaacttcaagaacctgcgcgagttcgtgtttaagaacatcgacggctacttcaagatctacagcaagcacacccctatcaacctcgtgcggggcctgcctcagggcttctctgctctggaacccctggtggatctgcccatcggcatcaacatcacccggtttcagacactgcacatcagctacctgacacctggcgatagcagcagcggatggacagctggtgccgccgcttactatgtgggctacctgcagcctagaaccttcctgctgaagtacaacgagaacggcaccatcaccgacgccgtggattgtgctctggatcctctgagcgagacaaagtgcaccctgaagtccttcaccgtggaaaagggcatctaccagaccagcaacttccgggtgcagcccaccgaatccatcgtgcggttccccaatatcaccaatctgtgccccttcggcgaggtgttcaatgccaccagattcgcctctgtgtacgcctggaaccggaagcggatcagcaattgcgtggccgactactccgtgctgtacaactccgccagcttcagcaccttcaagtgctacggcgtgtcccctaccaagctgaacgacctgtgcttcacaaacgtgtacgccgacagcttcgtgatccggggagatgaagtgcggcagattgcccctggacagacaggcaacatcgccgactacaactacaagctgcccgacgacttcaccggctgtgtgattgcctggaacagcaacaacctggactccaaagtcggcggcaactacaattacctgtaccggctgttccggaagtccaatctgaagcccttcgagcgggacatctccaccgagatctatcaggccggcagcaccccttgtaacggcgtgaagggcttcaactgctacttcccactgcagtcctacggctttcagcccacatacggcgtgggctatcagccctacagagtggtggtgctgagcttcgaactgctgcatgcccctgccacagtgtgcggccctaagaaaagcaccaatctcgtgaagaacaaatgcgtgaacttcaacttcaacggcctgaccggcaccggcgtgctgacagagagcaacaagaagttcctgccattccagcagtttggccgggatatcgccgataccacagacgccgttagagatccccagacactggaaatcctggacatcaccccttgcagcttcggcggagtgtctgtgatcacccctggcaccaacaccagcaatcaggtggcagtgctgtaccagggcgtgaactgtaccgaagtgcccgtggccattcacgccgatcagctgacacctacatggcgggtgtactccaccggcagcaatgtgtttcagaccagagccggctgtctgatcggagccgagcacgtgaacaatagctacgagtgcgacatccccatcggcgctggaatctgcgccagctaccagacacagacaaacagccctcggagagccagaagcgtggccagccagagcatcattgcctacacaatgtctctgggcgtcgagaacagcgtggcctactccaacaactctatcgctatccccaccaacttcaccatcagcgtgaccacagagatcctgcctgtgtccatgaccaagaccagcgtggactgcaccatgtacatctgcggcgattccaccgagtgctccaacctgctgctgcagtacggcagcttctgcacccagctgaatagagccctgacagggatcgccgtggaacaggacaagaacacccaagaggtgttcgcccaagtgaagcagatctacaagacccctcctatcaaggacttcggcggcttcaatttcagccagattctgcccgatcctagcaagcccagcaagcggagcttcatcgaggacctgctgttcaacaaagtgacactggccgacgccggcttcatcaagcagtatggcgattgtctgggcgacattgccgccagggatctgatttgcgcccagaagtttaacggactgacagtgctgcctcctctgctgaccgatgagatgatcgcccagtacacatctgccctgctggccggcacaatcacaagcggctggacatttggagcaggcgccgctctgcagatcccctttgctatgcagatggcctaccggttcaacggcatcggagtgacccagaatgtgctgtacgagaaccagaagctgatcgccaaccagttcaacagcgccatcggcaagatccaggacagcctgagcagcacagcaagcgccctgggaaagctgcaggacgtggtcaaccagaatgcccaggcactgaacaccctggtcaagcagctgtcctccaacttcggcgccatcagctctgtgctgaacgatatcctgagcagactggaccctcctgaggccgaggtgcagatcgacagactgatcacaggcagactgcagagcctccagacatacgtgacccagcagctgatcagagccgccgagattagagcctctgccaatctggccgccaccaagatgtctgagtgtgtgctgggccagagcaagagagtggacttttgcggcaagggctaccacctgatgagcttccctcagtctgcccctcacggcgtggtgtttctgcacgtgacatatgtgcccgctcaagagaagaatttcaccaccgctccagccatctgccacgacggcaaagcccactttcctagagaaggcgtgttcgtgtccaacggcacccattggttcgtgacacagcggaacttctacgagccccagatcatcaccaccgacaacaccttcgtgtctggcaactgcgacgtcgtgatcggcattgtgaacaataccgtgtacgaccctctgcagcccgagctggacagcttcaaagaggaactggacaagtactttaagaaccacacaagccccgacgtggacctgggcgatatcagcggaatcaatgccagcgtcgtgaacatccagaaagagatcgaccggctgaacgaggtggccaagaatctgaacgagagcctgatcgacctgcaagaactggggaagtacgagcagtacatcaagtggccctggtacatctggctgggctttatcgccggactgattgccatcgtgatggtcacaatcatgctgtgttgcatgaccagctgctgtagctgcctgaagggctgttgtagctgtggcagctgctgcaagttcgacgaggacgattctgagcccgtgctgaagggcgtgaaactgcactacacatgatgac

SEQ ID NO: 153 - DNA, 4274 bp, synthetic construct
  source 1..4274: mol_type = other DNA
agaataaactagtattcttctggtccccacagactcagagagaacccgccaccatgttcgtgttcctggtgctgctgcctctggtgtccagccagtgtgtgaacttcaccaccagaacacagctgcctccagcctacaccaacagctttaccagaggcgtgtactaccccgacaaggtgttcagatccagcgtgctgcactctacccaggacctgttcctgcctttcttcagcaacgtgacctggttccacgccatccacgtgtccggcaccaatggcaccaagagattcgccaaccccgtgctgcccttcaacgacggggtgtactttgccagcaccgagaagtccaacatcatcagaggctggatcttcggcaccacactggacagcaagacccagagcctgctgatcgtgaacaacgccaccaacgtggtcatcaaagtgtgcgagttccagttctgcaacgaccccttcctgggcgtctactaccacaagaacaacaagagctggatggaaagcgagttccgggtgtacagcagcgccaacaactgcaccttcgagtacgtgtcccagcctttcctgatggacctggaaggcaagcagggcaacttcaagaacctgcgcgagttcgtgtttaagaacatcgacggctacttcaagatctacagcaagcacacccctatcaacctcgtgcggggcctgcctcagggcttctctgctctggaacccctggtggatctgcccatcggcatcaacatcacccggtttcagacactgcacatcagctacctgacacctggcgatagcagcagcggatggacagctggtgccgccgcttactatgtgggctacctgcagcctagaaccttcctgctgaagtacaacgagaacggcaccatcaccgacgccgtggattgtgctctggatcctctgagcgagacaaagtgcaccctgaagtccttcaccgtggaaaagggcatctaccagaccagcaacttccgggtgcagcccaccgaatccatcgtgcggttccccaatatcaccaatctgtgccccttcggcgaggtgttcaatgccaccagattcgcctctgtgtacgcctggaaccggaagcggatcagcaattgcgtggccgactactccgtgctgtacaactccgccagcttcagcaccttcaagtgctacggcgtgtcccctaccaagctgaacgacctgtgcttcacaaacgtgtacgccgacagcttcgtgatccggggagatgaagtgcggcagattgcccctggacagacaggcaacatcgccgactacaactacaagctgcccgacgacttcaccggctgtgtgattgcctggaacagcaacaacctggactccaaagtcggcggcaactacaattacctgtaccggctgttccggaagtccaatctgaagcccttcgagcgggacatctccaccgagatctatcaggccggcagcaccccttgtaacggcgtgaagggcttcaactgctacttcccactgcagtcctacggctttcagcccacatacggcgtgggctatcagccctacagagtggtggtgctgagcttcgaactgctgcatgcccctgccacagtgtgcggccctaagaaaagcaccaatctcgtgaagaacaaatgcgtgaacttcaacttcaacggcctgaccggcaccggcgtgctgacagagagcaacaagaagttcctgccattccagcagtttggccgggatatcgccgataccacagacgccgttagagatccccagacactggaaatcctggacatcaccccttgcagcttcggcggagtgtctgtgatcacccctggcaccaacaccagcaatcaggtggcagtgctgtaccagggcgtgaactgtaccgaagtgcccgtggccattcacgccgatcagctgacacctacatggcgggtgtactccaccggcagcaatgtgtttcagaccagagccggctgtctgatcggagccgagcacgtgaacaatagctacgagtgcgacatccccatcggcgctggaatctgcgccagctaccagacacagacaaacagccctcggagagccagaagcgtggccagccagagcatcattgcctacacaatgtctctgggcgtcgagaacagcgtggcctactccaacaactctatcgctatccccaccaacttcaccatcagcgtgaccacagagatcctgcctgtgtccatgaccaagaccagcgtggactgcaccatgtacatctgcggcgattccaccgagtgctccaacctgctgctgcagtacggcagcttctgcacccagctgaatagagccctgacagggatcgccgtggaacaggacaagaacacccaagaggtgttcgcccaagtgaagcagatctacaagacccctcctatcaaggacttcggcggcttcaatttcagccagattctgcccgatcctagcaagcccagcaagcggagcttcatcgaggacctgctgttcaacaaagtgacactggccgacgccggcttcatcaagcagtatggcgattgtctgggcgacattgccgccagggatctgatttgcgcccagaagtttaacggactgacagtgctgcctcctctgctgaccgatgagatgatcgcccagtacacatctgccctgctggccggcacaatcacaagcggctggacatttggagcaggcgccgctctgcagatcccctttgctatgcagatggcctaccggttcaacggcatcggagtgacccagaatgtgctgtacgagaaccagaagctgatcgccaaccagttcaacagcgccatcggcaagatccaggacagcctgagcagcacagcaagcgccctgggaaagctgcaggacgtggtcaaccagaatgcccaggcactgaacaccctggtcaagcagctgtcctccaacttcggcgccatcagctctgtgctgaacgatatcctgagcagactggaccctcctgaggccgaggtgcagatcgacagactgatcacaggcagactgcagagcctccagacatacgtgacccagcagctgatcagagccgccgagattagagcctctgccaatctggccgccaccaagatgtctgagtgtgtgctgggccagagcaagagagtggacttttgcggcaagggctaccacctgatgagcttccctcagtctgcccctcacggcgtggtgtttctgcacgtgacatatgtgcccgctcaagagaagaatttcaccaccgctccagccatctgccacgacggcaaagcccactttcctagagaaggcgtgttcgtgtccaacggcacccattggttcgtgacacagcggaacttctacgagccccagatcatcaccaccgacaacaccttcgtgtctggcaactgcgacgtcgtgatcggcattgtgaacaataccgtgtacgaccctctgcagcccgagctggacagcttcaaagaggaactggacaagtactttaagaaccacacaagccccgacgtggacctgggcgatatcagcggaatcaatgccagcgtcgtgaacatccagaaagagatcgaccggctgaacgaggtggccaagaatctgaacgagagcctgatcgacctgcaagaactggggaagtacgagcagtacatcaagtggccctggtacatctggctgggctttatcgccggactgattgccatcgtgatggtcacaatcatgctgtgttgcatgaccagctgctgtagctgcctgaagggctgttgtagctgtggcagctgctgcaagttcgacgaggacgattctgagcccgtgctgaagggcgtgaaactgcactacacatgatgactcgagctggtactgcatgcacgcaatgctagctgcccctttcccgtcctgggtaccccgagtctcccccgacctcgggtcccaggtatgctcccacctccacctgccccactcaccacctctgctagttccagacacctcccaagcacgcagcaatgcagctcaaaacgcttagcctagccacacccccacgggaaacagcagtgattaacctttagcaataaacgaaagtttaactaagctatactaaccccagggttggtcaatttcgtgccagccacaccctggagctagcaaaaaaaaaaaaaaaaaaaaaaaaaaaaaagcatatgactaaaaaaaaaaaaaaaaaaaaaaaaaaaaaaaaaaaaaaaaaaaaaaaaaaaaaaaaaaaaaaaaaaaaaa

SEQ ID NO: 154 - DNA, 3816 bp, synthetic construct
  source 1..3816: mol_type = other DNA
atgttcgtgttcctggtgctgctgcctctggtgtccagccagtgtgtgaacctgaccaccagaacacagctgcctccagcctacaccaacagctttaccagaggcgtgtactaccccgacaaggtgttcagatccagcgtgctgcactctacccaggacctgttcctgcctttcttcagcaacgtgacctggttccacgccatctccggcaccaatggcaccaagagattcgacaaccccgtgctgcccttcaacgacggggtgtactttgccagcaccgagaagtccaacatcatcagaggctggatcttcggcaccacactggacagcaagacccagagcctgctgatcgtgaacaacgccaccaacgtggtcatcaaagtgtgcgagttccagttctgcaacgaccccttcctgggcgtctaccacaagaacaacaagagctggatggaaagcgagttccgggtgtacagcagcgccaacaactgcaccttcgagtacgtgtcccagcctttcctgatggacctggaaggcaagcagggcaacttcaagaacctgcgcgagttcgtgtttaagaacatcgacggctacttcaagatctacagcaagcacacccctatcaacctcgtgcgggatctgcctcagggcttctctgctctggaacccctggtggatctgcccatcggcatcaacatcacccggtttcagacactgctggccctgcacagaagctacctgacacctggcgatagcagcagcggatggacagctggtgccgccgcttactatgtgggctacctgcagcctagaaccttcctgctgaagtacaacgagaacggcaccatcaccgacgccgtggattgtgctctggatcctctgagcgagacaaagtgcaccctgaagtccttcaccgtggaaaagggcatctaccagaccagcaacttccgggtgcagcccaccgaatccatcgtgcggttccccaatatcaccaatctgtgccccttcggcgaggtgttcaatgccaccagattcgcctctgtgtacgcctggaaccggaagcggatcagcaattgcgtggccgactactccgtgctgtacaactccgccagcttcagcaccttcaagtgctacggcgtgtcccctaccaagctgaacgacctgtgcttcacaaacgtgtacgccgacagcttcgtgatccggggagatgaagtgcggcagattgcccctggacagacaggcaagatcgccgactacaactacaagctgcccgacgacttcaccggctgtgtgattgcctggaacagcaacaacctggactccaaagtcggcggcaactacaattacctgtaccggctgttccggaagtccaatctgaagcccttcgagcgggacatctccaccgagatctatcaggccggcagcaccccttgtaacggcgtggaaggcttcaactgctacttcccactgcagtcctacggctttcagcccacatacggcgtgggctatcagccctacagagtggtggtgctgagcttcgaactgctgcatgcccctgccacagtgtgcggccctaagaaaagcaccaatctcgtgaagaacaaatgcgtgaacttcaacttcaacggcctgaccggcaccggcgtgctgacagagagcaacaagaagttcctgccattccagcagtttggccgggatatcgacgataccacagacgccgttagagatccccagacactggaaatcctggacatcaccccttgcagcttcggcggagtgtctgtgatcacccctggcaccaacaccagcaatcaggtggcagtgctgtaccagggcgtgaactgtaccgaagtgcccgtggccattcacgccgatcagctgacacctacatggcgggtgtactccaccggcagcaatgtgtttcagaccagagccggctgtctgatcggagccgagcacgtgaacaatagctacgagtgcgacatccccatcggcgctggaatctgcgccagctaccagacacagacaaacagccaccggagagccagaagcgtggccagccagagcatcattgcctacacaatgtctctgggcgccgagaacagcgtggcctactccaacaactctatcgctatccccatcaacttcaccatcagcgtgaccacagagatcctgcctgtgtccatgaccaagaccagcgtggactgcaccatgtacatctgcggcgattccaccgagtgctccaacctgctgctgcagtacggcagcttctgcacccagctgaatagagccctgacagggatcgccgtggaacaggacaagaacacccaagaggtgttcgcccaagtgaagcagatctacaagacccctcctatcaaggacttcggcggcttcaatttcagccagattctgcccgatcctagcaagcccagcaagcggagcttcatcgaggacctgctgttcaacaaagtgacactggccgacgccggcttcatcaagcagtatggcgattgtctgggcgacattgccgccagggatctgatttgcgcccagaagtttaacggactgacagtgctgcctcctctgctgaccgatgagatgatcgcccagtacacatctgccctgctggccggcacaatcacaagcggctggacatttggagcaggcgccgctctgcagatcccctttgctatgcagatggcctaccggttcaacggcatcggagtgacccagaatgtgctgtacgagaaccagaagctgatcgccaaccagttcaacagcgccatcggcaagatccaggacagcctgagcagcacagcaagcgccctgggaaagctgcaggacgtggtcaaccagaatgcccaggcactgaacaccctggtcaagcagctgtcctccaacttcggcgccatcagctctgtgctgaacgatatcctggccagactggaccctcctgaggccgaggtgcagatcgacagactgatcacaggcagactgcagagcctccagacatacgtgacccagcagctgatcagagccgccgagattagagcctctgccaatctggccgccaccaagatgtctgagtgtgtgctgggccagagcaagagagtggacttttgcggcaagggctaccacctgatgagcttccctcagtctgcccctcacggcgtggtgtttctgcacgtgacatatgtgcccgctcaagagaagaatttcaccaccgctccagccatctgccacgacggcaaagcccactttcctagagaaggcgtgttcgtgtccaacggcacccattggttcgtgacacagcggaacttctacgagccccagatcatcaccacccacaacaccttcgtgtctggcaactgcgacgtcgtgatcggcattgtgaacaataccgtgtacgaccctctgcagcccgagctggacagcttcaaagaggaactggacaagtactttaagaaccacacaagccccgacgtggacctgggcgatatcagcggaatcaatgccagcgtcgtgaacatccagaaagagatcgaccggctgaacgaggtggccaagaatctgaacgagagcctgatcgacctgcaagaactggggaagtacgagcagtacatcaagtggccctggtacatctggctgggctttatcgccggactgattgccatcgtgatggtcacaatcatgctgtgttgcatgaccagctgctgtagctgcctgaagggctgttgtagctgtggcagctgctgcaagttcgacgaggacgattctgagcccgtgctgaagggcgtgaaactgcactacacatgatga

SEQ ID NO: 155 - DNA, 4274 bp, synthetic construct
  source 1..4274: mol_type = other DNA
agaataaactagtattcttctggtccccacagactcagagagaacccgccaccatgttcgtgttcctggtgctgctgcctctggtgtccagccagtgtgtgaacctgaccaccagaacacagctgcctccagcctacaccaacagctttaccagaggcgtgtactaccccgacaaggtgttcagatccagcgtgctgcactctacccaggacctgttcctgcctttcttcagcaacgtgacctggttccacgccatctccggcaccaatggcaccaagagattcgacaaccccgtgctgcccttcaacgacggggtgtactttgccagcaccgagaagtccaacatcatcagaggctggatcttcggcaccacactggacagcaagacccagagcctgctgatcgtgaacaacgccaccaacgtggtcatcaaagtgtgcgagttccagttctgcaacgaccccttcctgggcgtctaccacaagaacaacaagagctggatggaaagcgagttccgggtgtacagcagcgccaacaactgcaccttcgagtacgtgtcccagcctttcctgatggacctggaaggcaagcagggcaacttcaagaacctgcgcgagttcgtgtttaagaacatcgacggctacttcaagatctacagcaagcacacccctatcaacctcgtgcgggatctgcctcagggcttctctgctctggaacccctggtggatctgcccatcggcatcaacatcacccggtttcagacactgctggccctgcacagaagctacctgacacctggcgatagcagcagcggatggacagctggtgccgccgcttactatgtgggctacctgcagcctagaaccttcctgctgaagtacaacgagaacggcaccatcaccgacgccgtggattgtgctctggatcctctgagcgagacaaagtgcaccctgaagtccttcaccgtggaaaagggcatctaccagaccagcaacttccgggtgcagcccaccgaatccatcgtgcggttccccaatatcaccaatctgtgccccttcggcgaggtgttcaatgccaccagattcgcctctgtgtacgcctggaaccggaagcggatcagcaattgcgtggccgactactccgtgctgtacaactccgccagcttcagcaccttcaagtgctacggcgtgtcccctaccaagctgaacgacctgtgcttcacaaacgtgtacgccgacagcttcgtgatccggggagatgaagtgcggcagattgcccctggacagacaggcaagatcgccgactacaactacaagctgcccgacgacttcaccggctgtgtgattgcctggaacagcaacaacctggactccaaagtcggcggcaactacaattacctgtaccggctgttccggaagtccaatctgaagcccttcgagcgggacatctccaccgagatctatcaggccggcagcaccccttgtaacggcgtggaaggcttcaactgctacttcccactgcagtcctacggctttcagcccacatacggcgtgggctatcagccctacagagtggtggtgctgagcttcgaactgctgcatgcccctgccacagtgtgcggccctaagaaaagcaccaatctcgtgaagaacaaatgcgtgaacttcaacttcaacggcctgaccggcaccggcgtgctgacagagagcaacaagaagttcctgccattccagcagtttggccgggatatcgacgataccacagacgccgttagagatccccagacactggaaatcctggacatcaccccttgcagcttcggcggagtgtctgtgatcacccctggcaccaacaccagcaatcaggtggcagtgctgtaccagggcgtgaactgtaccgaagtgcccgtggccattcacgccgatcagctgacacctacatggcgggtgtactccaccggcagcaatgtgtttcagaccagagccggctgtctgatcggagccgagcacgtgaacaatagctacgagtgcgacatccccatcggcgctggaatctgcgccagctaccagacacagacaaacagccaccggagagccagaagcgtggccagccagagcatcattgcctacacaatgtctctgggcgccgagaacagcgtggcctactccaacaactctatcgctatccccatcaacttcaccatcagcgtgaccacagagatcctgcctgtgtccatgaccaagaccagcgtggactgcaccatgtacatctgcggcgattccaccgagtgctccaacctgctgctgcagtacggcagcttctgcacccagctgaatagagccctgacagggatcgccgtggaacaggacaagaacacccaagaggtgttcgcccaagtgaagcagatctacaagacccctcctatcaaggacttcggcggcttcaatttcagccagattctgcccgatcctagcaagcccagcaagcggagcttcatcgaggacctgctgttcaacaaagtgacactggccgacgccggcttcatcaagcagtatggcgattgtctgggcgacattgccgccagggatctgatttgcgcccagaagtttaacggactgacagtgctgcctcctctgctgaccgatgagatgatcgcccagtacacatctgccctgctggccggcacaatcacaagcggctggacatttggagcaggcgccgctctgcagatcccctttgctatgcagatggcctaccggttcaacggcatcggagtgacccagaatgtgctgtacgagaaccagaagctgatcgccaaccagttcaacagcgccatcggcaagatccaggacagcctgagcagcacagcaagcgccctgggaaagctgcaggacgtggtcaaccagaatgcccaggcactgaacaccctggtcaagcagctgtcctccaacttcggcgccatcagctctgtgctgaacgatatcctggccagactggaccctcctgaggccgaggtgcagatcgacagactgatcacaggcagactgcagagcctccagacatacgtgacccagcagctgatcagagccgccgagattagagcctctgccaatctggccgccaccaagatgtctgagtgtgtgctgggccagagcaagagagtggacttttgcggcaagggctaccacctgatgagcttccctcagtctgcccctcacggcgtggtgtttctgcacgtgacatatgtgcccgctcaagagaagaatttcaccaccgctccagccatctgccacgacggcaaagcccactttcctagagaaggcgtgttcgtgtccaacggcacccattggttcgtgacacagcggaacttctacgagccccagatcatcaccacccacaacaccttcgtgtctggcaactgcgacgtcgtgatcggcattgtgaacaataccgtgtacgaccctctgcagcccgagctggacagcttcaaagaggaactggacaagtactttaagaaccacacaagccccgacgtggacctgggcgatatcagcggaatcaatgccagcgtcgtgaacatccagaaagagatcgaccggctgaacgaggtggccaagaatctgaacgagagcctgatcgacctgcaagaactggggaagtacgagcagtacatcaagtggccctggtacatctggctgggctttatcgccggactgattgccatcgtgatggtcacaatcatgctgtgttgcatgaccagctgctgtagctgcctgaagggctgttgtagctgtggcagctgctgcaagttcgacgaggacgattctgagcccgtgctgaagggcgtgaaactgcactacacatgatgagatctgctggtactgcatgcacgcaatgctagctgcccctttcccgtcctgggtaccccgagtctcccccgacctcgggtcccaggtatgctcccacctccacctgccccactcaccacctctgctagttccagacacctcccaagcacgcagcaatgcagctcaaaacgcttagcctagccacacccccacgggaaacagcagtgattaacctttagcaataaacgaaagtttaactaagctatactaaccccagggttggtcaatttcgtgccagccacaccctggagctagcaaaaaaaaaaaaaaaaaaaaaaaaaaaaaagcatatgactaaaaaaaaaaaaaaaaaaaaaaaaaaaaaaaaaaaaaaaaaaaaaaaaaaaaaaaaaaaaaaaaaaaaaa

SEQ ID NO: 156 - RNA, 3819 nt, synthetic construct
  source 1..3819: mol_type = other RNA
atgttcgtgttcctggtgctgctgcctctggtgtccagccagtgtgtgaacctgagaaccagaacacagctgcctccagcctacaccaacagctttaccagaggcgtgtactaccccgacaaggtgttcagatccagcgtgctgcactctacccaggacctgttcctgcctttcttcagcaacgtgacctggttccacgccatccacgtgtccggcaccaatggcaccaagagattcgacaaccccgtgctgcccttcaacgacggggtgtactttgccagcaccgagaagtccaacatcatcagaggctggatcttcggcaccacactggacagcaagacccagagcctgctgatcgtgaacaacgccaccaacgtggtcatcaaagtgtgcgagttccagttctgcaacgaccccttcctggacgtctactaccacaagaacaacaagagctggatggaaagcggcgtgtacagcagcgccaacaactgcaccttcgagtacgtgtcccagcctttcctgatggacctggaaggcaagcagggcaacttcaagaacctgcgcgagttcgtgtttaagaacatcgacggctacttcaagatctacagcaagcacacccctatcaacctcgtgcgggatctgcctcagggcttctctgctctggaacccctggtggatctgcccatcggcatcaacatcacccggtttcagacactgctggccctgcacagaagctacctgacacctggcgatagcagcagcggatggacagctggtgccgccgcttactatgtgggctacctgcagcctagaaccttcctgctgaagtacaacgagaacggcaccatcaccgacgccgtggattgtgctctggatcctctgagcgagacaaagtgcaccctgaagtccttcaccgtggaaaagggcatctaccagaccagcaacttccgggtgcagcccaccgaatccatcgtgcggttccccaatatcaccaatctgtgccccttcggcgaggtgttcaatgccaccagattcgcctctgtgtacgcctggaaccggaagcggatcagcaattgcgtggccgactactccgtgctgtacaactccgccagcttcagcaccttcaagtgctacggcgtgtcccctaccaagctgaacgacctgtgcttcacaaacgtgtacgccgacagcttcgtgatccggggagatgaagtgcggcagattgcccctggacagacaggcaagatcgccgactacaactacaagctgcccgacgacttcaccggctgtgtgattgcctggaacagcaacaacctggactccaaagtcggcggcaactacaattacaggtaccggctgttccggaagtccaatctgaagcccttcgagcgggacatctccaccgagatctatcaggccggcagcaagccttgtaacggcgtggaaggcttcaactgctacttcccactgcagtcctacggctttcagcccacaaatggcgtgggctatcagccctacagagtggtggtgctgagcttcgaactgctgcatgcccctgccacagtgtgcggccctaagaaaagcaccaatctcgtgaagaacaaatgcgtgaacttcaacttcaacggcctgaccggcaccggcgtgctgacagagagcaacaagaagttcctgccattccagcagtttggccgggatatcgccgataccacagacgccgttagagatccccagacactggaaatcctggacatcaccccttgcagcttcggcggagtgtctgtgatcacccctggcaccaacaccagcaatcaggtggcagtgctgtaccagggcgtgaactgtaccgaagtgcccgtggccattcacgccgatcagctgacacctacatggcgggtgtactccaccggcagcaatgtgtttcagaccagagccggctgtctgatcggagccgagcacgtgaacaatagctacgagtgcgacatccccatcggcgctggaatctgcgccagctaccagacacagacaaacagcaggcggagagccagaagcgtggccagccagagcatcattgcctacacaatgtctctgggcgccgagaacagcgtggcctactccaacaactctatcgctatccccaccaacttcaccatcagcgtgaccacagagatcctgcctgtgtccatgaccaagaccagcgtggactgcaccatgtacatctgcggcgattccaccgagtgctccaacctgctgctgcagtacggcagcttctgcacccagctgaatagagccctgacagggatcgccgtggaacaggacaagaacacccaagaggtgttcgcccaagtgaagcagatctacaagacccctcctatcaaggacttcggcggcttcaatttcagccagattctgcccgatcctagcaagcccagcaagcggagcttcatcgaggacctgctgttcaacaaagtgacactggccgacgccggcttcatcaagcagtatggcgattgtctgggcgacattgccgccagggatctgatttgcgcccagaagtttaacggactgacagtgctgcctcctctgctgaccgatgagatgatcgcccagtacacatctgccctgctggccggcacaatcacaagcggctggacatttggagcaggcgccgctctgcagatcccctttgctatgcagatggcctaccggttcaacggcatcggagtgacccagaatgtgctgtacgagaaccagaagctgatcgccaaccagttcaacagcgccatcggcaagatccaggacagcctgagcagcacagcaagcgccctgggaaagctgcagaacgtggtcaaccagaatgcccaggcactgaacaccctggtcaagcagctgtcctccaacttcggcgccatcagctctgtgctgaacgatatcctgagcagactggaccctcctgaggccgaggtgcagatcgacagactgatcacaggcagactgcagagcctccagacatacgtgacccagcagctgatcagagccgccgagattagagcctctgccaatctggccgccaccaagatgtctgagtgtgtgctgggccagagcaagagagtggacttttgcggcaagggctaccacctgatgagcttccctcagtctgcccctcacggcgtggtgtttctgcacgtgacatatgtgcccgctcaagagaagaatttcaccaccgctccagccatctgccacgacggcaaagcccactttcctagagaaggcgtgttcgtgtccaacggcacccattggttcgtgacacagcggaacttctacgagccccagatcatcaccaccgacaacaccttcgtgtctggcaactgcgacgtcgtgatcggcattgtgaacaataccgtgtacgaccctctgcagcccgagctggacagcttcaaagaggaactggacaagtactttaagaaccacacaagccccgacgtggacctgggcgatatcagcggaatcaatgccagcgtcgtgaacatccagaaagagatcgaccggctgaacgaggtggccaagaatctgaacgagagcctgatcgacctgcaagaactggggaagtacgagcagtacatcaagtggccctggtacatctggctgggctttatcgccggactgattgccatcgtgatggtcacaatcatgctgtgttgcatgaccagctgctgtagctgcctgaagggctgttgtagctgtggcagctgctgcaagttcgacgaggacgattctgagcccgtgctgaagggcgtgaaactgcactacacatgatga

SEQ ID NO: 157 - RNA, 4277 nt, synthetic construct
  source 1..4277: mol_type = other RNA
agaataaactagtattcttctggtccccacagactcagagagaacccgccaccatgttcgtgttcctggtgctgctgcctctggtgtccagccagtgtgtgaacctgagaaccagaacacagctgcctccagcctacaccaacagctttaccagaggcgtgtactaccccgacaaggtgttcagatccagcgtgctgcactctacccaggacctgttcctgcctttcttcagcaacgtgacctggttccacgccatccacgtgtccggcaccaatggcaccaagagattcgacaaccccgtgctgcccttcaacgacggggtgtactttgccagcaccgagaagtccaacatcatcagaggctggatcttcggcaccacactggacagcaagacccagagcctgctgatcgtgaacaacgccaccaacgtggtcatcaaagtgtgcgagttccagttctgcaacgaccccttcctggacgtctactaccacaagaacaacaagagctggatggaaagcggcgtgtacagcagcgccaacaactgcaccttcgagtacgtgtcccagcctttcctgatggacctggaaggcaagcagggcaacttcaagaacctgcgcgagttcgtgtttaagaacatcgacggctacttcaagatctacagcaagcacacccctatcaacctcgtgcgggatctgcctcagggcttctctgctctggaacccctggtggatctgcccatcggcatcaacatcacccggtttcagacactgctggccctgcacagaagctacctgacacctggcgatagcagcagcggatggacagctggtgccgccgcttactatgtgggctacctgcagcctagaaccttcctgctgaagtacaacgagaacggcaccatcaccgacgccgtggattgtgctctggatcctctgagcgagacaaagtgcaccctgaagtccttcaccgtggaaaagggcatctaccagaccagcaacttccgggtgcagcccaccgaatccatcgtgcggttccccaatatcaccaatctgtgccccttcggcgaggtgttcaatgccaccagattcgcctctgtgtacgcctggaaccggaagcggatcagcaattgcgtggccgactactccgtgctgtacaactccgccagcttcagcaccttcaagtgctacggcgtgtcccctaccaagctgaacgacctgtgcttcacaaacgtgtacgccgacagcttcgtgatccggggagatgaagtgcggcagattgcccctggacagacaggcaagatcgccgactacaactacaagctgcccgacgacttcaccggctgtgtgattgcctggaacagcaacaacctggactccaaagtcggcggcaactacaattacaggtaccggctgttccggaagtccaatctgaagcccttcgagcgggacatctccaccgagatctatcaggccggcagcaagccttgtaacggcgtggaaggcttcaactgctacttcccactgcagtcctacggctttcagcccacaaatggcgtgggctatcagccctacagagtggtggtgctgagcttcgaactgctgcatgcccctgccacagtgtgcggccctaagaaaagcaccaatctcgtgaagaacaaatgcgtgaacttcaacttcaacggcctgaccggcaccggcgtgctgacagagagcaacaagaagttcctgccattccagcagtttggccgggatatcgccgataccacagacgccgttagagatccccagacactggaaatcctggacatcaccccttgcagcttcggcggagtgtctgtgatcacccctggcaccaacaccagcaatcaggtggcagtgctgtaccagggcgtgaactgtaccgaagtgcccgtggccattcacgccgatcagctgacacctacatggcgggtgtactccaccggcagcaatgtgtttcagaccagagccggctgtctgatcggagccgagcacgtgaacaatagctacgagtgcgacatccccatcggcgctggaatctgcgccagctaccagacacagacaaacagcaggcggagagccagaagcgtggccagccagagcatcattgcctacacaatgtctctgggcgccgagaacagcgtggcctactccaacaactctatcgctatccccaccaacttcaccatcagcgtgaccacagagatcctgcctgtgtccatgaccaagaccagcgtggactgcaccatgtacatctgcggcgattccaccgagtgctccaacctgctgctgcagtacggcagcttctgcacccagctgaatagagccctgacagggatcgccgtggaacaggacaagaacacccaagaggtgttcgcccaagtgaagcagatctacaagacccctcctatcaaggacttcggcggcttcaatttcagccagattctgcccgatcctagcaagcccagcaagcggagcttcatcgaggacctgctgttcaacaaagtgacactggccgacgccggcttcatcaagcagtatggcgattgtctgggcgacattgccgccagggatctgatttgcgcccagaagtttaacggactgacagtgctgcctcctctgctgaccgatgagatgatcgcccagtacacatctgccctgctggccggcacaatcacaagcggctggacatttggagcaggcgccgctctgcagatcccctttgctatgcagatggcctaccggttcaacggcatcggagtgacccagaatgtgctgtacgagaaccagaagctgatcgccaaccagttcaacagcgccatcggcaagatccaggacagcctgagcagcacagcaagcgccctgggaaagctgcagaacgtggtcaaccagaatgcccaggcactgaacaccctggtcaagcagctgtcctccaacttcggcgccatcagctctgtgctgaacgatatcctgagcagactggaccctcctgaggccgaggtgcagatcgacagactgatcacaggcagactgcagagcctccagacatacgtgacccagcagctgatcagagccgccgagattagagcctctgccaatctggccgccaccaagatgtctgagtgtgtgctgggccagagcaagagagtggacttttgcggcaagggctaccacctgatgagcttccctcagtctgcccctcacggcgtggtgtttctgcacgtgacatatgtgcccgctcaagagaagaatttcaccaccgctccagccatctgccacgacggcaaagcccactttcctagagaaggcgtgttcgtgtccaacggcacccattggttcgtgacacagcggaacttctacgagccccagatcatcaccaccgacaacaccttcgtgtctggcaactgcgacgtcgtgatcggcattgtgaacaataccgtgtacgaccctctgcagcccgagctggacagcttcaaagaggaactggacaagtactttaagaaccacacaagccccgacgtggacctgggcgatatcagcggaatcaatgccagcgtcgtgaacatccagaaagagatcgaccggctgaacgaggtggccaagaatctgaacgagagcctgatcgacctgcaagaactggggaagtacgagcagtacatcaagtggccctggtacatctggctgggctttatcgccggactgattgccatcgtgatggtcacaatcatgctgtgttgcatgaccagctgctgtagctgcctgaagggctgttgtagctgtggcagctgctgcaagttcgacgaggacgattctgagcccgtgctgaagggcgtgaaactgcactacacatgatgatttcacctggtactgcatgcacgcaatgctagctgcccctttcccgtcctgggtaccccgagtctcccccgacctcgggtcccaggtatgctcccacctccacctgccccactcaccacctctgctagttccagacacctcccaagcacgcagcaatgcagctcaaaacgcttagcctagccacacccccacgggaaacagcagtgattaacctttagcaataaacgaaagtttaactaagctatactaaccccagggttggtcaatttcgtgccagccacaccctggagctagcaaaaaaaaaaaaaaaaaaaaaaaaaaaaaagcatatgactaaaaaaaaaaaaaaaaaaaaaaaaaaaaaaaaaaaaaaaaaaaaaaaaaaaaaaaaaaaaaaaaaaaaaa

SEQ ID NO: 158 - protein, 1269 aa, synthetic construct
MFVFLVLLPLVSSQCVNLITRTQSYTNSFTRGVYYPDKVFRSSVLHSTQDLFLPFFSNVTWFHAIHVSGTNGTKRFDNPALPFNDGVYFASTEKSNIIRGWIFGTTLDSKTQSLLIVNNATNVVIKVCEFQFCNDPFLDVYQKNNKSWMESEFRVYSSANNCTFEYVSQPFLMDLEGKEGNFKNLREFVFKNIDGYFKIYSKHTPINLERDLPQGFSALEPLVDLPIGINITRFQTLLALHRSYLTPVDSSSGWTAGAAAYYVGYLQPRTFLLKYNENGTITDAVDCALDPLSETKCTLKSFTVEKGIYQTSNFRVQPTESIVRFPNITNLCPFHEVFNATTFASVYAWNRKRISNCVADYSVIYNFAPFFAFKCYGVSPTKLNDLCFTNVYADSFVIRGNEVSQIAPGQTGNIADYNYKLPDDFTGCVIAWNSNKLDSKPSGNYNYLYRLFRKSKLKPFERDISTEIYQAGNKPCNGVAGPNCYSPLQSYGFRPTYGVGHQPYRVVVLSFELLHAPATVCGPKKSTNLVKNKCVNFNFNGLTGTGVLTESNKKFLPFQQFGRDIADTTDAVRDPQTLEILDITPCSFGGVSVITPGTNTSNQVAVLYQGVNCTEVPVAIHADQLTPTWRVYSTGSNVFQTRAGCLIGAEYVNNSYECDIPIGAGICASYQTQTKSHRRARSVASQSIIAYTMSLGAENSVAYSNNSIAIPTNFTISVTTEILPVSMTKTSVDCTMYICGDSTECSNLLLQYGSFCTQLKRALTGIAVEQDKNTQEVFAQVKQIYKTPPIKYFGGFNFSQILPDPSKPSKRSFIEDLLFNKVTLADAGFIKQYGDCLGDIAARDLICAQKFNGLTVLPPLLTDEMIAQYTSALLAGTITSGWTFGAGAALQIPFAMQMAYRFNGIGVTQNVLYENQKLIANQFNSAIGKIQDSLSSTASALGKLQDVVNHNAQALNTLVKQLSSKFGAISSVLNDILSRLDPPEAEVQIDRLITGRLQSLQTYVTQQLIRAAEIRASANLAATKMSECVLGQSKRVDFCGKGYHLMSFPQSAPHGVVFLHVTYVPAQEKNFTTAPAICHDGKAHFPREGVFVSNGTHWFVTQRNFYEPQIITTDNTFVSGNCDVVIGIVNNTVYDPLQPELDSFKEELDKYFKNHTSPDVDLGDISGINASVVNIQKEIDRLNEVAKNLNESLIDLQELGKYEQYIKWPWYIWLGFIAGLIAIVMVTIMLCCMTSCCSCLKGCCSCGSCCKFDEDDSEPVLKGVKLHYT

SEQ ID NO: 159 - RNA, 3813 nt, synthetic construct
  source 1..3813: mol_type = other RNA
atgttcgtgttcctggtgctgctgcctctggtgtccagccagtgtgtgaacctgatcaccagaacacagtcatacaccaacagctttaccagaggcgtgtactaccccgacaaggtgttcagatccagcgtgctgcactctacccaggacctgttcctgcctttcttcagcaacgtgacctggttccacgccatccacgtgtccggcaccaatggcaccaagagattcgacaaccccgccctgcccttcaacgacggggtgtactttgccagcaccgagaagtccaacatcatcagaggctggatcttcggcaccacactggacagcaagacccagagcctgctgatcgtgaacaacgccaccaacgtggtcatcaaagtgtgcgagttccagttctgcaacgaccccttcctggacgtctaccagaagaacaacaagagctggatggaaagcgagttccgggtgtacagcagcgccaacaactgcaccttcgagtacgtgtcccagcctttcctgatggacctggaaggcaaggagggcaacttcaagaacctgcgcgagttcgtgtttaagaacatcgacggctacttcaagatctacagcaagcacacccctatcaacctcgagcgggatctgcctcagggcttctctgctctggaacccctggtggatctgcccatcggcatcaacatcacccggtttcagacactgctggccctgcacagaagctacctgacacctgtggatagcagcagcggatggacagctggtgccgccgcttactatgtgggctacctgcagcctagaaccttcctgctgaagtacaacgagaacggcaccatcaccgacgccgtggattgtgctctggatcctctgagcgagacaaagtgcaccctgaagtccttcaccgtggaaaagggcatctaccagaccagcaacttccgggtgcagcccaccgaatccatcgtgcggttccccaatatcaccaatctgtgccccttccacgaggtgttcaatgccaccaccttcgcctctgtgtacgcctggaaccggaagcggatcagcaattgcgtggccgactactccgtgatctacaacttcgcccccttcttcgcattcaagtgctacggcgtgtcccctaccaagctgaacgacctgtgcttcacaaacgtgtacgccgacagcttcgtgatccggggaaacgaagtgtcacagattgcccctggacagacaggcaacatcgccgactacaactacaagctgcccgacgacttcaccggctgtgtgattgcctggaacagcaacaagctggactccaaacccagcggcaactacaattacctgtaccggctgttccggaagtccaagctgaagcccttcgagcgggacatctccaccgagatctatcaggccggcaacaagccttgtaacggcgtggcaggccccaactgctacagcccactgcagtcctacggctttaggcccacatacggcgtgggccaccagccctacagagtggtggtgctgagcttcgaactgctgcatgcccctgccacagtgtgcggccctaagaaaagcaccaatctcgtgaagaacaaatgcgtgaacttcaacttcaacggcctgaccggcaccggcgtgctgacagagagcaacaagaagttcctgccattccagcagtttggccgggatatcgccgataccacagacgccgttagagatccccagacactggaaatcctggacatcaccccttgcagcttcggcggagtgtctgtgatcacccctggcaccaacaccagcaatcaggtggcagtgctgtaccagggcgtgaactgtaccgaagtgcccgtggccattcacgccgatcagctgacacctacatggcgggtgtactccaccggcagcaatgtgtttcagaccagagccggctgtctgatcggagccgagtacgtgaacaatagctacgagtgcgacatccccatcggcgctggaatctgcgccagctaccagacacagacaaagagccaccggagagccagaagcgtggccagccagagcatcattgcctacacaatgtctctgggcgccgagaacagcgtggcctactccaacaactctatcgctatccccaccaacttcaccatcagcgtgaccacagagatcctgcctgtgtccatgaccaagaccagcgtggactgcaccatgtacatctgcggcgattccaccgagtgctccaacctgctgctgcagtacggcagcttctgcacccagctgaaaagagccctgacagggatcgccgtggaacaggacaagaacacccaagaggtgttcgcccaagtgaagcagatctacaagacccctcctatcaagtacttcggcggcttcaatttcagccagattctgcccgatcctagcaagcccagcaagcggagcttcatcgaggacctgctgttcaacaaagtgacactggccgacgccggcttcatcaagcagtatggcgattgtctgggcgacattgccgccagggatctgatttgcgcccagaagtttaacggactgacagtgctgcctcctctgctgaccgatgagatgatcgcccagtacacatctgccctgctggccggcacaatcacaagcggctggacatttggagcaggcgccgctctgcagatcccctttgctatgcagatggcctaccggttcaacggcatcggagtgacccagaatgtgctgtacgagaaccagaagctgatcgccaaccagttcaacagcgccatcggcaagatccaggacagcctgagcagcacagcaagcgccctgggaaagctgcaggacgtggtcaaccacaatgcccaggcactgaacaccctggtcaagcagctgtcctccaagttcggcgccatcagctctgtgctgaacgatatcctgagcagactggaccctcctgaggccgaggtgcagatcgacagactgatcacaggcagactgcagagcctccagacatacgtgacccagcagctgatcagagccgccgagattagagcctctgccaatctggccgccaccaagatgtctgagtgtgtgctgggccagagcaagagagtggacttttgcggcaagggctaccacctgatgagcttccctcagtctgcccctcacggcgtggtgtttctgcacgtgacatatgtgcccgctcaagagaagaatttcaccaccgctccagccatctgccacgacggcaaagcccactttcctagagaaggcgtgttcgtgtccaacggcacccattggttcgtgacacagcggaacttctacgagccccagatcatcaccaccgacaacaccttcgtgtctggcaactgcgacgtcgtgatcggcattgtgaacaataccgtgtacgaccctctgcagcccgagctggacagcttcaaagaggaactggacaagtactttaagaaccacacaagccccgacgtggacctgggcgatatcagcggaatcaatgccagcgtcgtgaacatccagaaagagatcgaccggctgaacgaggtggccaagaatctgaacgagagcctgatcgacctgcaagaactggggaagtacgagcagtacatcaagtggccctggtacatctggctgggctttatcgccggactgattgccatcgtgatggtcacaatcatgctgtgttgcatgaccagctgctgtagctgcctgaagggctgttgtagctgtggcagctgctgcaagttcgacgaggacgattctgagcccgtgctgaagggcgtgaaactgcactacacatgatga

SEQ ID NO: 160 - DNA, 3813 bp, synthetic construct
  source 1..3813: mol_type = other DNA
atgttcgtgttcctggtgctgctgcctctggtgtccagccagtgtgtgaacctgatcaccagaacacagtcatacaccaacagctttaccagaggcgtgtactaccccgacaaggtgttcagatccagcgtgctgcactctacccaggacctgttcctgcctttcttcagcaacgtgacctggttccacgccatccacgtgtccggcaccaatggcaccaagagattcgacaaccccgccctgcccttcaacgacggggtgtactttgccagcaccgagaagtccaacatcatcagaggctggatcttcggcaccacactggacagcaagacccagagcctgctgatcgtgaacaacgccaccaacgtggtcatcaaagtgtgcgagttccagttctgcaacgaccccttcctggacgtctaccagaagaacaacaagagctggatggaaagcgagttccgggtgtacagcagcgccaacaactgcaccttcgagtacgtgtcccagcctttcctgatggacctggaaggcaaggagggcaacttcaagaacctgcgcgagttcgtgtttaagaacatcgacggctacttcaagatctacagcaagcacacccctatcaacctcgagcgggatctgcctcagggcttctctgctctggaacccctggtggatctgcccatcggcatcaacatcacccggtttcagacactgctggccctgcacagaagctacctgacacctgtggatagcagcagcggatggacagctggtgccgccgcttactatgtgggctacctgcagcctagaaccttcctgctgaagtacaacgagaacggcaccatcaccgacgccgtggattgtgctctggatcctctgagcgagacaaagtgcaccctgaagtccttcaccgtggaaaagggcatctaccagaccagcaacttccgggtgcagcccaccgaatccatcgtgcggttccccaatatcaccaatctgtgccccttccacgaggtgttcaatgccaccaccttcgcctctgtgtacgcctggaaccggaagcggatcagcaattgcgtggccgactactccgtgatctacaacttcgcccccttcttcgcattcaagtgctacggcgtgtcccctaccaagctgaacgacctgtgcttcacaaacgtgtacgccgacagcttcgtgatccggggaaacgaagtgtcacagattgcccctggacagacaggcaacatcgccgactacaactacaagctgcccgacgacttcaccggctgtgtgattgcctggaacagcaacaagctggactccaaacccagcggcaactacaattacctgtaccggctgttccggaagtccaagctgaagcccttcgagcgggacatctccaccgagatctatcaggccggcaacaagccttgtaacggcgtggcaggccccaactgctacagcccactgcagtcctacggctttaggcccacatacggcgtgggccaccagccctacagagtggtggtgctgagcttcgaactgctgcatgcccctgccacagtgtgcggccctaagaaaagcaccaatctcgtgaagaacaaatgcgtgaacttcaacttcaacggcctgaccggcaccggcgtgctgacagagagcaacaagaagttcctgccattccagcagtttggccgggatatcgccgataccacagacgccgttagagatccccagacactggaaatcctggacatcaccccttgcagcttcggcggagtgtctgtgatcacccctggcaccaacaccagcaatcaggtggcagtgctgtaccagggcgtgaactgtaccgaagtgcccgtggccattcacgccgatcagctgacacctacatggcgggtgtactccaccggcagcaatgtgtttcagaccagagccggctgtctgatcggagccgagtacgtgaacaatagctacgagtgcgacatccccatcggcgctggaatctgcgccagctaccagacacagacaaagagccaccggagagccagaagcgtggccagccagagcatcattgcctacacaatgtctctgggcgccgagaacagcgtggcctactccaacaactctatcgctatccccaccaacttcaccatcagcgtgaccacagagatcctgcctgtgtccatgaccaagaccagcgtggactgcaccatgtacatctgcggcgattccaccgagtgctccaacctgctgctgcagtacggcagcttctgcacccagctgaaaagagccctgacagggatcgccgtggaacaggacaagaacacccaagaggtgttcgcccaagtgaagcagatctacaagacccctcctatcaagtacttcggcggcttcaatttcagccagattctgcccgatcctagcaagcccagcaagcggagcttcatcgaggacctgctgttcaacaaagtgacactggccgacgccggcttcatcaagcagtatggcgattgtctgggcgacattgccgccagggatctgatttgcgcccagaagtttaacggactgacagtgctgcctcctctgctgaccgatgagatgatcgcccagtacacatctgccctgctggccggcacaatcacaagcggctggacatttggagcaggcgccgctctgcagatcccctttgctatgcagatggcctaccggttcaacggcatcggagtgacccagaatgtgctgtacgagaaccagaagctgatcgccaaccagttcaacagcgccatcggcaagatccaggacagcctgagcagcacagcaagcgccctgggaaagctgcaggacgtggtcaaccacaatgcccaggcactgaacaccctggtcaagcagctgtcctccaagttcggcgccatcagctctgtgctgaacgatatcctgagcagactggaccctcctgaggccgaggtgcagatcgacagactgatcacaggcagactgcagagcctccagacatacgtgacccagcagctgatcagagccgccgagattagagcctctgccaatctggccgccaccaagatgtctgagtgtgtgctgggccagagcaagagagtggacttttgcggcaagggctaccacctgatgagcttccctcagtctgcccctcacggcgtggtgtttctgcacgtgacatatgtgcccgctcaagagaagaatttcaccaccgctccagccatctgccacgacggcaaagcccactttcctagagaaggcgtgttcgtgtccaacggcacccattggttcgtgacacagcggaacttctacgagccccagatcatcaccaccgacaacaccttcgtgtctggcaactgcgacgtcgtgatcggcattgtgaacaataccgtgtacgaccctctgcagcccgagctggacagcttcaaagaggaactggacaagtactttaagaaccacacaagccccgacgtggacctgggcgatatcagcggaatcaatgccagcgtcgtgaacatccagaaagagatcgaccggctgaacgaggtggccaagaatctgaacgagagcctgatcgacctgcaagaactggggaagtacgagcagtacatcaagtggccctggtacatctggctgggctttatcgccggactgattgccatcgtgatggtcacaatcatgctgtgttgcatgaccagctgctgtagctgcctgaagggctgttgtagctgtggcagctgctgcaagttcgacgaggacgattctgagcccgtgctgaagggcgtgaaactgcactacacatgatga

SEQ ID NO: 161 - RNA, 4270 nt, synthetic construct
  source 1..4270: mol_type = other RNA
agaataaactagtattcttctggtccccacagactcagagagaacccgccaccatgttcgtgttcctggtgctgctgcctctggtgtccagccagtgtgtgaacctgatcaccagaacacagtcatacaccaacagctttaccagaggcgtgtactaccccgacaaggtgttcagatccagcgtgctgcactctacccaggacctgttcctgcctttcttcagcaacgtgacctggttccacgccatccacgtgtccggcaccaatggcaccaagagattcgacaaccccgccctgcccttcaacgacggggtgtactttgccagcaccgagaagtccaacatcatcagaggctggatcttcggcaccacactggacagcaagacccagagcctgctgatcgtgaacaacgccaccaacgtggtcatcaaagtgtgcgagttccagttctgcaacgaccccttcctggacgtctaccagaagaacaacaagagctggatggaaagcgagttccgggtgtacagcagcgccaacaactgcaccttcgagtacgtgtcccagcctttcctgatggacctggaaggcaaggagggcaacttcaagaacctgcgcgagttcgtgtttaagaacatcgacggctacttcaagatctacagcaagcacacccctatcaacctcgagcgggatctgcctcagggcttctctgctctggaacccctggtggatctgcccatcggcatcaacatcacccggtttcagacactgctggccctgcacagaagctacctgacacctgtggatagcagcagcggatggacagctggtgccgccgcttactatgtgggctacctgcagcctagaaccttcctgctgaagtacaacgagaacggcaccatcaccgacgccgtggattgtgctctggatcctctgagcgagacaaagtgcaccctgaagtccttcaccgtggaaaagggcatctaccagaccagcaacttccgggtgcagcccaccgaatccatcgtgcggttccccaatatcaccaatctgtgccccttccacgaggtgttcaatgccaccaccttcgcctctgtgtacgcctggaaccggaagcggatcagcaattgcgtggccgactactccgtgatctacaacttcgcccccttcttcgcattcaagtgctacggcgtgtcccctaccaagctgaacgacctgtgcttcacaaacgtgtacgccgacagcttcgtgatccggggaaacgaagtgtcacagattgcccctggacagacaggcaacatcgccgactacaactacaagctgcccgacgacttcaccggctgtgtgattgcctggaacagcaacaagctggactccaaacccagcggcaactacaattacctgtaccggctgttccggaagtccaagctgaagcccttcgagcgggacatctccaccgagatctatcaggccggcaacaagccttgtaacggcgtggcaggccccaactgctacagcccactgcagtcctacggctttaggcccacatacggcgtgggccaccagccctacagagtggtggtgctgagcttcgaactgctgcatgcccctgccacagtgtgcggccctaagaaaagcaccaatctcgtgaagaacaaatgcgtgaacttcaacttcaacggcctgaccggcaccggcgtgctgacagagagcaacaagaagttcctgccattccagcagtttggccgggatatcgccgataccacagacgccgttagagatccccagacactggaaatcctggacatcaccccttgcagcttcggcggagtgtctgtgatcacccctggcaccaacaccagcaatcaggtggcagtgctgtaccagggcgtgaactgtaccgaagtgcccgtggccattcacgccgatcagctgacacctacatggcgggtgtactccaccggcagcaatgtgtttcagaccagagccggctgtctgatcggagccgagtacgtgaacaatagctacgagtgcgacatccccatcggcgctggaatctgcgccagctaccagacacagacaaagagccaccggagagccagaagcgtggccagccagagcatcattgcctacacaatgtctctgggcgccgagaacagcgtggcctactccaacaactctatcgctatccccaccaacttcaccatcagcgtgaccacagagatcctgcctgtgtccatgaccaagaccagcgtggactgcaccatgtacatctgcggcgattccaccgagtgctccaacctgctgctgcagtacggcagcttctgcacccagctgaaaagagccctgacagggatcgccgtggaacaggacaagaacacccaagaggtgttcgcccaagtgaagcagatctacaagacccctcctatcaagtacttcggcggcttcaatttcagccagattctgcccgatcctagcaagcccagcaagcggagcttcatcgaggacctgctgttcaacaaagtgacactggccgacgccggcttcatcaagcagtatggcgattgtctgggcgacattgccgccagggatctgatttgcgcccagaagtttaacggactgacagtgctgcctcctctgctgaccgatgagatgatcgcccagtacacatctgccctgctggccggcacaatcacaagcggctggacatttggagcaggcgccgctctgcagatcccctttgctatgcagatggcctaccggttcaacggcatcggagtgacccagaatgtgctgtacgagaaccagaagctgatcgccaaccagttcaacagcgccatcggcaagatccaggacagcctgagcagcacagcaagcgccctgggaaagctgcaggacgtggtcaaccacaatgcccaggcactgaacaccctggtcaagcagctgtcctccaagttcggcgccatcagctctgtgctgaacgatatcctgagcagactggaccctcctgaggccgaggtgcagatcgacagactgatcacaggcagactgcagagcctccagacatacgtgacccagcagctgatcagagccgccgagattagagcctctgccaatctggccgccaccaagatgtctgagtgtgtgctgggccagagcaagagagtggacttttgcggcaagggctaccacctgatgagcttccctcagtctgcccctcacggcgtggtgtttctgcacgtgacatatgtgcccgctcaagagaagaatttcaccaccgctccagccatctgccacgacggcaaagcccactttcctagagaaggcgtgttcgtgtccaacggcacccattggttcgtgacacagcggaacttctacgagccccagatcatcaccaccgacaacaccttcgtgtctggcaactgcgacgtcgtgatcggcattgtgaacaataccgtgtacgaccctctgcagcccgagctggacagcttcaaagaggaactggacaagtactttaagaaccacacaagccccgacgtggacctgggcgatatcagcggaatcaatgccagcgtcgtgaacatccagaaagagatcgaccggctgaacgaggtggccaagaatctgaacgagagcctgatcgacctgcaagaactggggaagtacgagcagtacatcaagtggccctggtacatctggctgggctttatcgccggactgattgccatcgtgatggtcacaatcatgctgtgttgcatgaccagctgctgtagctgcctgaagggctgttgtagctgtggcagctgctgcaagttcgacgaggacgattctgagcccgtgctgaagggcgtgaaactgcactacacatgatgactcgagctggtactgcatgcacgcaatgctagctgcccctttcccgtcctgggtaccccgagtctcccccgacctcgggtcccaggtatgctcccacctccacctgccccactcaccacctctgctagttccagacacctcccaagcacgcagcaatgcagctcaaaacgcttagcctagccacacccccacgggaaacagcagtgattaacctttagcaataaacgaaagtttaactaagctatactaaccccagggttggtcaatttcgtgccagccacaccctggagctagcaaaaaaaaaaaaaaaaaaaaaaaaaaaaaagcatatgactaaaaaaaaaaaaaaaaaaaaaaaaaaaaaaaaaaaaaaaaaaaaaaaaaaaaaaaaaaaaaaaaaaaaa

SEQ ID NO: 162 - DNA, 4270 bp, synthetic construct
  source 1..4270: mol_type = other DNA
agaataaactagtattcttctggtccccacagactcagagagaacccgccaccatgttcgtgttcctggtgctgctgcctctggtgtccagccagtgtgtgaacctgatcaccagaacacagtcatacaccaacagctttaccagaggcgtgtactaccccgacaaggtgttcagatccagcgtgctgcactctacccaggacctgttcctgcctttcttcagcaacgtgacctggttccacgccatccacgtgtccggcaccaatggcaccaagagattcgacaaccccgccctgcccttcaacgacggggtgtactttgccagcaccgagaagtccaacatcatcagaggctggatcttcggcaccacactggacagcaagacccagagcctgctgatcgtgaacaacgccaccaacgtggtcatcaaagtgtgcgagttccagttctgcaacgaccccttcctggacgtctaccagaagaacaacaagagctggatggaaagcgagttccgggtgtacagcagcgccaacaactgcaccttcgagtacgtgtcccagcctttcctgatggacctggaaggcaaggagggcaacttcaagaacctgcgcgagttcgtgtttaagaacatcgacggctacttcaagatctacagcaagcacacccctatcaacctcgagcgggatctgcctcagggcttctctgctctggaacccctggtggatctgcccatcggcatcaacatcacccggtttcagacactgctggccctgcacagaagctacctgacacctgtggatagcagcagcggatggacagctggtgccgccgcttactatgtgggctacctgcagcctagaaccttcctgctgaagtacaacgagaacggcaccatcaccgacgccgtggattgtgctctggatcctctgagcgagacaaagtgcaccctgaagtccttcaccgtggaaaagggcatctaccagaccagcaacttccgggtgcagcccaccgaatccatcgtgcggttccccaatatcaccaatctgtgccccttccacgaggtgttcaatgccaccaccttcgcctctgtgtacgcctggaaccggaagcggatcagcaattgcgtggccgactactccgtgatctacaacttcgcccccttcttcgcattcaagtgctacggcgtgtcccctaccaagctgaacgacctgtgcttcacaaacgtgtacgccgacagcttcgtgatccggggaaacgaagtgtcacagattgcccctggacagacaggcaacatcgccgactacaactacaagctgcccgacgacttcaccggctgtgtgattgcctggaacagcaacaagctggactccaaacccagcggcaactacaattacctgtaccggctgttccggaagtccaagctgaagcccttcgagcgggacatctccaccgagatctatcaggccggcaacaagccttgtaacggcgtggcaggccccaactgctacagcccactgcagtcctacggctttaggcccacatacggcgtgggccaccagccctacagagtggtggtgctgagcttcgaactgctgcatgcccctgccacagtgtgcggccctaagaaaagcaccaatctcgtgaagaacaaatgcgtgaacttcaacttcaacggcctgaccggcaccggcgtgctgacagagagcaacaagaagttcctgccattccagcagtttggccgggatatcgccgataccacagacgccgttagagatccccagacactggaaatcctggacatcaccccttgcagcttcggcggagtgtctgtgatcacccctggcaccaacaccagcaatcaggtggcagtgctgtaccagggcgtgaactgtaccgaagtgcccgtggccattcacgccgatcagctgacacctacatggcgggtgtactccaccggcagcaatgtgtttcagaccagagccggctgtctgatcggagccgagtacgtgaacaatagctacgagtgcgacatccccatcggcgctggaatctgcgccagctaccagacacagacaaagagccaccggagagccagaagcgtggccagccagagcatcattgcctacacaatgtctctgggcgccgagaacagcgtggcctactccaacaactctatcgctatccccaccaacttcaccatcagcgtgaccacagagatcctgcctgtgtccatgaccaagaccagcgtggactgcaccatgtacatctgcggcgattccaccgagtgctccaacctgctgctgcagtacggcagcttctgcacccagctgaaaagagccctgacagggatcgccgtggaacaggacaagaacacccaagaggtgttcgcccaagtgaagcagatctacaagacccctcctatcaagtacttcggcggcttcaatttcagccagattctgcccgatcctagcaagcccagcaagcggagcttcatcgaggacctgctgttcaacaaagtgacactggccgacgccggcttcatcaagcagtatggcgattgtctgggcgacattgccgccagggatctgatttgcgcccagaagtttaacggactgacagtgctgcctcctctgctgaccgatgagatgatcgcccagtacacatctgccctgctggccggcacaatcacaagcggctggacatttggagcaggcgccgctctgcagatcccctttgctatgcagatggcctaccggttcaacggcatcggagtgacccagaatgtgctgtacgagaaccagaagctgatcgccaaccagttcaacagcgccatcggcaagatccaggacagcctgagcagcacagcaagcgccctgggaaagctgcaggacgtggtcaaccacaatgcccaggcactgaacaccctggtcaagcagctgtcctccaagttcggcgccatcagctctgtgctgaacgatatcctgagcagactggaccctcctgaggccgaggtgcagatcgacagactgatcacaggcagactgcagagcctccagacatacgtgacccagcagctgatcagagccgccgagattagagcctctgccaatctggccgccaccaagatgtctgagtgtgtgctgggccagagcaagagagtggacttttgcggcaagggctaccacctgatgagcttccctcagtctgcccctcacggcgtggtgtttctgcacgtgacatatgtgcccgctcaagagaagaatttcaccaccgctccagccatctgccacgacggcaaagcccactttcctagagaaggcgtgttcgtgtccaacggcacccattggttcgtgacacagcggaacttctacgagccccagatcatcaccaccgacaacaccttcgtgtctggcaactgcgacgtcgtgatcggcattgtgaacaataccgtgtacgaccctctgcagcccgagctggacagcttcaaagaggaactggacaagtactttaagaaccacacaagccccgacgtggacctgggcgatatcagcggaatcaatgccagcgtcgtgaacatccagaaagagatcgaccggctgaacgaggtggccaagaatctgaacgagagcctgatcgacctgcaagaactggggaagtacgagcagtacatcaagtggccctggtacatctggctgggctttatcgccggactgattgccatcgtgatggtcacaatcatgctgtgttgcatgaccagctgctgtagctgcctgaagggctgttgtagctgtggcagctgctgcaagttcgacgaggacgattctgagcccgtgctgaagggcgtgaaactgcactacacatgatgactcgagctggtactgcatgcacgcaatgctagctgcccctttcccgtcctgggtaccccgagtctcccccgacctcgggtcccaggtatgctcccacctccacctgccccactcaccacctctgctagttccagacacctcccaagcacgcagcaatgcagctcaaaacgcttagcctagccacacccccacgggaaacagcagtgattaacctttagcaataaacgaaagtttaactaagctatactaaccccagggttggtcaatttcgtgccagccacaccctggagctagcaaaaaaaaaaaaaaaaaaaaaaaaaaaaaagcatatgactaaaaaaaaaaaaaaaaaaaaaaaaaaaaaaaaaaaaaaaaaaaaaaaaaaaaaaaaaaaaaaaaaaaaa

SEQ ID NO: 163 - protein, 1269 aa, synthetic construct
MFVFLVLLPLVSSQCVNLITRTQSYTNSFTRGVYYPDKVFRSSVLHSTQDLFLPFFSNVTWFHAIHVSGTNGTKRFDNPALPFNDGVYFASTEKSNIIRGWIFGTTLDSKTQSLLIVNNATNVVIKVCEFQFCNDPFLDVYQKNNKSWMESEFRVYSSANNCTFEYVSQPFLMDLVGKEGNFKNLREFVFKNIDGYFKIYSKHTPINLERDLPQGFSALEPLVDLPIGINITRFQTLLALHRSYLTPVDSSSGWTAGAAAYYVGYLQPRTFLLKYNENGTITDAVDCALDPLSETKCTLKSFTVEKGIYQTSNFRVQPTESIVRFPNITNLCPFHEVFNATTFASVYAWNRKRISNCVADYSVIYNFAPFFAFKCYGVSPTKLNDLCFTNVYADSFVIRGNEVSQIAPGQTGNIADYNYKLPDDFTGCVIAWNSNKLDSKPSGNYNYLYRLFRKSKLKPFERDISTEIYQAGNRPCNGVAGPNCYSPLQSYGFRPTYGVGHQPYRVVVLSFELLHAPATVCGPKKSTNLVKNKCVNFNFNGLTGTGVLTESNKKFLPFQQFGRDIADTTDAVRDPQTLEILDITPCSFGGVSVITPGTNTSNQVAVLYQGVNCTEVPVAIHADQLTPTWRVYSTGSNVFQTRAGCLIGAEYVNNSYECDIPIGAGICASYQTQTKSHRRARSVASQSIIAYTMSLGAENSVAYSNNSIAIPTNFTISVTTEILPVSMTKTSVDCTMYICGDSTECSNLLLQYGSFCTQLKRALTGIAVEQDKNTQEVFAQVKQIYKTPPIKYFGGFNFSQILPDPSKPSKRSFIEDLLFNKVTLADAGFIKQYGDCLGDIAARDLICAQKFNGLTVLPPLLTDEMIAQYTSALLAGTITSGWTFGAGAALQIPFAMQMAYRFNGIGVTQNVLYENQKLIANQFNSAIGKIQDSLSSTASALGKLQDVVNHNAQALNTLVKQLSSKFGAISSVLNDILSRLDPPEAEVQIDRLITGRLQSLQTYVTQQLIRAAEIRASANLAATKMSECVLGQSKRVDFCGKGYHLMSFPQSAPHGVVFLHVTYVPAQEKNFTTAPAICHDGKAHFPREGVFVSNGTHWFVTQRNFYEPQIITTDNTFVSGNCDVVIGIVNNTVYDPLQPELDSFKEELDKYFKNHTSPDVDLGDISGINASVVNIQKEIDRLNEVAKNLNESLIDLQELGKYEQYIKWPWYIWLGFIAGLIAIVMVTIMLCCMTSCCSCLKGCCSCGSCCKFDEDDSEPVLKGVKLHYT

SEQ ID NO: 164 - RNA, 3813 nt, synthetic construct
  source 1..3813: mol_type = other RNA
atgttcgtgttcctggtgctgctgcctctggtgtccagccagtgtgtgaacctgatcaccagaacacagtcatacaccaacagctttaccagaggcgtgtactaccccgacaaggtgttcagatccagcgtgctgcactctacccaggacctgttcctgcctttcttcagcaacgtgacctggttccacgccatccacgtgtccggcaccaatggcaccaagagattcgacaaccccgccctgcccttcaacgacggggtgtactttgccagcaccgagaagtccaacatcatcagaggctggatcttcggcaccacactggacagcaagacccagagcctgctgatcgtgaacaacgccaccaacgtggtcatcaaagtgtgcgagttccagttctgcaacgaccccttcctggacgtctaccagaagaacaacaagagctggatggaaagcgagttccgggtgtacagcagcgccaacaactgcaccttcgagtacgtgtcccagcctttcctgatggacctggtgggcaaggagggcaacttcaagaacctgcgcgagttcgtgtttaagaacatcgacggctacttcaagatctacagcaagcacacccctatcaacctcgagcgggatctgcctcagggcttctctgctctggaacccctggtggatctgcccatcggcatcaacatcacccggtttcagacactgctggccctgcacagaagctacctgacacctgtggatagcagcagcggatggacagctggtgccgccgcttactatgtgggctacctgcagcctagaaccttcctgctgaagtacaacgagaacggcaccatcaccgacgccgtggattgtgctctggatcctctgagcgagacaaagtgcaccctgaagtccttcaccgtggaaaagggcatctaccagaccagcaacttccgggtgcagcccaccgaatccatcgtgcggttccccaatatcaccaatctgtgccccttccacgaggtgttcaatgccaccaccttcgcctctgtgtacgcctggaaccggaagcggatcagcaattgcgtggccgactactccgtgatctacaacttcgcccccttcttcgcattcaagtgctacggcgtgtcccctaccaagctgaacgacctgtgcttcacaaacgtgtacgccgacagcttcgtgatccggggaaacgaagtgtcacagattgcccctggacagacaggcaacatcgccgactacaactacaagctgcccgacgacttcaccggctgtgtgattgcctggaacagcaacaagctggactccaaacccagcggcaactacaattacctgtaccggctgttccggaagtccaagctgaagcccttcgagcgggacatctccaccgagatctatcaggccggcaacaggccttgtaacggcgtggcaggccccaactgctacagcccactgcagtcctacggctttaggcccacatacggcgtgggccaccagccctacagagtggtggtgctgagcttcgaactgctgcatgcccctgccacagtgtgcggccctaagaaaagcaccaatctcgtgaagaacaaatgcgtgaacttcaacttcaacggcctgaccggcaccggcgtgctgacagagagcaacaagaagttcctgccattccagcagtttggccgggatatcgccgataccacagacgccgttagagatccccagacactggaaatcctggacatcaccccttgcagcttcggcggagtgtctgtgatcacccctggcaccaacaccagcaatcaggtggcagtgctgtaccagggcgtgaactgtaccgaagtgcccgtggccattcacgccgatcagctgacacctacatggcgggtgtactccaccggcagcaatgtgtttcagaccagagccggctgtctgatcggagccgagtacgtgaacaatagctacgagtgcgacatccccatcggcgctggaatctgcgccagctaccagacacagacaaagagccaccggagagccagaagcgtggccagccagagcatcattgcctacacaatgtctctgggcgccgagaacagcgtggcctactccaacaactctatcgctatccccaccaacttcaccatcagcgtgaccacagagatcctgcctgtgtccatgaccaagaccagcgtggactgcaccatgtacatctgcggcgattccaccgagtgctccaacctgctgctgcagtacggcagcttctgcacccagctgaaaagagccctgacagggatcgccgtggaacaggacaagaacacccaagaggtgttcgcccaagtgaagcagatctacaagacccctcctatcaagtacttcggcggcttcaatttcagccagattctgcccgatcctagcaagcccagcaagcggagcttcatcgaggacctgctgttcaacaaagtgacactggccgacgccggcttcatcaagcagtatggcgattgtctgggcgacattgccgccagggatctgatttgcgcccagaagtttaacggactgacagtgctgcctcctctgctgaccgatgagatgatcgcccagtacacatctgccctgctggccggcacaatcacaagcggctggacatttggagcaggcgccgctctgcagatcccctttgctatgcagatggcctaccggttcaacggcatcggagtgacccagaatgtgctgtacgagaaccagaagctgatcgccaaccagttcaacagcgccatcggcaagatccaggacagcctgagcagcacagcaagcgccctgggaaagctgcaggacgtggtcaaccacaatgcccaggcactgaacaccctggtcaagcagctgtcctccaagttcggcgccatcagctctgtgctgaacgatatcctgagcagactggaccctcctgaggccgaggtgcagatcgacagactgatcacaggcagactgcagagcctccagacatacgtgacccagcagctgatcagagccgccgagattagagcctctgccaatctggccgccaccaagatgtctgagtgtgtgctgggccagagcaagagagtggacttttgcggcaagggctaccacctgatgagcttccctcagtctgcccctcacggcgtggtgtttctgcacgtgacatatgtgcccgctcaagagaagaatttcaccaccgctccagccatctgccacgacggcaaagcccactttcctagagaaggcgtgttcgtgtccaacggcacccattggttcgtgacacagcggaacttctacgagccccagatcatcaccaccgacaacaccttcgtgtctggcaactgcgacgtcgtgatcggcattgtgaacaataccgtgtacgaccctctgcagcccgagctggacagcttcaaagaggaactggacaagtactttaagaaccacacaagccccgacgtggacctgggcgatatcagcggaatcaatgccagcgtcgtgaacatccagaaagagatcgaccggctgaacgaggtggccaagaatctgaacgagagcctgatcgacctgcaagaactggggaagtacgagcagtacatcaagtggccctggtacatctggctgggctttatcgccggactgattgccatcgtgatggtcacaatcatgctgtgttgcatgaccagctgctgtagctgcctgaagggctgttgtagctgtggcagctgctgcaagttcgacgaggacgattctgagcccgtgctgaagggcgtgaaactgcactacacatgatga

SEQ ID NO: 165 - DNA, 3813 bp, synthetic construct
  source 1..3813: mol_type = other DNA
atgttcgtgttcctggtgctgctgcctctggtgtccagccagtgtgtgaacctgatcaccagaacacagtcatacaccaacagctttaccagaggcgtgtactaccccgacaaggtgttcagatccagcgtgctgcactctacccaggacctgttcctgcctttcttcagcaacgtgacctggttccacgccatccacgtgtccggcaccaatggcaccaagagattcgacaaccccgccctgcccttcaacgacggggtgtactttgccagcaccgagaagtccaacatcatcagaggctggatcttcggcaccacactggacagcaagacccagagcctgctgatcgtgaacaacgccaccaacgtggtcatcaaagtgtgcgagttccagttctgcaacgaccccttcctggacgtctaccagaagaacaacaagagctggatggaaagcgagttccgggtgtacagcagcgccaacaactgcaccttcgagtacgtgtcccagcctttcctgatggacctggtgggcaaggagggcaacttcaagaacctgcgcgagttcgtgtttaagaacatcgacggctacttcaagatctacagcaagcacacccctatcaacctcgagcgggatctgcctcagggcttctctgctctggaacccctggtggatctgcccatcggcatcaacatcacccggtttcagacactgctggccctgcacagaagctacctgacacctgtggatagcagcagcggatggacagctggtgccgccgcttactatgtgggctacctgcagcctagaaccttcctgctgaagtacaacgagaacggcaccatcaccgacgccgtggattgtgctctggatcctctgagcgagacaaagtgcaccctgaagtccttcaccgtggaaaagggcatctaccagaccagcaacttccgggtgcagcccaccgaatccatcgtgcggttccccaatatcaccaatctgtgccccttccacgaggtgttcaatgccaccaccttcgcctctgtgtacgcctggaaccggaagcggatcagcaattgcgtggccgactactccgtgatctacaacttcgcccccttcttcgcattcaagtgctacggcgtgtcccctaccaagctgaacgacctgtgcttcacaaacgtgtacgccgacagcttcgtgatccggggaaacgaagtgtcacagattgcccctggacagacaggcaacatcgccgactacaactacaagctgcccgacgacttcaccggctgtgtgattgcctggaacagcaacaagctggactccaaacccagcggcaactacaattacctgtaccggctgttccggaagtccaagctgaagcccttcgagcgggacatctccaccgagatctatcaggccggcaacaggccttgtaacggcgtggcaggccccaactgctacagcccactgcagtcctacggctttaggcccacatacggcgtgggccaccagccctacagagtggtggtgctgagcttcgaactgctgcatgcccctgccacagtgtgcggccctaagaaaagcaccaatctcgtgaagaacaaatgcgtgaacttcaacttcaacggcctgaccggcaccggcgtgctgacagagagcaacaagaagttcctgccattccagcagtttggccgggatatcgccgataccacagacgccgttagagatccccagacactggaaatcctggacatcaccccttgcagcttcggcggagtgtctgtgatcacccctggcaccaacaccagcaatcaggtggcagtgctgtaccagggcgtgaactgtaccgaagtgcccgtggccattcacgccgatcagctgacacctacatggcgggtgtactccaccggcagcaatgtgtttcagaccagagccggctgtctgatcggagccgagtacgtgaacaatagctacgagtgcgacatccccatcggcgctggaatctgcgccagctaccagacacagacaaagagccaccggagagccagaagcgtggccagccagagcatcattgcctacacaatgtctctgggcgccgagaacagcgtggcctactccaacaactctatcgctatccccaccaacttcaccatcagcgtgaccacagagatcctgcctgtgtccatgaccaagaccagcgtggactgcaccatgtacatctgcggcgattccaccgagtgctccaacctgctgctgcagtacggcagcttctgcacccagctgaaaagagccctgacagggatcgccgtggaacaggacaagaacacccaagaggtgttcgcccaagtgaagcagatctacaagacccctcctatcaagtacttcggcggcttcaatttcagccagattctgcccgatcctagcaagcccagcaagcggagcttcatcgaggacctgctgttcaacaaagtgacactggccgacgccggcttcatcaagcagtatggcgattgtctgggcgacattgccgccagggatctgatttgcgcccagaagtttaacggactgacagtgctgcctcctctgctgaccgatgagatgatcgcccagtacacatctgccctgctggccggcacaatcacaagcggctggacatttggagcaggcgccgctctgcagatcccctttgctatgcagatggcctaccggttcaacggcatcggagtgacccagaatgtgctgtacgagaaccagaagctgatcgccaaccagttcaacagcgccatcggcaagatccaggacagcctgagcagcacagcaagcgccctgggaaagctgcaggacgtggtcaaccacaatgcccaggcactgaacaccctggtcaagcagctgtcctccaagttcggcgccatcagctctgtgctgaacgatatcctgagcagactggaccctcctgaggccgaggtgcagatcgacagactgatcacaggcagactgcagagcctccagacatacgtgacccagcagctgatcagagccgccgagattagagcctctgccaatctggccgccaccaagatgtctgagtgtgtgctgggccagagcaagagagtggacttttgcggcaagggctaccacctgatgagcttccctcagtctgcccctcacggcgtggtgtttctgcacgtgacatatgtgcccgctcaagagaagaatttcaccaccgctccagccatctgccacgacggcaaagcccactttcctagagaaggcgtgttcgtgtccaacggcacccattggttcgtgacacagcggaacttctacgagccccagatcatcaccaccgacaacaccttcgtgtctggcaactgcgacgtcgtgatcggcattgtgaacaataccgtgtacgaccctctgcagcccgagctggacagcttcaaagaggaactggacaagtactttaagaaccacacaagccccgacgtggacctgggcgatatcagcggaatcaatgccagcgtcgtgaacatccagaaagagatcgaccggctgaacgaggtggccaagaatctgaacgagagcctgatcgacctgcaagaactggggaagtacgagcagtacatcaagtggccctggtacatctggctgggctttatcgccggactgattgccatcgtgatggtcacaatcatgctgtgttgcatgaccagctgctgtagctgcctgaagggctgttgtagctgtggcagctgctgcaagttcgacgaggacgattctgagcccgtgctgaagggcgtgaaactgcactacacatgatga

SEQ ID NO: 166 - RNA, 4270 nt, synthetic construct
  source 1..4270: mol_type = other RNA
agaataaactagtattcttctggtccccacagactcagagagaacccgccaccatgttcgtgttcctggtgctgctgcctctggtgtccagccagtgtgtgaacctgatcaccagaacacagtcatacaccaacagctttaccagaggcgtgtactaccccgacaaggtgttcagatccagcgtgctgcactctacccaggacctgttcctgcctttcttcagcaacgtgacctggttccacgccatccacgtgtccggcaccaatggcaccaagagattcgacaaccccgccctgcccttcaacgacggggtgtactttgccagcaccgagaagtccaacatcatcagaggctggatcttcggcaccacactggacagcaagacccagagcctgctgatcgtgaacaacgccaccaacgtggtcatcaaagtgtgcgagttccagttctgcaacgaccccttcctggacgtctaccagaagaacaacaagagctggatggaaagcgagttccgggtgtacagcagcgccaacaactgcaccttcgagtacgtgtcccagcctttcctgatggacctggtgggcaaggagggcaacttcaagaacctgcgcgagttcgtgtttaagaacatcgacggctacttcaagatctacagcaagcacacccctatcaacctcgagcgggatctgcctcagggcttctctgctctggaacccctggtggatctgcccatcggcatcaacatcacccggtttcagacactgctggccctgcacagaagctacctgacacctgtggatagcagcagcggatggacagctggtgccgccgcttactatgtgggctacctgcagcctagaaccttcctgctgaagtacaacgagaacggcaccatcaccgacgccgtggattgtgctctggatcctctgagcgagacaaagtgcaccctgaagtccttcaccgtggaaaagggcatctaccagaccagcaacttccgggtgcagcccaccgaatccatcgtgcggttccccaatatcaccaatctgtgccccttccacgaggtgttcaatgccaccaccttcgcctctgtgtacgcctggaaccggaagcggatcagcaattgcgtggccgactactccgtgatctacaacttcgcccccttcttcgcattcaagtgctacggcgtgtcccctaccaagctgaacgacctgtgcttcacaaacgtgtacgccgacagcttcgtgatccggggaaacgaagtgtcacagattgcccctggacagacaggcaacatcgccgactacaactacaagctgcccgacgacttcaccggctgtgtgattgcctggaacagcaacaagctggactccaaacccagcggcaactacaattacctgtaccggctgttccggaagtccaagctgaagcccttcgagcgggacatctccaccgagatctatcaggccggcaacaggccttgtaacggcgtggcaggccccaactgctacagcccactgcagtcctacggctttaggcccacatacggcgtgggccaccagccctacagagtggtggtgctgagcttcgaactgctgcatgcccctgccacagtgtgcggccctaagaaaagcaccaatctcgtgaagaacaaatgcgtgaacttcaacttcaacggcctgaccggcaccggcgtgctgacagagagcaacaagaagttcctgccattccagcagtttggccgggatatcgccgataccacagacgccgttagagatccccagacactggaaatcctggacatcaccccttgcagcttcggcggagtgtctgtgatcacccctggcaccaacaccagcaatcaggtggcagtgctgtaccagggcgtgaactgtaccgaagtgcccgtggccattcacgccgatcagctgacacctacatggcgggtgtactccaccggcagcaatgtgtttcagaccagagccggctgtctgatcggagccgagtacgtgaacaatagctacgagtgcgacatccccatcggcgctggaatctgcgccagctaccagacacagacaaagagccaccggagagccagaagcgtggccagccagagcatcattgcctacacaatgtctctgggcgccgagaacagcgtggcctactccaacaactctatcgctatccccaccaacttcaccatcagcgtgaccacagagatcctgcctgtgtccatgaccaagaccagcgtggactgcaccatgtacatctgcggcgattccaccgagtgctccaacctgctgctgcagtacggcagcttctgcacccagctgaaaagagccctgacagggatcgccgtggaacaggacaagaacacccaagaggtgttcgcccaagtgaagcagatctacaagacccctcctatcaagtacttcggcggcttcaatttcagccagattctgcccgatcctagcaagcccagcaagcggagcttcatcgaggacctgctgttcaacaaagtgacactggccgacgccggcttcatcaagcagtatggcgattgtctgggcgacattgccgccagggatctgatttgcgcccagaagtttaacggactgacagtgctgcctcctctgctgaccgatgagatgatcgcccagtacacatctgccctgctggccggcacaatcacaagcggctggacatttggagcaggcgccgctctgcagatcccctttgctatgcagatggcctaccggttcaacggcatcggagtgacccagaatgtgctgtacgagaaccagaagctgatcgccaaccagttcaacagcgccatcggcaagatccaggacagcctgagcagcacagcaagcgccctgggaaagctgcaggacgtggtcaaccacaatgcccaggcactgaacaccctggtcaagcagctgtcctccaagttcggcgccatcagctctgtgctgaacgatatcctgagcagactggaccctcctgaggccgaggtgcagatcgacagactgatcacaggcagactgcagagcctccagacatacgtgacccagcagctgatcagagccgccgagattagagcctctgccaatctggccgccaccaagatgtctgagtgtgtgctgggccagagcaagagagtggacttttgcggcaagggctaccacctgatgagcttccctcagtctgcccctcacggcgtggtgtttctgcacgtgacatatgtgcccgctcaagagaagaatttcaccaccgctccagccatctgccacgacggcaaagcccactttcctagagaaggcgtgttcgtgtccaacggcacccattggttcgtgacacagcggaacttctacgagccccagatcatcaccaccgacaacaccttcgtgtctggcaactgcgacgtcgtgatcggcattgtgaacaataccgtgtacgaccctctgcagcccgagctggacagcttcaaagaggaactggacaagtactttaagaaccacacaagccccgacgtggacctgggcgatatcagcggaatcaatgccagcgtcgtgaacatccagaaagagatcgaccggctgaacgaggtggccaagaatctgaacgagagcctgatcgacctgcaagaactggggaagtacgagcagtacatcaagtggccctggtacatctggctgggctttatcgccggactgattgccatcgtgatggtcacaatcatgctgtgttgcatgaccagctgctgtagctgcctgaagggctgttgtagctgtggcagctgctgcaagttcgacgaggacgattctgagcccgtgctgaagggcgtgaaactgcactacacatgatgactcgagctggtactgcatgcacgcaatgctagctgcccctttcccgtcctgggtaccccgagtctcccccgacctcgggtcccaggtatgctcccacctccacctgccccactcaccacctctgctagttccagacacctcccaagcacgcagcaatgcagctcaaaacgcttagcctagccacacccccacgggaaacagcagtgattaacctttagcaataaacgaaagtttaactaagctatactaaccccagggttggtcaatttcgtgccagccacaccctggagctagcaaaaaaaaaaaaaaaaaaaaaaaaaaaaaagcatatgactaaaaaaaaaaaaaaaaaaaaaaaaaaaaaaaaaaaaaaaaaaaaaaaaaaaaaaaaaaaaaaaaaaaaa

SEQ ID NO: 167 - DNA, 4270 bp, synthetic construct
  source 1..4270: mol_type = other DNA
agaataaactagtattcttctggtccccacagactcagagagaacccgccaccatgttcgtgttcctggtgctgctgcctctggtgtccagccagtgtgtgaacctgatcaccagaacacagtcatacaccaacagctttaccagaggcgtgtactaccccgacaaggtgttcagatccagcgtgctgcactctacccaggacctgttcctgcctttcttcagcaacgtgacctggttccacgccatccacgtgtccggcaccaatggcaccaagagattcgacaaccccgccctgcccttcaacgacggggtgtactttgccagcaccgagaagtccaacatcatcagaggctggatcttcggcaccacactggacagcaagacccagagcctgctgatcgtgaacaacgccaccaacgtggtcatcaaagtgtgcgagttccagttctgcaacgaccccttcctggacgtctaccagaagaacaacaagagctggatggaaagcgagttccgggtgtacagcagcgccaacaactgcaccttcgagtacgtgtcccagcctttcctgatggacctggtgggcaaggagggcaacttcaagaacctgcgcgagttcgtgtttaagaacatcgacggctacttcaagatctacagcaagcacacccctatcaacctcgagcgggatctgcctcagggcttctctgctctggaacccctggtggatctgcccatcggcatcaacatcacccggtttcagacactgctggccctgcacagaagctacctgacacctgtggatagcagcagcggatggacagctggtgccgccgcttactatgtgggctacctgcagcctagaaccttcctgctgaagtacaacgagaacggcaccatcaccgacgccgtggattgtgctctggatcctctgagcgagacaaagtgcaccctgaagtccttcaccgtggaaaagggcatctaccagaccagcaacttccgggtgcagcccaccgaatccatcgtgcggttccccaatatcaccaatctgtgccccttccacgaggtgttcaatgccaccaccttcgcctctgtgtacgcctggaaccggaagcggatcagcaattgcgtggccgactactccgtgatctacaacttcgcccccttcttcgcattcaagtgctacggcgtgtcccctaccaagctgaacgacctgtgcttcacaaacgtgtacgccgacagcttcgtgatccggggaaacgaagtgtcacagattgcccctggacagacaggcaacatcgccgactacaactacaagctgcccgacgacttcaccggctgtgtgattgcctggaacagcaacaagctggactccaaacccagcggcaactacaattacctgtaccggctgttccggaagtccaagctgaagcccttcgagcgggacatctccaccgagatctatcaggccggcaacaggccttgtaacggcgtggcaggccccaactgctacagcccactgcagtcctacggctttaggcccacatacggcgtgggccaccagccctacagagtggtggtgctgagcttcgaactgctgcatgcccctgccacagtgtgcggccctaagaaaagcaccaatctcgtgaagaacaaatgcgtgaacttcaacttcaacggcctgaccggcaccggcgtgctgacagagagcaacaagaagttcctgccattccagcagtttggccgggatatcgccgataccacagacgccgttagagatccccagacactggaaatcctggacatcaccccttgcagcttcggcggagtgtctgtgatcacccctggcaccaacaccagcaatcaggtggcagtgctgtaccagggcgtgaactgtaccgaagtgcccgtggccattcacgccgatcagctgacacctacatggcgggtgtactccaccggcagcaatgtgtttcagaccagagccggctgtctgatcggagccgagtacgtgaacaatagctacgagtgcgacatccccatcggcgctggaatctgcgccagctaccagacacagacaaagagccaccggagagccagaagcgtggccagccagagcatcattgcctacacaatgtctctgggcgccgagaacagcgtggcctactccaacaactctatcgctatccccaccaacttcaccatcagcgtgaccacagagatcctgcctgtgtccatgaccaagaccagcgtggactgcaccatgtacatctgcggcgattccaccgagtgctccaacctgctgctgcagtacggcagcttctgcacccagctgaaaagagccctgacagggatcgccgtggaacaggacaagaacacccaagaggtgttcgcccaagtgaagcagatctacaagacccctcctatcaagtacttcggcggcttcaatttcagccagattctgcccgatcctagcaagcccagcaagcggagcttcatcgaggacctgctgttcaacaaagtgacactggccgacgccggcttcatcaagcagtatggcgattgtctgggcgacattgccgccagggatctgatttgcgcccagaagtttaacggactgacagtgctgcctcctctgctgaccgatgagatgatcgcccagtacacatctgccctgctggccggcacaatcacaagcggctggacatttggagcaggcgccgctctgcagatcccctttgctatgcagatggcctaccggttcaacggcatcggagtgacccagaatgtgctgtacgagaaccagaagctgatcgccaaccagttcaacagcgccatcggcaagatccaggacagcctgagcagcacagcaagcgccctgggaaagctgcaggacgtggtcaaccacaatgcccaggcactgaacaccctggtcaagcagctgtcctccaagttcggcgccatcagctctgtgctgaacgatatcctgagcagactggaccctcctgaggccgaggtgcagatcgacagactgatcacaggcagactgcagagcctccagacatacgtgacccagcagctgatcagagccgccgagattagagcctctgccaatctggccgccaccaagatgtctgagtgtgtgctgggccagagcaagagagtggacttttgcggcaagggctaccacctgatgagcttccctcagtctgcccctcacggcgtggtgtttctgcacgtgacatatgtgcccgctcaagagaagaatttcaccaccgctccagccatctgccacgacggcaaagcccactttcctagagaaggcgtgttcgtgtccaacggcacccattggttcgtgacacagcggaacttctacgagccccagatcatcaccaccgacaacaccttcgtgtctggcaactgcgacgtcgtgatcggcattgtgaacaataccgtgtacgaccctctgcagcccgagctggacagcttcaaagaggaactggacaagtactttaagaaccacacaagccccgacgtggacctgggcgatatcagcggaatcaatgccagcgtcgtgaacatccagaaagagatcgaccggctgaacgaggtggccaagaatctgaacgagagcctgatcgacctgcaagaactggggaagtacgagcagtacatcaagtggccctggtacatctggctgggctttatcgccggactgattgccatcgtgatggtcacaatcatgctgtgttgcatgaccagctgctgtagctgcctgaagggctgttgtagctgtggcagctgctgcaagttcgacgaggacgattctgagcccgtgctgaagggcgtgaaactgcactacacatgatgactcgagctggtactgcatgcacgcaatgctagctgcccctttcccgtcctgggtaccccgagtctcccccgacctcgggtcccaggtatgctcccacctccacctgccccactcaccacctctgctagttccagacacctcccaagcacgcagcaatgcagctcaaaacgcttagcctagccacacccccacgggaaacagcagtgattaacctttagcaataaacgaaagtttaactaagctatactaaccccagggttggtcaatttcgtgccagccacaccctggagctagcaaaaaaaaaaaaaaaaaaaaaaaaaaaaaagcatatgactaaaaaaaaaaaaaaaaaaaaaaaaaaaaaaaaaaaaaaaaaaaaaaaaaaaaaaaaaaaaaaaaaaaaa

SEQ ID NO: 168 - protein, 1269 aa, synthetic construct
MFVFLVLLPLVSSQCVNLITRTQSYTNSFTRGVYYPDKVFRSSVLHSTQDLFLPFFSNVTWFHAIHVSGTNGTKRFDNPALPFNDGVYFASTEKSNIIRGWIFGTTLDSKTQSLLIVNNATNVVIKVCEFQFCNDPFLDVYQKNNKSWMESEFRVYSSANNCTFEYVSQPFLMDLEGKEGNFKNLREFVFKNIDGYFKIYSKHTPINLERDLPQGFSALEPLVDLPIGINITRFQTLLALHRSYLTPGGSSSGWTAGAAAYYVGYLQPRTFLLKYNENGTITDAVDCALDPLSETKCTLKSFTVEKGIYQTSNFRVQPTESIVRFPNITNLCPFHEVFNATTFASVYAWNRKRISNCVADYSVIYNFAPFFAFKCYGVSPTKLNDLCFTNVYADSFVIRGNEVSQIAPGQTGNIADYNYKLPDDFTGCVIAWNSNKLDSKPSGNYNYLYRLFRKSKLKPFERDISTEIYQAGNKPCNGVAGPNCYSPLQSYGFRPTYGVGHQPYRVVVLSFELLHASATVCGPKKSTNLVKNKCVNFNFNGLTGTGVLTESNKKFLPFQQFGRDIADTTDAVRDPQTLEILDITPCSFGGVSVITPGTNTSNQVAVLYQGVNCTEVPVAIHADQLTPTWRVYSTGSNVFQTRAGCLIGAEYVNNSYECDIPIGAGICASYQTQTKSHRRARSVASQSIIAYTMSLGAENSVAYSNNSIAIPTNFTISVTTEILPVSMTKTSVDCTMYICGDSTECSNLLLQYGSFCTQLKRALTGIAVEQDKNTQEVFAQVKQIYKTPPIKYFGGFNFSQILPDPSKPSKRSFIEDLLFNKVTLADAGFIKQYGDCLGDIAARDLICAQKFNGLTVLPPLLTDEMIAQYTSALLAGTITSGWTFGAGAALQIPFAMQMAYRFNGIGVTQNVLYENQKLIANQFNSAIGKIQDSLSSTASALGKLQDVVNHNAQALNTLVKQLSSKFGAISSVLNDILSRLDPPEAEVQIDRLITGRLQSLQTYVTQQLIRAAEIRASANLAATKMSECVLGQSKRVDFCGKGYHLMSFPQSAPHGVVFLHVTYVPAQEKNFTTAPAICHDGKAHFPREGVFVSNGTHWFVTQRNFYEPQIITTDNTFVSGNCDVVIGIVNNTVYDPLQPELDSFKEELDKYFKNHTSPDVDLGDISGINASVVNIQKEIDRLNEVAKNLNESLIDLQELGKYEQYIKWPWYIWLGFIAGLIAIVMVTIMLCCMTSCCSCLKGCCSCGSCCKFDEDDSEPVLKGVKLHYT

SEQ ID NO: 169 - RNA, 3813 nt, synthetic construct
  source 1..3813: mol_type = other RNA
atgttcgtgttcctggtgctgctgcctctggtgtccagccagtgtgtgaacctgatcaccagaacacagtcatacaccaacagctttaccagaggcgtgtactaccccgacaaggtgttcagatccagcgtgctgcactctacccaggacctgttcctgcctttcttcagcaacgtgacctggttccacgccatccacgtgtccggcaccaatggcaccaagagattcgacaaccccgccctgcccttcaacgacggggtgtactttgccagcaccgagaagtccaacatcatcagaggctggatcttcggcaccacactggacagcaagacccagagcctgctgatcgtgaacaacgccaccaacgtggtcatcaaagtgtgcgagttccagttctgcaacgaccccttcctggacgtctaccagaagaacaacaagagctggatggaaagcgagttccgggtgtacagcagcgccaacaactgcaccttcgagtacgtgtcccagcctttcctgatggacctggaaggcaaggagggcaacttcaagaacctgcgcgagttcgtgtttaagaacatcgacggctacttcaagatctacagcaagcacacccctatcaacctcgagcgggatctgcctcagggcttctctgctctggaacccctggtggatctgcccatcggcatcaacatcacccggtttcagacactgctggccctgcacagaagctacctgacacctggcggcagcagcagcggatggacagctggtgccgccgcttactatgtgggctacctgcagcctagaaccttcctgctgaagtacaacgagaacggcaccatcaccgacgccgtggattgtgctctggatcctctgagcgagacaaagtgcaccctgaagtccttcaccgtggaaaagggcatctaccagaccagcaacttccgggtgcagcccaccgaatccatcgtgcggttccccaatatcaccaatctgtgccccttccacgaggtgttcaatgccaccaccttcgcctctgtgtacgcctggaaccggaagcggatcagcaattgcgtggccgactactccgtgatctacaacttcgcccccttcttcgcattcaagtgctacggcgtgtcccctaccaagctgaacgacctgtgcttcacaaacgtgtacgccgacagcttcgtgatccggggaaacgaagtgtcacagattgcccctggacagacaggcaacatcgccgactacaactacaagctgcccgacgacttcaccggctgtgtgattgcctggaacagcaacaagctggactccaaacccagcggcaactacaattacctgtaccggctgttccggaagtccaagctgaagcccttcgagcgggacatctccaccgagatctatcaggccggcaacaagccttgtaacggcgtggcaggccccaactgctacagcccactgcagtcctacggctttaggcccacatacggcgtgggccaccagccctacagagtggtggtgctgagcttcgaactgctgcatgcctcagccacagtgtgcggccctaagaaaagcaccaatctcgtgaagaacaaatgcgtgaacttcaacttcaacggcctgaccggcaccggcgtgctgacagagagcaacaagaagttcctgccattccagcagtttggccgggatatcgccgataccacagacgccgttagagatccccagacactggaaatcctggacatcaccccttgcagcttcggcggagtgtctgtgatcacccctggcaccaacaccagcaatcaggtggcagtgctgtaccagggcgtgaactgtaccgaagtgcccgtggccattcacgccgatcagctgacacctacatggcgggtgtactccaccggcagcaatgtgtttcagaccagagccggctgtctgatcggagccgagtacgtgaacaatagctacgagtgcgacatccccatcggcgctggaatctgcgccagctaccagacacagacaaagagccaccggagagccagaagcgtggccagccagagcatcattgcctacacaatgtctctgggcgccgagaacagcgtggcctactccaacaactctatcgctatccccaccaacttcaccatcagcgtgaccacagagatcctgcctgtgtccatgaccaagaccagcgtggactgcaccatgtacatctgcggcgattccaccgagtgctccaacctgctgctgcagtacggcagcttctgcacccagctgaaaagagccctgacagggatcgccgtggaacaggacaagaacacccaagaggtgttcgcccaagtgaagcagatctacaagacccctcctatcaagtacttcggcggcttcaatttcagccagattctgcccgatcctagcaagcccagcaagcggagcttcatcgaggacctgctgttcaacaaagtgacactggccgacgccggcttcatcaagcagtatggcgattgtctgggcgacattgccgccagggatctgatttgcgcccagaagtttaacggactgacagtgctgcctcctctgctgaccgatgagatgatcgcccagtacacatctgccctgctggccggcacaatcacaagcggctggacatttggagcaggcgccgctctgcagatcccctttgctatgcagatggcctaccggttcaacggcatcggagtgacccagaatgtgctgtacgagaaccagaagctgatcgccaaccagttcaacagcgccatcggcaagatccaggacagcctgagcagcacagcaagcgccctgggaaagctgcaggacgtggtcaaccacaatgcccaggcactgaacaccctggtcaagcagctgtcctccaagttcggcgccatcagctctgtgctgaacgatatcctgagcagactggaccctcctgaggccgaggtgcagatcgacagactgatcacaggcagactgcagagcctccagacatacgtgacccagcagctgatcagagccgccgagattagagcctctgccaatctggccgccaccaagatgtctgagtgtgtgctgggccagagcaagagagtggacttttgcggcaagggctaccacctgatgagcttccctcagtctgcccctcacggcgtggtgtttctgcacgtgacatatgtgcccgctcaagagaagaatttcaccaccgctccagccatctgccacgacggcaaagcccactttcctagagaaggcgtgttcgtgtccaacggcacccattggttcgtgacacagcggaacttctacgagccccagatcatcaccaccgacaacaccttcgtgtctggcaactgcgacgtcgtgatcggcattgtgaacaataccgtgtacgaccctctgcagcccgagctggacagcttcaaagaggaactggacaagtactttaagaaccacacaagccccgacgtggacctgggcgatatcagcggaatcaatgccagcgtcgtgaacatccagaaagagatcgaccggctgaacgaggtggccaagaatctgaacgagagcctgatcgacctgcaagaactggggaagtacgagcagtacatcaagtggccctggtacatctggctgggctttatcgccggactgattgccatcgtgatggtcacaatcatgctgtgttgcatgaccagctgctgtagctgcctgaagggctgttgtagctgtggcagctgctgcaagttcgacgaggacgattctgagcccgtgctgaagggcgtgaaactgcactacacatgatga

SEQ ID NO: 170 - DNA, 3813 bp, synthetic construct
  source 1..3813: mol_type = other DNA
atgttcgtgttcctggtgctgctgcctctggtgtccagccagtgtgtgaacctgatcaccagaacacagtcatacaccaacagctttaccagaggcgtgtactaccccgacaaggtgttcagatccagcgtgctgcactctacccaggacctgttcctgcctttcttcagcaacgtgacctggttccacgccatccacgtgtccggcaccaatggcaccaagagattcgacaaccccgccctgcccttcaacgacggggtgtactttgccagcaccgagaagtccaacatcatcagaggctggatcttcggcaccacactggacagcaagacccagagcctgctgatcgtgaacaacgccaccaacgtggtcatcaaagtgtgcgagttccagttctgcaacgaccccttcctggacgtctaccagaagaacaacaagagctggatggaaagcgagttccgggtgtacagcagcgccaacaactgcaccttcgagtacgtgtcccagcctttcctgatggacctggaaggcaaggagggcaacttcaagaacctgcgcgagttcgtgtttaagaacatcgacggctacttcaagatctacagcaagcacacccctatcaacctcgagcgggatctgcctcagggcttctctgctctggaacccctggtggatctgcccatcggcatcaacatcacccggtttcagacactgctggccctgcacagaagctacctgacacctggcggcagcagcagcggatggacagctggtgccgccgcttactatgtgggctacctgcagcctagaaccttcctgctgaagtacaacgagaacggcaccatcaccgacgccgtggattgtgctctggatcctctgagcgagacaaagtgcaccctgaagtccttcaccgtggaaaagggcatctaccagaccagcaacttccgggtgcagcccaccgaatccatcgtgcggttccccaatatcaccaatctgtgccccttccacgaggtgttcaatgccaccaccttcgcctctgtgtacgcctggaaccggaagcggatcagcaattgcgtggccgactactccgtgatctacaacttcgcccccttcttcgcattcaagtgctacggcgtgtcccctaccaagctgaacgacctgtgcttcacaaacgtgtacgccgacagcttcgtgatccggggaaacgaagtgtcacagattgcccctggacagacaggcaacatcgccgactacaactacaagctgcccgacgacttcaccggctgtgtgattgcctggaacagcaacaagctggactccaaacccagcggcaactacaattacctgtaccggctgttccggaagtccaagctgaagcccttcgagcgggacatctccaccgagatctatcaggccggcaacaagccttgtaacggcgtggcaggccccaactgctacagcccactgcagtcctacggctttaggcccacatacggcgtgggccaccagccctacagagtggtggtgctgagcttcgaactgctgcatgcctcagccacagtgtgcggccctaagaaaagcaccaatctcgtgaagaacaaatgcgtgaacttcaacttcaacggcctgaccggcaccggcgtgctgacagagagcaacaagaagttcctgccattccagcagtttggccgggatatcgccgataccacagacgccgttagagatccccagacactggaaatcctggacatcaccccttgcagcttcggcggagtgtctgtgatcacccctggcaccaacaccagcaatcaggtggcagtgctgtaccagggcgtgaactgtaccgaagtgcccgtggccattcacgccgatcagctgacacctacatggcgggtgtactccaccggcagcaatgtgtttcagaccagagccggctgtctgatcggagccgagtacgtgaacaatagctacgagtgcgacatccccatcggcgctggaatctgcgccagctaccagacacagacaaagagccaccggagagccagaagcgtggccagccagagcatcattgcctacacaatgtctctgggcgccgagaacagcgtggcctactccaacaactctatcgctatccccaccaacttcaccatcagcgtgaccacagagatcctgcctgtgtccatgaccaagaccagcgtggactgcaccatgtacatctgcggcgattccaccgagtgctccaacctgctgctgcagtacggcagcttctgcacccagctgaaaagagccctgacagggatcgccgtggaacaggacaagaacacccaagaggtgttcgcccaagtgaagcagatctacaagacccctcctatcaagtacttcggcggcttcaatttcagccagattctgcccgatcctagcaagcccagcaagcggagcttcatcgaggacctgctgttcaacaaagtgacactggccgacgccggcttcatcaagcagtatggcgattgtctgggcgacattgccgccagggatctgatttgcgcccagaagtttaacggactgacagtgctgcctcctctgctgaccgatgagatgatcgcccagtacacatctgccctgctggccggcacaatcacaagcggctggacatttggagcaggcgccgctctgcagatcccctttgctatgcagatggcctaccggttcaacggcatcggagtgacccagaatgtgctgtacgagaaccagaagctgatcgccaaccagttcaacagcgccatcggcaagatccaggacagcctgagcagcacagcaagcgccctgggaaagctgcaggacgtggtcaaccacaatgcccaggcactgaacaccctggtcaagcagctgtcctccaagttcggcgccatcagctctgtgctgaacgatatcctgagcagactggaccctcctgaggccgaggtgcagatcgacagactgatcacaggcagactgcagagcctccagacatacgtgacccagcagctgatcagagccgccgagattagagcctctgccaatctggccgccaccaagatgtctgagtgtgtgctgggccagagcaagagagtggacttttgcggcaagggctaccacctgatgagcttccctcagtctgcccctcacggcgtggtgtttctgcacgtgacatatgtgcccgctcaagagaagaatttcaccaccgctccagccatctgccacgacggcaaagcccactttcctagagaaggcgtgttcgtgtccaacggcacccattggttcgtgacacagcggaacttctacgagccccagatcatcaccaccgacaacaccttcgtgtctggcaactgcgacgtcgtgatcggcattgtgaacaataccgtgtacgaccctctgcagcccgagctggacagcttcaaagaggaactggacaagtactttaagaaccacacaagccccgacgtggacctgggcgatatcagcggaatcaatgccagcgtcgtgaacatccagaaagagatcgaccggctgaacgaggtggccaagaatctgaacgagagcctgatcgacctgcaagaactggggaagtacgagcagtacatcaagtggccctggtacatctggctgggctttatcgccggactgattgccatcgtgatggtcacaatcatgctgtgttgcatgaccagctgctgtagctgcctgaagggctgttgtagctgtggcagctgctgcaagttcgacgaggacgattctgagcccgtgctgaagggcgtgaaactgcactacacatgatga

SEQ ID NO: 171 - RNA, 4270 nt, synthetic construct
  source 1..4270: mol_type = other RNA
agaataaactagtattcttctggtccccacagactcagagagaacccgccaccatgttcgtgttcctggtgctgctgcctctggtgtccagccagtgtgtgaacctgatcaccagaacacagtcatacaccaacagctttaccagaggcgtgtactaccccgacaaggtgttcagatccagcgtgctgcactctacccaggacctgttcctgcctttcttcagcaacgtgacctggttccacgccatccacgtgtccggcaccaatggcaccaagagattcgacaaccccgccctgcccttcaacgacggggtgtactttgccagcaccgagaagtccaacatcatcagaggctggatcttcggcaccacactggacagcaagacccagagcctgctgatcgtgaacaacgccaccaacgtggtcatcaaagtgtgcgagttccagttctgcaacgaccccttcctggacgtctaccagaagaacaacaagagctggatggaaagcgagttccgggtgtacagcagcgccaacaactgcaccttcgagtacgtgtcccagcctttcctgatggacctggaaggcaaggagggcaacttcaagaacctgcgcgagttcgtgtttaagaacatcgacggctacttcaagatctacagcaagcacacccctatcaacctcgagcgggatctgcctcagggcttctctgctctggaacccctggtggatctgcccatcggcatcaacatcacccggtttcagacactgctggccctgcacagaagctacctgacacctggcggcagcagcagcggatggacagctggtgccgccgcttactatgtgggctacctgcagcctagaaccttcctgctgaagtacaacgagaacggcaccatcaccgacgccgtggattgtgctctggatcctctgagcgagacaaagtgcaccctgaagtccttcaccgtggaaaagggcatctaccagaccagcaacttccgggtgcagcccaccgaatccatcgtgcggttccccaatatcaccaatctgtgccccttccacgaggtgttcaatgccaccaccttcgcctctgtgtacgcctggaaccggaagcggatcagcaattgcgtggccgactactccgtgatctacaacttcgcccccttcttcgcattcaagtgctacggcgtgtcccctaccaagctgaacgacctgtgcttcacaaacgtgtacgccgacagcttcgtgatccggggaaacgaagtgtcacagattgcccctggacagacaggcaacatcgccgactacaactacaagctgcccgacgacttcaccggctgtgtgattgcctggaacagcaacaagctggactccaaacccagcggcaactacaattacctgtaccggctgttccggaagtccaagctgaagcccttcgagcgggacatctccaccgagatctatcaggccggcaacaagccttgtaacggcgtggcaggccccaactgctacagcccactgcagtcctacggctttaggcccacatacggcgtgggccaccagccctacagagtggtggtgctgagcttcgaactgctgcatgcctcagccacagtgtgcggccctaagaaaagcaccaatctcgtgaagaacaaatgcgtgaacttcaacttcaacggcctgaccggcaccggcgtgctgacagagagcaacaagaagttcctgccattccagcagtttggccgggatatcgccgataccacagacgccgttagagatccccagacactggaaatcctggacatcaccccttgcagcttcggcggagtgtctgtgatcacccctggcaccaacaccagcaatcaggtggcagtgctgtaccagggcgtgaactgtaccgaagtgcccgtggccattcacgccgatcagctgacacctacatggcgggtgtactccaccggcagcaatgtgtttcagaccagagccggctgtctgatcggagccgagtacgtgaacaatagctacgagtgcgacatccccatcggcgctggaatctgcgccagctaccagacacagacaaagagccaccggagagccagaagcgtggccagccagagcatcattgcctacacaatgtctctgggcgccgagaacagcgtggcctactccaacaactctatcgctatccccaccaacttcaccatcagcgtgaccacagagatcctgcctgtgtccatgaccaagaccagcgtggactgcaccatgtacatctgcggcgattccaccgagtgctccaacctgctgctgcagtacggcagcttctgcacccagctgaaaagagccctgacagggatcgccgtggaacaggacaagaacacccaagaggtgttcgcccaagtgaagcagatctacaagacccctcctatcaagtacttcggcggcttcaatttcagccagattctgcccgatcctagcaagcccagcaagcggagcttcatcgaggacctgctgttcaacaaagtgacactggccgacgccggcttcatcaagcagtatggcgattgtctgggcgacattgccgccagggatctgatttgcgcccagaagtttaacggactgacagtgctgcctcctctgctgaccgatgagatgatcgcccagtacacatctgccctgctggccggcacaatcacaagcggctggacatttggagcaggcgccgctctgcagatcccctttgctatgcagatggcctaccggttcaacggcatcggagtgacccagaatgtgctgtacgagaaccagaagctgatcgccaaccagttcaacagcgccatcggcaagatccaggacagcctgagcagcacagcaagcgccctgggaaagctgcaggacgtggtcaaccacaatgcccaggcactgaacaccctggtcaagcagctgtcctccaagttcggcgccatcagctctgtgctgaacgatatcctgagcagactggaccctcctgaggccgaggtgcagatcgacagactgatcacaggcagactgcagagcctccagacatacgtgacccagcagctgatcagagccgccgagattagagcctctgccaatctggccgccaccaagatgtctgagtgtgtgctgggccagagcaagagagtggacttttgcggcaagggctaccacctgatgagcttccctcagtctgcccctcacggcgtggtgtttctgcacgtgacatatgtgcccgctcaagagaagaatttcaccaccgctccagccatctgccacgacggcaaagcccactttcctagagaaggcgtgttcgtgtccaacggcacccattggttcgtgacacagcggaacttctacgagccccagatcatcaccaccgacaacaccttcgtgtctggcaactgcgacgtcgtgatcggcattgtgaacaataccgtgtacgaccctctgcagcccgagctggacagcttcaaagaggaactggacaagtactttaagaaccacacaagccccgacgtggacctgggcgatatcagcggaatcaatgccagcgtcgtgaacatccagaaagagatcgaccggctgaacgaggtggccaagaatctgaacgagagcctgatcgacctgcaagaactggggaagtacgagcagtacatcaagtggccctggtacatctggctgggctttatcgccggactgattgccatcgtgatggtcacaatcatgctgtgttgcatgaccagctgctgtagctgcctgaagggctgttgtagctgtggcagctgctgcaagttcgacgaggacgattctgagcccgtgctgaagggcgtgaaactgcactacacatgatgactcgagctggtactgcatgcacgcaatgctagctgcccctttcccgtcctgggtaccccgagtctcccccgacctcgggtcccaggtatgctcccacctccacctgccccactcaccacctctgctagttccagacacctcccaagcacgcagcaatgcagctcaaaacgcttagcctagccacacccccacgggaaacagcagtgattaacctttagcaataaacgaaagtttaactaagctatactaaccccagggttggtcaatttcgtgccagccacaccctggagctagcaaaaaaaaaaaaaaaaaaaaaaaaaaaaaagcatatgactaaaaaaaaaaaaaaaaaaaaaaaaaaaaaaaaaaaaaaaaaaaaaaaaaaaaaaaaaaaaaaaaaaaaa

SEQ ID NO: 172 - DNA, 4270 bp, synthetic construct
  source 1..4270: mol_type = other DNA
agaataaactagtattcttctggtccccacagactcagagagaacccgccaccatgttcgtgttcctggtgctgctgcctctggtgtccagccagtgtgtgaacctgatcaccagaacacagtcatacaccaacagctttaccagaggcgtgtactaccccgacaaggtgttcagatccagcgtgctgcactctacccaggacctgttcctgcctttcttcagcaacgtgacctggttccacgccatccacgtgtccggcaccaatggcaccaagagattcgacaaccccgccctgcccttcaacgacggggtgtactttgccagcaccgagaagtccaacatcatcagaggctggatcttcggcaccacactggacagcaagacccagagcctgctgatcgtgaacaacgccaccaacgtggtcatcaaagtgtgcgagttccagttctgcaacgaccccttcctggacgtctaccagaagaacaacaagagctggatggaaagcgagttccgggtgtacagcagcgccaacaactgcaccttcgagtacgtgtcccagcctttcctgatggacctggaaggcaaggagggcaacttcaagaacctgcgcgagttcgtgtttaagaacatcgacggctacttcaagatctacagcaagcacacccctatcaacctcgagcgggatctgcctcagggcttctctgctctggaacccctggtggatctgcccatcggcatcaacatcacccggtttcagacactgctggccctgcacagaagctacctgacacctggcggcagcagcagcggatggacagctggtgccgccgcttactatgtgggctacctgcagcctagaaccttcctgctgaagtacaacgagaacggcaccatcaccgacgccgtggattgtgctctggatcctctgagcgagacaaagtgcaccctgaagtccttcaccgtggaaaagggcatctaccagaccagcaacttccgggtgcagcccaccgaatccatcgtgcggttccccaatatcaccaatctgtgccccttccacgaggtgttcaatgccaccaccttcgcctctgtgtacgcctggaaccggaagcggatcagcaattgcgtggccgactactccgtgatctacaacttcgcccccttcttcgcattcaagtgctacggcgtgtcccctaccaagctgaacgacctgtgcttcacaaacgtgtacgccgacagcttcgtgatccggggaaacgaagtgtcacagattgcccctggacagacaggcaacatcgccgactacaactacaagctgcccgacgacttcaccggctgtgtgattgcctggaacagcaacaagctggactccaaacccagcggcaactacaattacctgtaccggctgttccggaagtccaagctgaagcccttcgagcgggacatctccaccgagatctatcaggccggcaacaagccttgtaacggcgtggcaggccccaactgctacagcccactgcagtcctacggctttaggcccacatacggcgtgggccaccagccctacagagtggtggtgctgagcttcgaactgctgcatgcctcagccacagtgtgcggccctaagaaaagcaccaatctcgtgaagaacaaatgcgtgaacttcaacttcaacggcctgaccggcaccggcgtgctgacagagagcaacaagaagttcctgccattccagcagtttggccgggatatcgccgataccacagacgccgttagagatccccagacactggaaatcctggacatcaccccttgcagcttcggcggagtgtctgtgatcacccctggcaccaacaccagcaatcaggtggcagtgctgtaccagggcgtgaactgtaccgaagtgcccgtggccattcacgccgatcagctgacacctacatggcgggtgtactccaccggcagcaatgtgtttcagaccagagccggctgtctgatcggagccgagtacgtgaacaatagctacgagtgcgacatccccatcggcgctggaatctgcgccagctaccagacacagacaaagagccaccggagagccagaagcgtggccagccagagcatcattgcctacacaatgtctctgggcgccgagaacagcgtggcctactccaacaactctatcgctatccccaccaacttcaccatcagcgtgaccacagagatcctgcctgtgtccatgaccaagaccagcgtggactgcaccatgtacatctgcggcgattccaccgagtgctccaacctgctgctgcagtacggcagcttctgcacccagctgaaaagagccctgacagggatcgccgtggaacaggacaagaacacccaagaggtgttcgcccaagtgaagcagatctacaagacccctcctatcaagtacttcggcggcttcaatttcagccagattctgcccgatcctagcaagcccagcaagcggagcttcatcgaggacctgctgttcaacaaagtgacactggccgacgccggcttcatcaagcagtatggcgattgtctgggcgacattgccgccagggatctgatttgcgcccagaagtttaacggactgacagtgctgcctcctctgctgaccgatgagatgatcgcccagtacacatctgccctgctggccggcacaatcacaagcggctggacatttggagcaggcgccgctctgcagatcccctttgctatgcagatggcctaccggttcaacggcatcggagtgacccagaatgtgctgtacgagaaccagaagctgatcgccaaccagttcaacagcgccatcggcaagatccaggacagcctgagcagcacagcaagcgccctgggaaagctgcaggacgtggtcaaccacaatgcccaggcactgaacaccctggtcaagcagctgtcctccaagttcggcgccatcagctctgtgctgaacgatatcctgagcagactggaccctcctgaggccgaggtgcagatcgacagactgatcacaggcagactgcagagcctccagacatacgtgacccagcagctgatcagagccgccgagattagagcctctgccaatctggccgccaccaagatgtctgagtgtgtgctgggccagagcaagagagtggacttttgcggcaagggctaccacctgatgagcttccctcagtctgcccctcacggcgtggtgtttctgcacgtgacatatgtgcccgctcaagagaagaatttcaccaccgctccagccatctgccacgacggcaaagcccactttcctagagaaggcgtgttcgtgtccaacggcacccattggttcgtgacacagcggaacttctacgagccccagatcatcaccaccgacaacaccttcgtgtctggcaactgcgacgtcgtgatcggcattgtgaacaataccgtgtacgaccctctgcagcccgagctggacagcttcaaagaggaactggacaagtactttaagaaccacacaagccccgacgtggacctgggcgatatcagcggaatcaatgccagcgtcgtgaacatccagaaagagatcgaccggctgaacgaggtggccaagaatctgaacgagagcctgatcgacctgcaagaactggggaagtacgagcagtacatcaagtggccctggtacatctggctgggctttatcgccggactgattgccatcgtgatggtcacaatcatgctgtgttgcatgaccagctgctgtagctgcctgaagggctgttgtagctgtggcagctgctgcaagttcgacgaggacgattctgagcccgtgctgaagggcgtgaaactgcactacacatgatgactcgagctggtactgcatgcacgcaatgctagctgcccctttcccgtcctgggtaccccgagtctcccccgacctcgggtcccaggtatgctcccacctccacctgccccactcaccacctctgctagttccagacacctcccaagcacgcagcaatgcagctcaaaacgcttagcctagccacacccccacgggaaacagcagtgattaacctttagcaataaacgaaagtttaactaagctatactaaccccagggttggtcaatttcgtgccagccacaccctggagctagcaaaaaaaaaaaaaaaaaaaaaaaaaaaaaagcatatgactaaaaaaaaaaaaaaaaaaaaaaaaaaaaaaaaaaaaaaaaaaaaaaaaaaaaaaaaaaaaaaaaaaaaa

SEQ ID NO: 173 - protein, 1269 aa, synthetic construct
MFVFLVLLPLVSSQCVNLITRTQSYTNSFTRGVYYPDKVFRSSVLHSTQDLFLPFFSNVTWFHAIHVSGTNGTKRFDNPALPFNDGVYFASTEKSNIIRGWIFGTTLDSKTQSLLIVNNATNVVIKVCEFQFCNDPFLDVYQKNNKSWMESEFRVYSSANNCTFEYVSQPFLMDLEGKEVNFKNLREFVFKNIDGYFKIYSKHTPINLERDLPQGFSALEPLVDLPIGINITRFQTLLALHRSYLTPGGSSSGWTAGAAAYYVGYLQPRTFLLKYNENGTITDAVDCALDPLSETKCTLKSFTVEKGIYQTSNFRVQPTESIVRFPNITNLCPFHEVFNATTFASVYAWNRKRISNCVADYSVIYNFAPFFAFKCYGVSPTKLNDLCFTNVYADSFVIRGNEVSQIAPGQTGNIADYNYKLPDDFTGCVIAWNSNKLDSKPSGNYNYLYRLFRKSKLKPFERDISTEIYQAGNKPCNGVAGPNCYSPLQSYGFRPTYGVGHQPYRVVVLSFELLHASATVCGPKKSTNLVKNKCVNFNFNGLTGTGVLTESNKKFLPFQQFGRDIADTTDAVRDPQTLEILDITPCSFGGVSVITPGTNTSNQVAVLYQGVNCTEVPVAIHADQLTPTWRVYSTGSNVFQTRAGCLIGAEYVNNSYECDIPIGAGICASYQTQTKSHRRARSVASQSIIAYTMSLGAENSVAYSNNSIAIPTNFTISVTTEILPVSMTKTSVDCTMYICGDSTECSNLLLQYGSFCTQLKRALTGIAVEQDKNTQEVFAQVKQIYKTPPIKYFGGFNFSQILPDPSKPSKRSFIEDLLFNKVTLADAGFIKQYGDCLGDIAARDLICAQKFNGLTVLPPLLTDEMIAQYTSALLAGTITSGWTFGAGAALQIPFAMQMAYRFNGIGVTQNVLYENQKLIANQFNSAIGKIQDSLSSTASALGKLQDVVNHNAQALNTLVKQLSSKFGAISSVLNDILSRLDPPEAEVQIDRLITGRLQSLQTYVTQQLIRAAEIRASANLAATKMSECVLGQSKRVDFCGKGYHLMSFPQSAPHGVVFLHVTYVPAQEKNFTTAPAICHDGKAHFPREGVFVSNGTHWFVTQRNFYEPQIITTDNTFVSGNCDVVIGIVNNTVYDPLQPELDSFKEELDKYFKNHTSPDVDLGDISGINASVVNIQKEIDRLNEVAKNLNESLIDLQELGKYEQYIKWPWYIWLGFIAGLIAIVMVTIMLCCMTSCCSCLKGCCSCGSCCKFDEDDSEPVLKGVKLHYT

SEQ ID NO: 174 - RNA, 3813 nt, synthetic construct
  source 1..3813: mol_type = other RNA
atgttcgtgttcctggtgctgctgcctctggtgtccagccagtgtgtgaacctgatcaccagaacacagtcatacaccaacagctttaccagaggcgtgtactaccccgacaaggtgttcagatccagcgtgctgcactctacccaggacctgttcctgcctttcttcagcaacgtgacctggttccacgccatccacgtgtccggcaccaatggcaccaagagattcgacaaccccgccctgcccttcaacgacggggtgtactttgccagcaccgagaagtccaacatcatcagaggctggatcttcggcaccacactggacagcaagacccagagcctgctgatcgtgaacaacgccaccaacgtggtcatcaaagtgtgcgagttccagttctgcaacgaccccttcctggacgtctaccagaagaacaacaagagctggatggaaagcgagttccgggtgtacagcagcgccaacaactgcaccttcgagtacgtgtcccagcctttcctgatggacctggaaggcaaggaggtgaacttcaagaacctgcgcgagttcgtgtttaagaacatcgacggctacttcaagatctacagcaagcacacccctatcaacctcgagcgggatctgcctcagggcttctctgctctggaacccctggtggatctgcccatcggcatcaacatcacccggtttcagacactgctggccctgcacagaagctacctgacacctggcggcagcagcagcggatggacagctggtgccgccgcttactatgtgggctacctgcagcctagaaccttcctgctgaagtacaacgagaacggcaccatcaccgacgccgtggattgtgctctggatcctctgagcgagacaaagtgcaccctgaagtccttcaccgtggaaaagggcatctaccagaccagcaacttccgggtgcagcccaccgaatccatcgtgcggttccccaatatcaccaatctgtgccccttccacgaggtgttcaatgccaccaccttcgcctctgtgtacgcctggaaccggaagcggatcagcaattgcgtggccgactactccgtgatctacaacttcgcccccttcttcgcattcaagtgctacggcgtgtcccctaccaagctgaacgacctgtgcttcacaaacgtgtacgccgacagcttcgtgatccggggaaacgaagtgtcacagattgcccctggacagacaggcaacatcgccgactacaactacaagctgcccgacgacttcaccggctgtgtgattgcctggaacagcaacaagctggactccaaacccagcggcaactacaattacctgtaccggctgttccggaagtccaagctgaagcccttcgagcgggacatctccaccgagatctatcaggccggcaacaagccttgtaacggcgtggcaggccccaactgctacagcccactgcagtcctacggctttaggcccacatacggcgtgggccaccagccctacagagtggtggtgctgagcttcgaactgctgcatgcctcagccacagtgtgcggccctaagaaaagcaccaatctcgtgaagaacaaatgcgtgaacttcaacttcaacggcctgaccggcaccggcgtgctgacagagagcaacaagaagttcctgccattccagcagtttggccgggatatcgccgataccacagacgccgttagagatccccagacactggaaatcctggacatcaccccttgcagcttcggcggagtgtctgtgatcacccctggcaccaacaccagcaatcaggtggcagtgctgtaccagggcgtgaactgtaccgaagtgcccgtggccattcacgccgatcagctgacacctacatggcgggtgtactccaccggcagcaatgtgtttcagaccagagccggctgtctgatcggagccgagtacgtgaacaatagctacgagtgcgacatccccatcggcgctggaatctgcgccagctaccagacacagacaaagagccaccggagagccagaagcgtggccagccagagcatcattgcctacacaatgtctctgggcgccgagaacagcgtggcctactccaacaactctatcgctatccccaccaacttcaccatcagcgtgaccacagagatcctgcctgtgtccatgaccaagaccagcgtggactgcaccatgtacatctgcggcgattccaccgagtgctccaacctgctgctgcagtacggcagcttctgcacccagctgaaaagagccctgacagggatcgccgtggaacaggacaagaacacccaagaggtgttcgcccaagtgaagcagatctacaagacccctcctatcaagtacttcggcggcttcaatttcagccagattctgcccgatcctagcaagcccagcaagcggagcttcatcgaggacctgctgttcaacaaagtgacactggccgacgccggcttcatcaagcagtatggcgattgtctgggcgacattgccgccagggatctgatttgcgcccagaagtttaacggactgacagtgctgcctcctctgctgaccgatgagatgatcgcccagtacacatctgccctgctggccggcacaatcacaagcggctggacatttggagcaggcgccgctctgcagatcccctttgctatgcagatggcctaccggttcaacggcatcggagtgacccagaatgtgctgtacgagaaccagaagctgatcgccaaccagttcaacagcgccatcggcaagatccaggacagcctgagcagcacagcaagcgccctgggaaagctgcaggacgtggtcaaccacaatgcccaggcactgaacaccctggtcaagcagctgtcctccaagttcggcgccatcagctctgtgctgaacgatatcctgagcagactggaccctcctgaggccgaggtgcagatcgacagactgatcacaggcagactgcagagcctccagacatacgtgacccagcagctgatcagagccgccgagattagagcctctgccaatctggccgccaccaagatgtctgagtgtgtgctgggccagagcaagagagtggacttttgcggcaagggctaccacctgatgagcttccctcagtctgcccctcacggcgtggtgtttctgcacgtgacatatgtgcccgctcaagagaagaatttcaccaccgctccagccatctgccacgacggcaaagcccactttcctagagaaggcgtgttcgtgtccaacggcacccattggttcgtgacacagcggaacttctacgagccccagatcatcaccaccgacaacaccttcgtgtctggcaactgcgacgtcgtgatcggcattgtgaacaataccgtgtacgaccctctgcagcccgagctggacagcttcaaagaggaactggacaagtactttaagaaccacacaagccccgacgtggacctgggcgatatcagcggaatcaatgccagcgtcgtgaacatccagaaagagatcgaccggctgaacgaggtggccaagaatctgaacgagagcctgatcgacctgcaagaactggggaagtacgagcagtacatcaagtggccctggtacatctggctgggctttatcgccggactgattgccatcgtgatggtcacaatcatgctgtgttgcatgaccagctgctgtagctgcctgaagggctgttgtagctgtggcagctgctgcaagttcgacgaggacgattctgagcccgtgctgaagggcgtgaaactgcactacacatgatga

SEQ ID NO: 175 - DNA, 3813 bp, synthetic construct
  source 1..3813: mol_type = other DNA
atgttcgtgttcctggtgctgctgcctctggtgtccagccagtgtgtgaacctgatcaccagaacacagtcatacaccaacagctttaccagaggcgtgtactaccccgacaaggtgttcagatccagcgtgctgcactctacccaggacctgttcctgcctttcttcagcaacgtgacctggttccacgccatccacgtgtccggcaccaatggcaccaagagattcgacaaccccgccctgcccttcaacgacggggtgtactttgccagcaccgagaagtccaacatcatcagaggctggatcttcggcaccacactggacagcaagacccagagcctgctgatcgtgaacaacgccaccaacgtggtcatcaaagtgtgcgagttccagttctgcaacgaccccttcctggacgtctaccagaagaacaacaagagctggatggaaagcgagttccgggtgtacagcagcgccaacaactgcaccttcgagtacgtgtcccagcctttcctgatggacctggaaggcaaggaggtgaacttcaagaacctgcgcgagttcgtgtttaagaacatcgacggctacttcaagatctacagcaagcacacccctatcaacctcgagcgggatctgcctcagggcttctctgctctggaacccctggtggatctgcccatcggcatcaacatcacccggtttcagacactgctggccctgcacagaagctacctgacacctggcggcagcagcagcggatggacagctggtgccgccgcttactatgtgggctacctgcagcctagaaccttcctgctgaagtacaacgagaacggcaccatcaccgacgccgtggattgtgctctggatcctctgagcgagacaaagtgcaccctgaagtccttcaccgtggaaaagggcatctaccagaccagcaacttccgggtgcagcccaccgaatccatcgtgcggttccccaatatcaccaatctgtgccccttccacgaggtgttcaatgccaccaccttcgcctctgtgtacgcctggaaccggaagcggatcagcaattgcgtggccgactactccgtgatctacaacttcgcccccttcttcgcattcaagtgctacggcgtgtcccctaccaagctgaacgacctgtgcttcacaaacgtgtacgccgacagcttcgtgatccggggaaacgaagtgtcacagattgcccctggacagacaggcaacatcgccgactacaactacaagctgcccgacgacttcaccggctgtgtgattgcctggaacagcaacaagctggactccaaacccagcggcaactacaattacctgtaccggctgttccggaagtccaagctgaagcccttcgagcgggacatctccaccgagatctatcaggccggcaacaagccttgtaacggcgtggcaggccccaactgctacagcccactgcagtcctacggctttaggcccacatacggcgtgggccaccagccctacagagtggtggtgctgagcttcgaactgctgcatgcctcagccacagtgtgcggccctaagaaaagcaccaatctcgtgaagaacaaatgcgtgaacttcaacttcaacggcctgaccggcaccggcgtgctgacagagagcaacaagaagttcctgccattccagcagtttggccgggatatcgccgataccacagacgccgttagagatccccagacactggaaatcctggacatcaccccttgcagcttcggcggagtgtctgtgatcacccctggcaccaacaccagcaatcaggtggcagtgctgtaccagggcgtgaactgtaccgaagtgcccgtggccattcacgccgatcagctgacacctacatggcgggtgtactccaccggcagcaatgtgtttcagaccagagccggctgtctgatcggagccgagtacgtgaacaatagctacgagtgcgacatccccatcggcgctggaatctgcgccagctaccagacacagacaaagagccaccggagagccagaagcgtggccagccagagcatcattgcctacacaatgtctctgggcgccgagaacagcgtggcctactccaacaactctatcgctatccccaccaacttcaccatcagcgtgaccacagagatcctgcctgtgtccatgaccaagaccagcgtggactgcaccatgtacatctgcggcgattccaccgagtgctccaacctgctgctgcagtacggcagcttctgcacccagctgaaaagagccctgacagggatcgccgtggaacaggacaagaacacccaagaggtgttcgcccaagtgaagcagatctacaagacccctcctatcaagtacttcggcggcttcaatttcagccagattctgcccgatcctagcaagcccagcaagcggagcttcatcgaggacctgctgttcaacaaagtgacactggccgacgccggcttcatcaagcagtatggcgattgtctgggcgacattgccgccagggatctgatttgcgcccagaagtttaacggactgacagtgctgcctcctctgctgaccgatgagatgatcgcccagtacacatctgccctgctggccggcacaatcacaagcggctggacatttggagcaggcgccgctctgcagatcccctttgctatgcagatggcctaccggttcaacggcatcggagtgacccagaatgtgctgtacgagaaccagaagctgatcgccaaccagttcaacagcgccatcggcaagatccaggacagcctgagcagcacagcaagcgccctgggaaagctgcaggacgtggtcaaccacaatgcccaggcactgaacaccctggtcaagcagctgtcctccaagttcggcgccatcagctctgtgctgaacgatatcctgagcagactggaccctcctgaggccgaggtgcagatcgacagactgatcacaggcagactgcagagcctccagacatacgtgacccagcagctgatcagagccgccgagattagagcctctgccaatctggccgccaccaagatgtctgagtgtgtgctgggccagagcaagagagtggacttttgcggcaagggctaccacctgatgagcttccctcagtctgcccctcacggcgtggtgtttctgcacgtgacatatgtgcccgctcaagagaagaatttcaccaccgctccagccatctgccacgacggcaaagcccactttcctagagaaggcgtgttcgtgtccaacggcacccattggttcgtgacacagcggaacttctacgagccccagatcatcaccaccgacaacaccttcgtgtctggcaactgcgacgtcgtgatcggcattgtgaacaataccgtgtacgaccctctgcagcccgagctggacagcttcaaagaggaactggacaagtactttaagaaccacacaagccccgacgtggacctgggcgatatcagcggaatcaatgccagcgtcgtgaacatccagaaagagatcgaccggctgaacgaggtggccaagaatctgaacgagagcctgatcgacctgcaagaactggggaagtacgagcagtacatcaagtggccctggtacatctggctgggctttatcgccggactgattgccatcgtgatggtcacaatcatgctgtgttgcatgaccagctgctgtagctgcctgaagggctgttgtagctgtggcagctgctgcaagttcgacgaggacgattctgagcccgtgctgaagggcgtgaaactgcactacacatgatga

SEQ ID NO: 176 - RNA, 4270 nt, synthetic construct
  source 1..4270: mol_type = other RNA
agaataaactagtattcttctggtccccacagactcagagagaacccgccaccatgttcgtgttcctggtgctgctgcctctggtgtccagccagtgtgtgaacctgatcaccagaacacagtcatacaccaacagctttaccagaggcgtgtactaccccgacaaggtgttcagatccagcgtgctgcactctacccaggacctgttcctgcctttcttcagcaacgtgacctggttccacgccatccacgtgtccggcaccaatggcaccaagagattcgacaaccccgccctgcccttcaacgacggggtgtactttgccagcaccgagaagtccaacatcatcagaggctggatcttcggcaccacactggacagcaagacccagagcctgctgatcgtgaacaacgccaccaacgtggtcatcaaagtgtgcgagttccagttctgcaacgaccccttcctggacgtctaccagaagaacaacaagagctggatggaaagcgagttccgggtgtacagcagcgccaacaactgcaccttcgagtacgtgtcccagcctttcctgatggacctggaaggcaaggaggtgaacttcaagaacctgcgcgagttcgtgtttaagaacatcgacggctacttcaagatctacagcaagcacacccctatcaacctcgagcgggatctgcctcagggcttctctgctctggaacccctggtggatctgcccatcggcatcaacatcacccggtttcagacactgctggccctgcacagaagctacctgacacctggcggcagcagcagcggatggacagctggtgccgccgcttactatgtgggctacctgcagcctagaaccttcctgctgaagtacaacgagaacggcaccatcaccgacgccgtggattgtgctctggatcctctgagcgagacaaagtgcaccctgaagtccttcaccgtggaaaagggcatctaccagaccagcaacttccgggtgcagcccaccgaatccatcgtgcggttccccaatatcaccaatctgtgccccttccacgaggtgttcaatgccaccaccttcgcctctgtgtacgcctggaaccggaagcggatcagcaattgcgtggccgactactccgtgatctacaacttcgcccccttcttcgcattcaagtgctacggcgtgtcccctaccaagctgaacgacctgtgcttcacaaacgtgtacgccgacagcttcgtgatccggggaaacgaagtgtcacagattgcccctggacagacaggcaacatcgccgactacaactacaagctgcccgacgacttcaccggctgtgtgattgcctggaacagcaacaagctggactccaaacccagcggcaactacaattacctgtaccggctgttccggaagtccaagctgaagcccttcgagcgggacatctccaccgagatctatcaggccggcaacaagccttgtaacggcgtggcaggccccaactgctacagcccactgcagtcctacggctttaggcccacatacggcgtgggccaccagccctacagagtggtggtgctgagcttcgaactgctgcatgcctcagccacagtgtgcggccctaagaaaagcaccaatctcgtgaagaacaaatgcgtgaacttcaacttcaacggcctgaccggcaccggcgtgctgacagagagcaacaagaagttcctgccattccagcagtttggccgggatatcgccgataccacagacgccgttagagatccccagacactggaaatcctggacatcaccccttgcagcttcggcggagtgtctgtgatcacccctggcaccaacaccagcaatcaggtggcagtgctgtaccagggcgtgaactgtaccgaagtgcccgtggccattcacgccgatcagctgacacctacatggcgggtgtactccaccggcagcaatgtgtttcagaccagagccggctgtctgatcggagccgagtacgtgaacaatagctacgagtgcgacatccccatcggcgctggaatctgcgccagctaccagacacagacaaagagccaccggagagccagaagcgtggccagccagagcatcattgcctacacaatgtctctgggcgccgagaacagcgtggcctactccaacaactctatcgctatccccaccaacttcaccatcagcgtgaccacagagatcctgcctgtgtccatgaccaagaccagcgtggactgcaccatgtacatctgcggcgattccaccgagtgctccaacctgctgctgcagtacggcagcttctgcacccagctgaaaagagccctgacagggatcgccgtggaacaggacaagaacacccaagaggtgttcgcccaagtgaagcagatctacaagacccctcctatcaagtacttcggcggcttcaatttcagccagattctgcccgatcctagcaagcccagcaagcggagcttcatcgaggacctgctgttcaacaaagtgacactggccgacgccggcttcatcaagcagtatggcgattgtctgggcgacattgccgccagggatctgatttgcgcccagaagtttaacggactgacagtgctgcctcctctgctgaccgatgagatgatcgcccagtacacatctgccctgctggccggcacaatcacaagcggctggacatttggagcaggcgccgctctgcagatcccctttgctatgcagatggcctaccggttcaacggcatcggagtgacccagaatgtgctgtacgagaaccagaagctgatcgccaaccagttcaacagcgccatcggcaagatccaggacagcctgagcagcacagcaagcgccctgggaaagctgcaggacgtggtcaaccacaatgcccaggcactgaacaccctggtcaagcagctgtcctccaagttcggcgccatcagctctgtgctgaacgatatcctgagcagactggaccctcctgaggccgaggtgcagatcgacagactgatcacaggcagactgcagagcctccagacatacgtgacccagcagctgatcagagccgccgagattagagcctctgccaatctggccgccaccaagatgtctgagtgtgtgctgggccagagcaagagagtggacttttgcggcaagggctaccacctgatgagcttccctcagtctgcccctcacggcgtggtgtttctgcacgtgacatatgtgcccgctcaagagaagaatttcaccaccgctccagccatctgccacgacggcaaagcccactttcctagagaaggcgtgttcgtgtccaacggcacccattggttcgtgacacagcggaacttctacgagccccagatcatcaccaccgacaacaccttcgtgtctggcaactgcgacgtcgtgatcggcattgtgaacaataccgtgtacgaccctctgcagcccgagctggacagcttcaaagaggaactggacaagtactttaagaaccacacaagccccgacgtggacctgggcgatatcagcggaatcaatgccagcgtcgtgaacatccagaaagagatcgaccggctgaacgaggtggccaagaatctgaacgagagcctgatcgacctgcaagaactggggaagtacgagcagtacatcaagtggccctggtacatctggctgggctttatcgccggactgattgccatcgtgatggtcacaatcatgctgtgttgcatgaccagctgctgtagctgcctgaagggctgttgtagctgtggcagctgctgcaagttcgacgaggacgattctgagcccgtgctgaagggcgtgaaactgcactacacatgatgactcgagctggtactgcatgcacgcaatgctagctgcccctttcccgtcctgggtaccccgagtctcccccgacctcgggtcccaggtatgctcccacctccacctgccccactcaccacctctgctagttccagacacctcccaagcacgcagcaatgcagctcaaaacgcttagcctagccacacccccacgggaaacagcagtgattaacctttagcaataaacgaaagtttaactaagctatactaaccccagggttggtcaatttcgtgccagccacaccctggagctagcaaaaaaaaaaaaaaaaaaaaaaaaaaaaaagcatatgactaaaaaaaaaaaaaaaaaaaaaaaaaaaaaaaaaaaaaaaaaaaaaaaaaaaaaaaaaaaaaaaaaaaaa

SEQ ID NO: 177 - DNA, 4270 bp, synthetic construct
  source 1..4270: mol_type = other DNA
agaataaactagtattcttctggtccccacagactcagagagaacccgccaccatgttcgtgttcctggtgctgctgcctctggtgtccagccagtgtgtgaacctgatcaccagaacacagtcatacaccaacagctttaccagaggcgtgtactaccccgacaaggtgttcagatccagcgtgctgcactctacccaggacctgttcctgcctttcttcagcaacgtgacctggttccacgccatccacgtgtccggcaccaatggcaccaagagattcgacaaccccgccctgcccttcaacgacggggtgtactttgccagcaccgagaagtccaacatcatcagaggctggatcttcggcaccacactggacagcaagacccagagcctgctgatcgtgaacaacgccaccaacgtggtcatcaaagtgtgcgagttccagttctgcaacgaccccttcctggacgtctaccagaagaacaacaagagctggatggaaagcgagttccgggtgtacagcagcgccaacaactgcaccttcgagtacgtgtcccagcctttcctgatggacctggaaggcaaggaggtgaacttcaagaacctgcgcgagttcgtgtttaagaacatcgacggctacttcaagatctacagcaagcacacccctatcaacctcgagcgggatctgcctcagggcttctctgctctggaacccctggtggatctgcccatcggcatcaacatcacccggtttcagacactgctggccctgcacagaagctacctgacacctggcggcagcagcagcggatggacagctggtgccgccgcttactatgtgggctacctgcagcctagaaccttcctgctgaagtacaacgagaacggcaccatcaccgacgccgtggattgtgctctggatcctctgagcgagacaaagtgcaccctgaagtccttcaccgtggaaaagggcatctaccagaccagcaacttccgggtgcagcccaccgaatccatcgtgcggttccccaatatcaccaatctgtgccccttccacgaggtgttcaatgccaccaccttcgcctctgtgtacgcctggaaccggaagcggatcagcaattgcgtggccgactactccgtgatctacaacttcgcccccttcttcgcattcaagtgctacggcgtgtcccctaccaagctgaacgacctgtgcttcacaaacgtgtacgccgacagcttcgtgatccggggaaacgaagtgtcacagattgcccctggacagacaggcaacatcgccgactacaactacaagctgcccgacgacttcaccggctgtgtgattgcctggaacagcaacaagctggactccaaacccagcggcaactacaattacctgtaccggctgttccggaagtccaagctgaagcccttcgagcgggacatctccaccgagatctatcaggccggcaacaagccttgtaacggcgtggcaggccccaactgctacagcccactgcagtcctacggctttaggcccacatacggcgtgggccaccagccctacagagtggtggtgctgagcttcgaactgctgcatgcctcagccacagtgtgcggccctaagaaaagcaccaatctcgtgaagaacaaatgcgtgaacttcaacttcaacggcctgaccggcaccggcgtgctgacagagagcaacaagaagttcctgccattccagcagtttggccgggatatcgccgataccacagacgccgttagagatccccagacactggaaatcctggacatcaccccttgcagcttcggcggagtgtctgtgatcacccctggcaccaacaccagcaatcaggtggcagtgctgtaccagggcgtgaactgtaccgaagtgcccgtggccattcacgccgatcagctgacacctacatggcgggtgtactccaccggcagcaatgtgtttcagaccagagccggctgtctgatcggagccgagtacgtgaacaatagctacgagtgcgacatccccatcggcgctggaatctgcgccagctaccagacacagacaaagagccaccggagagccagaagcgtggccagccagagcatcattgcctacacaatgtctctgggcgccgagaacagcgtggcctactccaacaactctatcgctatccccaccaacttcaccatcagcgtgaccacagagatcctgcctgtgtccatgaccaagaccagcgtggactgcaccatgtacatctgcggcgattccaccgagtgctccaacctgctgctgcagtacggcagcttctgcacccagctgaaaagagccctgacagggatcgccgtggaacaggacaagaacacccaagaggtgttcgcccaagtgaagcagatctacaagacccctcctatcaagtacttcggcggcttcaatttcagccagattctgcccgatcctagcaagcccagcaagcggagcttcatcgaggacctgctgttcaacaaagtgacactggccgacgccggcttcatcaagcagtatggcgattgtctgggcgacattgccgccagggatctgatttgcgcccagaagtttaacggactgacagtgctgcctcctctgctgaccgatgagatgatcgcccagtacacatctgccctgctggccggcacaatcacaagcggctggacatttggagcaggcgccgctctgcagatcccctttgctatgcagatggcctaccggttcaacggcatcggagtgacccagaatgtgctgtacgagaaccagaagctgatcgccaaccagttcaacagcgccatcggcaagatccaggacagcctgagcagcacagcaagcgccctgggaaagctgcaggacgtggtcaaccacaatgcccaggcactgaacaccctggtcaagcagctgtcctccaagttcggcgccatcagctctgtgctgaacgatatcctgagcagactggaccctcctgaggccgaggtgcagatcgacagactgatcacaggcagactgcagagcctccagacatacgtgacccagcagctgatcagagccgccgagattagagcctctgccaatctggccgccaccaagatgtctgagtgtgtgctgggccagagcaagagagtggacttttgcggcaagggctaccacctgatgagcttccctcagtctgcccctcacggcgtggtgtttctgcacgtgacatatgtgcccgctcaagagaagaatttcaccaccgctccagccatctgccacgacggcaaagcccactttcctagagaaggcgtgttcgtgtccaacggcacccattggttcgtgacacagcggaacttctacgagccccagatcatcaccaccgacaacaccttcgtgtctggcaactgcgacgtcgtgatcggcattgtgaacaataccgtgtacgaccctctgcagcccgagctggacagcttcaaagaggaactggacaagtactttaagaaccacacaagccccgacgtggacctgggcgatatcagcggaatcaatgccagcgtcgtgaacatccagaaagagatcgaccggctgaacgaggtggccaagaatctgaacgagagcctgatcgacctgcaagaactggggaagtacgagcagtacatcaagtggccctggtacatctggctgggctttatcgccggactgattgccatcgtgatggtcacaatcatgctgtgttgcatgaccagctgctgtagctgcctgaagggctgttgtagctgtggcagctgctgcaagttcgacgaggacgattctgagcccgtgctgaagggcgtgaaactgcactacacatgatgactcgagctggtactgcatgcacgcaatgctagctgcccctttcccgtcctgggtaccccgagtctcccccgacctcgggtcccaggtatgctcccacctccacctgccccactcaccacctctgctagttccagacacctcccaagcacgcagcaatgcagctcaaaacgcttagcctagccacacccccacgggaaacagcagtgattaacctttagcaataaacgaaagtttaactaagctatactaaccccagggttggtcaatttcgtgccagccacaccctggagctagcaaaaaaaaaaaaaaaaaaaaaaaaaaaaaagcatatgactaaaaaaaaaaaaaaaaaaaaaaaaaaaaaaaaaaaaaaaaaaaaaaaaaaaaaaaaaaaaaaaaaaaaa